European Patent Specification EP 3 520 813 B1, published April 19, 2023. Title: ANTIGEN DELIVERY PLATFORMS. Applicant: GLAXOSMITHKLINE BIOLOGICALS SA. The sequence listing filed with the application follows.

SEQUENCE LISTING (85 sequences)

SEQ ID NO: 1 - DNA, 24 bp, Venezuelan equine encephalitis virus
ctctctacggctaacctgaatgga

SEQ ID NO: 2 - protein, 8 aa, Artificial Sequence
  source: /note="Description of Artificial Sequence: Synthetic consensus sequence"
  VARIANT (2)..(2): /replace="Ile"
  MOD_RES (4)..(4): Any amino acid
DVEXNPGP

SEQ ID NO: 3 - protein, 8 aa, Foot and mouth disease virus
DVESNPGP

SEQ ID NO: 4 - protein, 100 aa, Artificial Sequence
  source: /note="Description of Artificial Sequence: Synthetic polypeptide"
  misc_feature (1)..(100): /note="This sequence may encompass 3 to 100 'Lys' residues"
KKKKKKKKKKKKKKKKKKKKKKKKKKKKKKKKKKKKKKKKKKKKKKKKKKKKKKKKKKKKKKKKKKKKKKKKKKKKKKKKKKKKKKKKKKKKKKKKKKKK

SEQ ID NO: 5 - protein, 3 aa, Unknown
  source: /note="Description of Unknown: integrin receptor-binding moiety peptide"
RGD

SEQ ID NO: 6 - protein, 6 aa, Artificial Sequence
  source: /note="Description of Artificial Sequence: Synthetic 6xHis tag"
HHHHHH

SEQ ID NO: 7 - DNA, 6 bp, Artificial Sequence
  source: /note="Description of Artificial Sequence: Synthetic oligonucleotide"
gggccc

SEQ ID NO: 8 - DNA, 6 bp, Artificial Sequence
  source: /note="Description of Artificial Sequence: Synthetic oligonucleotide"
ggcgcc

SEQ ID NO: 9 - DNA, 28 bp, Artificial Sequence
  source: /note="Description of Artificial Sequence: Synthetic oligonucleotide"
ctcgatgtacttccgaggaactgatgtg

SEQ ID NO: 10 - DNA, 28 bp, Artificial Sequence
  source: /note="Description of Artificial Sequence: Synthetic oligonucleotide"
atcgatgtacttccgaggaactcacgtg

SEQ ID NO: 11 - DNA, 6 bp, Artificial Sequence
  source: /note="Description of Artificial Sequence: Synthetic oligonucleotide"
gtcgac

SEQ ID NO: 12 - DNA, 6 bp, Artificial Sequence
  source: /note="Description of Artificial Sequence: Synthetic oligonucleotide"
gtctac

SEQ ID NO: 13 - DNA, 6 bp, Artificial Sequence
  source: /note="Description of Artificial Sequence: Synthetic oligonucleotide"
tctaga

SEQ ID NO: 14 - DNA, 6 bp, Artificial Sequence
  source: /note="Description of Artificial Sequence: Synthetic oligonucleotide"
tcaaga

SEQ ID NO: 15 - DNA, 14 bp, Artificial Sequence
  source: /note="Description of Artificial Sequence: Synthetic oligonucleotide"
ctggatatctgcag

SEQ ID NO: 16 - DNA, 14 bp, Artificial Sequence
  source: /note="Description of Artificial Sequence: Synthetic oligonucleotide"
atcgatatccgcgg

SEQ ID NO: 17 - DNA, 78 bp, Artificial Sequence
  source: /note="Description of Artificial Sequence: Synthetic oligonucleotide"
ctataactctctacggctaacctgaatggactacgacatagtctagtcgaccaagcctctagacggcgcgcccaccca

SEQ ID NO: 18 - DNA, 38 bp, Artificial Sequence
  source: /note="Description of Artificial Sequence: Synthetic primer"
ataagaatgcggccgcctataactctctacggctaacc

SEQ ID NO: 19 - DNA, 28 bp, Artificial Sequence
  source: /note="Description of Artificial Sequence: Synthetic primer"
ccatcgattgggtgggcgcgccgtctag

SEQ ID NO: 20 - DNA, 30 bp, Artificial Sequence
  source: /note="Description of Artificial Sequence: Synthetic primer"
ccatcgatctataactctctacggctaacc

SEQ ID NO: 21 - DNA, 29 bp, Artificial Sequence
  source: /note="Description of Artificial Sequence: Synthetic primer"
tccccgcggtgggtgggcgcgccgtctag

SEQ ID NO: 22 - DNA, 12 bp, Artificial Sequence
  source: /note="Description of Artificial Sequence: Synthetic oligonucleotide"
ccactgtgatcg

SEQ ID NO: 23 - DNA, 6 bp, Artificial Sequence
  source: /note="Description of Artificial Sequence: Synthetic oligonucleotide"
cacgtg

SEQ ID NO: 24 - DNA, 6 bp, Artificial Sequence
  source: /note="Description of Artificial Sequence: Synthetic oligonucleotide"
actgtg

SEQ ID NO: 25 - DNA, 2727 bp, Human herpesvirus 5
atggaaagccggatctggtgcctggtcgtgtgcgtgaacctgtgcatcgtgtgcctgggagccgccgtgagcagcagcagcaccagaggcaccagcgccacacacagccaccacagcagccacaccacctctgccgcccacagcagatccggcagcgtgtcccagagagtgaccagcagccagaccgtgtcccacggcgtgaacgagacaatctacaacaccaccctgaagtacggcgacgtcgtgggcgtgaataccaccaagtacccctacagagtgtgcagcatggcccagggcaccgacctgatcagattcgagcggaacatcgtgtgcaccagcatgaagcccatcaacgaggacctggacgagggcatcatggtggtgtacaagagaaacatcgtggcccacaccttcaaagtgcgggtgtaccagaaggtgctgaccttccggcggagctacgcctacatccacaccacatacctgctgggcagcaacaccgagtacgtggcccctcccatgtgggagatccaccacatcaacagccacagccagtgctacagcagctacagccgcgtgatcgccggcacagtgttcgtggcctaccaccgggacagctacgagaacaagaccatgcagctgatgcccgacgactacagcaacacccacagcaccagatacgtgaccgtgaaggaccagtggcacagcagaggcagcacctggctgtaccgggagacatgcaacctgaactgcatggtcaccatcaccaccgccagaagcaagtacccttaccacttcttcgccacctccaccggcgacgtggtggacatcagccccttctacaacggcaccaaccggaacgccagctacttcggcgagaacgccgacaagttcttcatcttccccaactacaccatcgtgtccgacttcggcagacccaacagcgctctggaaacccacagactggtggcctttctggaacgggccgacagcgtgatcagctgggacatccaggacgagaagaacgtgacctgccagctgaccttctgggaggcctctgagagaaccatcagaagcgaggccgaggacagctaccacttcagcagcgccaagatgaccgccaccttcctgagcaagaaacaggaagtgaacatgagcgactccgccctggactgcgtgagggacgaggccatcaacaagctgcagcagatcttcaacaccagctacaaccagacctacgagaagtatggcaatgtgtccgtgttcgagacaacaggcggcctggtggtgttctggcagggcatcaagcagaaaagcctggtggagctggaacggctcgccaaccggtccagcctgaacctgacccacaaccggaccaagcggagcaccgacggcaacaacgcaacccacctgtccaacatggaaagcgtgcacaacctggtgtacgcacagctgcagttcacctacgacaccctgcggggctacatcaacagagccctggcccagatcgccgaggcttggtgcgtggaccagcggcggaccctggaagtgttcaaagagctgtccaagatcaaccccagcgccatcctgagcgccatctacaacaagcctatcgccgccagattcatgggcgacgtgctgggcctggccagctgcgtgaccatcaaccagaccagcgtgaaggtgctgcgggacatgaacgtgaaagagagcccaggccgctgctactccagacccgtggtcatcttcaacttcgccaacagctcctacgtgcagtacggccagctgggcgaggacaacgagatcctgctggggaaccaccggaccgaggaatgccagctgcccagcctgaagatctttatcgccggcaacagcgcctacgagtatgtggactacctgttcaagcggatgatcgacctgagcagcatctccaccgtggacagcatgatcgccctggacatcgaccccctggaaaacaccgacttccgggtgctggaactgtacagccagaaagagctgcggagcagcaacgtgttcgacctggaagagatcatgcgggagttcaacagctacaagcagcgcgtgaaatacgtggaggacaaggtggtggaccccctgcctccttacctgaagggcctggacgacctgatgagcggactgggcgctgccggaaaagccgtgggagtggccattggagctgtgggcggagctgtggcctctgtcgtggaaggcgtcgccacctttctgaagaaccccttcggcgccttcaccatcatcctggtggccattgccgtcgtgatcatcacctacctgatctacacccggcagcggagactgtgtacccagcccctgcagaacctgttcccctacctggtgtccgccgatggcaccacagtgaccagcggctccaccaaggataccagcctgcaggccccacccagctacgaagagagcgtgtacaacagcggcagaaagggccctggccctcccagctctgatgccagcacagccgcccctccctacaccaacgagcaggcctaccagatgctgctggccctggctagactggatgccgagcagagggcccagcagaacggcaccgacagcctggatggcagaaccggcacccaggacaagggccagaagcccaacctgctggaccggctgcggcaccggaagaacggctaccggcacctgaaggacagcgacgaggaagagaacgtctgataa

SEQ ID NO: 26 - protein, 907 aa, Human herpesvirus 5
MESRIWCLVVCVNLCIVCLGAAVSSSSTRGTSATHSHHSSHTTSAAHSRSGSVSQRVTSSQTVSHGVNETIYNTTLKYGDVVGVNTTKYPYRVCSMAQGTDLIRFERNIVCTSMKPINEDLDEGIMVVYKRNIVAHTFKVRVYQKVLTFRRSYAYIHTTYLLGSNTEYVAPPMWEIHHINSHSQCYSSYSRVIAGTVFVAYHRDSYENKTMQLMPDDYSNTHSTRYVTVKDQWHSRGSTWLYRETCNLNCMVTITTARSKYPYHFFATSTGDVVDISPFYNGTNRNASYFGENADKFFIFPNYTIVSDFGRPNSALETHRLVAFLERADSVISWDIQDEKNVTCQLTFWEASERTIRSEAEDSYHFSSAKMTATFLSKKQEVNMSDSALDCVRDEAINKLQQIFNTSYNQTYEKYGNVSVFETTGGLVVFWQGIKQKSLVELERLANRSSLNLTHNRTKRSTDGNNATHLSNMESVHNLVYAQLQFTYDTLRGYINRALAQIAEAWCVDQRRTLEVFKELSKINPSAILSAIYNKPIAARFMGDVLGLASCVTINQTSVKVLRDMNVKESPGRCYSRPVVIFNFANSSYVQYGQLGEDNEILLGNHRTEECQLPSLKIFIAGNSAYEYVDYLFKRMIDLSSISTVDSMIALDIDPLENTDFRVLELYSQKELRSSNVFDLEEIMREFNSYKQRVKYVEDKVVDPLPPYLKGLDDLMSGLGAAGKAVGVAIGAVGGAVASVVEGVATFLKNPFGAFTIILVAIAVVIITYLIYTRQRRLCTQPLQNLFPYLVSADGTTVTSGSTKDTSLQAPPSYEESVYNSGRKGPGPPSSDASTAAPPYTNEQAYQMLLALARLDAEQRAQQNGTDSLDGRTGTQDKGQKPNLLDRLRHRKNGYRHLKDSDEEENV

SEQ ID NO: 27 - DNA, 2256 bp, Human herpesvirus 5
atggaaagccggatctggtgcctggtcgtgtgcgtgaacctgtgcatcgtgtgcctgggagccgccgtgagcagcagcagcaccagaggcaccagcgccacacacagccaccacagcagccacaccacctctgccgcccacagcagatccggcagcgtgtcccagagagtgaccagcagccagaccgtgtcccacggcgtgaacgagacaatctacaacaccaccctgaagtacggcgacgtcgtgggcgtgaataccaccaagtacccctacagagtgtgcagcatggcccagggcaccgacctgatcagattcgagcggaacatcgtgtgcaccagcatgaagcccatcaacgaggacctggacgagggcatcatggtggtgtacaagagaaacatcgtggcccacaccttcaaagtgcgggtgtaccagaaggtgctgaccttccggcggagctacgcctacatccacaccacatacctgctgggcagcaacaccgagtacgtggcccctcccatgtgggagatccaccacatcaacagccacagccagtgctacagcagctacagccgcgtgatcgccggcacagtgttcgtggcctaccaccgggacagctacgagaacaagaccatgcagctgatgcccgacgactacagcaacacccacagcaccagatacgtgaccgtgaaggaccagtggcacagcagaggcagcacctggctgtaccgggagacatgcaacctgaactgcatggtcaccatcaccaccgccagaagcaagtacccttaccacttcttcgccacctccaccggcgacgtggtggacatcagccccttctacaacggcaccaaccggaacgccagctacttcggcgagaacgccgacaagttcttcatcttccccaactacaccatcgtgtccgacttcggcagacccaacagcgctctggaaacccacagactggtggcctttctggaacgggccgacagcgtgatcagctgggacatccaggacgagaagaacgtgacctgccagctgaccttctgggaggcctctgagagaaccatcagaagcgaggccgaggacagctaccacttcagcagcgccaagatgaccgccaccttcctgagcaagaaacaggaagtgaacatgagcgactccgccctggactgcgtgagggacgaggccatcaacaagctgcagcagatcttcaacaccagctacaaccagacctacgagaagtatggcaatgtgtccgtgttcgagacaacaggcggcctggtggtgttctggcagggcatcaagcagaaaagcctggtggagctggaacggctcgccaaccggtccagcctgaacctgacccacaaccggaccaagcggagcaccgacggcaacaacgcaacccacctgtccaacatggaaagcgtgcacaacctggtgtacgcacagctgcagttcacctacgacaccctgcggggctacatcaacagagccctggcccagatcgccgaggcttggtgcgtggaccagcggcggaccctggaagtgttcaaagagctgtccaagatcaaccccagcgccatcctgagcgccatctacaacaagcctatcgccgccagattcatgggcgacgtgctgggcctggccagctgcgtgaccatcaaccagaccagcgtgaaggtgctgcgggacatgaacgtgaaagagagcccaggccgctgctactccagacccgtggtcatcttcaacttcgccaacagctcctacgtgcagtacggccagctgggcgaggacaacgagatcctgctggggaaccaccggaccgaggaatgccagctgcccagcctgaagatctttatcgccggcaacagcgcctacgagtatgtggactacctgttcaagcggatgatcgacctgagcagcatctccaccgtggacagcatgatcgccctggacatcgaccccctggaaaacaccgacttccgggtgctggaactgtacagccagaaagagctgcggagcagcaacgtgttcgacctggaagagatcatgcgggagttcaacagctacaagcagcgcgtgaaatacgtggaggacaaggtggtggaccccctgcctccttacctgaagggcctggacgacctgatgagcggactgggcgctgccggaaaagccgtgggagtggccattggagctgtgggcggagctgtggcctctgtcgtggaaggcgtcgccacctttctgaagaactgataa

SEQ ID NO: 28 - protein, 750 aa, Human herpesvirus 5
MESRIWCLVVCVNLCIVCLGAAVSSSSTRGTSATHSHHSSHTTSAAHSRSGSVSQRVTSSQTVSHGVNETIYNTTLKYGDVVGVNTTKYPYRVCSMAQGTDLIRFERNIVCTSMKPINEDLDEGIMVVYKRNIVAHTFKVRVYQKVLTFRRSYAYIHTTYLLGSNTEYVAPPMWEIHHINSHSQCYSSYSRVIAGTVFVAYHRDSYENKTMQLMPDDYSNTHSTRYVTVKDQWHSRGSTWLYRETCNLNCMVTITTARSKYPYHFFATSTGDVVDISPFYNGTNRNASYFGENADKFFIFPNYTIVSDFGRPNSALETHRLVAFLERADSVISWDIQDEKNVTCQLTFWEASERTIRSEAEDSYHFSSAKMTATFLSKKQEVNMSDSALDCVRDEAINKLQQIFNTSYNQTYEKYGNVSVFETTGGLVVFWQGIKQKSLVELERLANRSSLNLTHNRTKRSTDGNNATHLSNMESVHNLVYAQLQFTYDTLRGYINRALAQIAEAWCVDQRRTLEVFKELSKINPSAILSAIYNKPIAARFMGDVLGLASCVTINQTSVKVLRDMNVKESPGRCYSRPVVIFNFANSSYVQYGQLGEDNEILLGNHRTEECQLPSLKIFIAGNSAYEYVDYLFKRMIDLSSISTVDSMIALDIDPLENTDFRVLELYSQKELRSSNVFDLEEIMREFNSYKQRVKYVEDKVVDPLPPYLKGLDDLMSGLGAAGKAVGVAIGAVGGAVASVVEGVATFLKN

SEQ ID NO: 29 - DNA, 2082 bp, Human herpesvirus 5
atggaaagccggatctggtgcctggtcgtgtgcgtgaacctgtgcatcgtgtgcctgggagccgccgtgagcagcagcagcaccagaggcaccagcgccacacacagccaccacagcagccacaccacctctgccgcccacagcagatccggcagcgtgtcccagagagtgaccagcagccagaccgtgtcccacggcgtgaacgagacaatctacaacaccaccctgaagtacggcgacgtcgtgggcgtgaataccaccaagtacccctacagagtgtgcagcatggcccagggcaccgacctgatcagattcgagcggaacatcgtgtgcaccagcatgaagcccatcaacgaggacctggacgagggcatcatggtggtgtacaagagaaacatcgtggcccacaccttcaaagtgcgggtgtaccagaaggtgctgaccttccggcggagctacgcctacatccacaccacatacctgctgggcagcaacaccgagtacgtggcccctcccatgtgggagatccaccacatcaacagccacagccagtgctacagcagctacagccgcgtgatcgccggcacagtgttcgtggcctaccaccgggacagctacgagaacaagaccatgcagctgatgcccgacgactacagcaacacccacagcaccagatacgtgaccgtgaaggaccagtggcacagcagaggcagcacctggctgtaccgggagacatgcaacctgaactgcatggtcaccatcaccaccgccagaagcaagtacccttaccacttcttcgccacctccaccggcgacgtggtggacatcagccccttctacaacggcaccaaccggaacgccagctacttcggcgagaacgccgacaagttcttcatcttccccaactacaccatcgtgtccgacttcggcagacccaacagcgctctggaaacccacagactggtggcctttctggaacgggccgacagcgtgatcagctgggacatccaggacgagaagaacgtgacctgccagctgaccttctgggaggcctctgagagaaccatcagaagcgaggccgaggacagctaccacttcagcagcgccaagatgaccgccaccttcctgagcaagaaacaggaagtgaacatgagcgactccgccctggactgcgtgagggacgaggccatcaacaagctgcagcagatcttcaacaccagctacaaccagacctacgagaagtatggcaatgtgtccgtgttcgagacaacaggcggcctggtggtgttctggcagggcatcaagcagaaaagcctggtggagctggaacggctcgccaaccggtccagcctgaacctgacccacaaccggaccaagcggagcaccgacggcaacaacgcaacccacctgtccaacatggaaagcgtgcacaacctggtgtacgcacagctgcagttcacctacgacaccctgcggggctacatcaacagagccctggcccagatcgccgaggcttggtgcgtggaccagcggcggaccctggaagtgttcaaagagctgtccaagatcaaccccagcgccatcctgagcgccatctacaacaagcctatcgccgccagattcatgggcgacgtgctgggcctggccagctgcgtgaccatcaaccagaccagcgtgaaggtgctgcgggacatgaacgtgaaagagagcccaggccgctgctactccagacccgtggtcatcttcaacttcgccaacagctcctacgtgcagtacggccagctgggcgaggacaacgagatcctgctggggaaccaccggaccgaggaatgccagctgcccagcctgaagatctttatcgccggcaacagcgcctacgagtatgtggactacctgttcaagcggatgatcgacctgagcagcatctccaccgtggacagcatgatcgccctggacatcgaccccctggaaaacaccgacttccgggtgctggaactgtacagccagaaagagctgcggagcagcaacgtgttcgacctggaagagatcatgcgggagttcaacagctacaagcagtgataa

SEQ ID NO: 30 - protein, 692 aa, Human herpesvirus 5
MESRIWCLVVCVNLCIVCLGAAVSSSSTRGTSATHSHHSSHTTSAAHSRSGSVSQRVTSSQTVSHGVNETIYNTTLKYGDVVGVNTTKYPYRVCSMAQGTDLIRFERNIVCTSMKPINEDLDEGIMVVYKRNIVAHTFKVRVYQKVLTFRRSYAYIHTTYLLGSNTEYVAPPMWEIHHINSHSQCYSSYSRVIAGTVFVAYHRDSYENKTMQLMPDDYSNTHSTRYVTVKDQWHSRGSTWLYRETCNLNCMVTITTARSKYPYHFFATSTGDVVDISPFYNGTNRNASYFGENADKFFIFPNYTIVSDFGRPNSALETHRLVAFLERADSVISWDIQDEKNVTCQLTFWEASERTIRSEAEDSYHFSSAKMTATFLSKKQEVNMSDSALDCVRDEAINKLQQIFNTSYNQTYEKYGNVSVFETTGGLVVFWQGIKQKSLVELERLANRSSLNLTHNRTKRSTDGNNATHLSNMESVHNLVYAQLQFTYDTLRGYINRALAQIAEAWCVDQRRTLEVFKELSKINPSAILSAIYNKPIAARFMGDVLGLASCVTINQTSVKVLRDMNVKESPGRCYSRPVVIFNFANSSYVQYGQLGEDNEILLGNHRTEECQLPSLKIFIAGNSAYEYVDYLFKRMIDLSSISTVDSMIALDIDPLENTDFRVLELYSQKELRSSNVFDLEEIMREFNSYKQ

SEQ ID NO: 31 - DNA, 2232 bp, Human herpesvirus 5
atgaggcctggcctgccctcctacctgatcatcctggccgtgtgcctgttcagccacctgctgtccagcagatacggcgccgaggccgtgagcgagcccctggacaaggctttccacctgctgctgaacacctacggcagacccatccggtttctgcgggagaacaccacccagtgcacctacaacagcagcctgcggaacagcaccgtcgtgagagagaacgccatcagcttcaactttttccagagctacaaccagtactacgtgttccacatgcccagatgcctgtttgccggccctctggccgagcagttcctgaaccaggtggacctgaccgagacactggaaagataccagcagcggctgaatacctacgccctggtgtccaaggacctggccagctaccggtcctttagccagcagctcaaggctcaggatagcctcggcgagcagcctaccaccgtgccccctcccatcgacctgagcatcccccacgtgtggatgcctccccagaccacccctcacggctggaccgagagccacaccacctccggcctgcacagaccccacttcaaccagacctgcatcctgttcgacggccacgacctgctgtttagcaccgtgaccccctgcctgcaccagggcttctacctgatcgacgagctgagatacgtgaagatcaccctgaccgaggatttcttcgtggtcaccgtgtccatcgacgacgacacccccatgctgctgatcttcggccacctgcccagagtgctgttcaaggccccctaccagcgggacaacttcatcctgcggcagaccgagaagcacgagctgctggtgctggtcaagaaggaccagctgaaccggcactcctacctgaaggaccccgacttcctggacgccgccctggacttcaactacctggacctgagcgccctgctgagaaacagcttccacagatacgccgtggacgtgctgaagtccggacggtgccagatgctcgatcggcggaccgtggagatggccttcgcctatgccctcgccctgttcgccgctgccagacaggaagaggctggcgcccaggtgtcagtgcccagagccctggatagacaggccgccctgctgcagatccaggaattcatgatcacctgcctgagccagaccccccctagaaccaccctgctgctgtaccccacagccgtggatctggccaagagggccctgtggacccccaaccagatcaccgacatcacaagcctcgtgcggctcgtgtacatcctgagcaagcagaaccagcagcacctgatcccccagtgggccctgagacagatcgccgacttcgccctgaagctgcacaagacccatctggccagctttctgagcgccttcgccaggcaggaactgtacctgatgggcagcctggtccacagcatgctggtgcataccaccgagcggcgggagatcttcatcgtggagacaggcctgtgtagcctggccgagctgtcccactttacccagctgctggcccaccctcaccacgagtacctgagcgacctgtacaccccctgcagcagcagcggcagacgggaccacagcctggaacggctgaccagactgttccccgatgccaccgtgcctgctacagtgcctgccgccctgtccatcctgtccaccatgcagcccagcaccctggaaaccttccccgacctgttctgcctgcccctgggcgagagctttagcgccctgaccgtgtccgagcacgtgtcctacatcgtgaccaatcagtacctgatcaagggcatcagctaccccgtgtccaccacagtcgtgggccagagcctgatcatcacccagaccgacagccagaccaagtgcgagctgacccggaacatgcacaccacacacagcatcaccgtggccctgaacatcagcctggaaaactgcgctttctgtcagtctgccctgctggaatacgacgatacccagggcgtgatcaacatcatgtacatgcacgacagcgacgacgtgctgttcgccctggacccctacaacgaggtggtggtgtccagcccccggacccactacctgatgctgctgaagaacggcaccgtgctggaagtgaccgacgtggtggtggacgccaccgacagcagactgctgatgatgagcgtgtacgccctgagcgccatcatcggcatctacctgctgtaccggatgctgaaaacctgctgataa

SEQ ID NO: 32 - protein, 742 aa, Human herpesvirus 5
MRPGLPSYLIILAVCLFSHLLSSRYGAEAVSEPLDKAFHLLLNTYGRPIRFLRENTTQCTYNSSLRNSTVVRENAISFNFFQSYNQYYVFHMPRCLFAGPLAEQFLNQVDLTETLERYQQRLNTYALVSKDLASYRSFSQQLKAQDSLGEQPTTVPPPIDLSIPHVWMPPQTTPHGWTESHTTSGLHRPHFNQTCILFDGHDLLFSTVTPCLHQGFYLIDELRYVKITLTEDFFVVTVSIDDDTPMLLIFGHLPRVLFKAPYQRDNFILRQTEKHELLVLVKKDQLNRHSYLKDPDFLDAALDFNYLDLSALLRNSFHRYAVDVLKSGRCQMLDRRTVEMAFAYALALFAAARQEEAGAQVSVPRALDRQAALLQIQEFMITCLSQTPPRTTLLLYPTAVDLAKRALWTPNQITDITSLVRLVYILSKQNQQHLIPQWALRQIADFALKLHKTHLASFLSAFARQELYLMGSLVHSMLVHTTERREIFIVETGLCSLAELSHFTQLLAHPHHEYLSDLYTPCSSSGRRDHSLERLTRLFPDATVPATVPAALSILSTMQPSTLETFPDLFCLPLGESFSALTVSEHVSYIVTNQYLIKGISYPVSTTVVGQSLIITQTDSQTKCELTRNMHTTHSITVALNISLENCAFCQSALLEYDDTQGVINIMYMHDSDDVLFALDPYNEVVVSSPRTHYLMLLKNGTVLEVTDVVVDATDSRLLMMSVYALSAIIGIYLLYRMLKTC

SEQ ID NO: 33 - DNA, 2151 bp, Human herpesvirus 5
atgaggcctggcctgccctcctacctgatcatcctggccgtgtgcctgttcagccacctgctgtccagcagatacggcgccgaggccgtgagcgagcccctggacaaggctttccacctgctgctgaacacctacggcagacccatccggtttctgcgggagaacaccacccagtgcacctacaacagcagcctgcggaacagcaccgtcgtgagagagaacgccatcagcttcaactttttccagagctacaaccagtactacgtgttccacatgcccagatgcctgtttgccggccctctggccgagcagttcctgaaccaggtggacctgaccgagacactggaaagataccagcagcggctgaatacctacgccctggtgtccaaggacctggccagctaccggtcctttagccagcagctcaaggctcaggatagcctcggcgagcagcctaccaccgtgccccctcccatcgacctgagcatcccccacgtgtggatgcctccccagaccacccctcacggctggaccgagagccacaccacctccggcctgcacagaccccacttcaaccagacctgcatcctgttcgacggccacgacctgctgtttagcaccgtgaccccctgcctgcaccagggcttctacctgatcgacgagctgagatacgtgaagatcaccctgaccgaggatttcttcgtggtcaccgtgtccatcgacgacgacacccccatgctgctgatcttcggccacctgcccagagtgctgttcaaggccccctaccagcgggacaacttcatcctgcggcagaccgagaagcacgagctgctggtgctggtcaagaaggaccagctgaaccggcactcctacctgaaggaccccgacttcctggacgccgccctggacttcaactacctggacctgagcgccctgctgagaaacagcttccacagatacgccgtggacgtgctgaagtccggacggtgccagatgctcgatcggcggaccgtggagatggccttcgcctatgccctcgccctgttcgccgctgccagacaggaagaggctggcgcccaggtgtcagtgcccagagccctggatagacaggccgccctgctgcagatccaggaattcatgatcacctgcctgagccagaccccccctagaaccaccctgctgctgtaccccacagccgtggatctggccaagagggccctgtggacccccaaccagatcaccgacatcacaagcctcgtgcggctcgtgtacatcctgagcaagcagaaccagcagcacctgatcccccagtgggccctgagacagatcgccgacttcgccctgaagctgcacaagacccatctggccagctttctgagcgccttcgccaggcaggaactgtacctgatgggcagcctggtccacagcatgctggtgcataccaccgagcggcgggagatcttcatcgtggagacaggcctgtgtagcctggccgagctgtcccactttacccagctgctggcccaccctcaccacgagtacctgagcgacctgtacaccccctgcagcagcagcggcagacgggaccacagcctggaacggctgaccagactgttccccgatgccaccgtgcctgctacagtgcctgccgccctgtccatcctgtccaccatgcagcccagcaccctggaaaccttccccgacctgttctgcctgcccctgggcgagagctttagcgccctgaccgtgtccgagcacgtgtcctacatcgtgaccaatcagtacctgatcaagggcatcagctaccccgtgtccaccacagtcgtgggccagagcctgatcatcacccagaccgacagccagaccaagtgcgagctgacccggaacatgcacaccacacacagcatcaccgtggccctgaacatcagcctggaaaactgcgctttctgtcagtctgccctgctggaatacgacgatacccagggcgtgatcaacatcatgtacatgcacgacagcgacgacgtgctgttcgccctggacccctacaacgaggtggtggtgtccagcccccggacccactacctgatgctgctgaagaacggcaccgtgctggaagtgaccgacgtggtggtggacgccaccgactgataa

SEQ ID NO: 34 - protein, 715 aa, Human herpesvirus 5
MRPGLPSYLIILAVCLFSHLLSSRYGAEAVSEPLDKAFHLLLNTYGRPIRFLRENTTQCTYNSSLRNSTVVRENAISFNFFQSYNQYYVFHMPRCLFAGPLAEQFLNQVDLTETLERYQQRLNTYALVSKDLASYRSFSQQLKAQDSLGEQPTTVPPPIDLSIPHVWMPPQTTPHGWTESHTTSGLHRPHFNQTCILFDGHDLLFSTVTPCLHQGFYLIDELRYVKITLTEDFFVVTVSIDDDTPMLLIFGHLPRVLFKAPYQRDNFILRQTEKHELLVLVKKDQLNRHSYLKDPDFLDAALDFNYLDLSALLRNSFHRYAVDVLKSGRCQMLDRRTVEMAFAYALALFAAARQEEAGAQVSVPRALDRQAALLQIQEFMITCLSQTPPRTTLLLYPTAVDLAKRALWTPNQITDITSLVRLVYILSKQNQQHLIPQWALRQIADFALKLHKTHLASFLSAFARQELYLMGSLVHSMLVHTTERREIFIVETGLCSLAELSHFTQLLAHPHHEYLSDLYTPCSSSGRRDHSLERLTRLFPDATVPATVPAALSILSTMQPSTLETFPDLFCLPLGESFSALTVSEHVSYIVTNQYLIKGISYPVSTTVVGQSLIITQTDSQTKCELTRNMHTTHSITVALNISLENCAFCQSALLEYDDTQGVINIMYMHDSDDVLFALDPYNEVVVSSPRTHYLMLLKNGTVLEVTDVVVDATD

SEQ ID NO: 35 - DNA, 840 bp, Human herpesvirus 5
atgtgcagaaggcccgactgcggcttcagcttcagccctggacccgtgatcctgctgtggtgctgcctgctgctgcctatcgtgtcctctgccgccgtgtctgtggcccctacagccgccgagaaggtgccagccgagtgccccgagctgaccagaagatgcctgctgggcgaggtgttcgagggcgacaagtacgagagctggctgcggcccctggtcaacgtgaccggcagagatggccccctgagccagctgatccggtacagacccgtgacccccgaggccgccaatagcgtgctgctggacgaggccttcctggataccctggccctgctgtacaacaaccccgaccagctgagagccctgctgaccctgctgtccagcgacaccgcccccagatggatgaccgtgatgcggggctacagcgagtgtggagatggcagccctgccgtgtacacctgcgtggacgacctgtgcagaggctacgacctgaccagactgagctacggccggtccatcttcacagagcacgtgctgggcttcgagctggtgccccccagcctgttcaacgtggtggtggccatccggaacgaggccaccagaaccaacagagccgtgcggctgcctgtgtctacagccgctgcacctgagggcatcacactgttctacggcctgtacaacgccgtgaaagagttctgcctccggcaccagctggatccccccctgctgagacacctggacaagtactacgccggcctgcccccagagctgaagcagaccagagtgaacctgcccgcccacagcagatatggccctcaggccgtggacgccagatgataa

SEQ ID NO: 36 - protein, 278 aa, Human herpesvirus 5
MCRRPDCGFSFSPGPVILLWCCLLLPIVSSAAVSVAPTAAEKVPAECPELTRRCLLGEVFEGDKYESWLRPLVNVTGRDGPLSQLIRYRPVTPEAANSVLLDEAFLDTLALLYNNPDQLRALLTLLSSDTAPRWMTVMRGYSECGDGSPAVYTCVDDLCRGYDLTRLSYGRSIFTEHVLGFELVPPSLFNVVVAIRNEATRTNRAVRLPVSTAAAPEGITLFYGLYNAVKEFCLRHQLDPPLLRHLDKYYAGLPPELKQTRVNLPAHSRYGPQAVDAR

SEQ ID NO: 37 - DNA, 1119 bp, Human herpesvirus 5
atggcccccagccacgtggacaaagtgaacacccggacttggagcgccagcatcgtgttcatggtgctgaccttcgtgaacgtgtccgtgcacctggtgctgtccaacttcccccacctgggctacccctgcgtgtactaccacgtggtggacttcgagcggctgaacatgagcgcctacaacgtgatgcacctgcacacccccatgctgtttctggacagcgtgcagctcgtgtgctacgccgtgttcatgcagctggtgtttctggccgtgaccatctactacctcgtgtgctggatcaagatcagcatgcggaaggacaagggcatgagcctgaaccagagcacccgggacatcagctacatgggcgacagcctgaccgccttcctgttcatcctgagcatggacaccttccagctgttcaccctgaccatgagcttccggctgcccagcatgatcgccttcatggccgccgtgcactttttctgtctgaccatcttcaacgtgtccatggtcacccagtaccggtcctacaagcggagcctgttcttcttctcccggctgcaccccaagctgaagggcaccgtgcagttccggaccctgatcgtgaacctggtggaggtggccctgggcttcaataccaccgtggtggctatggccctgtgctacggcttcggcaacaacttcttcgtgcggaccggccatatggtgctggccgtgttcgtggtgtacgccatcatcagcatcatctactttctgctgatcgaggccgtgttcttccagtacgtgaaggtgcagttcggctaccatctgggcgcctttttcggcctgtgcggcctgatctaccccatcgtgcagtacgacaccttcctgagcaacgagtaccggaccggcatcagctggtccttcggaatgctgttcttcatctgggccatgttcaccacctgcagagccgtgcggtacttcagaggcagaggcagcggctccgtgaagtaccaggccctggccacagcctctggcgaagaggtggccgccctgagccaccacgacagcctggaaagcagacggctgcgggaggaagaggacgacgacgacgaggacttcgaggacgcctgataa

SEQ ID NO: 38 - protein, 371 aa, Human herpesvirus 5
MAPSHVDKVNTRTWSASIVFMVLTFVNVSVHLVLSNFPHLGYPCVYYHVVDFERLNMSAYNVMHLHTPMLFLDSVQLVCYAVFMQLVFLAVTIYYLVCWIKISMRKDKGMSLNQSTRDISYMGDSLTAFLFILSMDTFQLFTLTMSFRLPSMIAFMAAVHFFCLTIFNVSMVTQYRSYKRSLFFFSRLHPKLKGTVQFRTLIVNLVEVALGFNTTVVAMALCYGFGNNFFVRTGHMVLAVFVVYAIISIIYFLLIEAVFFQYVKVQFGYHLGAFFGLCGLIYPIVQYDTFLSNEYRTGISWSFGMLFFIWAMFTTCRAVRYFRGRGSGSVKYQALATASGEEVAALSHHDSLESRRLREEEDDDDEDFEDA

SEQ ID NO: 39 - DNA, 411 bp, Human herpesvirus 5
atggaatggaacaccctggtcctgggcctgctggtgctgtctgtcgtggccagcagcaacaacacatccacagccagcacccctagacctagcagcagcacccacgccagcactaccgtgaaggctaccaccgtggccaccacaagcaccaccactgctaccagcaccagctccaccacctctgccaagcctggctctaccacacacgaccccaacgtgatgaggccccacgcccacaacgacttctacaacgctcactgcaccagccacatgtacgagctgtccctgagcagctttgccgcctggtggaccatgctgaacgccctgatcctgatgggcgccttctgcatcgtgctgcggcactgctgcttccagaacttcaccgccaccaccaccaagggctactgataa

SEQ ID NO: 40 - protein, 135 aa, Human herpesvirus 5
MEWNTLVLGLLVLSVVASSNNTSTASTPRPSSSTHASTTVKATTVATTSTTTATSTSSTTSAKPGSTTHDPNVMRPHAHNDFYNAHCTSHMYELSLSSFAAWWTMLNALILMGAFCIVLRHCCFQNFTATTTKGY

SEQ ID NO: 41 - DNA, 1422 bp, Human herpesvirus 5
atgggcaagaaagaaatgatcatggtcaagggcatccccaagatcatgctgctgattagcatcacctttctgctgctgtccctgatcaactgcaacgtgctggtcaacagccggggcaccagaagatcctggccctacaccgtgctgtcctaccggggcaaagagatcctgaagaagcagaaagaggacatcctgaagcggctgatgagcaccagcagcgacggctaccggttcctgatgtaccccagccagcagaaattccacgccatcgtgatcagcatggacaagttcccccaggactacatcctggccggacccatccggaacgacagcatcacccacatgtggttcgacttctacagcacccagctgcggaagcccgccaaatacgtgtacagcgagtacaaccacaccgcccacaagatcaccctgaggcctcccccttgtggcaccgtgcccagcatgaactgcctgagcgagatgctgaacgtgtccaagcggaacgacaccggcgagaagggctgcggcaacttcaccaccttcaaccccatgttcttcaacgtgccccggtggaacaccaagctgtacatcggcagcaacaaagtgaacgtggacagccagaccatctactttctgggcctgaccgccctgctgctgagatacgcccagcggaactgcacccggtccttctacctggtcaacgccatgagccggaacctgttccgggtgcccaagtacatcaacggcaccaagctgaagaacaccatgcggaagctgaagcggaagcaggccctggtcaaagagcagccccagaagaagaacaagaagtcccagagcaccaccaccccctacctgagctacaccacctccaccgccttcaacgtgaccaccaacgtgacctacagcgccacagccgccgtgaccagagtggccacaagcaccaccggctaccggcccgacagcaactttatgaagtccatcatggccacccagctgagagatctggccacctgggtgtacaccaccctgcggtacagaaacgagcccttctgcaagcccgaccggaacagaaccgccgtgagcgagttcatgaagaatacccacgtgctgatcagaaacgagacaccctacaccatctacggcaccctggacatgagcagcctgtactacaacgagacaatgagcgtggagaacgagacagccagcgacaacaacgaaaccacccccacctcccccagcacccggttccagcggaccttcatcgaccccctgtgggactacctggacagcctgctgttcctggacaagatccggaacttcagcctgcagctgcccgcctacggcaatctgaccccccctgagcacagaagggccgccaacctgagcaccctgaacagcctgtggtggtggagccagtgataa

SEQ ID NO: 42 - protein, 472 aa, Human herpesvirus 5
MGKKEMIMVKGIPKIMLLISITFLLLSLINCNVLVNSRGTRRSWPYTVLSYRGKEILKKQKEDILKRLMSTSSDGYRFLMYPSQQKFHAIVISMDKFPQDYILAGPIRNDSITHMWFDFYSTQLRKPAKYVYSEYNHTAHKITLRPPPCGTVPSMNCLSEMLNVSKRNDTGEKGCGNFTTFNPMFFNVPRWNTKLYIGSNKVNVDSQTIYFLGLTALLLRYAQRNCTRSFYLVNAMSRNLFRVPKYINGTKLKNTMRKLKRKQALVKEQPQKKNKKSQSTTTPYLSYTTSTAFNVTTNVTYSATAAVTRVATSTTGYRPDSNFMKSIMATQLRDLATWVYTTLRYRNEPFCKPDRNRTAVSEFMKNTHVLIRNETPYTIYGTLDMSSLYYNETMSVENETASDNNETTPTSPSTRFQRTFIDPLWDYLDSLLFLDKIRNFSLQLPAYGNLTPPEHRRAANLSTLNSLWWWSQ

SEQ ID NO: 43 - DNA, 519 bp, Human herpesvirus 5
atgagccccaaggacctgacccccttcctgacaaccctgtggctgctcctgggccatagcagagtgcctagagtgcgggccgaggaatgctgcgagttcatcaacgtgaaccacccccccgagcggtgctacgacttcaagatgtgcaaccggttcaccgtggccctgagatgccccgacggcgaagtgtgctacagccccgagaaaaccgccgagatccggggcatcgtgaccaccatgacccacagcctgacccggcaggtggtgcacaacaagctgaccagctgcaactacaaccccctgtacctggaagccgacggccggatcagatgcggcaaagtgaacgacaaggcccagtacctgctgggagccgccggaagcgtgccctaccggtggatcaacctggaatacgacaagatcacccggatcgtgggcctggaccagtacctggaaagcgtgaagaagcacaagcggctggacgtgtgcagagccaagatgggctacatgctgcagtgataa

SEQ ID NO: 44 - protein, 171 aa, Human herpesvirus 5
MSPKDLTPFLTTLWLLLGHSRVPRVRAEECCEFINVNHPPERCYDFKMCNRFTVALRCPDGEVCYSPEKTAEIRGIVTTMTHSLTRQVVHNKLTSCNYNPLYLEADGRIRCGKVNDKAQYLLGAAGSVPYRWINLEYDKITRIVGLDQYLESVKKHKRLDVCRAKMGYMLQ

SEQ ID NO: 45 - DNA, 648 bp, Human herpesvirus 5
atgctgcggctgctgctgagacaccacttccactgcctgctgctgtgtgccgtgtgggccaccccttgtctggccagcccttggagcaccctgaccgccaaccagaaccctagccccccttggtccaagctgacctacagcaagccccacgacgccgccaccttctactgcccctttctgtaccccagccctcccagaagccccctgcagttcagcggcttccagagagtgtccaccggccctgagtgccggaacgagacactgtacctgctgtacaaccgggagggccagacactggtggagcggagcagcacctgggtgaaaaaagtgatctggtatctgagcggccggaaccagaccatcctgcagcggatgcccagaaccgccagcaagcccagcgacggcaacgtgcagatcagcgtggaggacgccaaaatcttcggcgcccacatggtgcccaagcagaccaagctgctgagattcgtggtcaacgacggcaccagatatcagatgtgcgtgatgaagctggaaagctgggcccacgtgttccgggactactccgtgagcttccaggtccggctgaccttcaccgaggccaacaaccagacctacaccttctgcacccaccccaacctgatcgtgtgataa

SEQ ID NO: 46 - protein, 214 aa, Human herpesvirus 5
MLRLLLRHHFHCLLLCAVWATPCLASPWSTLTANQNPSPPWSKLTYSKPHDAATFYCPFLYPSPPRSPLQFSGFQRVSTGPECRNETLYLLYNREGQTLVERSSTWVKKVIWYLSGRNQTILQRMPRTASKPSDGNVQISVEDAKIFGAHMVPKQTKLLRFVVNDGTRYQMCVMKLESWAHVFRDYSVSFQVRLTFTEANNQTYTFCTHPNLIV

SEQ ID NO: 47 - DNA, 393 bp, Human herpesvirus 5
atgcggctgtgcagagtgtggctgtccgtgtgcctgtgtgccgtggtgctgggccagtgccagagagagacagccgagaagaacgactactaccgggtgccccactactgggatgcctgcagcagagccctgcccgaccagacccggtacaaatacgtggagcagctcgtggacctgaccctgaactaccactacgacgccagccacggcctggacaacttcgacgtgctgaagcggatcaacgtgaccgaggtgtccctgctgatcagcgacttccggcggcagaacagaagaggcggcaccaacaagcggaccaccttcaacgccgctggctctctggcccctcacgccagatccctggaattcagcgtgcggctgttcgccaactgataa

SEQ ID NO: 48 - protein, 129 aa, Human herpesvirus 5
MRLCRVWLSVCLCAVVLGQCQRETAEKNDYYRVPHYWDACSRALPDQTRYKYVEQLVDLTLNYHYDASHGLDNFDVLKRINVTEVSLLISDFRRQNRRGGTNKRTTFNAAGSLAPHARSLEFSVRLFAN

SEQ ID NO: 49 - DNA, 550 bp, Encephalomyocarditis virus
aacgttactggccgaagccgcttggaataaggccggtgtgcgtttgtctatatgttattttccaccatattgccgtcttttggcaatgtgagggcccggaaacctggccctgtcttcttgacgagcattcctaggggtctttcccctctcgccaaaggaatgcaaggtctgttgaatgtcgtgaaggaagcagttcctctggaagcttcttgaagacaaacaacgtctgtagcgaccctttgcaggcagcggaaccccccacctggcgacaggtgcctctgcggccaaaagccacgtgtataagatacacctgcaaaggcggcacaaccccagtgccacgttgtgagttggatagttgtggaaagagtcaaatggctctcctcaagcgtattcaacaaggggctgaaggatgcccagaaggtaccccattgtatgggatctgatctggggcctcggtgcacatgctttacatgtgtttagtcgaggttaaaaaaacgtctaggccccccgaaccacggggacgtggttttcctttgaaaaacacgataat

SEQ ID NO: 50 - DNA, 678 bp, Human enterovirus 71
gtacctttgtacgcctgttttataccccctccctgatttgcaacttagaagcaacgcaaaccagatcaatagtaggtgtgacataccagtcgcatcttgatcaagcacttctgtatccccggaccgagtatcaatagactgtgcacacggttgaaggagaaaacgtccgttacccggctaactacttcgagaagcctagtaacgccattgaagttgcagagtgtttcgctcagcactccccccgtgtagatcaggtcgatgagtcaccgcattccccacgggcgaccgtggcggtggctgcgttggcggcctgcctatggggtaacccataggacgctctaatacggacatggcgtgaagagtctattgagctagttagtagtcctccggcccctgaatgcggctaatcctaactgcggagcacatacccttaatccaaagggcagtgtgtcgtaacgggcaactctgcagcggaaccgactactttgggtgtccgtgtttctttttattcttgtattggctgcttatggtgacaattaaagaattgttaccatatagctattggattggccatccagtgtcaaacagagctattgtatatctctttgttggattcacacctctcactcttgaaacgttacacaccctcaattacattatactgctgaacacgaagcg

SEQ ID NO: 51 - DNA, 24 bp, Venezuelan equine encephalitis virus
ctctctacggctaacctgaatgga

SEQ ID NO: 52 - DNA, 14071 bp, Artificial Sequence
  source: /note="Description of Artificial Sequence: Synthetic polynucleotide"
cgcgtcggctacaattaatacataaccttatgtatcatacacatacgatttaggtgacactatagatgggcggcgcatgagagaagcccagaccaattacctacccaaaatggagaaagttcacgttgacatcgaggaagacagcccattcctcagagctttgcagcggagcttcccgcagtttgaggtagaagccaagcaggtcactgataatgaccatgctaatgccagagcgttttcgcatctggcttcaaaactgatcgaaacggaggtggacccatccgacacgatccttgacattggaagtgcgcccgcccgcagaatgtattctaagcacaagtatcattgtatctgtccgatgagatgtgcggaagatccggacagattgtataagtatgcaactaagctgaagaaaaactgtaaggaaataactgataaggaattggacaagaaaatgaaggagctcgccgccgtcatgagcgaccctgacctggaaactgagactatgtgcctccacgacgacgagtcgtgtcgctacgaagggcaagtcgctgtttaccaggatgtatacgcggttgacggaccgacaagtctctatcaccaagccaataagggagttagagtcgcctactggataggctttgacaccaccccttttatgtttaagaacttggctggagcatatccatcatactctaccaactgggccgacgaaaccgtgttaacggctcgtaacataggcctatgcagctctgacgttatggagcggtcacgtagagggatgtccattcttagaaagaagtatttgaaaccatccaacaatgttctattctctgttggctcgaccatctaccacgagaagagggacttactgaggagctggcacctgccgtctgtatttcacttacgtggcaagcaaaattacacatgtcggtgtgagactatagttagttgcgacgggtacgtcgttaaaagaatagctatcagtccaggcctgtatgggaagccttcaggctatgctgctacgatgcaccgcgagggattcttgtgctgcaaagtgacagacacattgaacggggagagggtctcttttcccgtgtgcacgtatgtgccagctacattgtgtgaccaaatgactggcatactggcaacagatgtcagtgcggacgacgcgcaaaaactgctggttgggctcaaccagcgtatagtcgtcaacggtcgcacccagagaaacaccaataccatgaaaaattaccttttgcccgtagtggcccaggcatttgctaggtgggcaaaggaatataaggaagatcaagaagatgaaaggccactaggactacgagatagacagttagtcatggggtgttgttgggcttttagaaggcacaagataacatctatttataagcgcccggatacccaaaccatcatcaaagtgaacagcgatttccactcattcgtgctgcccaggataggcagtaacacattggagatcgggctgagaacaagaatcaggaaaatgttagaggagcacaaggagccgtcacctctcattaccgccgaggacgtacaagaagctaagtgcgcagccgatgaggctaaggaggtgcgtgaagccgaggagttgcgcgcagctctaccacctttggcagctgatgttgaggagcccactctggaagccgatgtagacttgatgttacaagaggctggggccggctcagtggagacacctcgtggcttgataaaggttaccagctacgctggcgaggacaagatcggctcttacgctgtgctttctccgcaggctgtactcaagagtgaaaaattatcttgcatccaccctctcgctgaacaagtcatagtgataacacactctggccgaaaagggcgttatgccgtggaaccataccatggtaaagtagtggtgccagagggacatgcaatacccgtccaggactttcaagctctgagtgaaagtgccaccattgtgtacaacgaacgtgagttcgtaaacaggtacctgcaccatattgccacacatggaggagcgctgaacactgatgaagaatattacaaaactgtcaagcccagcgagcacgacggcgaatacctgtacgacatcgacaggaaacagtgcgtcaagaaagaactagtcactgggctagggctcacaggcgagctggtggatcctcccttccatgaattcgcctacgagagtctgagaacacgaccagccgctccttaccaagtaccaaccataggggtgtatggcgtgccaggatcaggcaagtctggcatcattaaaagcgcagtcaccaaaaaagatctagtggtgagcgccaagaaagaaaactgtgcagaaattataagggacgtcaagaaaatgaaagggctggacgtcaatgccagaactgtggactcagtgctcttgaatggatgcaaacaccccgtagagaccctgtatattgacgaagcttttgcttgtcatgcaggtactctcagagcgctcatagccattataagacctaaaaaggcagtgctctgcggggatcccaaacagtgcggtttttttaacatgatgtgcctgaaagtgcattttaaccacgagatttgcacacaagtcttccacaaaagcatctctcgccgttgcactaaatctgtgacttcggtcgtctcaaccttgttttacgacaaaaaaatgagaacgacgaatccgaaagagactaagattgtgattgacactaccggcagtaccaaacctaagcaggacgatctcattctcacttgtttcagagggtgggtgaagcagttgcaaatagattacaaaggcaacgaaataatgacggcagctgcctctcaagggctgacccgtaaaggtgtgtatgccgttcggtacaaggtgaatgaaaatcctctgtacgcacccacctcagaacatgtgaacgtcctactgacccgcacggaggaccgcatcgtgtggaaaacactagccggcgacccatggataaaaacactgactgccaagtaccctgggaatttcactgccacgatagaggagtggcaagcagagcatgatgccatcatgaggcacatcttggagagaccggaccctaccgacgtcttccagaataaggcaaacgtgtgttgggccaaggctttagtgccggtgctgaagaccgctggcatagacatgaccactgaacaatggaacactgtggattattttgaaacggacaaagctcactcagcagagatagtattgaaccaactatgcgtgaggttctttggactcgatctggactccggtctattttctgcacccactgttccgttatccattaggaataatcactgggataactccccgtcgcctaacatgtacgggctgaataaagaagtggtccgtcagctctctcgcaggtacccacaactgcctcgggcagttgccactggaagagtctatgacatgaacactggtacactgcgcaattatgatccgcgcataaacctagtacctgtaaacagaagactgcctcatgctttagtcctccaccataatgaacacccacagagtgacttttcttcattcgtcagcaaattgaagggcagaactgtcctggtggtcggggaaaagttgtccgtcccaggcaaaatggttgactggttgtcagaccggcctgaggctaccttcagagctcggctggatttaggcatcccaggtgatgtgcccaaatatgacataatatttgttaatgtgaggaccccatataaataccatcactatcagcagtgtgaagaccatgccattaagcttagcatgttgaccaagaaagcttgtctgcatctgaatcccggcggaacctgtgtcagcataggttatggttacgctgacagggccagcgaaagcatcattggtgctatagcgcggcagttcaagttttcccgggtatgcaaaccgaaatcctcacttgaagagacggaagttctgtttgtattcattgggtacgatcgcaaggcccgtacgcacaatccttacaagctttcatcaaccttgaccaacatttatacaggttccagactccacgaagccggatgtgcaccctcatatcatgtggtgcgaggggatattgccacggccaccgaaggagtgattataaatgctgctaacagcaaaggacaacctggcggaggggtgtgcggagcgctgtataagaaattcccggaaagcttcgatttacagccgatcgaagtaggaaaagcgcgactggtcaaaggtgcagctaaacatatcattcatgccgtaggaccaaacttcaacaaagtttcggaggttgaaggtgacaaacagttggcagaggcttatgagtccatcgctaagattgtcaacgataacaattacaagtcagtagcgattccactgttgtccaccggcatcttttccgggaacaaagatcgactaacccaatcattgaaccatttgctgacagctttagacaccactgatgcagatgtagccatatactgcagggacaagaaatgggaaatgactctcaaggaagcagtggctaggagagaagcagtggaggagatatgcatatccgacgactcttcagtgacagaacctgatgcagagctggtgagggtgcatccgaagagttctttggctggaaggaagggctacagcacaagcgatggcaaaactttctcatatttggaagggaccaagtttcaccaggcggccaaggatatagcagaaattaatgccatgtggcccgttgcaacggaggccaatgagcaggtatgcatgtatatcctcggagaaagcatgagcagtattaggtcgaaatgccccgtcgaagagtcggaagcctcctcaccacctagcacgctgccttgcttgtgcatccatgccatgactccagaaagagtacagcgcctaaaagcctcacgtccagaacaaattactgtgtgctcatcctttccattgccgaagtatagaatcactggtgtgcagaagatccaatgctcccagcctatattgttctcaccgaaagtgcctgcgtatattcatccaaggaagtatctcgtggaaacaccaccggtagacgagactccggagccatcggcagagaaccaatccacagaggggacacctgaacaaccaccacttataaccgaggatgagaccaggactagaacgcctgagccgatcatcatcgaagaggaagaagaggatagcataagtttgctgtcagatggcccgacccaccaggtgctgcaagtcgaggcagacattcacgggccgccctctgtatctagctcatcctggtccattcctcatgcatccgactttgatgtggacagtttatccatacttgacaccctggagggagctagcgtgaccagcggggcaacgtcagccgagactaactcttacttcgcaaagagtatggagtttctggcgcgaccggtgcctgcgcctcgaacagtattcaggaaccctccacatcccgctccgcgcacaagaacaccgtcacttgcacccagcagggcctgctcgagagggatcacgggagaaaccgtgggatacgcggttacacacaatagcgagggcttcttgctatgcaaagttactgacacagtaaaaggagaacgggtatcgttccctgtgtgcacgtacatcccggccaccataaactcgagaaccagcctggtctccaacccgccaggcgtaaatagggtgattacaagagaggagtttgaggcgttcgtagcacaacaacaatgacggtttgatgcgggtgcatacatcttttcctccgacaccggtcaagggcatttacaacaaaaatcagtaaggcaaacggtgctatccgaagtggtgttggagaggaccgaattggagatttcgtatgccccgcgcctcgaccaagaaaaagaagaattactacgcaagaaattacagttaaatcccacacctgctaacagaagcagataccagtccaggaaggtggagaacatgaaagccataacagctagacgtattctgcaaggcctagggcattatttgaaggcagaaggaaaagtggagtgctaccgaaccctgcatcctgttcctttgtattcatctagtgtgaaccgtgccttttcaagccccaaggtcgcagtggaagcctgtaacgccatgttgaaagagaactttccgactgtggcttcttactgtattattccagagtacgatgcctatttggacatggttgacggagcttcatgctgcttagacactgccagtttttgccctgcaaagctgcgcagctttccaaagaaacactcctatttggaacccacaatacgatcggcagtgccttcagcgatccagaacacgctccagaacgtcctggcagctgccacaaaaagaaattgcaatgtcacgcaaatgagagaattgcccgtattggattcggcggcctttaatgtggaatgcttcaagaaatatgcgtgtaataatgaatattgggaaacgtttaaagaaaaccccatcaggcttactgaagaaaacgtggtaaattacattaccaaattaaaaggaccaaaagctgctgctctttttgcgaagacacataatttgaatatgttgcaggacataccaatggacaggtttgtaatggacttaaagagagacgtgaaagtgactccaggaacaaaacatactgaagaacggcccaaggtacaggtgatccaggctgccgatccgctagcaacagcgtatctgtgcggaatccaccgagagctggttaggagattaaatgcggtcctgcttccgaacattcatacactgtttgatatgtcggctgaagactttgacgctattatagccgagcacttccagcctggggattgtgttctggaaactgacatcgcgtcgtttgataaaagtgaggacgacgccatggctctgaccgcgttaatgattctggaagacttaggtgtggacgcagagctgttgacgctgattgaggcggctttcggcgaaatttcatcaatacatttgcccactaaaactaaatttaaattcggagccatgatgaaatctggaatgttcctcacactgtttgtgaacacagtcattaacattgtaatcgcaagcagagtgttgagagaacggctaaccggatcaccatgtgcagcattcattggagatgacaatatcgtgaaaggagtcaaatcggacaaattaatggcagacaggtgcgccacctggttgaatatggaagtcaagattatagatgctgtggtgggcgagaaagcgccttatttctgtggagggtttattttgtgtgactccgtgaccggcacagcgtgccgtgtggcagaccccctaaaaaggctgtttaagcttggcaaacctctggcagcagacgatgaacatgatgatgacaggagaagggcattgcatgaagagtcaacacgctggaaccgagtgggtattctttcagagctgtgcaaggcagtagaatcaaggtatgaaaccgtaggaacttccatcatagttatggccatgactactctagctagcagtgttaaatcattcagctacctgagaggggcccctataactctctacggctaacctgaatggactacgacatagtctagtcgacgccaccatgaggcctggcctgccctcctacctgatcatcctggccgtgtgcctgttcagccacctgctgtccagcagatacggcgccgaggccgtgagcgagcccctggacaaggctttccacctgctgctgaacacctacggcagacccatccggtttctgcgggagaacaccacccagtgcacctacaacagcagcctgcggaacagcaccgtcgtgagagagaacgccatcagcttcaactttttccagagctacaaccagtactacgtgttccacatgcccagatgcctgtttgccggccctctggccgagcagttcctgaaccaggtggacctgaccgagacactggaaagataccagcagcggctgaatacctacgccctggtgtccaaggacctggccagctaccggtcctttagccagcagctcaaggctcaggatagcctcggcgagcagcctaccaccgtgccccctcccatcgacctgagcatcccccacgtgtggatgcctccccagaccacccctcacggctggaccgagagccacaccacctccggcctgcacagaccccacttcaaccagacctgcatcctgttcgacggccacgacctgctgtttagcaccgtgaccccctgcctgcaccagggcttctacctgatcgacgagctgagatacgtgaagatcaccctgaccgaggatttcttcgtggtcaccgtgtccatcgacgacgacacccccatgctgctgatcttcggccacctgcccagagtgctgttcaaggccccctaccagcgggacaacttcatcctgcggcagaccgagaagcacgagctgctggtgctggtcaagaaggaccagctgaaccggcactcctacctgaaggaccccgacttcctggacgccgccctggacttcaactacctggacctgagcgccctgctgagaaacagcttccacagatacgccgtggacgtgctgaagtccggacggtgccagatgctcgatcggcggaccgtggagatggccttcgcctatgccctcgccctgttcgccgctgccagacaggaagaggctggcgcccaggtgtcagtgcccagagccctggatagacaggccgccctgctgcagatccaggaattcatgatcacctgcctgagccagaccccccctagaaccaccctgctgctgtaccccacagccgtggatctggccaagagggccctgtggacccccaaccagatcaccgacatcacaagcctcgtgcggctcgtgtacatcctgagcaagcagaaccagcagcacctgatcccccagtgggccctgagacagatcgccgacttcgccctgaagctgcacaagacccatctggccagctttctgagcgccttcgccaggcaggaactgtacctgatgggcagcctggtccacagcatgctggtgcataccaccgagcggcgggagatcttcatcgtggagacaggcctgtgtagcctggccgagctgtcccactttacccagctgctggcccaccctcaccacgagtacctgagcgacctgtacaccccctgcagcagcagcggcagacgggaccacagcctggaacggctgaccagactgttccccgatgccaccgtgcctgctacagtgcctgccgccctgtccatcctgtccaccatgcagcccagcaccctggaaaccttccccgacctgttctgcctgcccctgggcgagagctttagcgccctgaccgtgtccgagcacgtgtcctacatcgtgaccaatcagtacctgatcaagggcatcagctaccccgtgtccaccacagtcgtgggccagagcctgatcatcacccagaccgacagccagaccaagtgcgagctgacccggaacatgcacaccacacacagcatcaccgtggccctgaacatcagcctggaaaactgcgctttctgtcagtctgccctgctggaatacgacgatacccagggcgtgatcaacatcatgtacatgcacgacagcgacgacgtgctgttcgccctggacccctacaacgaggtggtggtgtccagcccccggacccactacctgatgctgctgaagaacggcaccgtgctggaagtgaccgacgtggtggtggacgccaccgactgataatctagacggcgcgcccacccagcggccgcctataactctctacggctaacctgaatggactacgacatagtctagtcgacgccaccatgtgcagaaggcccgactgcggcttcagcttcagccctggacccgtgatcctgctgtggtgctgcctgctgctgcctatcgtgtcctctgccgccgtgtctgtggcccctacagccgccgagaaggtgccagccgagtgccccgagctgaccagaagatgcctgctgggcgaggtgttcgagggcgacaagtacgagagctggctgcggcccctggtcaacgtgaccggcagagatggccccctgagccagctgatccggtacagacccgtgacccccgaggccgccaatagcgtgctgctggacgaggccttcctggataccctggccctgctgtacaacaaccccgaccagctgagagccctgctgaccctgctgtccagcgacaccgcccccagatggatgaccgtgatgcggggctacagcgagtgtggagatggcagccctgccgtgtacacctgcgtggacgacctgtgcagaggctacgacctgaccagactgagctacggccggtccatcttcacagagcacgtgctgggcttcgagctggtgccccccagcctgttcaacgtggtggtggccatccggaacgaggccaccagaaccaacagagccgtgcggctgcctgtgtctacagccgctgcacctgagggcatcacactgttctacggcctgtacaacgccgtgaaagagttctgcctccggcaccagctggatccccccctgctgagacacctggacaagtactacgccggcctgcccccagagctgaagcagaccagagtgaacctgcccgcccacagcagatatggccctcaggccgtggacgccagatgataatctagacggcgcgcccacccaatcgatgtacttccgaggaactcacgtgcataatgcatcaggctggtacattagatccccgcttaccgcgggcaatatagcaacactaaaaactcgatgtacttccgaggaagcgcagtgcataatgctgcgcagtgttgccacataaccactatattaaccatttatctagcggacgccaaaaactcaatgtatttctgaggaagcgtggtgcataatgccacgcagcgtctgcataacttttattatttcttttattaatcaacaaaattttgtttttaacatttcaaaaaaaaaaaaaaaaaaaaaaaaaaaaaaaaaaaaaaaagggtcggcatggcatctccacctcctcgcggtccgacctgggcatccgaaggaggacgcacgtccactcggatggctaagggagagccacgagctcctgtttaaaccagctccaattcgccctatagtgagtcgtattacgcgcgctcactggccgtcgttttacaacgtcgtgactgggaaaaccctggcgttacccaacttaatcgccttgcagcacatccccctttcgccagctggcgtaatagcgaagaggcccgcaccgatcgcccttcccaacagttgcgcagcctgaatggcgaatgggacgcgccctgtagcggcgcattaagcgcggcgggtgtggtggttacgcgcagcgtgaccgctacacttgccagcgccctagcgcccgctcctttcgctttcttcccttcctttctcgccacgttcgccggctttccccgtcaagctctaaatcgggggctccctttagggttccgatttagtgctttacggcacctcgaccccaaaaaacttgattagggtgatggttcacgtagtgggccatcgccctgatagacggtttttcgccctttgacgttggagtccacgttctttaatagtggactcttgttccaaactggaacaacactcaaccctatctcggtctattcttttgatttataagggattttgccgatttcggcctattggttaaaaaatgagctgatttaacaaaaatttaacgcgaattttaacaaaatattaacgcttacaatttaggtggcacttttcggggaaatgtgcgcggaacccctatttgtttatttttctaaatacattcaaatatgtatccgctcatgagacaataaccctgataaatgcttcaataatattgaaaaaggaagagtatgagtattcaacatttccgtgtcgcccttattcccttttttgcggcattttgccttcctgtttttgctcacccagaaacgctggtgaaagtaaaagatgctgaagatcagttgggtgcacgagtgggttacatcgaactggatctcaacagcggtaagatccttgagagttttcgccccgaagaacgttttccaatgatgagcacttttaaagttctgctatgtggcgcggtattatcccgtattgacgccgggcaagagcaactcggtcgccgcatacactattctcagaatgacttggttgagtactcaccagtcacagaaaagcatcttacggatggcatgacagtaagagaattatgcagtgctgccataaccatgagtgataacactgcggccaacttacttctgacaacgatcggaggaccgaaggagctaaccgcttttttgcacaacatgggggatcatgtaactcgccttgatcgttgggaaccggagctgaatgaagccataccaaacgacgagcgtgacaccacgatgcctgtagcaatggcaacaacgttgcgcaaactattaactggcgaactacttactctagcttcccggcaacaattaatagactggatggaggcggataaagttgcaggaccacttctgcgctcggcccttccggctggctggtttattgctgataaatctggagccggtgagcgtgggtctcgcggtatcattgcagcactggggccagatggtaagccctcccgtatcgtagttatctacacgacggggagtcaggcaactatggatgaacgaaatagacagatcgctgagataggtgcctcactgattaagcattggtaactgtcagaccaagtttactcatatatactttagattgatttaaaacttcatttttaatttaaaaggatctaggtgaagatcctttttgataatctcatgaccaaaatcccttaacgtgagttttcgttccactgagcgtcagaccccgtagaaaagatcaaaggatcttcttgagatcctttttttctgcgcgtaatctgctgcttgcaaacaaaaaaaccaccgctaccagcggtggtttgtttgccggatcaagagctaccaactctttttccgaaggtaactggcttcagcagagcgcagataccaaatactgttcttctagtgtagccgtagttaggccaccacttcaagaactctgtagcaccgcctacatacctcgctctgctaatcctgttaccagtggctgctgccagtggcgataagtcgtgtcttaccgggttggactcaagacgatagttaccggataaggcgcagcggtcgggctgaacggggggttcgtgcacacagcccagcttggagcgaacgacctacaccgaactgagatacctacagcgtgagctatgagaaagcgccacgcttcccgaagggagaaaggcggacaggtatccggtaagcggcagggtcggaacaggagagcgcacgagggagcttccagggggaaacgcctggtatctttatagtcctgtcgggtttcgccacctctgacttgagcgtcgatttttgtgatgctcgtcaggggggcggagcctatggaaaaacgccagcaacgcggcctttttacggttcctggccttttgctggccttttgctcacatgttctttcctgcgttatcccctgattctgtggataaccgtattaccgcctttgagtgagctgataccgctcgccgcagccgaacgaccgagcgcagcgagtcagtgagcgaggaagcggaagagcgcccaatacgcaaaccgcctctccccgcgcgttggccgattcattaatgcagctggcacgacaggtttcccgactggaaagcgggcagtgagcgcaacgcaattaatgtgagttagctcactcattaggcaccccaggctttacactttatgctcccggctcgtatgttgtgtggaattgtgagcggataacaatttcacacaggaaacagctatgaccatgattacgccaagcgcgcaattaaccctcactaaagggaacaaaagctgggtaccggcgcca

SEQ ID NO: 53 - DNA, 14152 bp, Artificial Sequence
  source: /note="Description of Artificial Sequence: Synthetic polynucleotide"
cgcgtcggctacaattaatacataaccttatgtatcatacacatacgatttaggtgacactatagatgggcggcgcatgagagaagcccagaccaattacctacccaaaatggagaaagttcacgttgacatcgaggaagacagcccattcctcagagctttgcagcggagcttcccgcagtttgaggtagaagccaagcaggtcactgataatgaccatgctaatgccagagcgttttcgcatctggcttcaaaactgatcgaaacggaggtggacccatccgacacgatccttgacattggaagtgcgcccgcccgcagaatgtattctaagcacaagtatcattgtatctgtccgatgagatgtgcggaagatccggacagattgtataagtatgcaactaagctgaagaaaaactgtaaggaaataactgataaggaattggacaagaaaatgaaggagctcgccgccgtcatgagcgaccctgacctggaaactgagactatgtgcctccacgacgacgagtcgtgtcgctacgaagggcaagtcgctgtttaccaggatgtatacgcggttgacggaccgacaagtctctatcaccaagccaataagggagttagagtcgcctactggataggctttgacaccaccccttttatgtttaagaacttggctggagcatatccatcatactctaccaactgggccgacgaaaccgtgttaacggctcgtaacataggcctatgcagctctgacgttatggagcggtcacgtagagggatgtccattcttagaaagaagtatttgaaaccatccaacaatgttctattctctgttggctcgaccatctaccacgagaagagggacttactgaggagctggcacctgccgtctgtatttcacttacgtggcaagcaaaattacacatgtcggtgtgagactatagttagttgcgacgggtacgtcgttaaaagaatagctatcagtccaggcctgtatgggaagccttcaggctatgctgctacgatgcaccgcgagggattcttgtgctgcaaagtgacagacacattgaacggggagagggtctcttttcccgtgtgcacgtatgtgccagctacattgtgtgaccaaatgactggcatactggcaacagatgtcagtgcggacgacgcgcaaaaactgctggttgggctcaaccagcgtatagtcgtcaacggtcgcacccagagaaacaccaataccatgaaaaattaccttttgcccgtagtggcccaggcatttgctaggtgggcaaaggaatataaggaagatcaagaagatgaaaggccactaggactacgagatagacagttagtcatggggtgttgttgggcttttagaaggcacaagataacatctatttataagcgcccggatacccaaaccatcatcaaagtgaacagcgatttccactcattcgtgctgcccaggataggcagtaacacattggagatcgggctgagaacaagaatcaggaaaatgttagaggagcacaaggagccgtcacctctcattaccgccgaggacgtacaagaagctaagtgcgcagccgatgaggctaaggaggtgcgtgaagccgaggagttgcgcgcagctctaccacctttggcagctgatgttgaggagcccactctggaagccgatgtagacttgatgttacaagaggctggggccggctcagtggagacacctcgtggcttgataaaggttaccagctacgctggcgaggacaagatcggctcttacgctgtgctttctccgcaggctgtactcaagagtgaaaaattatcttgcatccaccctctcgctgaacaagtcatagtgataacacactctggccgaaaagggcgttatgccgtggaaccataccatggtaaagtagtggtgccagagggacatgcaatacccgtccaggactttcaagctctgagtgaaagtgccaccattgtgtacaacgaacgtgagttcgtaaacaggtacctgcaccatattgccacacatggaggagcgctgaacactgatgaagaatattacaaaactgtcaagcccagcgagcacgacggcgaatacctgtacgacatcgacaggaaacagtgcgtcaagaaagaactagtcactgggctagggctcacaggcgagctggtggatcctcccttccatgaattcgcctacgagagtctgagaacacgaccagccgctccttaccaagtaccaaccataggggtgtatggcgtgccaggatcaggcaagtctggcatcattaaaagcgcagtcaccaaaaaagatctagtggtgagcgccaagaaagaaaactgtgcagaaattataagggacgtcaagaaaatgaaagggctggacgtcaatgccagaactgtggactcagtgctcttgaatggatgcaaacaccccgtagagaccctgtatattgacgaagcttttgcttgtcatgcaggtactctcagagcgctcatagccattataagacctaaaaaggcagtgctctgcggggatcccaaacagtgcggtttttttaacatgatgtgcctgaaagtgcattttaaccacgagatttgcacacaagtcttccacaaaagcatctctcgccgttgcactaaatctgtgacttcggtcgtctcaaccttgttttacgacaaaaaaatgagaacgacgaatccgaaagagactaagattgtgattgacactaccggcagtaccaaacctaagcaggacgatctcattctcacttgtttcagagggtgggtgaagcagttgcaaatagattacaaaggcaacgaaataatgacggcagctgcctctcaagggctgacccgtaaaggtgtgtatgccgttcggtacaaggtgaatgaaaatcctctgtacgcacccacctcagaacatgtgaacgtcctactgacccgcacggaggaccgcatcgtgtggaaaacactagccggcgacccatggataaaaacactgactgccaagtaccctgggaatttcactgccacgatagaggagtggcaagcagagcatgatgccatcatgaggcacatcttggagagaccggaccctaccgacgtcttccagaataaggcaaacgtgtgttgggccaaggctttagtgccggtgctgaagaccgctggcatagacatgaccactgaacaatggaacactgtggattattttgaaacggacaaagctcactcagcagagatagtattgaaccaactatgcgtgaggttctttggactcgatctggactccggtctattttctgcacccactgttccgttatccattaggaataatcactgggataactccccgtcgcctaacatgtacgggctgaataaagaagtggtccgtcagctctctcgcaggtacccacaactgcctcgggcagttgccactggaagagtctatgacatgaacactggtacactgcgcaattatgatccgcgcataaacctagtacctgtaaacagaagactgcctcatgctttagtcctccaccataatgaacacccacagagtgacttttcttcattcgtcagcaaattgaagggcagaactgtcctggtggtcggggaaaagttgtccgtcccaggcaaaatggttgactggttgtcagaccggcctgaggctaccttcagagctcggctggatttaggcatcccaggtgatgtgcccaaatatgacataatatttgttaatgtgaggaccccatataaataccatcactatcagcagtgtgaagaccatgccattaagcttagcatgttgaccaagaaagcttgtctgcatctgaatcccggcggaacctgtgtcagcataggttatggttacgctgacagggccagcgaaagcatcattggtgctatagcgcggcagttcaagttttcccgggtatgcaaaccgaaatcctcacttgaagagacggaagttctgtttgtattcattgggtacgatcgcaaggcccgtacgcacaatccttacaagctttcatcaaccttgaccaacatttatacaggttccagactccacgaagccggatgtgcaccctcatatcatgtggtgcgaggggatattgccacggccaccgaaggagtgattataaatgctgctaacagcaaaggacaacctggcggaggggtgtgcggagcgctgtataagaaattcccggaaagcttcgatttacagccgatcgaagtaggaaaagcgcgactggtcaaaggtgcagctaaacatatcattcatgccgtaggaccaaacttcaacaaagtttcggaggttgaaggtgacaaacagttggcagaggcttatgagtccatcgctaagattgtcaacgataacaattacaagtcagtagcgattccactgttgtccaccggcatcttttccgggaacaaagatcgactaacccaatcattgaaccatttgctgacagctttagacaccactgatgcagatgtagccatatactgcagggacaagaaatgggaaatgactctcaaggaagcagtggctaggagagaagcagtggaggagatatgcatatccgacgactcttcagtgacagaacctgatgcagagctggtgagggtgcatccgaagagttctttggctggaaggaagggctacagcacaagcgatggcaaaactttctcatatttggaagggaccaagtttcaccaggcggccaaggatatagcagaaattaatgccatgtggcccgttgcaacggaggccaatgagcaggtatgcatgtatatcctcggagaaagcatgagcagtattaggtcgaaatgccccgtcgaagagtcggaagcctcctcaccacctagcacgctgccttgcttgtgcatccatgccatgactccagaaagagtacagcgcctaaaagcctcacgtccagaacaaattactgtgtgctcatcctttccattgccgaagtatagaatcactggtgtgcagaagatccaatgctcccagcctatattgttctcaccgaaagtgcctgcgtatattcatccaaggaagtatctcgtggaaacaccaccggtagacgagactccggagccatcggcagagaaccaatccacagaggggacacctgaacaaccaccacttataaccgaggatgagaccaggactagaacgcctgagccgatcatcatcgaagaggaagaagaggatagcataagtttgctgtcagatggcccgacccaccaggtgctgcaagtcgaggcagacattcacgggccgccctctgtatctagctcatcctggtccattcctcatgcatccgactttgatgtggacagtttatccatacttgacaccctggagggagctagcgtgaccagcggggcaacgtcagccgagactaactcttacttcgcaaagagtatggagtttctggcgcgaccggtgcctgcgcctcgaacagtattcaggaaccctccacatcccgctccgcgcacaagaacaccgtcacttgcacccagcagggcctgctcgagagggatcacgggagaaaccgtgggatacgcggttacacacaatagcgagggcttcttgctatgcaaagttactgacacagtaaaaggagaacgggtatcgttccctgtgtgcacgtacatcccggccaccataaactcgagaaccagcctggtctccaacccgccaggcgtaaatagggtgattacaagagaggagtttgaggcgttcgtagcacaacaacaatgacggtttgatgcgggtgcatacatcttttcctccgacaccggtcaagggcatttacaacaaaaatcagtaaggcaaacggtgctatccgaagtggtgttggagaggaccgaattggagatttcgtatgccccgcgcctcgaccaagaaaaagaagaattactacgcaagaaattacagttaaatcccacacctgctaacagaagcagataccagtccaggaaggtggagaacatgaaagccataacagctagacgtattctgcaaggcctagggcattatttgaaggcagaaggaaaagtggagtgctaccgaaccctgcatcctgttcctttgtattcatctagtgtgaaccgtgccttttcaagccccaaggtcgcagtggaagcctgtaacgccatgttgaaagagaactttccgactgtggcttcttactgtattattccagagtacgatgcctatttggacatggttgacggagcttcatgctgcttagacactgccagtttttgccctgcaaagctgcgcagctttccaaagaaacactcctatttggaacccacaatacgatcggcagtgccttcagcgatccagaacacgctccagaacgtcctggcagctgccacaaaaagaaattgcaatgtcacgcaaatgagagaattgcccgtattggattcggcggcctttaatgtggaatgcttcaagaaatatgcgtgtaataatgaatattgggaaacgtttaaagaaaaccccatcaggcttactgaagaaaacgtggtaaattacattaccaaattaaaaggaccaaaagctgctgctctttttgcgaagacacataatttgaatatgttgcaggacataccaatggacaggtttgtaatggacttaaagagagacgtgaaagtgactccaggaacaaaacatactgaagaacggcccaaggtacaggtgatccaggctgccgatccgctagcaacagcgtatctgtgcggaatccaccgagagctggttaggagattaaatgcggtcctgcttccgaacattcatacactgtttgatatgtcggctgaagactttgacgctattatagccgagcacttccagcctggggattgtgttctggaaactgacatcgcgtcgtttgataaaagtgaggacgacgccatggctctgaccgcgttaatgattctggaagacttaggtgtggacgcagagctgttgacgctgattgaggcggctttcggcgaaatttcatcaatacatttgcccactaaaactaaatttaaattcggagccatgatgaaatctggaatgttcctcacactgtttgtgaacacagtcattaacattgtaatcgcaagcagagtgttgagagaacggctaaccggatcaccatgtgcagcattcattggagatgacaatatcgtgaaaggagtcaaatcggacaaattaatggcagacaggtgcgccacctggttgaatatggaagtcaagattatagatgctgtggtgggcgagaaagcgccttatttctgtggagggtttattttgtgtgactccgtgaccggcacagcgtgccgtgtggcagaccccctaaaaaggctgtttaagcttggcaaacctctggcagcagacgatgaacatgatgatgacaggagaagggcattgcatgaagagtcaacacgctggaaccgagtgggtattctttcagagctgtgcaaggcagtagaatcaaggtatgaaaccgtaggaacttccatcatagttatggccatgactactctagctagcagtgttaaatcattcagctacctgagaggggcccctataactctctacggctaacctgaatggactacgacatagtctagtcgacgccaccatgaggcctggcctgccctcctacctgatcatcctggccgtgtgcctgttcagccacctgctgtccagcagatacggcgccgaggccgtgagcgagcccctggacaaggctttccacctgctgctgaacacctacggcagacccatccggtttctgcgggagaacaccacccagtgcacctacaacagcagcctgcggaacagcaccgtcgtgagagagaacgccatcagcttcaactttttccagagctacaaccagtactacgtgttccacatgcccagatgcctgtttgccggccctctggccgagcagttcctgaaccaggtggacctgaccgagacactggaaagataccagcagcggctgaatacctacgccctggtgtccaaggacctggccagctaccggtcctttagccagcagctcaaggctcaggatagcctcggcgagcagcctaccaccgtgccccctcccatcgacctgagcatcccccacgtgtggatgcctccccagaccacccctcacggctggaccgagagccacaccacctccggcctgcacagaccccacttcaaccagacctgcatcctgttcgacggccacgacctgctgtttagcaccgtgaccccctgcctgcaccagggcttctacctgatcgacgagctgagatacgtgaagatcaccctgaccgaggatttcttcgtggtcaccgtgtccatcgacgacgacacccccatgctgctgatcttcggccacctgcccagagtgctgttcaaggccccctaccagcgggacaacttcatcctgcggcagaccgagaagcacgagctgctggtgctggtcaagaaggaccagctgaaccggcactcctacctgaaggaccccgacttcctggacgccgccctggacttcaactacctggacctgagcgccctgctgagaaacagcttccacagatacgccgtggacgtgctgaagtccggacggtgccagatgctcgatcggcggaccgtggagatggccttcgcctatgccctcgccctgttcgccgctgccagacaggaagaggctggcgcccaggtgtcagtgcccagagccctggatagacaggccgccctgctgcagatccaggaattcatgatcacctgcctgagccagaccccccctagaaccaccctgctgctgtaccccacagccgtggatctggccaagagggccctgtggacccccaaccagatcaccgacatcacaagcctcgtgcggctcgtgtacatcctgagcaagcagaaccagcagcacctgatcccccagtgggccctgagacagatcgccgacttcgccctgaagctgcacaagacccatctggccagctttctgagcgccttcgccaggcaggaactgtacctgatgggcagcctggtccacagcatgctggtgcataccaccgagcggcgggagatcttcatcgtggagacaggcctgtgtagcctggccgagctgtcccactttacccagctgctggcccaccctcaccacgagtacctgagcgacctgtacaccccctgcagcagcagcggcagacgggaccacagcctggaacggctgaccagactgttccccgatgccaccgtgcctgctacagtgcctgccgccctgtccatcctgtccaccatgcagcccagcaccctggaaaccttccccgacctgttctgcctgcccctgggcgagagctttagcgccctgaccgtgtccgagcacgtgtcctacatcgtgaccaatcagtacctgatcaagggcatcagctaccccgtgtccaccacagtcgtgggccagagcctgatcatcacccagaccgacagccagaccaagtgcgagctgacccggaacatgcacaccacacacagcatcaccgtggccctgaacatcagcctggaaaactgcgctttctgtcagtctgccctgctggaatacgacgatacccagggcgtgatcaacatcatgtacatgcacgacagcgacgacgtgctgttcgccctggacccctacaacgaggtggtggtgtccagcccccggacccactacctgatgctgctgaagaacggcaccgtgctggaagtgaccgacgtggtggtggacgccaccgacagcagactgctgatgatgagcgtgtacgccctgagcgccatcatcggcatctacctgctgtaccggatgctgaaaacctgctgataatctagacggcgcgcccacccagcggccgcctataactctctacggctaacctgaatggactacgacatagtctagtcgacgccaccatgtgcagaaggcccgactgcggcttcagcttcagccctggacccgtgatcctgctgtggtgctgcctgctgctgcctatcgtgtcctctgccgccgtgtctgtggcccctacagccgccgagaaggtgccagccgagtgccccgagctgaccagaagatgcctgctgggcgaggtgttcgagggcgacaagtacgagagctggctgcggcccctggtcaacgtgaccggcagagatggccccctgagccagctgatccggtacagacccgtgacccccgaggccgccaatagcgtgctgctggacgaggccttcctggataccctggccctgctgtacaacaaccccgaccagctgagagccctgctgaccctgctgtccagcgacaccgcccccagatggatgaccgtgatgcggggctacagcgagtgtggagatggcagccctgccgtgtacacctgcgtggacgacctgtgcagaggctacgacctgaccagactgagctacggccggtccatcttcacagagcacgtgctgggcttcgagctggtgccccccagcctgttcaacgtggtggtggccatccggaacgaggccaccagaaccaacagagccgtgcggctgcctgtgtctacagccgctgcacctgagggcatcacactgttctacggcctgtacaacgccgtgaaagagttctgcctccggcaccagctggatccccccctgctgagacacctggacaagtactacgccggcctgcccccagagctgaagcagaccagagtgaacctgcccgcccacagcagatatggccctcaggccgtggacgccagatgataatctagacggcgcgcccacccaatcgatgtacttccgaggaactcacgtgcataatgcatcaggctggtacattagatccccgcttaccgcgggcaatatagcaacactaaaaactcgatgtacttccgaggaagcgcagtgcataatgctgcgcagtgttgccacataaccactatattaaccatttatctagcggacgccaaaaactcaatgtatttctgaggaagcgtggtgcataatgccacgcagcgtctgcataacttttattatttcttttattaatcaacaaaattttgtttttaacatttcaaaaaaaaaaaaaaaaaaaaaaaaaaaaaaaaaaaaaaaagggtcggcatggcatctccacctcctcgcggtccgacctgggcatccgaaggaggacgcacgtccactcggatggctaagggagagccacgagctcctgtttaaaccagctccaattcgccctatagtgagtcgtattacgcgcgctcactggccgtcgttttacaacgtcgtgactgggaaaaccctggcgttacccaacttaatcgccttgcagcacatccccctttcgccagctggcgtaatagcgaagaggcccgcaccgatcgcccttcccaacagttgcgcagcctgaatggcgaatgggacgcgccctgtagcggcgcattaagcgcggcgggtgtggtggttacgcgcagcgtgaccgctacacttgccagcgccctagcgcccgctcctttcgctttcttcccttcctttctcgccacgttcgccggctttccccgtcaagctctaaatcgggggctccctttagggttccgatttagtgctttacggcacctcgaccccaaaaaacttgattagggtgatggttcacgtagtgggccatcgccctgatagacggtttttcgccctttgacgttggagtccacgttctttaatagtggactcttgttccaaactggaacaacactcaaccctatctcggtctattcttttgatttataagggattttgccgatttcggcctattggttaaaaaatgagctgatttaacaaaaatttaacgcgaattttaacaaaatattaacgcttacaatttaggtggcacttttcggggaaatgtgcgcggaacccctatttgtttatttttctaaatacattcaaatatgtatccgctcatgagacaataaccctgataaatgcttcaataatattgaaaaaggaagagtatgagtattcaacatttccgtgtcgcccttattcccttttttgcggcattttgccttcctgtttttgctcacccagaaacgctggtgaaagtaaaagatgctgaagatcagttgggtgcacgagtgggttacatcgaactggatctcaacagcggtaagatccttgagagttttcgccccgaagaacgttttccaatgatgagcacttttaaagttctgctatgtggcgcggtattatcccgtattgacgccgggcaagagcaactcggtcgccgcatacactattctcagaatgacttggttgagtactcaccagtcacagaaaagcatcttacggatggcatgacagtaagagaattatgcagtgctgccataaccatgagtgataacactgcggccaacttacttctgacaacgatcggaggaccgaaggagctaaccgcttttttgcacaacatgggggatcatgtaactcgccttgatcgttgggaaccggagctgaatgaagccataccaaacgacgagcgtgacaccacgatgcctgtagcaatggcaacaacgttgcgcaaactattaactggcgaactacttactctagcttcccggcaacaattaatagactggatggaggcggataaagttgcaggaccacttctgcgctcggcccttccggctggctggtttattgctgataaatctggagccggtgagcgtgggtctcgcggtatcattgcagcactggggccagatggtaagccctcccgtatcgtagttatctacacgacggggagtcaggcaactatggatgaacgaaatagacagatcgctgagataggtgcctcactgattaagcattggtaactgtcagaccaagtttactcatatatactttagattgatttaaaacttcatttttaatttaaaaggatctaggtgaagatcctttttgataatctcatgaccaaaatcccttaacgtgagttttcgttccactgagcgtcagaccccgtagaaaagatcaaaggatcttcttgagatcctttttttctgcgcgtaatctgctgcttgcaaacaaaaaaaccaccgctaccagcggtggtttgtttgccggatcaagagctaccaactctttttccgaaggtaactggcttcagcagagcgcagataccaaatactgttcttctagtgtagccgtagttaggccaccacttcaagaactctgtagcaccgcctacatacctcgctctgctaatcctgttaccagtggctgctgccagtggcgataagtcgtgtcttaccgggttggactcaagacgatagttaccggataaggcgcagcggtcgggctgaacggggggttcgtgcacacagcccagcttggagcgaacgacctacaccgaactgagatacctacagcgtgagctatgagaaagcgccacgcttcccgaagggagaaaggcggacaggtatccggtaagcggcagggtcggaacaggagagcgcacgagggagcttccagggggaaacgcctggtatctttatagtcctgtcgggtttcgccacctctgacttgagcgtcgatttttgtgatgctcgtcaggggggcggagcctatggaaaaacgccagcaacgcggcctttttacggttcctggccttttgctggccttttgctcacatgttctttcctgcgttatcccctgattctgtggataaccgtattaccgcctttgagtgagctgataccgctcgccgcagccgaacgaccgagcgcagcgagtcagtgagcgaggaagcggaagagcgcccaatacgcaaaccgcctctccccgcgcgttggccgattcattaatgcagctggcacgacaggtttcccgactggaaagcgggcagtgagcgcaacgcaattaatgtgagttagctcactcattaggcaccccaggctttacactttatgctcccggctcgtatgttgtgtggaattgtgagcggataacaatttcacacaggaaacagctatgaccatgattacgccaagcgcgcaattaaccctcactaaagggaacaaaagctgggtaccggcgcca

SEQ ID NO: 54 - DNA, 15512 bp, Artificial Sequence
  source: /note="Description of Artificial Sequence: Synthetic polynucleotide"
cgcgtcggctacaattaatacataaccttatgtatcatacacatacgatttaggtgacactatagatgggcggcgcatgagagaagcccagaccaattacctacccaaaatggagaaagttcacgttgacatcgaggaagacagcccattcctcagagctttgcagcggagcttcccgcagtttgaggtagaagccaagcaggtcactgataatgaccatgctaatgccagagcgttttcgcatctggcttcaaaactgatcgaaacggaggtggacccatccgacacgatccttgacattggaagtgcgcccgcccgcagaatgtattctaagcacaagtatcattgtatctgtccgatgagatgtgcggaagatccggacagattgtataagtatgcaactaagctgaagaaaaactgtaaggaaataactgataaggaattggacaagaaaatgaaggagctcgccgccgtcatgagcgaccctgacctggaaactgagactatgtgcctccacgacgacgagtcgtgtcgctacgaagggcaagtcgctgtttaccaggatgtatacgcggttgacggaccgacaagtctctatcaccaagccaataagggagttagagtcgcctactggataggctttgacaccaccccttttatgtttaagaacttggctggagcatatccatcatactctaccaactgggccgacgaaaccgtgttaacggctcgtaacataggcctatgcagctctgacgttatggagcggtcacgtagagggatgtccattcttagaaagaagtatttgaaaccatccaacaatgttctattctctgttggctcgaccatctaccacgagaagagggacttactgaggagctggcacctgccgtctgtatttcacttacgtggcaagcaaaattacacatgtcggtgtgagactatagttagttgcgacgggtacgtcgttaaaagaatagctatcagtccaggcctgtatgggaagccttcaggctatgctgctacgatgcaccgcgagggattcttgtgctgcaaagtgacagacacattgaacggggagagggtctcttttcccgtgtgcacgtatgtgccagctacattgtgtgaccaaatgactggcatactggcaacagatgtcagtgcggacgacgcgcaaaaactgctggttgggctcaaccagcgtatagtcgtcaacggtcgcacccagagaaacaccaataccatgaaaaattaccttttgcccgtagtggcccaggcatttgctaggtgggcaaaggaatataaggaagatcaagaagatgaaaggccactaggactacgagatagacagttagtcatggggtgttgttgggcttttagaaggcacaagataacatctatttataagcgcccggatacccaaaccatcatcaaagtgaacagcgatttccactcattcgtgctgcccaggataggcagtaacacattggagatcgggctgagaacaagaatcaggaaaatgttagaggagcacaaggagccgtcacctctcattaccgccgaggacgtacaagaagctaagtgcgcagccgatgaggctaaggaggtgcgtgaagccgaggagttgcgcgcagctctaccacctttggcagctgatgttgaggagcccactctggaagccgatgtagacttgatgttacaagaggctggggccggctcagtggagacacctcgtggcttgataaaggttaccagctacgctggcgaggacaagatcggctcttacgctgtgctttctccgcaggctgtactcaagagtgaaaaattatcttgcatccaccctctcgctgaacaagtcatagtgataacacactctggccgaaaagggcgttatgccgtggaaccataccatggtaaagtagtggtgccagagggacatgcaatacccgtccaggactttcaagctctgagtgaaagtgccaccattgtgtacaacgaacgtgagttcgtaaacaggtacctgcaccatattgccacacatggaggagcgctgaacactgatgaagaatattacaaaactgtcaagcccagcgagcacgacggcgaatacctgtacgacatcgacaggaaacagtgcgtcaagaaagaactagtcactgggctagggctcacaggcgagctggtggatcctcccttccatgaattcgcctacgagagtctgagaacacgaccagccgctccttaccaagtaccaaccataggggtgtatggcgtgccaggatcaggcaagtctggcatcattaaaagcgcagtcaccaaaaaagatctagtggtgagcgccaagaaagaaaactgtgcagaaattataagggacgtcaagaaaatgaaagggctggacgtcaatgccagaactgtggactcagtgctcttgaatggatgcaaacaccccgtagagaccctgtatattgacgaagcttttgcttgtcatgcaggtactctcagagcgctcatagccattataagacctaaaaaggcagtgctctgcggggatcccaaacagtgcggtttttttaacatgatgtgcctgaaagtgcattttaaccacgagatttgcacacaagtcttccacaaaagcatctctcgccgttgcactaaatctgtgacttcggtcgtctcaaccttgttttacgacaaaaaaatgagaacgacgaatccgaaagagactaagattgtgattgacactaccggcagtaccaaacctaagcaggacgatctcattctcacttgtttcagagggtgggtgaagcagttgcaaatagattacaaaggcaacgaaataatgacggcagctgcctctcaagggctgacccgtaaaggtgtgtatgccgttcggtacaaggtgaatgaaaatcctctgtacgcacccacctcagaacatgtgaacgtcctactgacccgcacggaggaccgcatcgtgtggaaaacactagccggcgacccatggataaaaacactgactgccaagtaccctgggaatttcactgccacgatagaggagtggcaagcagagcatgatgccatcatgaggcacatcttggagagaccggaccctaccgacgtcttccagaataaggcaaacgtgtgttgggccaaggctttagtgccggtgctgaagaccgctggcatagacatgaccactgaacaatggaacactgtggattattttgaaacggacaaagctcactcagcagagatagtattgaaccaactatgcgtgaggttctttggactcgatctggactccggtctattttctgcacccactgttccgttatccattaggaataatcactgggataactccccgtcgcctaacatgtacgggctgaataaagaagtggtccgtcagctctctcgcaggtacccacaactgcctcgggcagttgccactggaagagtctatgacatgaacactggtacactgcgcaattatgatccgcgcataaacctagtacctgtaaacagaagactgcctcatgctttagtcctccaccataatgaacacccacagagtgacttttcttcattcgtcagcaaattgaagggcagaactgtcctggtggtcggggaaaagttgtccgtcccaggcaaaatggttgactggttgtcagaccggcctgaggctaccttcagagctcggctggatttaggcatcccaggtgatgtgcccaaatatgacataatatttgttaatgtgaggaccccatataaataccatcactatcagcagtgtgaagaccatgccattaagcttagcatgttgaccaagaaagcttgtctgcatctgaatcccggcggaacctgtgtcagcataggttatggttacgctgacagggccagcgaaagcatcattggtgctatagcgcggcagttcaagttttcccgggtatgcaaaccgaaatcctcacttgaagagacggaagttctgtttgtattcattgggtacgatcgcaaggcccgtacgcacaatccttacaagctttcatcaaccttgaccaacatttatacaggttccagactccacgaagccggatgtgcaccctcatatcatgtggtgcgaggggatattgccacggccaccgaaggagtgattataaatgctgctaacagcaaaggacaacctggcggaggggtgtgcggagcgctgtataagaaattcccggaaagcttcgatttacagccgatcgaagtaggaaaagcgcgactggtcaaaggtgcagctaaacatatcattcatgccgtaggaccaaacttcaacaaagtttcggaggttgaaggtgacaaacagttggcagaggcttatgagtccatcgctaagattgtcaacgataacaattacaagtcagtagcgattccactgttgtccaccggcatcttttccgggaacaaagatcgactaacccaatcattgaaccatttgctgacagctttagacaccactgatgcagatgtagccatatactgcagggacaagaaatgggaaatgactctcaaggaagcagtggctaggagagaagcagtggaggagatatgcatatccgacgactcttcagtgacagaacctgatgcagagctggtgagggtgcatccgaagagttctttggctggaaggaagggctacagcacaagcgatggcaaaactttctcatatttggaagggaccaagtttcaccaggcggccaaggatatagcagaaattaatgccatgtggcccgttgcaacggaggccaatgagcaggtatgcatgtatatcctcggagaaagcatgagcagtattaggtcgaaatgccccgtcgaagagtcggaagcctcctcaccacctagcacgctgccttgcttgtgcatccatgccatgactccagaaagagtacagcgcctaaaagcctcacgtccagaacaaattactgtgtgctcatcctttccattgccgaagtatagaatcactggtgtgcagaagatccaatgctcccagcctatattgttctcaccgaaagtgcctgcgtatattcatccaaggaagtatctcgtggaaacaccaccggtagacgagactccggagccatcggcagagaaccaatccacagaggggacacctgaacaaccaccacttataaccgaggatgagaccaggactagaacgcctgagccgatcatcatcgaagaggaagaagaggatagcataagtttgctgtcagatggcccgacccaccaggtgctgcaagtcgaggcagacattcacgggccgccctctgtatctagctcatcctggtccattcctcatgcatccgactttgatgtggacagtttatccatacttgacaccctggagggagctagcgtgaccagcggggcaacgtcagccgagactaactcttacttcgcaaagagtatggagtttctggcgcgaccggtgcctgcgcctcgaacagtattcaggaaccctccacatcccgctccgcgcacaagaacaccgtcacttgcacccagcagggcctgctcgagagggatcacgggagaaaccgtgggatacgcggttacacacaatagcgagggcttcttgctatgcaaagttactgacacagtaaaaggagaacgggtatcgttccctgtgtgcacgtacatcccggccaccataaactcgagaaccagcctggtctccaacccgccaggcgtaaatagggtgattacaagagaggagtttgaggcgttcgtagcacaacaacaatgacggtttgatgcgggtgcatacatcttttcctccgacaccggtcaagggcatttacaacaaaaatcagtaaggcaaacggtgctatccgaagtggtgttggagaggaccgaattggagatttcgtatgccccgcgcctcgaccaagaaaaagaagaattactacgcaagaaattacagttaaatcccacacctgctaacagaagcagataccagtccaggaaggtggagaacatgaaagccataacagctagacgtattctgcaaggcctagggcattatttgaaggcagaaggaaaagtggagtgctaccgaaccctgcatcctgttcctttgtattcatctagtgtgaaccgtgccttttcaagccccaaggtcgcagtggaagcctgtaacgccatgttgaaagagaactttccgactgtggcttcttactgtattattccagagtacgatgcctatttggacatggttgacggagcttcatgctgcttagacactgccagtttttgccctgcaaagctgcgcagctttccaaagaaacactcctatttggaacccacaatacgatcggcagtgccttcagcgatccagaacacgctccagaacgtcctggcagctgccacaaaaagaaattgcaatgtcacgcaaatgagagaattgcccgtattggattcggcggcctttaatgtggaatgcttcaagaaatatgcgtgtaataatgaatattgggaaacgtttaaagaaaaccccatcaggcttactgaagaaaacgtggtaaattacattaccaaattaaaaggaccaaaagctgctgctctttttgcgaagacacataatttgaatatgttgcaggacataccaatggacaggtttgtaatggacttaaagagagacgtgaaagtgactccaggaacaaaacatactgaagaacggcccaaggtacaggtgatccaggctgccgatccgctagcaacagcgtatctgtgcggaatccaccgagagctggttaggagattaaatgcggtcctgcttccgaacattcatacactgtttgatatgtcggctgaagactttgacgctattatagccgagcacttccagcctggggattgtgttctggaaactgacatcgcgtcgtttgataaaagtgaggacgacgccatggctctgaccgcgttaatgattctggaagacttaggtgtggacgcagagctgttgacgctgattgaggcggctttcggcgaaatttcatcaatacatttgcccactaaaactaaatttaaattcggagccatgatgaaatctggaatgttcctcacactgtttgtgaacacagtcattaacattgtaatcgcaagcagagtgttgagagaacggctaaccggatcaccatgtgcagcattcattggagatgacaatatcgtgaaaggagtcaaatcggacaaattaatggcagacaggtgcgccacctggttgaatatggaagtcaagattatagatgctgtggtgggcgagaaagcgccttatttctgtggagggtttattttgtgtgactccgtgaccggcacagcgtgccgtgtggcagaccccctaaaaaggctgtttaagcttggcaaacctctggcagcagacgatgaacatgatgatgacaggagaagggcattgcatgaagagtcaacacgctggaaccgagtgggtattctttcagagctgtgcaaggcagtagaatcaaggtatgaaaccgtaggaacttccatcatagttatggccatgactactctagctagcagtgttaaatcattcagctacctgagaggggcccctataactctctacggctaacctgaatggactacgacatagtctagtcgacgccaccatgaggcctggcctgccctcctacctgatcatcctggccgtgtgcctgttcagccacctgctgtccagcagatacggcgccgaggccgtgagcgagcccctggacaaggctttccacctgctgctgaacacctacggcagacccatccggtttctgcgggagaacaccacccagtgcacctacaacagcagcctgcggaacagcaccgtcgtgagagagaacgccatcagcttcaactttttccagagctacaaccagtactacgtgttccacatgcccagatgcctgtttgccggccctctggccgagcagttcctgaaccaggtggacctgaccgagacactggaaagataccagcagcggctgaatacctacgccctggtgtccaaggacctggccagctaccggtcctttagccagcagctcaaggctcaggatagcctcggcgagcagcctaccaccgtgccccctcccatcgacctgagcatcccccacgtgtggatgcctccccagaccacccctcacggctggaccgagagccacaccacctccggcctgcacagaccccacttcaaccagacctgcatcctgttcgacggccacgacctgctgtttagcaccgtgaccccctgcctgcaccagggcttctacctgatcgacgagctgagatacgtgaagatcaccctgaccgaggatttcttcgtggtcaccgtgtccatcgacgacgacacccccatgctgctgatcttcggccacctgcccagagtgctgttcaaggccccctaccagcgggacaacttcatcctgcggcagaccgagaagcacgagctgctggtgctggtcaagaaggaccagctgaaccggcactcctacctgaaggaccccgacttcctggacgccgccctggacttcaactacctggacctgagcgccctgctgagaaacagcttccacagatacgccgtggacgtgctgaagtccggacggtgccagatgctcgatcggcggaccgtggagatggccttcgcctatgccctcgccctgttcgccgctgccagacaggaagaggctggcgcccaggtgtcagtgcccagagccctggatagacaggccgccctgctgcagatccaggaattcatgatcacctgcctgagccagaccccccctagaaccaccctgctgctgtaccccacagccgtggatctggccaagagggccctgtggacccccaaccagatcaccgacatcacaagcctcgtgcggctcgtgtacatcctgagcaagcagaaccagcagcacctgatcccccagtgggccctgagacagatcgccgacttcgccctgaagctgcacaagacccatctggccagctttctgagcgccttcgccaggcaggaactgtacctgatgggcagcctggtccacagcatgctggtgcataccaccgagcggcgggagatcttcatcgtggagacaggcctgtgtagcctggccgagctgtcccactttacccagctgctggcccaccctcaccacgagtacctgagcgacctgtacaccccctgcagcagcagcggcagacgggaccacagcctggaacggctgaccagactgttccccgatgccaccgtgcctgctacagtgcctgccgccctgtccatcctgtccaccatgcagcccagcaccctggaaaccttccccgacctgttctgcctgcccctgggcgagagctttagcgccctgaccgtgtccgagcacgtgtcctacatcgtgaccaatcagtacctgatcaagggcatcagctaccccgtgtccaccacagtcgtgggccagagcctgatcatcacccagaccgacagccagaccaagtgcgagctgacccggaacatgcacaccacacacagcatcaccgtggccctgaacatcagcctggaaaactgcgctttctgtcagtctgccctgctggaatacgacgatacccagggcgtgatcaacatcatgtacatgcacgacagcgacgacgtgctgttcgccctggacccctacaacgaggtggtggtgtccagcccccggacccactacctgatgctgctgaagaacggcaccgtgctggaagtgaccgacgtggtggtggacgccaccgactgataatctagacggcgcgcccacccagcggccgcctataactctctacggctaacctgaatggactacgacatagtctagtcgacgccaccatgtgcagaaggcccgactgcggcttcagcttcagccctggacccgtgatcctgctgtggtgctgcctgctgctgcctatcgtgtcctctgccgccgtgtctgtggcccctacagccgccgagaaggtgccagccgagtgccccgagctgaccagaagatgcctgctgggcgaggtgttcgagggcgacaagtacgagagctggctgcggcccctggtcaacgtgaccggcagagatggccccctgagccagctgatccggtacagacccgtgacccccgaggccgccaatagcgtgctgctggacgaggccttcctggataccctggccctgctgtacaacaaccccgaccagctgagagccctgctgaccctgctgtccagcgacaccgcccccagatggatgaccgtgatgcggggctacagcgagtgtggagatggcagccctgccgtgtacacctgcgtggacgacctgtgcagaggctacgacctgaccagactgagctacggccggtccatcttcacagagcacgtgctgggcttcgagctggtgccccccagcctgttcaacgtggtggtggccatccggaacgaggccaccagaaccaacagagccgtgcggctgcctgtgtctacagccgctgcacctgagggcatcacactgttctacggcctgtacaacgccgtgaaagagttctgcctccggcaccagctggatccccccctgctgagacacctggacaagtactacgccggcctgcccccagagctgaagcagaccagagtgaacctgcccgcccacagcagatatggccctcaggccgtggacgccagatgataatctagacggcgcgcccacccaatcgatctataactctctacggctaacctgaatggactacgacatagtctagtcgacgccaccatgggcaagaaagaaatgatcatggtcaagggcatccccaagatcatgctgctgattagcatcacctttctgctgctgtccctgatcaactgcaacgtgctggtcaacagccggggcaccagaagatcctggccctacaccgtgctgtcctaccggggcaaagagatcctgaagaagcagaaagaggacatcctgaagcggctgatgagcaccagcagcgacggctaccggttcctgatgtaccccagccagcagaaattccacgccatcgtgatcagcatggacaagttcccccaggactacatcctggccggacccatccggaacgacagcatcacccacatgtggttcgacttctacagcacccagctgcggaagcccgccaaatacgtgtacagcgagtacaaccacaccgcccacaagatcaccctgaggcctcccccttgtggcaccgtgcccagcatgaactgcctgagcgagatgctgaacgtgtccaagcggaacgacaccggcgagaagggctgcggcaacttcaccaccttcaaccccatgttcttcaacgtgccccggtggaacaccaagctgtacatcggcagcaacaaagtgaacgtggacagccagaccatctactttctgggcctgaccgccctgctgctgagatacgcccagcggaactgcacccggtccttctacctggtcaacgccatgagccggaacctgttccgggtgcccaagtacatcaacggcaccaagctgaagaacaccatgcggaagctgaagcggaagcaggccctggtcaaagagcagccccagaagaagaacaagaagtcccagagcaccaccaccccctacctgagctacaccacctccaccgccttcaacgtgaccaccaacgtgacctacagcgccacagccgccgtgaccagagtggccacaagcaccaccggctaccggcccgacagcaactttatgaagtccatcatggccacccagctgagagatctggccacctgggtgtacaccaccctgcggtacagaaacgagcccttctgcaagcccgaccggaacagaaccgccgtgagcgagttcatgaagaatacccacgtgctgatcagaaacgagacaccctacaccatctacggcaccctggacatgagcagcctgtactacaacgagacaatgagcgtggagaacgagacagccagcgacaacaacgaaaccacccccacctcccccagcacccggttccagcggaccttcatcgaccccctgtgggactacctggacagcctgctgttcctggacaagatccggaacttcagcctgcagctgcccgcctacggcaatctgaccccccctgagcacagaagggccgccaacctgagcaccctgaacagcctgtggtggtggagccagtgataatctagacggcgcgcccacccaccgcgggcaatatagcaacactaaaaactcgatgtacttccgaggaagcgcagtgcataatgctgcgcagtgttgccacataaccactatattaaccatttatctagcggacgccaaaaactcaatgtatttctgaggaagcgtggtgcataatgccacgcagcgtctgcataacttttattatttcttttattaatcaacaaaattttgtttttaacatttcaaaaaaaaaaaaaaaaaaaaaaaaaaaaaaaaaaaaaaaagggtcggcatggcatctccacctcctcgcggtccgacctgggcatccgaaggaggacgcacgtccactcggatggctaagggagagccacgagctcctgtttaaaccagctccaattcgccctatagtgagtcgtattacgcgcgctcactggccgtcgttttacaacgtcgtgactgggaaaaccctggcgttacccaacttaatcgccttgcagcacatccccctttcgccagctggcgtaatagcgaagaggcccgcaccgatcgcccttcccaacagttgcgcagcctgaatggcgaatgggacgcgccctgtagcggcgcattaagcgcggcgggtgtggtggttacgcgcagcgtgaccgctacacttgccagcgccctagcgcccgctcctttcgctttcttcccttcctttctcgccacgttcgccggctttccccgtcaagctctaaatcgggggctccctttagggttccgatttagtgctttacggcacctcgaccccaaaaaacttgattagggtgatggttcacgtagtgggccatcgccctgatagacggtttttcgccctttgacgttggagtccacgttctttaatagtggactcttgttccaaactggaacaacactcaaccctatctcggtctattcttttgatttataagggattttgccgatttcggcctattggttaaaaaatgagctgatttaacaaaaatttaacgcgaattttaacaaaatattaacgcttacaatttaggtggcacttttcggggaaatgtgcgcggaacccctatttgtttatttttctaaatacattcaaatatgtatccgctcatgagacaataaccctgataaatgcttcaataatattgaaaaaggaagagtatgagtattcaacatttccgtgtcgcccttattcccttttttgcggcattttgccttcctgtttttgctcacccagaaacgctggtgaaagtaaaagatgctgaagatcagttgggtgcacgagtgggttacatcgaactggatctcaacagcggtaagatccttgagagttttcgccccgaagaacgttttccaatgatgagcacttttaaagttctgctatgtggcgcggtattatcccgtattgacgccgggcaagagcaactcggtcgccgcatacactattctcagaatgacttggttgagtactcaccagtcacagaaaagcatcttacggatggcatgacagtaagagaattatgcagtgctgccataaccatgagtgataacactgcggccaacttacttctgacaacgatcggaggaccgaaggagctaaccgcttttttgcacaacatgggggatcatgtaactcgccttgatcgttgggaaccggagctgaatgaagccataccaaacgacgagcgtgacaccacgatgcctgtagcaatggcaacaacgttgcgcaaactattaactggcgaactacttactctagcttcccggcaacaattaatagactggatggaggcggataaagttgcaggaccacttctgcgctcggcccttccggctggctggtttattgctgataaatctggagccggtgagcgtgggtctcgcggtatcattgcagcactggggccagatggtaagccctcccgtatcgtagttatctacacgacggggagtcaggcaactatggatgaacgaaatagacagatcgctgagataggtgcctcactgattaagcattggtaactgtcagaccaagtttactcatatatactttagattgatttaaaacttcatttttaatttaaaaggatctaggtgaagatcctttttgataatctcatgaccaaaatcccttaacgtgagttttcgttccactgagcgtcagaccccgtagaaaagatcaaaggatcttcttgagatcctttttttctgcgcgtaatctgctgcttgcaaacaaaaaaaccaccgctaccagcggtggtttgtttgccggatcaagagctaccaactctttttccgaaggtaactggcttcagcagagcgcagataccaaatactgttcttctagtgtagccgtagttaggccaccacttcaagaactctgtagcaccgcctacatacctcgctctgctaatcctgttaccagtggctgctgccagtggcgataagtcgtgtcttaccgggttggactcaagacgatagttaccggataaggcgcagcggtcgggctgaacggggggttcgtgcacacagcccagcttggagcgaacgacctacaccgaactgagatacctacagcgtgagctatgagaaagcgccacgcttcccgaagggagaaaggcggacaggtatccggtaagcggcagggtcggaacaggagagcgcacgagggagcttccagggggaaacgcctggtatctttatagtcctgtcgggtttcgccacctctgacttgagcgtcgatttttgtgatgctcgtcaggggggcggagcctatggaaaaacgccagcaacgcggcctttttacggttcctggccttttgctggccttttgctcacatgttctttcctgcgttatcccctgattctgtggataaccgtattaccgcctttgagtgagctgataccgctcgccgcagccgaacgaccgagcgcagcgagtcagtgagcgaggaagcggaagagcgcccaatacgcaaaccgcctctccccgcgcgttggccgattcattaatgcagctggcacgacaggtttcccgactggaaagcgggcagtgagcgcaacgcaattaatgtgagttagctcactcattaggcaccccaggctttacactttatgctcccggctcgtatgttgtgtggaattgtgagcggataacaatttcacacaggaaacagctatgaccatgattacgccaagcgcgcaattaaccctcactaaagggaacaaaagctgggtaccggcgcca

SEQ ID NO: 55 - DNA, 15593 bp, Artificial Sequence
  source: /note="Description of Artificial Sequence: Synthetic polynucleotide"
cgcgtcggctacaattaatacataaccttatgtatcatacacatacgatttaggtgacactatagatgggcggcgcatgagagaagcccagaccaattacctacccaaaatggagaaagttcacgttgacatcgaggaagacagcccattcctcagagctttgcagcggagcttcccgcagtttgaggtagaagccaagcaggtcactgataatgaccatgctaatgccagagcgttttcgcatctggcttcaaaactgatcgaaacggaggtggacccatccgacacgatccttgacattggaagtgcgcccgcccgcagaatgtattctaagcacaagtatcattgtatctgtccgatgagatgtgcggaagatccggacagattgtataagtatgcaactaagctgaagaaaaactgtaaggaaataactgataaggaattggacaagaaaatgaaggagctcgccgccgtcatgagcgaccctgacctggaaactgagactatgtgcctccacgacgacgagtcgtgtcgctacgaagggcaagtcgctgtttaccaggatgtatacgcggttgacggaccgacaagtctctatcaccaagccaataagggagttagagtcgcctactggataggctttgacaccaccccttttatgtttaagaacttggctggagcatatccatcatactctaccaactgggccgacgaaaccgtgttaacggctcgtaacataggcctatgcagctctgacgttatggagcggtcacgtagagggatgtccattcttagaaagaagtatttgaaaccatccaacaatgttctattctctgttggctcgaccatctaccacgagaagagggacttactgaggagctggcacctgccgtctgtatttcacttacgtggcaagcaaaattacacatgtcggtgtgagactatagttagttgcgacgggtacgtcgttaaaagaatagctatcagtccaggcctgtatgggaagccttcaggctatgctgctacgatgcaccgcgagggattcttgtgctgcaaagtgacagacacattgaacggggagagggtctcttttcccgtgtgcacgtatgtgccagctacattgtgtgaccaaatgactggcatactggcaacagatgtcagtgcggacgacgcgcaaaaactgctggttgggctcaaccagcgtatagtcgtcaacggtcgcacccagagaaacaccaataccatgaaaaattaccttttgcccgtagtggcccaggcatttgctaggtgggcaaaggaatataaggaagatcaagaagatgaaaggccactaggactacgagatagacagttagtcatggggtgttgttgggcttttagaaggcacaagataacatctatttataagcgcccggatacccaaaccatcatcaaagtgaacagcgatttccactcattcgtgctgcccaggataggcagtaacacattggagatcgggctgagaacaagaatcaggaaaatgttagaggagcacaaggagccgtcacctctcattaccgccgaggacgtacaagaagctaagtgcgcagccgatgaggctaaggaggtgcgtgaagccgaggagttgcgcgcagctctaccacctttggcagctgatgttgaggagcccactctggaagccgatgtagacttgatgttacaagaggctggggccggctcagtggagacacctcgtggcttgataaaggttaccagctacgctggcgaggacaagatcggctcttacgctgtgctttctccgcaggctgtactcaagagtgaaaaattatcttgcatccaccctctcgctgaacaagtcatagtgataacacactctggccgaaaagggcgttatgccgtggaaccataccatggtaaagtagtggtgccagagggacatgcaatacccgtccaggactttcaagctctgagtgaaagtgccaccattgtgtacaacgaacgtgagttcgtaaacaggtacctgcaccatattgccacacatggaggagcgctgaacactgatgaagaatattacaaaactgtcaagcccagcgagcacgacggcgaatacctgtacgacatcgacaggaaacagtgcgtcaagaaagaactagtcactgggctagggctcacaggcgagctggtggatcctcccttccatgaattcgcctacgagagtctgagaacacgaccagccgctccttaccaagtaccaaccataggggtgtatggcgtgccaggatcaggcaagtctggcatcattaaaagcgcagtcaccaaaaaagatctagtggtgagcgccaagaaagaaaactgtgcagaaattataagggacgtcaagaaaatgaaagggctggacgtcaatgccagaactgtggactcagtgctcttgaatggatgcaaacaccccgtagagaccctgtatattgacgaagcttttgcttgtcatgcaggtactctcagagcgctcatagccattataagacctaaaaaggcagtgctctgcggggatcccaaacagtgcggtttttttaacatgatgtgcctgaaagtgcattttaaccacgagatttgcacacaagtcttccacaaaagcatctctcgccgttgcactaaatctgtgacttcggtcgtctcaaccttgttttacgacaaaaaaatgagaacgacgaatccgaaagagactaagattgtgattgacactaccggcagtaccaaacctaagcaggacgatctcattctcacttgtttcagagggtgggtgaagcagttgcaaatagattacaaaggcaacgaaataatgacggcagctgcctctcaagggctgacccgtaaaggtgtgtatgccgttcggtacaaggtgaatgaaaatcctctgtacgcacccacctcagaacatgtgaacgtcctactgacccgcacggaggaccgcatcgtgtggaaaacactagccggcgacccatggataaaaacactgactgccaagtaccctgggaatttcactgccacgatagaggagtggcaagcagagcatgatgccatcatgaggcacatcttggagagaccggaccctaccgacgtcttccagaataaggcaaacgtgtgttgggccaaggctttagtgccggtgctgaagaccgctggcatagacatgaccactgaacaatggaacactgtggattattttgaaacggacaaagctcactcagcagagatagtattgaaccaactatgcgtgaggttctttggactcgatctggactccggtctattttctgcacccactgttccgttatccattaggaataatcactgggataactccccgtcgcctaacatgtacgggctgaataaagaagtggtccgtcagctctctcgcaggtacccacaactgcctcgggcagttgccactggaagagtctatgacatgaacactggtacactgcgcaattatgatccgcgcataaacctagtacctgtaaacagaagactgcctcatgctttagtcctccaccataatgaacacccacagagtgacttttcttcattcgtcagcaaattgaagggcagaactgtcctggtggtcggggaaaagttgtccgtcccaggcaaaatggttgactggttgtcagaccggcctgaggctaccttcagagctcggctggatttaggcatcccaggtgatgtgcccaaatatgacataatatttgttaatgtgaggaccccatataaataccatcactatcagcagtgtgaagaccatgccattaagcttagcatgttgaccaagaaagcttgtctgcatctgaatcccggcggaacctgtgtcagcataggttatggttacgctgacagggccagcgaaagcatcattggtgctatagcgcggcagttcaagttttcccgggtatgcaaaccgaaatcctcacttgaagagacggaagttctgtttgtattcattgggtacgatcgcaaggcccgtacgcacaatccttacaagctttcatcaaccttgaccaacatttatacaggttccagactccacgaagccggatgtgcaccctcatatcatgtggtgcgaggggatattgccacggccaccgaaggagtgattataaatgctgctaacagcaaaggacaacctggcggaggggtgtgcggagcgctgtataagaaattcccggaaagcttcgatttacagccgatcgaagtaggaaaagcgcgactggtcaaaggtgcagctaaacatatcattcatgccgtaggaccaaacttcaacaaagtttcggaggttgaaggtgacaaacagttggcagaggcttatgagtccatcgctaagattgtcaacgataacaattacaagtcagtagcgattccactgttgtccaccggcatcttttccgggaacaaagatcgactaacccaatcattgaaccatttgctgacagctttagacaccactgatgcagatgtagccatatactgcagggacaagaaatgggaaatgactctcaaggaagcagtggctaggagagaagcagtggaggagatatgcatatccgacgactcttcagtgacagaacctgatgcagagctggtgagggtgcatccgaagagttctttggctggaaggaagggctacagcacaagcgatggcaaaactttctcatatttggaagggaccaagtttcaccaggcggccaaggatatagcagaaattaatgccatgtggcccgttgcaacggaggccaatgagcaggtatgcatgtatatcctcggagaaagcatgagcagtattaggtcgaaatgccccgtcgaagagtcggaagcctcctcaccacctagcacgctgccttgcttgtgcatccatgccatgactccagaaagagtacagcgcctaaaagcctcacgtccagaacaaattactgtgtgctcatcctttccattgccgaagtatagaatcactggtgtgcagaagatccaatgctcccagcctatattgttctcaccgaaagtgcctgcgtatattcatccaaggaagtatctcgtggaaacaccaccggtagacgagactccggagccatcggcagagaaccaatccacagaggggacacctgaacaaccaccacttataaccgaggatgagaccaggactagaacgcctgagccgatcatcatcgaagaggaagaagaggatagcataagtttgctgtcagatggcccgacccaccaggtgctgcaagtcgaggcagacattcacgggccgccctctgtatctagctcatcctggtccattcctcatgcatccgactttgatgtggacagtttatccatacttgacaccctggagggagctagcgtgaccagcggggcaacgtcagccgagactaactcttacttcgcaaagagtatggagtttctggcgcgaccggtgcctgcgcctcgaacagtattcaggaaccctccacatcccgctccgcgcacaagaacaccgtcacttgcacccagcagggcctgctcgagagggatcacgggagaaaccgtgggatacgcggttacacacaatagcgagggcttcttgctatgcaaagttactgacacagtaaaaggagaacgggtatcgttccctgtgtgcacgtacatcccggccaccataaactcgagaaccagcctggtctccaacccgccaggcgtaaatagggtgattacaagagaggagtttgaggcgttcgtagcacaacaacaatgacggtttgatgcgggtgcatacatcttttcctccgacaccggtcaagggcatttacaacaaaaatcagtaaggcaaacggtgctatccgaagtggtgttggagaggaccgaattggagatttcgtatgccccgcgcctcgaccaagaaaaagaagaattactacgcaagaaattacagttaaatcccacacctgctaacagaagcagataccagtccaggaaggtggagaacatgaaagccataacagctagacgtattctgcaaggcctagggcattatttgaaggcagaaggaaaagtggagtgctaccgaaccctgcatcctgttcctttgtattcatctagtgtgaaccgtgccttttcaagccccaaggtcgcagtggaagcctgtaacgccatgttgaaagagaactttccgactgtggcttcttactgtattattccagagtacgatgcctatttggacatggttgacggagcttcatgctgcttagacactgccagtttttgccctgcaaagctgcgcagctttccaaagaaacactcctatttggaacccacaatacgatcggcagtgccttcagcgatccagaacacgctccagaacgtcctggcagctgccacaaaaagaaattgcaatgtcacgcaaatgagagaattgcccgtattggattcggcggcctttaatgtggaatgcttcaagaaatatgcgtgtaataatgaatattgggaaacgtttaaagaaaaccccatcaggcttactgaagaaaacgtggtaaattacattaccaaattaaaaggaccaaaagctgctgctctttttgcgaagacacataatttgaatatgttgcaggacataccaatggacaggtttgtaatggacttaaagagagacgtgaaagtgactccaggaacaaaacatactgaagaacggcccaaggtacaggtgatccaggctgccgatccgctagcaacagcgtatctgtgcggaatccaccgagagctggttaggagattaaatgcggtcctgcttccgaacattcatacactgtttgatatgtcggctgaagactttgacgctattatagccgagcacttccagcctggggattgtgttctggaaactgacatcgcgtcgtttgataaaagtgaggacgacgccatggctctgaccgcgttaatgattctggaagacttaggtgtggacgcagagctgttgacgctgattgaggcggctttcggcgaaatttcatcaatacatttgcccactaaaactaaatttaaattcggagccatgatgaaatctggaatgttcctcacactgtttgtgaacacagtcattaacattgtaatcgcaagcagagtgttgagagaacggctaaccggatcaccatgtgcagcattcattggagatgacaatatcgtgaaaggagtcaaatcggacaaattaatggcagacaggtgcgccacctggttgaatatggaagtcaagattatagatgctgtggtgggcgagaaagcgccttatttctgtggagggtttattttgtgtgactccgtgaccggcacagcgtgccgtgtggcagaccccctaaaaaggctgtttaagcttggcaaacctctggcagcagacgatgaacatgatgatgacaggagaagggcattgcatgaagagtcaacacgctggaaccgagtgggtattctttcagagctgtgcaaggcagtagaatcaaggtatgaaaccgtaggaacttccatcatagttatggccatgactactctagctagcagtgttaaatcattcagctacctgagaggggcccctataactctctacggctaacctgaatggactacgacatagtctagtcgacgccaccatgaggcctggcctgccctcctacctgatcatcctggccgtgtgcctgttcagccacctgctgtccagcagatacggcgccgaggccgtgagcgagcccctggacaaggctttccacctgctgctgaacacctacggcagacccatccggtttctgcgggagaacaccacccagtgcacctacaacagcagcctgcggaacagcaccgtcgtgagagagaacgccatcagcttcaactttttccagagctacaaccagtactacgtgttccacatgcccagatgcctgtttgccggccctctggccgagcagttcctgaaccaggtggacctgaccgagacactggaaagataccagcagcggctgaatacctacgccctggtgtccaaggacctggccagctaccggtcctttagccagcagctcaaggctcaggatagcctcggcgagcagcctaccaccgtgccccctcccatcgacctgagcatcccccacgtgtggatgcctccccagaccacccctcacggctggaccgagagccacaccacctccggcctgcacagaccccacttcaaccagacctgcatcctgttcgacggccacgacctgctgtttagcaccgtgaccccctgcctgcaccagggcttctacctgatcgacgagctgagatacgtgaagatcaccctgaccgaggatttcttcgtggtcaccgtgtccatcgacgacgacacccccatgctgctgatcttcggccacctgcccagagtgctgttcaaggccccctaccagcgggacaacttcatcctgcggcagaccgagaagcacgagctgctggtgctggtcaagaaggaccagctgaaccggcactcctacctgaaggaccccgacttcctggacgccgccctggacttcaactacctggacctgagcgccctgctgagaaacagcttccacagatacgccgtggacgtgctgaagtccggacggtgccagatgctcgatcggcggaccgtggagatggccttcgcctatgccctcgccctgttcgccgctgccagacaggaagaggctggcgcccaggtgtcagtgcccagagccctggatagacaggccgccctgctgcagatccaggaattcatgatcacctgcctgagccagaccccccctagaaccaccctgctgctgtaccccacagccgtggatctggccaagagggccctgtggacccccaaccagatcaccgacatcacaagcctcgtgcggctcgtgtacatcctgagcaagcagaaccagcagcacctgatcccccagtgggccctgagacagatcgccgacttcgccctgaagctgcacaagacccatctggccagctttctgagcgccttcgccaggcaggaactgtacctgatgggcagcctggtccacagcatgctggtgcataccaccgagcggcgggagatcttcatcgtggagacaggcctgtgtagcctggccgagctgtcccactttacccagctgctggcccaccctcaccacgagtacctgagcgacctgtacaccccctgcagcagcagcggcagacgggaccacagcctggaacggctgaccagactgttccccgatgccaccgtgcctgctacagtgcctgccgccctgtccatcctgtccaccatgcagcccagcaccctggaaaccttccccgacctgttctgcctgcccctgggcgagagctttagcgccctgaccgtgtccgagcacgtgtcctacatcgtgaccaatcagtacctgatcaagggcatcagctaccccgtgtccaccacagtcgtgggccagagcctgatcatcacccagaccgacagccagaccaagtgcgagctgacccggaacatgcacaccacacacagcatcaccgtggccctgaacatcagcctggaaaactgcgctttctgtcagtctgccctgctggaatacgacgatacccagggcgtgatcaacatcatgtacatgcacgacagcgacgacgtgctgttcgccctggacccctacaacgaggtggtggtgtccagcccccggacccactacctgatgctgctgaagaacggcaccgtgctggaagtgaccgacgtggtggtggacgccaccgacagcagactgctgatgatgagcgtgtacgccctgagcgccatcatcggcatctacctgctgtaccggatgctgaaaacctgctgataatctagacggcgcgcccacccagcggccgcctataactctctacggctaacctgaatggactacgacatagtctagtcgacgccaccatgtgcagaaggcccgactgcggcttcagcttcagccctggacccgtgatcctgctgtggtgctgcctgctgctgcctatcgtgtcctctgccgccgtgtctgtggcccctacagccgccgagaaggtgccagccgagtgccccgagctgaccagaagatgcctgctgggcgaggtgttcgagggcgacaagtacgagagctggctgcggcccctggtcaacgtgaccggcagagatggccccctgagccagctgatccggtacagacccgtgacccccgaggccgccaatagcgtgctgctggacgaggccttcctggataccctggccctgctgtacaacaaccccgaccagctgagagccctgctgaccctgctgtccagcgacaccgcccccagatggatgaccgtgatgcggggctacagcgagtgtggagatggcagccctgccgtgtacacctgcgtggacgacctgtgcagaggctacgacctgaccagactgagctacggccggtccatcttcacagagcacgtgctgggcttcgagctggtgccccccagcctgttcaacgtggtggtggccatccggaacgaggccaccagaaccaacagagccgtgcggctgcctgtgtctacagccgctgcacctgagggcatcacactgttctacggcctgtacaacgccgtgaaagagttctgcctccggcaccagctggatccccccctgctgagacacctggacaagtactacgccggcctgcccccagagctgaagcagaccagagtgaacctgcccgcccacagcagatatggccctcaggccgtggacgccagatgataatctagacggcgcgcccacccaatcgatctataactctctacggctaacctgaatggactacgacatagtctagtcgacgccaccatgggcaagaaagaaatgatcatggtcaagggcatccccaagatcatgctgctgattagcatcacctttctgctgctgtccctgatcaactgcaacgtgctggtcaacagccggggcaccagaagatcctggccctacaccgtgctgtcctaccggggcaaagagatcctgaagaagcagaaagaggacatcctgaagcggctgatgagcaccagcagcgacggctaccggttcctgatgtaccccagccagcagaaattccacgccatcgtgatcagcatggacaagttcccccaggactacatcctggccggacccatccggaacgacagcatcacccacatgtggttcgacttctacagcacccagctgcggaagcccgccaaatacgtgtacagcgagtacaaccacaccgcccacaagatcaccctgaggcctcccccttgtggcaccgtgcccagcatgaactgcctgagcgagatgctgaacgtgtccaagcggaacgacaccggcgagaagggctgcggcaacttcaccaccttcaaccccatgttcttcaacgtgccccggtggaacaccaagctgtacatcggcagcaacaaagtgaacgtggacagccagaccatctactttctgggcctgaccgccctgctgctgagatacgcccagcggaactgcacccggtccttctacctggtcaacgccatgagccggaacctgttccgggtgcccaagtacatcaacggcaccaagctgaagaacaccatgcggaagctgaagcggaagcaggccctggtcaaagagcagccccagaagaagaacaagaagtcccagagcaccaccaccccctacctgagctacaccacctccaccgccttcaacgtgaccaccaacgtgacctacagcgccacagccgccgtgaccagagtggccacaagcaccaccggctaccggcccgacagcaactttatgaagtccatcatggccacccagctgagagatctggccacctgggtgtacaccaccctgcggtacagaaacgagcccttctgcaagcccgaccggaacagaaccgccgtgagcgagttcatgaagaatacccacgtgctgatcagaaacgagacaccctacaccatctacggcaccctggacatgagcagcctgtactacaacgagacaatgagcgtggagaacgagacagccagcgacaacaacgaaaccacccccacctcccccagcacccggttccagcggaccttcatcgaccccctgtgggactacctggacagcctgctgttcctggacaagatccggaacttcagcctgcagctgcccgcctacggcaatctgaccccccctgagcacagaagggccgccaacctgagcaccctgaacagcctgtggtggtggagccagtgataatctagacggcgcgcccacccaccgcgggcaatatagcaacactaaaaactcgatgtacttccgaggaagcgcagtgcataatgctgcgcagtgttgccacataaccactatattaaccatttatctagcggacgccaaaaactcaatgtatttctgaggaagcgtggtgcataatgccacgcagcgtctgcataacttttattatttcttttattaatcaacaaaattttgtttttaacatttcaaaaaaaaaaaaaaaaaaaaaaaaaaaaaaaaaaaaaaaagggtcggcatggcatctccacctcctcgcggtccgacctgggcatccgaaggaggacgcacgtccactcggatggctaagggagagccacgagctcctgtttaaaccagctccaattcgccctatagtgagtcgtattacgcgcgctcactggccgtcgttttacaacgtcgtgactgggaaaaccctggcgttacccaacttaatcgccttgcagcacatccccctttcgccagctggcgtaatagcgaagaggcccgcaccgatcgcccttcccaacagttgcgcagcctgaatggcgaatgggacgcgccctgtagcggcgcattaagcgcggcgggtgtggtggttacgcgcagcgtgaccgctacacttgccagcgccctagcgcccgctcctttcgctttcttcccttcctttctcgccacgttcgccggctttccccgtcaagctctaaatcgggggctccctttagggttccgatttagtgctttacggcacctcgaccccaaaaaacttgattagggtgatggttcacgtagtgggccatcgccctgatagacggtttttcgccctttgacgttggagtccacgttctttaatagtggactcttgttccaaactggaacaacactcaaccctatctcggtctattcttttgatttataagggattttgccgatttcggcctattggttaaaaaatgagctgatttaacaaaaatttaacgcgaattttaacaaaatattaacgcttacaatttaggtggcacttttcggggaaatgtgcgcggaacccctatttgtttatttttctaaatacattcaaatatgtatccgctcatgagacaataaccctgataaatgcttcaataatattgaaaaaggaagagtatgagtattcaacatttccgtgtcgcccttattcccttttttgcggcattttgccttcctgtttttgctcacccagaaacgctggtgaaagtaaaagatgctgaagatcagttgggtgcacgagtgggttacatcgaactggatctcaacagcggtaagatccttgagagttttcgccccgaagaacgttttccaatgatgagcacttttaaagttctgctatgtggcgcggtattatcccgtattgacgccgggcaagagcaactcggtcgccgcatacactattctcagaatgacttggttgagtactcaccagtcacagaaaagcatcttacggatggcatgacagtaagagaattatgcagtgctgccataaccatgagtgataacactgcggccaacttacttctgacaacgatcggaggaccgaaggagctaaccgcttttttgcacaacatgggggatcatgtaactcgccttgatcgttgggaaccggagctgaatgaagccataccaaacgacgagcgtgacaccacgatgcctgtagcaatggcaacaacgttgcgcaaactattaactggcgaactacttactctagcttcccggcaacaattaatagactggatggaggcggataaagttgcaggaccacttctgcgctcggcccttccggctggctggtttattgctgataaatctggagccggtgagcgtgggtctcgcggtatcattgcagcactggggccagatggtaagccctcccgtatcgtagttatctacacgacggggagtcaggcaactatggatgaacgaaatagacagatcgctgagataggtgcctcactgattaagcattggtaactgtcagaccaagtttactcatatatactttagattgatttaaaacttcatttttaatttaaaaggatctaggtgaagatcctttttgataatctcatgaccaaaatcccttaacgtgagttttcgttccactgagcgtcagaccccgtagaaaagatcaaaggatcttcttgagatcctttttttctgcgcgtaatctgctgcttgcaaacaaaaaaaccaccgctaccagcggtggtttgtttgccggatcaagagctaccaactctttttccgaaggtaactggcttcagcagagcgcagataccaaatactgttcttctagtgtagccgtagttaggccaccacttcaagaactctgtagcaccgcctacatacctcgctctgctaatcctgttaccagtggctgctgccagtggcgataagtcgtgtcttaccgggttggactcaagacgatagttaccggataaggcgcagcggtcgggctgaacggggggttcgtgcacacagcccagcttggagcgaacgacctacaccgaactgagatacctacagcgtgagctatgagaaagcgccacgcttcccgaagggagaaaggcggacaggtatccggtaagcggcagggtcggaacaggagagcgcacgagggagcttccagggggaaacgcctggtatctttatagtcctgtcgggtttcgccacctctgacttgagcgtcgatttttgtgatgctcgtcaggggggcggagcctatggaaaaacgccagcaacgcggcctttttacggttcctggccttttgctggccttttgctcacatgttctttcctgcgttatcccctgattctgtggataaccgtattaccgcctttgagtgagctgataccgctcgccgcagccgaacgaccgagcgcagcgagtcagtgagcgaggaagcggaagagcgcccaatacgcaaaccgcctctccccgcgcgttggccgattcattaatgcagctggcacgacaggtttcccgactggaaagcgggcagtgagcgcaacgcaattaatgtgagttagctcactcattaggcaccccaggctttacactttatgctcccggctcgtatgttgtgtggaattgtgagcggataacaatttcacacaggaaacagctatgaccatgattacgccaagcgcgcaattaaccctcactaaagggaacaaaagctgggtaccggcgcca

SEQ ID NO: 56 - DNA, 15271 bp, Artificial Sequence
  source: /note="Description of Artificial Sequence: Synthetic polynucleotide"
ataggcggcgcatgagagaagcccagaccaattacctacccaaaatggagaaagttcacgttgacatcgaggaagacagcccattcctcagagctttgcagcggagcttcccgcagtttgaggtagaagccaagcaggtcactgataatgaccatgctaatgccagagcgttttcgcatctggcttcaaaactgatcgaaacggaggtggacccatccgacacgatccttgacattggaagtgcgcccgcccgcagaatgtattctaagcacaagtatcattgtatctgtccgatgagatgtgcggaagatccggacagattgtataagtatgcaactaagctgaagaaaaactgtaaggaaataactgataaggaattggacaagaaaatgaaggagctcgccgccgtcatgagcgaccctgacctggaaactgagactatgtgcctccacgacgacgagtcgtgtcgctacgaagggcaagtcgctgtttaccaggatgtatacgcggttgacggaccgacaagtctctatcaccaagccaataagggagttagagtcgcctactggataggctttgacaccaccccttttatgtttaagaacttggctggagcatatccatcatactctaccaactgggccgacgaaaccgtgttaacggctcgtaacataggcctatgcagctctgacgttatggagcggtcacgtagagggatgtccattcttagaaagaagtatttgaaaccatccaacaatgttctattctctgttggctcgaccatctaccacgagaagagggacttactgaggagctggcacctgccgtctgtatttcacttacgtggcaagcaaaattacacatgtcggtgtgagactatagttagttgcgacgggtacgtcgttaaaagaatagctatcagtccaggcctgtatgggaagccttcaggctatgctgctacgatgcaccgcgagggattcttgtgctgcaaagtgacagacacattgaacggggagagggtctcttttcccgtgtgcacgtatgtgccagctacattgtgtgaccaaatgactggcatactggcaacagatgtcagtgcggacgacgcgcaaaaactgctggttgggctcaaccagcgtatagtcgtcaacggtcgcacccagagaaacaccaataccatgaaaaattaccttttgcccgtagtggcccaggcatttgctaggtgggcaaaggaatataaggaagatcaagaagatgaaaggccactaggactacgagatagacagttagtcatggggtgttgttgggcttttagaaggcacaagataacatctatttataagcgcccggatacccaaaccatcatcaaagtgaacagcgatttccactcattcgtgctgcccaggataggcagtaacacattggagatcgggctgagaacaagaatcaggaaaatgttagaggagcacaaggagccgtcacctctcattaccgccgaggacgtacaagaagctaagtgcgcagccgatgaggctaaggaggtgcgtgaagccgaggagttgcgcgcagctctaccacctttggcagctgatgttgaggagcccactctggaagccgatgtagacttgatgttacaagaggctggggccggctcagtggagacacctcgtggcttgataaaggttaccagctacgatggcgaggacaagatcggctcttacgctgtgctttctccgcaggctgtactcaagagtgaaaaattatcttgcatccaccctctcgctgaacaagtcatagtgataacacactctggccgaaaagggcgttatgccgtggaaccataccatggtaaagtagtggtgccagagggacatgcaatacccgtccaggactttcaagctctgagtgaaagtgccaccattgtgtacaacgaacgtgagttcgtaaacaggtacctgcaccatattgccacacatggaggagcgctgaacactgatgaagaatattacaaaactgtcaagcccagcgagcacgacggcgaatacctgtacgacatcgacaggaaacagtgcgtcaagaaagaactagtcactgggctagggctcacaggcgagctggtggatcctcccttccatgaattcgcctacgagagtctgagaacacgaccagccgctccttaccaagtaccaaccataggggtgtatggcgtgccaggatcaggcaagtctggcatcattaaaagcgcagtcaccaaaaaagatctagtggtgagcgccaagaaagaaaactgtgcagaaattataagggacgtcaagaaaatgaaagggctggacgtcaatgccagaactgtggactcagtgctcttgaatggatgcaaacaccccgtagagaccctgtatattgacgaagcttttgcttgtcatgcaggtactctcagagcgctcatagccattataagacctaaaaaggcagtgctctgcggggatcccaaacagtgcggtttttttaacatgatgtgcctgaaagtgcattttaaccacgagatttgcacacaagtcttccacaaaagcatctctcgccgttgcactaaatctgtgacttcggtcgtctcaaccttgttttacgacaaaaaaatgagaacgacgaatccgaaagagactaagattgtgattgacactaccggcagtaccaaacctaagcaggacgatctcattctcacttgtttcagagggtgggtgaagcagttgcaaatagattacaaaggcaacgaaataatgacggcagctgcctctcaagggctgacccgtaaaggtgtgtatgccgttcggtacaaggtgaatgaaaatcctctgtacgcacccacctcagaacatgtgaacgtcctactgacccgcacggaggaccgcatcgtgtggaaaacactagccggcgacccatggataaaaacactgactgccaagtaccctgggaatttcactgccacgatagaggagtggcaagcagagcatgatgccatcatgaggcacatcttggagagaccggaccctaccgacgtcttccagaataaggcaaacgtgtgttgggccaaggctttagtgccggtgctgaagaccgctggcatagacatgaccactgaacaatggaacactgtggattattttgaaacggacaaagctcactcagcagagatagtattgaaccaactatgcgtgaggttctttggactcgatctggactccggtctattttctgcacccactgttccgttatccattaggaataatcactgggataactccccgtcgcctaacatgtacgggctgaataaagaagtggtccgtcagctctctcgcaggtacccacaactgcctcgggcagttgccactggaagagtctatgacatgaacactggtacactgcgcaattatgatccgcgcataaacctagtacctgtaaacagaagactgcctcatgctttagtcctccaccataatgaacacccacagagtgacttttcttcattcgtcagcaaattgaagggcagaactgtcctggtggtcggggaaaagttgtccgtcccaggcaaaatggttgactggttgtcagaccggcctgaggctaccttcagagctcggctggatttaggcatcccaggtgatgtgcccaaatatgacataatatttgttaatgtgaggaccccatataaataccatcactatcagcagtgtgaagaccatgccattaagcttagcatgttgaccaagaaagcttgtctgcatctgaatcccggcggaacctgtgtcagcataggttatggttacgctgacagggccagcgaaagcatcattggtgctatagcgcggcagttcaagttttcccgggtatgcaaaccgaaatcctcacttgaagagacggaagttctgtttgtattcattgggtacgatcgcaaggcccgtacgcacaatccttacaagctttcatcaaccttgaccaacatttatacaggttccagactccacgaagccggatgtgcaccctcatatcatgtggtgcgaggggatattgccacggccaccgaaggagtgattataaatgctgctaacagcaaaggacaacctggcggaggggtgtgcggagcgctgtataagaaattcccggaaagcttcgatttacagccgatcgaagtaggaaaagcgcgactggtcaaaggtgcagctaaacatatcattcatgccgtaggaccaaacttcaacaaagtttcggaggttgaaggtgacaaacagttggcagaggcttatgagtccatcgctaagattgtcaacgataacaattacaagtcagtagcgattccactgttgtccaccggcatcttttccgggaacaaagatcgactaacccaatcattgaaccatttgctgacagctttagacaccactgatgcagatgtagccatatactgcagggacaagaaatgggaaatgactctcaaggaagcagtggctaggagagaagcagtggaggagatatgcatatccgacgactcttcagtgacagaacctgatgcagagctggtgagggtgcatccgaagagttctttggctggaaggaagggctacagcacaagcgatggcaaaactttctcatatttggaagggaccaagtttcaccaggcggccaaggatatagcagaaattaatgccatgtggcccgttgcaacggaggccaatgagcaggtatgcatgtatatcctcggagaaagcatgagcagtattaggtcgaaatgccccgtcgaagagtcggaagcctccacaccacctagcacgctgccttgcttgtgcatccatgccatgactccagaaagagtacagcgcctaaaagcctcacgtccagaacaaattactgtgtgctcatcctttccattgccgaagtatagaatcactggtgtgcagaagatccaatgctcccagcctatattgttctcaccgaaagtgcctgcgtatattcatccaaggaagtatctcgtggaaacaccaccggtagacgagactccggagccatcggcagagaaccaatccacagaggggacacctgaacaaccaccacttataaccgaggatgagaccaggactagaacgcctgagccgatcatcatcgaagaggaagaagaggatagcataagtttgctgtcagatggcccgacccaccaggtgctgcaagtcgaggcagacattcacgggccgccctctgtatctagctcatcctggtccattcctcatgcatccgactttgatgtggacagtttatccatacttgacaccctggagggagctagcgtgaccagcggggcaacgtcagccgagactaactcttacttcgcaaagagtatggagtttctggcgcgaccggtgcctgcgcctcgaacagtattcaggaaccctccacatcccgctccgcgcacaagaacaccgtcacttgcacccagcagggcctgctcgagaaccagcctagtttccaccccgccaggcgtgaatagggtgatcactagagaggagctcgaggcgcttaccccgtcacgcactcctagcaggtcggtctcgagaaccagcctggtctccaacccgccaggcgtaaatagggtgattacaagagaggagtttgaggcgttcgtagcacaacaacaatgacggtttgatgcgggtgcatacatcttttcctccgacaccggtcaagggcatttacaacaaaaatcagtaaggcaaacggtgctatccgaagtggtgttggagaggaccgaattggagatttcgtatgccccgcgcctcgaccaagaaaaagaagaattactacgcaagaaattacagttaaatcccacacctgctaacagaagcagataccagtccaggaaggtggagaacatgaaagccataacagctagacgtattctgcaaggcctagggcattatttgaaggcagaaggaaaagtggagtgctaccgaaccctgcatcctgttcctttgtattcatctagtgtgaaccgtgccttttcaagccccaaggtcgcagtggaagcctgtaacgccatgttgaaagagaactttccgactgtggcttcttactgtattattccagagtacgatgcctatttggacatggttgacggagcttcatgctgcttagacactgccagtttttgccctgcaaagctgcgcagctttccaaagaaacactcctatttggaacccacaatacgatcggcagtgccttcagcgatccagaacacgctccagaacgtcctggcagctgccacaaaaagaaattgcaatgtcacgcaaatgagagaattgcccgtattggattcggcggcctttaatgtggaatgcttcaagaaatatgcgtgtaataatgaatattgggaaacgtttaaagaaaaccccatcaggcttactgaagaaaacgtggtaaattacattaccaaattaaaaggaccaaaagctgctgctctttttgcgaagacacataatttgaatatgttgcaggacataccaatggacaggtttgtaatggacttaaagagagacgtgaaagtgactccaggaacaaaacatactgaagaacggcccaaggtacaggtgatccaggctgccgatccgctagcaacagcgtatctgtgcggaatccaccgagagctggttaggagattaaatgcggtcctgcttccgaacattcatacactgtttgatatgtcggctgaagactttgacgctattatagccgagcacttccagcctggggattgtgttctggaaactgacatcgcgtcgtttgataaaagtgaggacgacgccatggctctgaccgcgttaatgattctggaagacttaggtgtggacgcagagctgttgacgctgattgaggcggctttcggcgaaatttcatcaatacatttgcccactaaaactaaatttaaattcggagccatgatgaaatctggaatgttcctcacactgtttgtgaacacagtcattaacattgtaatcgcaagcagagtgttgagagaacggctaaccggatcaccatgtgcagcattcattggagatgacaatatcgtgaaaggagtcaaatcggacaaattaatggcagacaggtgcgccacctggttgaatatggaagtcaagattatagatgctgtggtgggcgagaaagcgccttatttctgtggagggtttattttgtgtgactccgtgaccggcacagcgtgccgtgtggcagaccccctaaaaaggctgtttaagcttggcaaacctctggcagcagacgatgaacatgatgatgacaggagaagggcattgcatgaagagtcaacacgctggaaccgagtgggtattctttcagagctgtgcaaggcagtagaatcaaggtatgaaaccgtaggaacttccatcatagttatggccatgactactctagctagcagtgttaaatcattcagctacctgagaggggcccctataactctctacggctaacctgaatggactacgacatagtctagtccgccaagatgaggcctggcctgccctcctacctgatcatcctggccgtgtgcctgttcagccacctgctgtccagcagatacggcgccgaggccgtgagcgagcccctggacaaggctttccacctgctgctgaacacctacggcagacccatccggtttctgcgggagaacaccacccagtgcacctacaacagcagcctgcggaacagcaccgtcgtgagagagaacgccatcagcttcaactttttccagagctacaaccagtactacgtgttccacatgcccagatgcctgtttgccggccctctggccgagcagttcctgaaccaggtggacctgaccgagacactggaaagataccagcagcggctgaatacctacgccctggtgtccaaggacctggccagctaccggtcctttagccagcagctcaaggctcaggatagcctcggcgagcagcctaccaccgtgccccctcccatcgacctgagcatcccccacgtgtggatgcctccccagaccacccctcacggctggaccgagagccacaccacctccggcctgcacagaccccacttcaaccagacctgcatcctgttcgacggccacgacctgctgtttagcaccgtgaccccctgcctgcaccagggcttctacctgatcgacgagctgagatacgtgaagatcaccctgaccgaggatttcttcgtggtcaccgtgtccatcgacgacgacacccccatgctgctgatcttcggccacctgcccagagtgctgttcaaggccccctaccagcgggacaacttcatcctgcggcagaccgagaagcacgagctgctggtgctggtcaagaaggaccagctgaaccggcactcctacctgaaggaccccgacttcctggacgccgccctggacttcaactacctggacctgagcgccctgctgagaaacagcttccacagatacgccgtggacgtgctgaagtccggacggtgccagatgctcgatcggcggaccgtggagatggccttcgcctatgccctcgccctgttcgccgctgccagacaggaagaggctggcgcccaggtgtcagtgcccagagccctggatagacaggccgccctgctgcagatccaggaattcatgatcacctgcctgagccagaccccccctagaaccaccctgctgctgtaccccacagccgtggatctggccaagagggccctgtggacccccaaccagatcaccgacatcacaagcctcgtgcggctcgtgtacatcctgagcaagcagaaccagcagcacctgatcccccagtgggccctgagacagatcgccgacttcgccctgaagctgcacaagacccatctggccagctttctgagcgccttcgccaggcaggaactgtacctgatgggcagcctggtccacagcatgctggtgcataccaccgagcggcgggagatcttcatcgtggagacaggcctgtgtagcctggccgagctgtcccactttacccagctgctggcccaccctcaccacgagtacctgagcgacctgtacaccccctgcagcagcagcggcagacgggaccacagcctggaacggctgaccagactgttccccgatgccaccgtgcctgctacagtgcctgccgccctgtccatcctgtccaccatgcagcccagcaccctggaaaccttccccgacctgttctgcctgcccctgggcgagagctttagcgccctgaccgtgtccgagcacgtgtcctacatcgtgaccaatcagtacctgatcaagggcatcagctaccccgtgtccaccacagtcgtgggccagagcctgatcatcacccagaccgacagccagaccaagtgcgagctgacccggaacatgcacaccacacacagcatcaccgtggccctgaacatcagcctggaaaactgcgctttctgtcagtctgccctgctggaatacgacgatacccagggcgtgatcaacatcatgtacatgcacgacagcgacgacgtgctgttcgccctggacccctacaacgaggtggtggtgtccagcccccggacccactacctgatgctgctgaagaacggcaccgtgctggaagtgaccgacgtggtggtggacgccaccgacagcagactgctgatgatgagcgtgtacgccctgagcgccatcatcggcatctacctgctgtaccggatgctgaaaacctgctgataatctagaggcccctataactctctacggctaacctgaatggactacgacatagtctagtccgccaagatgtgcagaaggcccgactgcggcttcagcttcagccctggacccgtgatcctgctgtggtgctgcctgctgctgcctatcgtgtcctctgccgccgtgtctgtggcccctacagccgccgagaaggtgccagccgagtgccccgagctgaccagaagatgcctgctgggcgaggtgttcgagggcgacaagtacgagagctggctgcggcccctggtcaacgtgaccggcagagatggccccctgagccagctgatccggtacagacccgtgacccccgaggccgccaatagcgtgctgctggacgaggccttcctggataccctggccctgctgtacaacaaccccgaccagctgagagccctgctgaccctgctgtccagcgacaccgcccccagatggatgaccgtgatgcggggctacagcgagtgtggagatggcagccctgccgtgtacacctgcgtggacgacctgtgcagaggctacgacctgaccagactgagctacggccggtccatcttcacagagcacgtgctgggcttcgagctggtgccccccagcctgttcaacgtggtggtggccatccggaacgaggccaccagaaccaacagagccgtgcggctgcctgtgtctacagccgctgcacctgagggcatcacactgttctacggcctgtacaacgccgtgaaagagttctgcctccggcaccagctggatccccccctgctgagacacctggacaagtactacgccggcctgcccccagagctgaagcagaccagagtgaacctgcccgcccacagcagatatggccctcaggccgtggacgccagatgataacgccggcggcccctataactctctacggctaacctgaatggactacgacatagtctagtccgccaagatgagccccaaggacctgacccccttcctgacaaccctgtggctgctcctgggccatagcagagtgcctagagtgcgggccgaggaatgctgcgagttcatcaacgtgaaccacccccccgagcggtgctacgacttcaagatgtgcaaccggttcaccgtggccctgagatgccccgacggcgaagtgtgctacagccccgagaaaaccgccgagatccggggcatcgtgaccaccatgacccacagcctgacccggcaggtggtgcacaacaagctgaccagctgcaactacaaccccctgtacctggaagccgacggccggatcagatgcggcaaagtgaacgacaaggcccagtacctgctgggagccgccggaagcgtgccctaccggtggatcaacctggaatacgacaagatcacccggatcgtgggcctggaccagtacctggaaagcgtgaagaagcacaagcggctggacgtgtgcagagccaagatgggctacatgctgcagctgttgaattttgaccttcttaagcttgcgggagacgtcgagtccaaccccgggcccatgctgcggctgctgctgagacaccacttccactgcctgctgctgtgtgccgtgtgggccaccccttgtctggccagcccttggagcaccctgaccgccaaccagaaccctagccccccttggtccaagctgacctacagcaagccccacgacgccgccaccttctactgcccctttctgtaccccagccctcccagaagccccctgcagttcagcggcttccagagagtgtccaccggccctgagtgccggaacgagacactgtacctgctgtacaaccgggagggccagacactggtggagcggagcagcacctgggtgaaaaaagtgatctggtatctgagcggccggaaccagaccatcctgcagcggatgcccagaaccgccagcaagcccagcgacggcaacgtgcagatcagcgtggaggacgccaaaatcttcggcgcccacatggtgcccaagcagaccaagctgctgagattcgtggtcaacgacggcaccagatatcagatgtgcgtgatgaagctggaaagctgggcccacgtgttccgggactactccgtgagcttccaggtccggctgaccttcaccgaggccaacaaccagacctacaccttctgcacccaccccaacctgatcgtgctgctgaacttcgacctgctgaagctggccggcgacgtggagagcaaccccggcccccatatgcggctgtgcagagtgtggctgtccgtgtgcctgtgtgccgtggtgctgggccagtgccagagagagacagccgagaagaacgactactaccgggtgccccactactgggatgcctgcagcagagccctgcccgaccagacccggtacaaatacgtggagcagctcgtggacctgaccctgaactaccactacgacgccagccacggcctggacaacttcgacgtgctgaagcggatcaacgtgaccgaggtgtccctgctgatcagcgacttccggcggcagaacagaagaggcggcaccaacaagcggaccaccttcaacgccgctggctctctggcccctcacgccagatccctggaattcagcgtgcggctgttcgccaactgataacgttgcatcctgcaggatacagcagcaattggcaagctgcttacatagaactcgcggcgattggcatgccgccttaaaatttttattttatttttcttttcttttccgaatcggattttgtttttaatatttcaaaaaaaaaaaaaaaaaaaaaaaaaaaaaaaaaaagggtcggcatggcatctccacctcctcgcggtccgacctgggcatccgaaggaggacgcacgtccactcggatggctaagggagagccacgtttaaacgctagagcaagacgtttcccgttgaatatggctcataacaccccttgtattactgtttatgtaagcagacagttttattgttcatgatgatatatttttatcttgtgcaatgtaacatcagagattttgagacacaacgtggctttgttgaataaatcgaacttttgctgagttgaaggatcagatcacgcatcttcccgacaacgcagaccgttccgtggcaaagcaaaagttcaaaatcaccaactggtccacctacaacaaagctctcatcaaccgtggctccctcactttctggctggatgatggggcgattcaggcctggtatgagtcagcaacaccttcttcacgaggcagacctcagcgctagcggagtgtatactggcttactatgttggcactgatgagggtgtcagtgaagtgcttcatgtggcaggagaaaaaaggctgcaccggtgcgtcagcagaatatgtgatacaggatatattccgcttcctcgctcactgactcgctacgctcggtcgttcgactgcggcgagcggaaatggcttacgaacggggcggagatttcctggaagatgccaggaagatacttaacagggaagtgagagggccgcggcaaagccgtttttccataggctccgcccccctgacaagcatcacgaaatctgacgctcaaatcagtggtggcgaaacccgacaggactataaagataccaggcgtttcccctggcggctccctcgtgcgctctcctgttcctgcctttcggtttaccggtgtcattccgctgttatggccgcgtttgtctcattccacgcctgacactcagttccgggtaggcagttcgctccaagctggactgtatgcacgaaccccccgttcagtccgaccgctgcgccttatccggtaactatcgtcttgagtccaacccggaaagacatgcaaaagcaccactggcagcagccactggtaattgatttagaggagttagtcttgaagtcatgcgccggttaaggctaaactgaaaggacaagttttggtgactgcgctcctccaagccagttacctcggttcaaagagttggtagctcagagaaccttcgaaaaaccgccctgcaaggcggttttttcgttttcagagcaagagattacgcgcagaccaaaacgatctcaagaagatcatcttattaaggggtctgacgctcagtggaacgaaaactcacgttaagggattttggtcatgagattatcaaaaaggatcttcacctagatccttttaaattaaaaatgaagttttaaatcaatctaaagtatatatgagtaaacttggtctgacagttattagaaaaattcatccagcagacgataaaacgcaatacgctggctatccggtgccgcaatgccatacagcaccagaaaacgatccgcccattcgccgcccagttcttccgcaatatcacgggtggccagcgcaatatcctgataacgatccgccacgcccagacggccgcaatcaataaagccgctaaaacggccattttccaccataatgttcggcaggcacgcatcaccatgggtcaccaccagatcttcgccatccggcatgctcgctttcagacgcgcaaacagctctgccggtgccaggccctgatgttcttcatccagatcatcctgatccaccaggcccgcttccatacgggtacgcgcacgttcaatacgatgtttcgcctgatgatcaaacggacaggtcgccgggtccagggtatgcagacgacgcatggcatccgccataatgctcactttttctgccggcgccagatggctagacagcagatcctgacccggcacttcgcccagcagcagccaatcacggcccgcttcggtcaccacatccagcaccgccgcacacggaacaccggtggtggccagccagctcagacgcgccgcttcatcctgcagctcgttcagcgcaccgctcagatcggttttcacaaacagcaccggacgaccctgcgcgctcagacgaaacaccgccgcatcagagcagccaatggtctgctgcgcccaatcatagccaaacagacgttccacccacgctgccgggctacccgcatgcaggccatcctgttcaatcatactcttcctttttcaatattattgaagcatttatcagggttattgtctcatgagcggatacatatttgaatgtatttagaaaaataaacaaataggggttccgcgcacatttccccgaaaagtgccacctaaattgtaagcgttaatattttgttaaaattcgcgttaaatttttgttaaatcagctcattttttaaccaataggccgaaatcggcaaaatcccttataaatcaaaagaatagaccgagatagggttgagtggccgctacagggcgctcccattcgccattcaggctgcgcaactgttgggaagggcgtttcggtgcgggcctcttcgctattacgccagctggcgaaagggggatgtgctgcaaggcgattaagttgggtaacgccagggttttcccagtcacacgcgtaatacgactcactatag

SEQ ID NO: 57 - DNA, 16405 bp, Artificial Sequence
  source: /note="Description of Artificial Sequence: Synthetic polynucleotide"
ataggcggcgcatgagagaagcccagaccaattacctacccaaaatggagaaagttcacgttgacatcgaggaagacagcccattcctcagagctttgcagcggagcttcccgcagtttgaggtagaagccaagcaggtcactgataatgaccatgctaatgccagagcgttttcgcatctggcttcaaaactgatcgaaacggaggtggacccatccgacacgatccttgacattggaagtgcgcccgcccgcagaatgtattctaagcacaagtatcattgtatctgtccgatgagatgtgcggaagatccggacagattgtataagtatgcaactaagctgaagaaaaactgtaaggaaataactgataaggaattggacaagaaaatgaaggagctcgccgccgtcatgagcgaccctgacctggaaactgagactatgtgcctccacgacgacgagtcgtgtcgctacgaagggcaagtcgctgtttaccaggatgtatacgcggttgacggaccgacaagtctctatcaccaagccaataagggagttagagtcgcctactggataggctttgacaccaccccttttatgtttaagaacttggctggagcatatccatcatactctaccaactgggccgacgaaaccgtgttaacggctcgtaacataggcctatgcagctctgacgttatggagcggtcacgtagagggatgtccattcttagaaagaagtatttgaaaccatccaacaatgttctattctctgttggctcgaccatctaccacgagaagagggacttactgaggagctggcacctgccgtctgtatttcacttacgtggcaagcaaaattacacatgtcggtgtgagactatagttagttgcgacgggtacgtcgttaaaagaatagctatcagtccaggcctgtatgggaagccttcaggctatgctgctacgatgcaccgcgagggattcttgtgctgcaaagtgacagacacattgaacggggagagggtctcttttcccgtgtgcacgtatgtgccagctacattgtgtgaccaaatgactggcatactggcaacagatgtcagtgcggacgacgcgcaaaaactgctggttgggctcaaccagcgtatagtcgtcaacggtcgcacccagagaaacaccaataccatgaaaaattaccttttgcccgtagtggcccaggcatttgctaggtgggcaaaggaatataaggaagatcaagaagatgaaaggccactaggactacgagatagacagttagtcatggggtgttgttgggcttttagaaggcacaagataacatctatttataagcgcccggatacccaaaccatcatcaaagtgaacagcgatttccactcattcgtgctgcccaggataggcagtaacacattggagatcgggctgagaacaagaatcaggaaaatgttagaggagcacaaggagccgtcacctctcattaccgccgaggacgtacaagaagctaagtgcgcagccgatgaggctaaggaggtgcgtgaagccgaggagttgcgcgcagctctaccacctttggcagctgatgttgaggagcccactctggaagccgatgtagacttgatgttacaagaggctggggccggctcagtggagacacctcgtggcttgataaaggttaccagctacgatggcgaggacaagatcggctcttacgctgtgctttctccgcaggctgtactcaagagtgaaaaattatcttgcatccaccctctcgctgaacaagtcatagtgataacacactctggccgaaaagggcgttatgccgtggaaccataccatggtaaagtagtggtgccagagggacatgcaatacccgtccaggactttcaagctctgagtgaaagtgccaccattgtgtacaacgaacgtgagttcgtaaacaggtacctgcaccatattgccacacatggaggagcgctgaacactgatgaagaatattacaaaactgtcaagcccagcgagcacgacggcgaatacctgtacgacatcgacaggaaacagtgcgtcaagaaagaactagtcactgggctagggctcacaggcgagctggtggatcctcccttccatgaattcgcctacgagagtctgagaacacgaccagccgctccttaccaagtaccaaccataggggtgtatggcgtgccaggatcaggcaagtctggcatcattaaaagcgcagtcaccaaaaaagatctagtggtgagcgccaagaaagaaaactgtgcagaaattataagggacgtcaagaaaatgaaagggctggacgtcaatgccagaactgtggactcagtgctcttgaatggatgcaaacaccccgtagagaccctgtatattgacgaagcttttgcttgtcatgcaggtactctcagagcgctcatagccattataagacctaaaaaggcagtgctctgcggggatcccaaacagtgcggtttttttaacatgatgtgcctgaaagtgcattttaaccacgagatttgcacacaagtcttccacaaaagcatctctcgccgttgcactaaatctgtgacttcggtcgtctcaaccttgttttacgacaaaaaaatgagaacgacgaatccgaaagagactaagattgtgattgacactaccggcagtaccaaacctaagcaggacgatctcattctcacttgtttcagagggtgggtgaagcagttgcaaatagattacaaaggcaacgaaataatgacggcagctgcctctcaagggctgacccgtaaaggtgtgtatgccgttcggtacaaggtgaatgaaaatcctctgtacgcacccacctcagaacatgtgaacgtcctactgacccgcacggaggaccgcatcgtgtggaaaacactagccggcgacccatggataaaaacactgactgccaagtaccctgggaatttcactgccacgatagaggagtggcaagcagagcatgatgccatcatgaggcacatcttggagagaccggaccctaccgacgtcttccagaataaggcaaacgtgtgttgggccaaggctttagtgccggtgctgaagaccgctggcatagacatgaccactgaacaatggaacactgtggattattttgaaacggacaaagctcactcagcagagatagtattgaaccaactatgcgtgaggttctttggactcgatctggactccggtctattttctgcacccactgttccgttatccattaggaataatcactgggataactccccgtcgcctaacatgtacgggctgaataaagaagtggtccgtcagctctctcgcaggtacccacaactgcctcgggcagttgccactggaagagtctatgacatgaacactggtacactgcgcaattatgatccgcgcataaacctagtacctgtaaacagaagactgcctcatgctttagtcctccaccataatgaacacccacagagtgacttttcttcattcgtcagcaaattgaagggcagaactgtcctggtggtcggggaaaagttgtccgtcccaggcaaaatggttgactggttgtcagaccggcctgaggctaccttcagagctcggctggatttaggcatcccaggtgatgtgcccaaatatgacataatatttgttaatgtgaggaccccatataaataccatcactatcagcagtgtgaagaccatgccattaagcttagcatgttgaccaagaaagcttgtctgcatctgaatcccggcggaacctgtgtcagcataggttatggttacgctgacagggccagcgaaagcatcattggtgctatagcgcggcagttcaagttttcccgggtatgcaaaccgaaatcctcacttgaagagacggaagttctgtttgtattcattgggtacgatcgcaaggcccgtacgcacaatccttacaagctttcatcaaccttgaccaacatttatacaggttccagactccacgaagccggatgtgcaccctcatatcatgtggtgcgaggggatattgccacggccaccgaaggagtgattataaatgctgctaacagcaaaggacaacctggcggaggggtgtgcggagcgctgtataagaaattcccggaaagcttcgatttacagccgatcgaagtaggaaaagcgcgactggtcaaaggtgcagctaaacatatcattcatgccgtaggaccaaacttcaacaaagtttcggaggttgaaggtgacaaacagttggcagaggcttatgagtccatcgctaagattgtcaacgataacaattacaagtcagtagcgattccactgttgtccaccggcatcttttccgggaacaaagatcgactaacccaatcattgaaccatttgctgacagctttagacaccactgatgcagatgtagccatatactgcagggacaagaaatgggaaatgactctcaaggaagcagtggctaggagagaagcagtggaggagatatgcatatccgacgactcttcagtgacagaacctgatgcagagctggtgagggtgcatccgaagagttctttggctggaaggaagggctacagcacaagcgatggcaaaactttctcatatttggaagggaccaagtttcaccaggcggccaaggatatagcagaaattaatgccatgtggcccgttgcaacggaggccaatgagcaggtatgcatgtatatcctcggagaaagcatgagcagtattaggtcgaaatgccccgtcgaagagtcggaagcctccacaccacctagcacgctgccttgcttgtgcatccatgccatgactccagaaagagtacagcgcctaaaagcctcacgtccagaacaaattactgtgtgctcatcctttccattgccgaagtatagaatcactggtgtgcagaagatccaatgctcccagcctatattgttctcaccgaaagtgcctgcgtatattcatccaaggaagtatctcgtggaaacaccaccggtagacgagactccggagccatcggcagagaaccaatccacagaggggacacctgaacaaccaccacttataaccgaggatgagaccaggactagaacgcctgagccgatcatcatcgaagaggaagaagaggatagcataagtttgctgtcagatggcccgacccaccaggtgctgcaagtcgaggcagacattcacgggccgccctctgtatctagctcatcctggtccattcctcatgcatccgactttgatgtggacagtttatccatacttgacaccctggagggagctagcgtgaccagcggggcaacgtcagccgagactaactcttacttcgcaaagagtatggagtttctggcgcgaccggtgcctgcgcctcgaacagtattcaggaaccctccacatcccgctccgcgcacaagaacaccgtcacttgcacccagcagggcctgctcgagaaccagcctagtttccaccccgccaggcgtgaatagggtgatcactagagaggagctcgaggcgcttaccccgtcacgcactcctagcaggtcggtctcgagaaccagcctggtctccaacccgccaggcgtaaatagggtgattacaagagaggagtttgaggcgttcgtagcacaacaacaatgacggtttgatgcgggtgcatacatcttttcctccgacaccggtcaagggcatttacaacaaaaatcagtaaggcaaacggtgctatccgaagtggtgttggagaggaccgaattggagatttcgtatgccccgcgcctcgaccaagaaaaagaagaattactacgcaagaaattacagttaaatcccacacctgctaacagaagcagataccagtccaggaaggtggagaacatgaaagccataacagctagacgtattctgcaaggcctagggcattatttgaaggcagaaggaaaagtggagtgctaccgaaccctgcatcctgttcctttgtattcatctagtgtgaaccgtgccttttcaagccccaaggtcgcagtggaagcctgtaacgccatgttgaaagagaactttccgactgtggcttcttactgtattattccagagtacgatgcctatttggacatggttgacggagcttcatgctgcttagacactgccagtttttgccctgcaaagctgcgcagctttccaaagaaacactcctatttggaacccacaatacgatcggcagtgccttcagcgatccagaacacgctccagaacgtcctggcagctgccacaaaaagaaattgcaatgtcacgcaaatgagagaattgcccgtattggattcggcggcctttaatgtggaatgcttcaagaaatatgcgtgtaataatgaatattgggaaacgtttaaagaaaaccccatcaggcttactgaagaaaacgtggtaaattacattaccaaattaaaaggaccaaaagctgctgctctttttgcgaagacacataatttgaatatgttgcaggacataccaatggacaggtttgtaatggacttaaagagagacgtgaaagtgactccaggaacaaaacatactgaagaacggcccaaggtacaggtgatccaggctgccgatccgctagcaacagcgtatctgtgcggaatccaccgagagctggttaggagattaaatgcggtcctgcttccgaacattcatacactgtttgatatgtcggctgaagactttgacgctattatagccgagcacttccagcctggggattgtgttctggaaactgacatcgcgtcgtttgataaaagtgaggacgacgccatggctctgaccgcgttaatgattctggaagacttaggtgtggacgcagagctgttgacgctgattgaggcggctttcggcgaaatttcatcaatacatttgcccactaaaactaaatttaaattcggagccatgatgaaatctggaatgttcctcacactgtttgtgaacacagtcattaacattgtaatcgcaagcagagtgttgagagaacggctaaccggatcaccatgtgcagcattcattggagatgacaatatcgtgaaaggagtcaaatcggacaaattaatggcagacaggtgcgccacctggttgaatatggaagtcaagattatagatgctgtggtgggcgagaaagcgccttatttctgtggagggtttattttgtgtgactccgtgaccggcacagcgtgccgtgtggcagaccccctaaaaaggctgtttaagcttggcaaacctctggcagcagacgatgaacatgatgatgacaggagaagggcattgcatgaagagtcaacacgctggaaccgagtgggtattctttcagagctgtgcaaggcagtagaatcaaggtatgaaaccgtaggaacttccatcatagttatggccatgactactctagctagcagtgttaaatcattcagctacctgagaggggcccctataactctctacggctaacctgaatggactacgacatagtctagtccgccaagatgaggcctggcctgccctcctacctgatcatcctggccgtgtgcctgttcagccacctgctgtccagcagatacggcgccgaggccgtgagcgagcccctggacaaggctttccacctgctgctgaacacctacggcagacccatccggtttctgcgggagaacaccacccagtgcacctacaacagcagcctgcggaacagcaccgtcgtgagagagaacgccatcagcttcaactttttccagagctacaaccagtactacgtgttccacatgcccagatgcctgtttgccggccctctggccgagcagttcctgaaccaggtggacctgaccgagacactggaaagataccagcagcggctgaatacctacgccctggtgtccaaggacctggccagctaccggtcctttagccagcagctcaaggctcaggatagcctcggcgagcagcctaccaccgtgccccctcccatcgacctgagcatcccccacgtgtggatgcctccccagaccacccctcacggctggaccgagagccacaccacctccggcctgcacagaccccacttcaaccagacctgcatcctgttcgacggccacgacctgctgtttagcaccgtgaccccctgcctgcaccagggcttctacctgatcgacgagctgagatacgtgaagatcaccctgaccgaggatttcttcgtggtcaccgtgtccatcgacgacgacacccccatgctgctgatcttcggccacctgcccagagtgctgttcaaggccccctaccagcgggacaacttcatcctgcggcagaccgagaagcacgagctgctggtgctggtcaagaaggaccagctgaaccggcactcctacctgaaggaccccgacttcctggacgccgccctggacttcaactacctggacctgagcgccctgctgagaaacagcttccacagatacgccgtggacgtgctgaagtccggacggtgccagatgctcgatcggcggaccgtggagatggccttcgcctatgccctcgccctgttcgccgctgccagacaggaagaggctggcgcccaggtgtcagtgcccagagccctggatagacaggccgccctgctgcagatccaggaattcatgatcacctgcctgagccagaccccccctagaaccaccctgctgctgtaccccacagccgtggatctggccaagagggccctgtggacccccaaccagatcaccgacatcacaagcctcgtgcggctcgtgtacatcctgagcaagcagaaccagcagcacctgatcccccagtgggccctgagacagatcgccgacttcgccctgaagctgcacaagacccatctggccagctttctgagcgccttcgccaggcaggaactgtacctgatgggcagcctggtccacagcatgctggtgcataccaccgagcggcgggagatcttcatcgtggagacaggcctgtgtagcctggccgagctgtcccactttacccagctgctggcccaccctcaccacgagtacctgagcgacctgtacaccccctgcagcagcagcggcagacgggaccacagcctggaacggctgaccagactgttccccgatgccaccgtgcctgctacagtgcctgccgccctgtccatcctgtccaccatgcagcccagcaccctggaaaccttccccgacctgttctgcctgcccctgggcgagagctttagcgccctgaccgtgtccgagcacgtgtcctacatcgtgaccaatcagtacctgatcaagggcatcagctaccccgtgtccaccacagtcgtgggccagagcctgatcatcacccagaccgacagccagaccaagtgcgagctgacccggaacatgcacaccacacacagcatcaccgtggccctgaacatcagcctggaaaactgcgctttctgtcagtctgccctgctggaatacgacgatacccagggcgtgatcaacatcatgtacatgcacgacagcgacgacgtgctgttcgccctggacccctacaacgaggtggtggtgtccagcccccggacccactacctgatgctgctgaagaacggcaccgtgctggaagtgaccgacgtggtggtggacgccaccgacagcagactgctgatgatgagcgtgtacgccctgagcgccatcatcggcatctacctgctgtaccggatgctgaaaacctgctgataatctagaggcccctataactctctacggctaacctgaatggactacgacatagtctagtccgccaagatgtgcagaaggcccgactgcggcttcagcttcagccctggacccgtgatcctgctgtggtgctgcctgctgctgcctatcgtgtcctctgccgccgtgtctgtggcccctacagccgccgagaaggtgccagccgagtgccccgagctgaccagaagatgcctgctgggcgaggtgttcgagggcgacaagtacgagagctggctgcggcccctggtcaacgtgaccggcagagatggccccctgagccagctgatccggtacagacccgtgacccccgaggccgccaatagcgtgctgctggacgaggccttcctggataccctggccctgctgtacaacaaccccgaccagctgagagccctgctgaccctgctgtccagcgacaccgcccccagatggatgaccgtgatgcggggctacagcgagtgtggagatggcagccctgccgtgtacacctgcgtggacgacctgtgcagaggctacgacctgaccagactgagctacggccggtccatcttcacagagcacgtgctgggcttcgagctggtgccccccagcctgttcaacgtggtggtggccatccggaacgaggccaccagaaccaacagagccgtgcggctgcctgtgtctacagccgctgcacctgagggcatcacactgttctacggcctgtacaacgccgtgaaagagttctgcctccggcaccagctggatccccccctgctgagacacctggacaagtactacgccggcctgcccccagagctgaagcagaccagagtgaacctgcccgcccacagcagatatggccctcaggccgtggacgccagatgataacgccggcggcccctataactctctacggctaacctgaatggactacgacatagtctagtccgccaagatgagccccaaggacctgacccccttcctgacaaccctgtggctgctcctgggccatagcagagtgcctagagtgcgggccgaggaatgctgcgagttcatcaacgtgaaccacccccccgagcggtgctacgacttcaagatgtgcaaccggttcaccgtggccctgagatgccccgacggcgaagtgtgctacagccccgagaaaaccgccgagatccggggcatcgtgaccaccatgacccacagcctgacccggcaggtggtgcacaacaagctgaccagctgcaactacaaccccctgtacctggaagccgacggccggatcagatgcggcaaagtgaacgacaaggcccagtacctgctgggagccgccggaagcgtgccctaccggtggatcaacctggaatacgacaagatcacccggatcgtgggcctggaccagtacctggaaagcgtgaagaagcacaagcggctggacgtgtgcagagccaagatgggctacatgctgcagtgataaggcgcgccaacgttactggccgaagccgcttggaataaggccggtgtgcgtttgtctatatgttattttccaccatattgccgtcttttggcaatgtgagggcccggaaacctggccctgtcttcttgacgagcattcctaggggtctttcccctctcgccaaaggaatgcaaggtctgttgaatgtcgtgaaggaagcagttcctctggaagcttcttgaagacaaacaacgtctgtagcgaccctttgcaggcagcggaaccccccacctggcgacaggtgcctctgcggccaaaagccacgtgtataagatacacctgcaaaggcggcacaaccccagtgccacgttgtgagttggatagttgtggaaagagtcaaatggctctcctcaagcgtattcaacaaggggctgaaggatgcccagaaggtaccccattgtatgggatctgatctggggcctcggtgcacatgctttacatgtgtttagtcgaggttaaaaaaacgtctaggccccccgaaccacggggacgtggttttcctttgaaaaacacgataatatgctgcggctgctgctgagacaccacttccactgcctgctgctgtgtgccgtgtgggccaccccttgtctggccagcccttggagcaccctgaccgccaaccagaaccctagccccccttggtccaagctgacctacagcaagccccacgacgccgccaccttctactgcccctttctgtaccccagccctcccagaagccccctgcagttcagcggcttccagagagtgtccaccggccctgagtgccggaacgagacactgtacctgctgtacaaccgggagggccagacactggtggagcggagcagcacctgggtgaaaaaagtgatctggtatctgagcggccggaaccagaccatcctgcagcggatgcccagaaccgccagcaagcccagcgacggcaacgtgcagatcagcgtggaggacgccaaaatcttcggagcccacatggtgcccaagcagaccaagctgctgagattcgtggtcaacgacggcaccagatatcagatgtgcgtgatgaagctggaaagctgggcccacgtgttccgggactactccgtgagcttccaggtccggctgaccttcaccgaggccaacaaccagacctacaccttctgcacccaccccaacctgatcgtgtgataagtacctttgtacgcctgttttataccccctccctgatttgcaacttagaagcaacgcaaaccagatcaatagtaggtgtgacataccagtcgcatcttgatcaagcacttctgtatccccggaccgagtatcaatagactgtgcacacggttgaaggagaaaacgtccgttacccggctaactacttcgagaagcctagtaacgccattgaagttgcagagtgtttcgctcagcactccccccgtgtagatcaggtcgatgagtcaccgcattccccacgggcgaccgtggcggtggctgcgttggcggcctgcctatggggtaacccataggacgctctaatacggacatggcgtgaagagtctattgagctagttagtagtcctccggcccctgaatgcggctaatcctaactgcggagcacatacccttaatccaaagggcagtgtgtcgtaacgggcaactctgcagcggaaccgactactttgggtgtccgtgtttctttttattcttgtattggctgcttatggtgacaattaaagaattgttaccatatagctattggattggccatccagtgtcaaacagagctattgtatatctctttgttggattcacacctctcactcttgaaacgttacacaccctcaattacattatactgctgaacacgaagcgcatatgcggctgtgcagagtgtggctgtccgtgtgcctgtgtgccgtggtgctgggccagtgccagagagagacagccgagaagaacgactactaccgggtgccccactactgggatgcctgcagcagagccctgcccgaccagacccggtacaaatacgtggagcagctcgtggacctgaccctgaactaccactacgacgccagccacggcctggacaacttcgacgtgctgaagcggatcaacgtgaccgaggtgtccctgctgatcagcgacttccggcggcagaacagaagaggcggcaccaacaagcggaccaccttcaacgccgctggctctctggcccctcacgccagatccctggaattcagcgtgcggctgttcgccaactgataacgttgcatcctgcaggatacagcagcaattggcaagctgcttacatagaactcgcggcgattggcatgccgccttaaaatttttattttatttttcttttcttttccgaatcggattttgtttttaatatttcaaaaaaaaaaaaaaaaaaaaaaaaaaaaaaaaaaagggtcggcatggcatctccacctcctcgcggtccgacctgggcatccgaaggaggacgcacgtccactcggatggctaagggagagccacgtttaaacgctagagcaagacgtttcccgttgaatatggctcataacaccccttgtattactgtttatgtaagcagacagttttattgttcatgatgatatatttttatcttgtgcaatgtaacatcagagattttgagacacaacgtggctttgttgaataaatcgaacttttgctgagttgaaggatcagatcacgcatcttcccgacaacgcagaccgttccgtggcaaagcaaaagttcaaaatcaccaactggtccacctacaacaaagctctcatcaaccgtggctccctcactttctggctggatgatggggcgattcaggcctggtatgagtcagcaacaccttcttcacgaggcagacctcagcgctagcggagtgtatactggcttactatgttggcactgatgagggtgtcagtgaagtgcttcatgtggcaggagaaaaaaggctgcaccggtgcgtcagcagaatatgtgatacaggatatattccgcttcctcgctcactgactcgctacgctcggtcgttcgactgcggcgagcggaaatggcttacgaacggggcggagatttcctggaagatgccaggaagatacttaacagggaagtgagagggccgcggcaaagccgtttttccataggctccgcccccctgacaagcatcacgaaatctgacgctcaaatcagtggtggcgaaacccgacaggactataaagataccaggcgtttcccctggcggctccctcgtgcgctctcctgttcctgcctttcggtttaccggtgtcattccgctgttatggccgcgtttgtctcattccacgcctgacactcagttccgggtaggcagttcgctccaagctggactgtatgcacgaaccccccgttcagtccgaccgctgcgccttatccggtaactatcgtcttgagtccaacccggaaagacatgcaaaagcaccactggcagcagccactggtaattgatttagaggagttagtcttgaagtcatgcgccggttaaggctaaactgaaaggacaagttttggtgactgcgctcctccaagccagttacctcggttcaaagagttggtagctcagagaaccttcgaaaaaccgccctgcaaggcggttttttcgttttcagagcaagagattacgcgcagaccaaaacgatctcaagaagatcatcttattaaggggtctgacgctcagtggaacgaaaactcacgttaagggattttggtcatgagattatcaaaaaggatcttcacctagatccttttaaattaaaaatgaagttttaaatcaatctaaagtatatatgagtaaacttggtctgacagttattagaaaaattcatccagcagacgataaaacgcaatacgctggctatccggtgccgcaatgccatacagcaccagaaaacgatccgcccattcgccgcccagttcttccgcaatatcacgggtggccagcgcaatatcctgataacgatccgccacgcccagacggccgcaatcaataaagccgctaaaacggccattttccaccataatgttcggcaggcacgcatcaccatgggtcaccaccagatcttcgccatccggcatgctcgctttcagacgcgcaaacagctctgccggtgccaggccctgatgttcttcatccagatcatcctgatccaccaggcccgcttccatacgggtacgcgcacgttcaatacgatgtttcgcctgatgatcaaacggacaggtcgccgggtccagggtatgcagacgacgcatggcatccgccataatgctcactttttctgccggcgccagatggctagacagcagatcctgacccggcacttcgcccagcagcagccaatcacggcccgcttcggtcaccacatccagcaccgccgcacacggaacaccggtggtggccagccagctcagacgcgccgcttcatcctgcagctcgttcagcgcaccgctcagatcggttttcacaaacagcaccggacgaccctgcgcgctcagacgaaacaccgccgcatcagagcagccaatggtctgctgcgcccaatcatagccaaacagacgttccacccacgctgccgggctacccgcatgcaggccatcctgttcaatcatactcttcctttttcaatattattgaagcatttatcagggttattgtctcatgagcggatacatatttgaatgtatttagaaaaataaacaaataggggttccgcgcacatttccccgaaaagtgccacctaaattgtaagcgttaatattttgttaaaattcgcgttaaatttttgttaaatcagctcattttttaaccaataggccgaaatcggcaaaatcccttataaatcaaaagaatagaccgagatagggttgagtggccgctacagggcgctcccattcgccattcaggctgcgcaactgttgggaagggcgtttcggtgcgggcctcttcgctattacgccagctggcgaaagggggatgtgctgcaaggcgattaagttgggtaacgccagggttttcccagtcacacgcgtaatacgactcactatag

SEQ ID NO: 58 - DNA, 13102 bp, Artificial Sequence
  source: /note="Description of Artificial Sequence: Synthetic polynucleotide"
ataggcggcgcatgagagaagcccagaccaattacctacccaaaatggagaaagttcacgttgacatcgaggaagacagcccattcctcagagctttgcagcggagcttcccgcagtttgaggtagaagccaagcaggtcactgataatgaccatgctaatgccagagcgttttcgcatctggcttcaaaactgatcgaaacggaggtggacccatccgacacgatccttgacattggaagtgcgcccgcccgcagaatgtattctaagcacaagtatcattgtatctgtccgatgagatgtgcggaagatccggacagattgtataagtatgcaactaagctgaagaaaaactgtaaggaaataactgataaggaattggacaagaaaatgaaggagctcgccgccgtcatgagcgaccctgacctggaaactgagactatgtgcctccacgacgacgagtcgtgtcgctacgaagggcaagtcgctgtttaccaggatgtatacgcggttgacggaccgacaagtctctatcaccaagccaataagggagttagagtcgcctactggataggctttgacaccaccccttttatgtttaagaacttggctggagcatatccatcatactctaccaactgggccgacgaaaccgtgttaacggctcgtaacataggcctatgcagctctgacgttatggagcggtcacgtagagggatgtccattcttagaaagaagtatttgaaaccatccaacaatgttctattctctgttggctcgaccatctaccacgagaagagggacttactgaggagctggcacctgccgtctgtatttcacttacgtggcaagcaaaattacacatgtcggtgtgagactatagttagttgcgacgggtacgtcgttaaaagaatagctatcagtccaggcctgtatgggaagccttcaggctatgctgctacgatgcaccgcgagggattcttgtgctgcaaagtgacagacacattgaacggggagagggtctcttttcccgtgtgcacgtatgtgccagctacattgtgtgaccaaatgactggcatactggcaacagatgtcagtgcggacgacgcgcaaaaactgctggttgggctcaaccagcgtatagtcgtcaacggtcgcacccagagaaacaccaataccatgaaaaattaccttttgcccgtagtggcccaggcatttgctaggtgggcaaaggaatataaggaagatcaagaagatgaaaggccactaggactacgagatagacagttagtcatggggtgttgttgggcttttagaaggcacaagataacatctatttataagcgcccggatacccaaaccatcatcaaagtgaacagcgatttccactcattcgtgctgcccaggataggcagtaacacattggagatcgggctgagaacaagaatcaggaaaatgttagaggagcacaaggagccgtcacctctcattaccgccgaggacgtacaagaagctaagtgcgcagccgatgaggctaaggaggtgcgtgaagccgaggagttgcgcgcagctctaccacctttggcagctgatgttgaggagcccactctggaagccgatgtcgacttgatgttacaagaggctggggccggctcagtggagacacctcgtggcttgataaaggttaccagctacgatggcgaggacaagatcggctcttacgctgtgctttctccgcaggctgtactcaagagtgaaaaattatcttgcatccaccctctcgctgaacaagtcatagtgataacacactctggccgaaaagggcgttatgccgtggaaccataccatggtaaagtagtggtgccagagggacatgcaatacccgtccaggactttcaagctctgagtgaaagtgccaccattgtgtacaacgaacgtgagttcgtaaacaggtacctgcaccatattgccacacatggaggagcgctgaacactgatgaagaatattacaaaactgtcaagcccagcgagcacgacggcgaatacctgtacgacatcgacaggaaacagtgcgtcaagaaagaactagtcactgggctagggctcacaggcgagctggtggatcctcccttccatgaattcgcctacgagagtctgagaacacgaccagccgctccttaccaagtaccaaccataggggtgtatggcgtgccaggatcaggcaagtctggcatcattaaaagcgcagtcaccaaaaaagatctagtggtgagcgccaagaaagaaaactgtgcagaaattataagggacgtcaagaaaatgaaagggctggacgtcaatgccagaactgtggactcagtgctcttgaatggatgcaaacaccccgtagagaccctgtatattgacgaagcttttgcttgtcatgcaggtactctcagagcgctcatagccattataagacctaaaaaggcagtgctctgcggggatcccaaacagtgcggtttttttaacatgatgtgcctgaaagtgcattttaaccacgagatttgcacacaagtcttccacaaaagcatctctcgccgttgcactaaatctgtgacttcggtcgtctcaaccttgttttacgacaaaaaaatgagaacgacgaatccgaaagagactaagattgtgattgacactaccggcagtaccaaacctaagcaggacgatctcattctcacttgtttcagagggtgggtgaagcagttgcaaatagattacaaaggcaacgaaataatgacggcagctgcctctcaagggctgacccgtaaaggtgtgtatgccgttcggtacaaggtgaatgaaaatcctctgtacgcacccacctcagaacatgtgaacgtcctactgacccgcacggaggaccgcatcgtgtggaaaacactagccggcgacccatggataaaaacactgactgccaagtaccctgggaatttcactgccacgatagaggagtggcaagcagagcatgatgccatcatgaggcacatcttggagagaccggaccctaccgacgtcttccagaataaggcaaacgtgtgttgggccaaggctttagtgccggtgctgaagaccgctggcatagacatgaccactgaacaatggaacactgtggattattttgaaacggacaaagctcactcagcagagatagtattgaaccaactatgcgtgaggttctttggactcgatctggactccggtctattttctgcacccactgttccgttatccattaggaataatcactgggataactccccgtcgcctaacatgtacgggctgaataaagaagtggtccgtcagctctctcgcaggtacccacaactgcctcgggcagttgccactggaagagtctatgacatgaacactggtacactgcgcaattatgatccgcgcataaacctagtacctgtaaacagaagactgcctcatgctttagtcctccaccataatgaacacccacagagtgacttttcttcattcgtcagcaaattgaagggcagaactgtcctggtggtcggggaaaagttgtccgtcccaggcaaaatggttgactggttgtcagaccggcctgaggctaccttcagagctcggctggatttaggcatcccaggtgatgtgcccaaatatgacataatatttgttaatgtgaggaccccatataaataccatcactatcagcagtgtgaagaccatgccattaagcttagcatgttgaccaagaaagcttgtctgcatctgaatcccggcggaacctgtgtcagcataggttatggttacgctgacagggccagcgaaagcatcattggtgctatagcgcggcagttcaagttttcccgggtatgcaaaccgaaatcctcacttgaagagacggaagttctgtttgtattcattgggtacgatcgcaaggcccgtacgcacaatccttacaagctttcatcaaccttgaccaacatttatacaggttccagactccacgaagccggatgtgcaccctcatatcatgtggtgcgaggggatattgccacggccaccgaaggagtgattataaatgctgctaacagcaaaggacaacctggcggaggggtgtgcggagcgctgtataagaaattcccggaaagcttcgatttacagccgatcgaagtaggaaaagcgcgactggtcaaaggtgcagctaaacatatcattcatgccgtaggaccaaacttcaacaaagtttcggaggttgaaggtgacaaacagttggcagaggcttatgagtccatcgctaagattgtcaacgataacaattacaagtcagtagcgattccactgttgtccaccggcatcttttccgggaacaaagatcgactaacccaatcattgaaccatttgctgacagctttagacaccactgatgcagatgtagccatatactgcagggacaagaaatgggaaatgactctcaaggaagcagtggctaggagagaagcagtggaggagatatgcatatccgacgactcttcagtgacagaacctgatgcagagctggtgagggtgcatccgaagagttctttggctggaaggaagggctacagcacaagcgatggcaaaactttctcatatttggaagggaccaagtttcaccaggcggccaaggatatagcagaaattaatgccatgtggcccgttgcaacggaggccaatgagcaggtatgcatgtatatcctcggagaaagcatgagcagtattaggtcgaaatgccccgtcgaagagtcggaagcctccacaccacctagcacgctgccttgcttgtgcatccatgccatgactccagaaagagtacagcgcctaaaagcctcacgtccagaacaaattactgtgtgctcatcctttccattgccgaagtatagaatcactggtgtgcagaagatccaatgctcccagcctatattgttctcaccgaaagtgcctgcgtatattcatccaaggaagtatctcgtggaaacaccaccggtagacgagactccggagccatcggcagagaaccaatccacagaggggacacctgaacaaccaccacttataaccgaggatgagaccaggactagaacgcctgagccgatcatcatcgaagaggaagaagaggatagcataagtttgctgtcagatggcccgacccaccaggtgctgcaagtcgaggcagacattcacgggccgccctctgtatctagctcatcctggtccattcctcatgcatccgactttgatgtggacagtttatccatacttgacaccctggagggagctagcgtgaccagcggggcaacgtcagccgagactaactcttacttcgcaaagagtatggagtttctggcgcgaccggtgcctgcgcctcgaacagtattcaggaaccctccacatcccgctccgcgcacaagaacaccgtcacttgcacccagcagggcctgctcgagaaccagcctagtttccaccccgccaggcgtgaatagggtgatcactagagaggagctcgaggcgcttaccccgtcacgcactcctagcaggtcggtctcgagaaccagcctggtctccaacccgccaggcgtaaatagggtgattacaagagaggagtttgaggcgttcgtagcacaacaacaatgacggtttgatgcgggtgcatacatcttttcctccgacaccggtcaagggcatttacaacaaaaatcagtaaggcaaacggtgctatccgaagtggtgttggagaggaccgaattggagatttcgtatgccccgcgcctcgaccaagaaaaagaagaattactacgcaagaaattacagttaaatcccacacctgctaacagaagcagataccagtccaggaaggtggagaacatgaaagccataacagctagacgtattctgcaaggcctagggcattatttgaaggcagaaggaaaagtggagtgctaccgaaccctgcatcctgttcctttgtattcatctagtgtgaaccgtgccttttcaagccccaaggtcgcagtggaagcctgtaacgccatgttgaaagagaactttccgactgtggcttcttactgtattattccagagtacgatgcctatttggacatggttgacggagcttcatgctgcttagacactgccagtttttgccctgcaaagctgcgcagctttccaaagaaacactcctatttggaacccacaatacgatcggcagtgccttcagcgatccagaacacgctccagaacgtcctggcagctgccacaaaaagaaattgcaatgtcacgcaaatgagagaattgcccgtattggattcggcggcctttaatgtggaatgcttcaagaaatatgcgtgtaataatgaatattgggaaacgtttaaagaaaaccccatcaggcttactgaagaaaacgtggtaaattacattaccaaattaaaaggaccaaaagctgctgctctttttgcgaagacacataatttgaatatgttgcaggacataccaatggacaggtttgtaatggacttaaagagagacgtgaaagtgactccaggaacaaaacatactgaagaacggcccaaggtacaggtgatccaggctgccgatccgctagcaacagcgtatctgtgcggaatccaccgagagctggttaggagattaaatgcggtcctgcttccgaacattcatacactgtttgatatgtcggctgaagactttgacgctattatagccgagcacttccagcctggggattgtgttctggaaactgacatcgcgtcgtttgataaaagtgaggacgacgccatggctctgaccgcgttaatgattctggaagacttaggtgtggacgcagagctgttgacgctgattgaggcggctttcggcgaaatttcatcaatacatttgcccactaaaactaaatttaaattcggagccatgatgaaatctggaatgttcctcacactgtttgtgaacacagtcattaacattgtaatcgcaagcagagtgttgagagaacggctaaccggatcaccatgtgcagcattcattggagatgacaatatcgtgaaaggagtcaaatcggacaaattaatggcagacaggtgcgccacctggttgaatatggaagtcaagattatagatgctgtggtgggcgagaaagcgccttatttctgtggagggtttattttgtgtgactccgtgaccggcacagcgtgccgtgtggcagaccccctaaaaaggctgtttaagcttggcaaacctctggcagcagacgatgaacatgatgatgacaggagaagggcattgcatgaagagtcaacacgctggaaccgagtgggtattctttcagagctgtgcaaggcagtagaatcaaggtatgaaaccgtaggaacttccatcatagttatggccatgactactctagctagcagtgttaaatcattcagctacctgagaggggcccctataactctctacggctaacctgaatggactacgacatagtctagtccgccaagatgaggcctggcctgccctcctacctgatcatcctggccgtgtgcctgttcagccacctgctgtccagcagatacggcgccgaggccgtgagcgagcccctggacaaggctttccacctgctgctgaacacctacggcagacccatccggtttctgcgggagaacaccacccagtgcacctacaacagcagcctgcggaacagcaccgtcgtgagagagaacgccatcagcttcaactttttccagagctacaaccagtactacgtgttccacatgcccagatgcctgtttgccggccctctggccgagcagttcctgaaccaggtggacctgaccgagacactggaaagataccagcagcggctgaatacctacgccctggtgtccaaggacctggccagctaccggtcctttagccagcagctcaaggctcaggatagcctcggcgagcagcctaccaccgtgccccctcccatcgacctgagcatcccccacgtgtggatgcctccccagaccacccctcacggctggaccgagagccacaccacctccggcctgcacagaccccacttcaaccagacctgcatcctgttcgacggccacgacctgctgtttagcaccgtgaccccctgcctgcaccagggcttctacctgatcgacgagctgagatacgtgaagatcaccctgaccgaggatttcttcgtggtcaccgtgtccatcgacgacgacacccccatgctgctgatcttcggccacctgcccagagtgctgttcaaggccccctaccagcgggacaacttcatcctgcggcagaccgagaagcacgagctgctggtgctggtcaagaaggaccagctgaaccggcactcctacctgaaggaccccgacttcctggacgccgccctggacttcaactacctggacctgagcgccctgctgagaaacagcttccacagatacgccgtggacgtgctgaagtccggacggtgccagatgctcgatcggcggaccgtggagatggccttcgcctatgccctcgccctgttcgccgctgccagacaggaagaggctggcgcccaggtgtcagtgcccagagccctggatagacaggccgccctgctgcagatccaggaattcatgatcacctgcctgagccagaccccccctagaaccaccctgctgctgtaccccacagccgtggatctggccaagagggccctgtggacccccaaccagatcaccgacatcacaagcctcgtgcggctcgtgtacatcctgagcaagcagaaccagcagcacctgatcccccagtgggccctgagacagatcgccgacttcgccctgaagctgcacaagacccatctggccagctttctgagcgccttcgccaggcaggaactgtacctgatgggcagcctggtccacagcatgctggtgcataccaccgagcggcgggagatcttcatcgtggagacaggcctgtgtagcctggccgagctgtcccactttacccagctgctggcccaccctcaccacgagtacctgagcgacctgtacaccccctgcagcagcagcggcagacgggaccacagcctggaacggctgaccagactgttccccgatgccaccgtgcctgctacagtgcctgccgccctgtccatcctgtccaccatgcagcccagcaccctggaaaccttccccgacctgttctgcctgcccctgggcgagagctttagcgccctgaccgtgtccgagcacgtgtcctacatcgtgaccaatcagtacctgatcaagggcatcagctaccccgtgtccaccacagtcgtgggccagagcctgatcatcacccagaccgacagccagaccaagtgcgagctgacccggaacatgcacaccacacacagcatcaccgtggccctgaacatcagcctggaaaactgcgctttctgtcagtctgccctgctggaatacgacgatacccagggcgtgatcaacatcatgtacatgcacgacagcgacgacgtgctgttcgccctggacccctacaacgaggtggtggtgtccagcccccggacccactacctgatgctgctgaagaacggcaccgtgctggaagtgaccgacgtggtggtggacgccaccgactgataatctagaggcccctataactctctacggctaacctgaatggactacgacatagtctagtccgccaagatgtgcagaaggcccgactgcggcttcagcttcagccctggacccgtgatcctgctgtggtgctgcctgctgctgcctatcgtgtcctctgccgccgtgtctgtggcccctacagccgccgagaaggtgccagccgagtgccccgagctgaccagaagatgcctgctgggcgaggtgttcgagggcgacaagtacgagagctggctgcggcccctggtcaacgtgaccggcagagatggccccctgagccagctgatccggtacagacccgtgacccccgaggccgccaatagcgtgctgctggacgaggccttcctggataccctggccctgctgtacaacaaccccgaccagctgagagccctgctgaccctgctgtccagcgacaccgcccccagatggatgaccgtgatgcggggctacagcgagtgtggagatggcagccctgccgtgtacacctgcgtggacgacctgtgcagaggctacgacctgaccagactgagctacggccggtccatcttcacagagcacgtgctgggcttcgagctggtgccccccagcctgttcaacgtggtggtggccatccggaacgaggccaccagaaccaacagagccgtgcggctgcctgtgtctacagccgctgcacctgagggcatcacactgttctacggcctgtacaacgccgtgaaagagttctgcctccggcaccagctggatccccccctgctgagacacctggacaagtactacgccggcctgcccccagagctgaagcagaccagagtgaacctgcccgcccacagcagatatggccctcaggccgtggacgccagatgataagcggccgcatacagcagcaattggcaagctgcttacatagaactcgcggcgattggcatgccgccttaaaatttttattttatttttcttttcttttccgaatcggattttgtttttaatatttcaaaaaaaaaaaaaaaaaaaaaaaaaaaaaaaaaaagggtcggcatggcatctccacctcctcgcggtccgacctgggcatccgaaggaggacgcacgtccactcggatggctaagggagagccacgtttaaacacgtgatatctggcctcatgggccttcctttcactgcccgctttccagtcgggaaacctgtcgtgccagctgcattaacatggtcatagctgtttccttgcgtattgggcgctctccgcttcctcgctcactgactcgctgcgctcggtcgttcgggtaaagcctggggtgcctaatgagcaaaaggccagcaaaaggccaggaaccgtaaaaaggccgcgttgctggcgtttttccataggctccgcccccctgacgagcatcacaaaaatcgacgctcaagtcagaggtggcgaaacccgacaggactataaagataccaggcgtttccccctggaagctccctcgtgcgctctcctgttccgaccctgccgcttaccggatacctgtccgcctttctcccttcgggaagcgtggcgctttctcatagctcacgctgtaggtatctcagttcggtgtaggtcgttcgctccaagctgggctgtgtgcacgaaccccccgttcagcccgaccgctgcgccttatccggtaactatcgtcttgagtccaacccggtaagacacgacttatcgccactggcagcagccactggtaacaggattagcagagcgaggtatgtaggcggtgctacagagttcttgaagtggtggcctaactacggctacactagaagaacagtatttggtatctgcgctctgctgaagccagttaccttcggaaaaagagttggtagctcttgatccggcaaacaaaccaccgctggtagcggtggtttttttgtttgcaagcagcagattacgcgcagaaaaaaaggatctcaagaagatcctttgatcttttctacggggtctgacgctcagtggaacgaaaactcacgttaagggattttggtcatgagattatcaaaaaggatcttcacctagatccttttaaattaaaaatgaagttttaaatcaatctaaagtatatatgagtaaacttggtctgacagttattagaaaaattcatccagcagacgataaaacgcaatacgctggctatccggtgccgcaatgccatacagcaccagaaaacgatccgcccattcgccgcccagttcttccgcaatatcacgggtggccagcgcaatatcctgataacgatccgccacgcccagacggccgcaatcaataaagccgctaaaacggccattttccaccataatgttcggcaggcacgcatcaccatgggtcaccaccagatcttcgccatccggcatgctcgctttcagacgcgcaaacagctctgccggtgccaggccctgatgttcttcatccagatcatcctgatccaccaggcccgcttccatacgggtacgcgcacgttcaatacgatgtttcgcctgatgatcaaacggacaggtcgccgggtccagggtatgcagacgacgcatggcatccgccataatgctcactttttctgccggcgccagatggctagacagcagatcctgacccggcacttcgcccagcagcagccaatcacggcccgcttcggtcaccacatccagcaccgccgcacacggaacaccggtggtggccagccagctcagacgcgccgcttcatcctgcagctcgttcagcgcaccgctcagatcggttttcacaaacagcaccggacgaccctgcgcgctcagacgaaacaccgccgcatcagagcagccaatggtctgctgcgcccaatcatagccaaacagacgttccacccacgctgccgggctacccgcatgcaggccatcctgttcaatcatactcttcctttttcaatattattgaagcatttatcagggttattgtctcatgagcggatacatatttgaatgtatttagaaaaataaacaaataggggttccgcgcacatttccccgaaaagtgccacctaaattgtaagcgttaatattttgttaaaattcgcgttaaatttttgttaaatcagctcattttttaaccaataggccgaaatcggcaaaatcccttataaatcaaaagaatagaccgagatagggttgagtggccgctacagggcgctcccattcgccattcaggctgcgcaactgttgggaagggcgtttcggtgcgggcctcttcgctattacgccagctggcgaaagggggatgtgctgcaaggcgattaagttgggtaacgccagggttttcccagtcacacgcgtaatacgactcactatag

SEQ ID NO: 59 - DNA, 13087 bp, Artificial Sequence
  source: /note="Description of Artificial Sequence: Synthetic polynucleotide"
ataggcggcgcatgagagaagcccagaccaattacctacccaaaatggagaaagttcacgttgacatcgaggaagacagcccattcctcagagctttgcagcggagcttcccgcagtttgaggtagaagccaagcaggtcactgataatgaccatgctaatgccagagcgttttcgcatctggcttcaaaactgatcgaaacggaggtggacccatccgacacgatccttgacattggaagtgcgcccgcccgcagaatgtattctaagcacaagtatcattgtatctgtccgatgagatgtgcggaagatccggacagattgtataagtatgcaactaagctgaagaaaaactgtaaggaaataactgataaggaattggacaagaaaatgaaggagctcgccgccgtcatgagcgaccctgacctggaaactgagactatgtgcctccacgacgacgagtcgtgtcgctacgaagggcaagtcgctgtttaccaggatgtatacgcggttgacggaccgacaagtctctatcaccaagccaataagggagttagagtcgcctactggataggctttgacaccaccccttttatgtttaagaacttggctggagcatatccatcatactctaccaactgggccgacgaaaccgtgttaacggctcgtaacataggcctatgcagctctgacgttatggagcggtcacgtagagggatgtccattcttagaaagaagtatttgaaaccatccaacaatgttctattctctgttggctcgaccatctaccacgagaagagggacttactgaggagctggcacctgccgtctgtatttcacttacgtggcaagcaaaattacacatgtcggtgtgagactatagttagttgcgacgggtacgtcgttaaaagaatagctatcagtccaggcctgtatgggaagccttcaggctatgctgctacgatgcaccgcgagggattcttgtgctgcaaagtgacagacacattgaacggggagagggtctcttttcccgtgtgcacgtatgtgccagctacattgtgtgaccaaatgactggcatactggcaacagatgtcagtgcggacgacgcgcaaaaactgctggttgggctcaaccagcgtatagtcgtcaacggtcgcacccagagaaacaccaataccatgaaaaattaccttttgcccgtagtggcccaggcatttgctaggtgggcaaaggaatataaggaagatcaagaagatgaaaggccactaggactacgagatagacagttagtcatggggtgttgttgggcttttagaaggcacaagataacatctatttataagcgcccggatacccaaaccatcatcaaagtgaacagcgatttccactcattcgtgctgcccaggataggcagtaacacattggagatcgggctgagaacaagaatcaggaaaatgttagaggagcacaaggagccgtcacctctcattaccgccgaggacgtacaagaagctaagtgcgcagccgatgaggctaaggaggtgcgtgaagccgaggagttgcgcgcagctctaccacctttggcagctgatgttgaggagcccactctggaagccgatgtcgacttgatgttacaagaggctggggccggctcagtggagacacctcgtggcttgataaaggttaccagctacgatggcgaggacaagatcggctcttacgctgtgctttctccgcaggctgtactcaagagtgaaaaattatcttgcatccaccctctcgctgaacaagtcatagtgataacacactctggccgaaaagggcgttatgccgtggaaccataccatggtaaagtagtggtgccagagggacatgcaatacccgtccaggactttcaagctctgagtgaaagtgccaccattgtgtacaacgaacgtgagttcgtaaacaggtacctgcaccatattgccacacatggaggagcgctgaacactgatgaagaatattacaaaactgtcaagcccagcgagcacgacggcgaatacctgtacgacatcgacaggaaacagtgcgtcaagaaagaactagtcactgggctagggctcacaggcgagctggtggatcctcccttccatgaattcgcctacgagagtctgagaacacgaccagccgctccttaccaagtaccaaccataggggtgtatggcgtgccaggatcaggcaagtctggcatcattaaaagcgcagtcaccaaaaaagatctagtggtgagcgccaagaaagaaaactgtgcagaaattataagggacgtcaagaaaatgaaagggctggacgtcaatgccagaactgtggactcagtgctcttgaatggatgcaaacaccccgtagagaccctgtatattgacgaagcttttgcttgtcatgcaggtactctcagagcgctcatagccattataagacctaaaaaggcagtgctctgcggggatcccaaacagtgcggtttttttaacatgatgtgcctgaaagtgcattttaaccacgagatttgcacacaagtcttccacaaaagcatctctcgccgttgcactaaatctgtgacttcggtcgtctcaaccttgttttacgacaaaaaaatgagaacgacgaatccgaaagagactaagattgtgattgacactaccggcagtaccaaacctaagcaggacgatctcattctcacttgtttcagagggtgggtgaagcagttgcaaatagattacaaaggcaacgaaataatgacggcagctgcctctcaagggctgacccgtaaaggtgtgtatgccgttcggtacaaggtgaatgaaaatcctctgtacgcacccacctcagaacatgtgaacgtcctactgacccgcacggaggaccgcatcgtgtggaaaacactagccggcgacccatggataaaaacactgactgccaagtaccctgggaatttcactgccacgatagaggagtggcaagcagagcatgatgccatcatgaggcacatcttggagagaccggaccctaccgacgtcttccagaataaggcaaacgtgtgttgggccaaggctttagtgccggtgctgaagaccgctggcatagacatgaccactgaacaatggaacactgtggattattttgaaacggacaaagctcactcagcagagatagtattgaaccaactatgcgtgaggttctttggactcgatctggactccggtctattttctgcacccactgttccgttatccattaggaataatcactgggataactccccgtcgcctaacatgtacgggctgaataaagaagtggtccgtcagctctctcgcaggtacccacaactgcctcgggcagttgccactggaagagtctatgacatgaacactggtacactgcgcaattatgatccgcgcataaacctagtacctgtaaacagaagactgcctcatgctttagtcctccaccataatgaacacccacagagtgacttttcttcattcgtcagcaaattgaagggcagaactgtcctggtggtcggggaaaagttgtccgtcccaggcaaaatggttgactggttgtcagaccggcctgaggctaccttcagagctcggctggatttaggcatcccaggtgatgtgcccaaatatgacataatatttgttaatgtgaggaccccatataaataccatcactatcagcagtgtgaagaccatgccattaagcttagcatgttgaccaagaaagcttgtctgcatctgaatcccggcggaacctgtgtcagcataggttatggttacgctgacagggccagcgaaagcatcattggtgctatagcgcggcagttcaagttttcccgggtatgcaaaccgaaatcctcacttgaagagacggaagttctgtttgtattcattgggtacgatcgcaaggcccgtacgcacaatccttacaagctttcatcaaccttgaccaacatttatacaggttccagactccacgaagccggatgtgcaccctcatatcatgtggtgcgaggggatattgccacggccaccgaaggagtgattataaatgctgctaacagcaaaggacaacctggcggaggggtgtgcggagcgctgtataagaaattcccggaaagcttcgatttacagccgatcgaagtaggaaaagcgcgactggtcaaaggtgcagctaaacatatcattcatgccgtaggaccaaacttcaacaaagtttcggaggttgaaggtgacaaacagttggcagaggcttatgagtccatcgctaagattgtcaacgataacaattacaagtcagtagcgattccactgttgtccaccggcatcttttccgggaacaaagatcgactaacccaatcattgaaccatttgctgacagctttagacaccactgatgcagatgtagccatatactgcagggacaagaaatgggaaatgactctcaaggaagcagtggctaggagagaagcagtggaggagatatgcatatccgacgactcttcagtgacagaacctgatgcagagctggtgagggtgcatccgaagagttctttggctggaaggaagggctacagcacaagcgatggcaaaactttctcatatttggaagggaccaagtttcaccaggcggccaaggatatagcagaaattaatgccatgtggcccgttgcaacggaggccaatgagcaggtatgcatgtatatcctcggagaaagcatgagcagtattaggtcgaaatgccccgtcgaagagtcggaagcctccacaccacctagcacgctgccttgcttgtgcatccatgccatgactccagaaagagtacagcgcctaaaagcctcacgtccagaacaaattactgtgtgctcatcctttccattgccgaagtatagaatcactggtgtgcagaagatccaatgctcccagcctatattgttctcaccgaaagtgcctgcgtatattcatccaaggaagtatctcgtggaaacaccaccggtagacgagactccggagccatcggcagagaaccaatccacagaggggacacctgaacaaccaccacttataaccgaggatgagaccaggactagaacgcctgagccgatcatcatcgaagaggaagaagaggatagcataagtttgctgtcagatggcccgacccaccaggtgctgcaagtcgaggcagacattcacgggccgccctctgtatctagctcatcctggtccattcctcatgcatccgactttgatgtggacagtttatccatacttgacaccctggagggagctagcgtgaccagcggggcaacgtcagccgagactaactcttacttcgcaaagagtatggagtttctggcgcgaccggtgcctgcgcctcgaacagtattcaggaaccctccacatcccgctccgcgcacaagaacaccgtcacttgcacccagcagggcctgctcgagaaccagcctagtttccaccccgccaggcgtgaatagggtgatcactagagaggagctcgaggcgcttaccccgtcacgcactcctagcaggtcggtctcgagaaccagcctggtctccaacccgccaggcgtaaatagggtgattacaagagaggagtttgaggcgttcgtagcacaacaacaatgacggtttgatgcgggtgcatacatcttttcctccgacaccggtcaagggcatttacaacaaaaatcagtaaggcaaacggtgctatccgaagtggtgttggagaggaccgaattggagatttcgtatgccccgcgcctcgaccaagaaaaagaagaattactacgcaagaaattacagttaaatcccacacctgctaacagaagcagataccagtccaggaaggtggagaacatgaaagccataacagctagacgtattctgcaaggcctagggcattatttgaaggcagaaggaaaagtggagtgctaccgaaccctgcatcctgttcctttgtattcatctagtgtgaaccgtgccttttcaagccccaaggtcgcagtggaagcctgtaacgccatgttgaaagagaactttccgactgtggcttcttactgtattattccagagtacgatgcctatttggacatggttgacggagcttcatgctgcttagacactgccagtttttgccctgcaaagctgcgcagctttccaaagaaacactcctatttggaacccacaatacgatcggcagtgccttcagcgatccagaacacgctccagaacgtcctggcagctgccacaaaaagaaattgcaatgtcacgcaaatgagagaattgcccgtattggattcggcggcctttaatgtggaatgcttcaagaaatatgcgtgtaataatgaatattgggaaacgtttaaagaaaaccccatcaggcttactgaagaaaacgtggtaaattacattaccaaattaaaaggaccaaaagctgctgctctttttgcgaagacacataatttgaatatgttgcaggacataccaatggacaggtttgtaatggacttaaagagagacgtgaaagtgactccaggaacaaaacatactgaagaacggcccaaggtacaggtgatccaggctgccgatccgctagcaacagcgtatctgtgcggaatccaccgagagctggttaggagattaaatgcggtcctgcttccgaacattcatacactgtttgatatgtcggctgaagactttgacgctattatagccgagcacttccagcctggggattgtgttctggaaactgacatcgcgtcgtttgataaaagtgaggacgacgccatggctctgaccgcgttaatgattctggaagacttaggtgtggacgcagagctgttgacgctgattgaggcggctttcggcgaaatttcatcaatacatttgcccactaaaactaaatttaaattcggagccatgatgaaatctggaatgttcctcacactgtttgtgaacacagtcattaacattgtaatcgcaagcagagtgttgagagaacggctaaccggatcaccatgtgcagcattcattggagatgacaatatcgtgaaaggagtcaaatcggacaaattaatggcagacaggtgcgccacctggttgaatatggaagtcaagattatagatgctgtggtgggcgagaaagcgccttatttctgtggagggtttattttgtgtgactccgtgaccggcacagcgtgccgtgtggcagaccccctaaaaaggctgtttaagcttggcaaacctctggcagcagacgatgaacatgatgatgacaggagaagggcattgcatgaagagtcaacacgctggaaccgagtgggtattctttcagagctgtgcaaggcagtagaatcaaggtatgaaaccgtaggaacttccatcatagttatggccatgactactctagctagcagtgttaaatcattcagctacctgagaggggcccctataactctctacggctaacctgaatggactacgacatagtctagtccgccaagatgaggcctggcctgccctcctacctgatcatcctggccgtgtgcctgttcagccacctgctgtccagcagatacggcgccgaggccgtgagcgagcccctggacaaggctttccacctgctgctgaacacctacggcagacccatccggtttctgcgggagaacaccacccagtgcacctacaacagcagcctgcggaacagcaccgtcgtgagagagaacgccatcagcttcaactttttccagagctacaaccagtactacgtgttccacatgcccagatgcctgtttgccggccctctggccgagcagttcctgaaccaggtggacctgaccgagacactggaaagataccagcagcggctgaatacctacgccctggtgtccaaggacctggccagctaccggtcctttagccagcagctcaaggctcaggatagcctcggcgagcagcctaccaccgtgccccctcccatcgacctgagcatcccccacgtgtggatgcctccccagaccacccctcacggctggaccgagagccacaccacctccggcctgcacagaccccacttcaaccagacctgcatcctgttcgacggccacgacctgctgtttagcaccgtgaccccctgcctgcaccagggcttctacctgatcgacgagctgagatacgtgaagatcaccctgaccgaggatttcttcgtggtcaccgtgtccatcgacgacgacacccccatgctgctgatcttcggccacctgcccagagtgctgttcaaggccccctaccagcgggacaacttcatcctgcggcagaccgagaagcacgagctgctggtgctggtcaagaaggaccagctgaaccggcactcctacctgaaggaccccgacttcctggacgccgccctggacttcaactacctggacctgagcgccctgctgagaaacagcttccacagatacgccgtggacgtgctgaagtccggacggtgccagatgctcgatcggcggaccgtggagatggccttcgcctatgccctcgccctgttcgccgctgccagacaggaagaggctggcgcccaggtgtcagtgcccagagccctggatagacaggccgccctgctgcagatccaggaattcatgatcacctgcctgagccagaccccccctagaaccaccctgctgctgtaccccacagccgtggatctggccaagagggccctgtggacccccaaccagatcaccgacatcacaagcctcgtgcggctcgtgtacatcctgagcaagcagaaccagcagcacctgatcccccagtgggccctgagacagatcgccgacttcgccctgaagctgcacaagacccatctggccagctttctgagcgccttcgccaggcaggaactgtacctgatgggcagcctggtccacagcatgctggtgcataccaccgagcggcgggagatcttcatcgtggagacaggcctgtgtagcctggccgagctgtcccactttacccagctgctggcccaccctcaccacgagtacctgagcgacctgtacaccccctgcagcagcagcggcagacgggaccacagcctggaacggctgaccagactgttccccgatgccaccgtgcctgctacagtgcctgccgccctgtccatcctgtccaccatgcagcccagcaccctggaaaccttccccgacctgttctgcctgcccctgggcgagagctttagcgccctgaccgtgtccgagcacgtgtcctacatcgtgaccaatcagtacctgatcaagggcatcagctaccccgtgtccaccacagtcgtgggccagagcctgatcatcacccagaccgacagccagaccaagtgcgagctgacccggaacatgcacaccacacacagcatcaccgtggccctgaacatcagcctggaaaactgcgctttctgtcagtctgccctgctggaatacgacgatacccagggcgtgatcaacatcatgtacatgcacgacagcgacgacgtgctgttcgccctggacccctacaacgaggtggtggtgtccagcccccggacccactacctgatgctgctgaagaacggcaccgtgctggaagtgaccgacgtggtggtggacgccaccgacctgttgaattttgaccttcttaagcttgcgggagacgtcgagtccaaccccgggcccatgtgcagaaggcccgactgcggcttcagcttcagccctggacccgtgatcctgctgtggtgctgcctgctgctgcctatcgtgtcctctgccgccgtgtctgtggcccctacagccgccgagaaggtgccagccgagtgccccgagctgaccagaagatgcctgctgggcgaggtgttcgagggcgacaagtacgagagctggctgcggcccctggtcaacgtgaccggcagagatggccccctgagccagctgatccggtacagacccgtgacccccgaggccgccaatagcgtgctgctggacgaggccttcctggataccctggccctgctgtacaacaaccccgaccagctgagagccctgctgaccctgctgtccagcgacaccgcccccagatggatgaccgtgatgcggggctacagcgagtgtggagatggcagccctgccgtgtacacctgcgtggacgacctgtgcagaggctacgacctgaccagactgagctacggccggtccatcttcacagagcacgtgctgggcttcgagctggtgccccccagcctgttcaacgtggtggtggccatccggaacgaggccaccagaaccaacagagccgtgcggctgcctgtgtctacagccgctgcacctgagggcatcacactgttctacggcctgtacaacgccgtgaaagagttctgcctccggcaccagctggatccccccctgctgagacacctggacaagtactacgccggcctgcccccagagctgaagcagaccagagtgaacctgcccgcccacagcagatatggccctcaggccgtggacgccagatgataagcggccgcatacagcagcaattggcaagctgcttacatagaactcgcggcgattggcatgccgccttaaaatttttattttatttttcttttcttttccgaatcggattttgtttttaatatttcaaaaaaaaaaaaaaaaaaaaaaaaaaaaaaaaaaagggtcggcatggcatctccacctcctcgcggtccgacctgggcatccgaaggaggacgcacgtccactcggatggctaagggagagccacgtttaaacacgtgatatctggcctcatgggccttcctttcactgcccgctttccagtcgggaaacctgtcgtgccagctgcattaacatggtcatagctgtttccttgcgtattgggcgctctccgcttcctcgctcactgactcgctgcgctcggtcgttcgggtaaagcctggggtgcctaatgagcaaaaggccagcaaaaggccaggaaccgtaaaaaggccgcgttgctggcgtttttccataggctccgcccccctgacgagcatcacaaaaatcgacgctcaagtcagaggtggcgaaacccgacaggactataaagataccaggcgtttccccctggaagctccctcgtgcgctctcctgttccgaccctgccgcttaccggatacctgtccgcctttctcccttcgggaagcgtggcgctttctcatagctcacgctgtaggtatctcagttcggtgtaggtcgttcgctccaagctgggctgtgtgcacgaaccccccgttcagcccgaccgctgcgccttatccggtaactatcgtcttgagtccaacccggtaagacacgacttatcgccactggcagcagccactggtaacaggattagcagagcgaggtatgtaggcggtgctacagagttcttgaagtggtggcctaactacggctacactagaagaacagtatttggtatctgcgctctgctgaagccagttaccttcggaaaaagagttggtagctcttgatccggcaaacaaaccaccgctggtagcggtggtttttttgtttgcaagcagcagattacgcgcagaaaaaaaggatctcaagaagatcctttgatcttttctacggggtctgacgctcagtggaacgaaaactcacgttaagggattttggtcatgagattatcaaaaaggatcttcacctagatccttttaaattaaaaatgaagttttaaatcaatctaaagtatatatgagtaaacttggtctgacagttattagaaaaattcatccagcagacgataaaacgcaatacgctggctatccggtgccgcaatgccatacagcaccagaaaacgatccgcccattcgccgcccagttcttccgcaatatcacgggtggccagcgcaatatcctgataacgatccgccacgcccagacggccgcaatcaataaagccgctaaaacggccattttccaccataatgttcggcaggcacgcatcaccatgggtcaccaccagatcttcgccatccggcatgctcgctttcagacgcgcaaacagctctgccggtgccaggccctgatgttcttcatccagatcatcctgatccaccaggcccgcttccatacgggtacgcgcacgttcaatacgatgtttcgcctgatgatcaaacggacaggtcgccgggtccagggtatgcagacgacgcatggcatccgccataatgctcactttttctgccggcgccagatggctagacagcagatcctgacccggcacttcgcccagcagcagccaatcacggcccgcttcggtcaccacatccagcaccgccgcacacggaacaccggtggtggccagccagctcagacgcgccgcttcatcctgcagctcgttcagcgcaccgctcagatcggttttcacaaacagcaccggacgaccctgcgcgctcagacgaaacaccgccgcatcagagcagccaatggtctgctgcgcccaatcatagccaaacagacgttccacccacgctgccgggctacccgcatgcaggccatcctgttcaatcatactcttcctttttcaatattattgaagcatttatcagggttattgtctcatgagcggatacatatttgaatgtatttagaaaaataaacaaataggggttccgcgcacatttccccgaaaagtgccacctaaattgtaagcgttaatattttgttaaaattcgcgttaaatttttgttaaatcagctcattttttaaccaataggccgaaatcggcaaaatcccttataaatcaaaagaatagaccgagatagggttgagtggccgctacagggcgctcccattcgccattcaggctgcgcaactgttgggaagggcgtttcggtgcgggcctcttcgctattacgccagctggcgaaagggggatgtgctgcaaggcgattaagttgggtaacgccagggttttcccagtcacacgcgtaatacgactcactatag

SEQ ID NO: 60 - DNA, 13788 bp, Artificial Sequence
  source: /note="Description of Artificial Sequence: Synthetic polynucleotide"
ataggcggcgcatgagagaagcccagaccaattacctacccaaaatggagaaagttcacgttgacatcgaggaagacagcccattcctcagagctttgcagcggagcttcccgcagtttgaggtagaagccaagcaggtcactgataatgaccatgctaatgccagagcgttttcgcatctggcttcaaaactgatcgaaacggaggtggacccatccgacacgatccttgacattggaagtgcgcccgcccgcagaatgtattctaagcacaagtatcattgtatctgtccgatgagatgtgcggaagatccggacagattgtataagtatgcaactaagctgaagaaaaactgtaaggaaataactgataaggaattggacaagaaaatgaaggagctcgccgccgtcatgagcgaccctgacctggaaactgagactatgtgcctccacgacgacgagtcgtgtcgctacgaagggcaagtcgctgtttaccaggatgtatacgcggttgacggaccgacaagtctctatcaccaagccaataagggagttagagtcgcctactggataggctttgacaccaccccttttatgtttaagaacttggctggagcatatccatcatactctaccaactgggccgacgaaaccgtgttaacggctcgtaacataggcctatgcagctctgacgttatggagcggtcacgtagagggatgtccattcttagaaagaagtatttgaaaccatccaacaatgttctattctctgttggctcgaccatctaccacgagaagagggacttactgaggagctggcacctgccgtctgtatttcacttacgtggcaagcaaaattacacatgtcggtgtgagactatagttagttgcgacgggtacgtcgttaaaagaatagctatcagtccaggcctgtatgggaagccttcaggctatgctgctacgatgcaccgcgagggattcttgtgctgcaaagtgacagacacattgaacggggagagggtctcttttcccgtgtgcacgtatgtgccagctacattgtgtgaccaaatgactggcatactggcaacagatgtcagtgcggacgacgcgcaaaaactgctggttgggctcaaccagcgtatagtcgtcaacggtcgcacccagagaaacaccaataccatgaaaaattaccttttgcccgtagtggcccaggcatttgctaggtgggcaaaggaatataaggaagatcaagaagatgaaaggccactaggactacgagatagacagttagtcatggggtgttgttgggcttttagaaggcacaagataacatctatttataagcgcccggatacccaaaccatcatcaaagtgaacagcgatttccactcattcgtgctgcccaggataggcagtaacacattggagatcgggctgagaacaagaatcaggaaaatgttagaggagcacaaggagccgtcacctctcattaccgccgaggacgtacaagaagctaagtgcgcagccgatgaggctaaggaggtgcgtgaagccgaggagttgcgcgcagctctaccacctttggcagctgatgttgaggagcccactctggaagccgatgtcgacttgatgttacaagaggctggggccggctcagtggagacacctcgtggcttgataaaggttaccagctacgatggcgaggacaagatcggctcttacgctgtgctttctccgcaggctgtactcaagagtgaaaaattatcttgcatccaccctctcgctgaacaagtcatagtgataacacactctggccgaaaagggcgttatgccgtggaaccataccatggtaaagtagtggtgccagagggacatgcaatacccgtccaggactttcaagctctgagtgaaagtgccaccattgtgtacaacgaacgtgagttcgtaaacaggtacctgcaccatattgccacacatggaggagcgctgaacactgatgaagaatattacaaaactgtcaagcccagcgagcacgacggcgaatacctgtacgacatcgacaggaaacagtgcgtcaagaaagaactagtcactgggctagggctcacaggcgagctggtggatcctcccttccatgaattcgcctacgagagtctgagaacacgaccagccgctccttaccaagtaccaaccataggggtgtatggcgtgccaggatcaggcaagtctggcatcattaaaagcgcagtcaccaaaaaagatctagtggtgagcgccaagaaagaaaactgtgcagaaattataagggacgtcaagaaaatgaaagggctggacgtcaatgccagaactgtggactcagtgctcttgaatggatgcaaacaccccgtagagaccctgtatattgacgaagcttttgcttgtcatgcaggtactctcagagcgctcatagccattataagacctaaaaaggcagtgctctgcggggatcccaaacagtgcggtttttttaacatgatgtgcctgaaagtgcattttaaccacgagatttgcacacaagtcttccacaaaagcatctctcgccgttgcactaaatctgtgacttcggtcgtctcaaccttgttttacgacaaaaaaatgagaacgacgaatccgaaagagactaagattgtgattgacactaccggcagtaccaaacctaagcaggacgatctcattctcacttgtttcagagggtgggtgaagcagttgcaaatagattacaaaggcaacgaaataatgacggcagctgcctctcaagggctgacccgtaaaggtgtgtatgccgttcggtacaaggtgaatgaaaatcctctgtacgcacccacctcagaacatgtgaacgtcctactgacccgcacggaggaccgcatcgtgtggaaaacactagccggcgacccatggataaaaacactgactgccaagtaccctgggaatttcactgccacgatagaggagtggcaagcagagcatgatgccatcatgaggcacatcttggagagaccggaccctaccgacgtcttccagaataaggcaaacgtgtgttgggccaaggctttagtgccggtgctgaagaccgctggcatagacatgaccactgaacaatggaacactgtggattattttgaaacggacaaagctcactcagcagagatagtattgaaccaactatgcgtgaggttctttggactcgatctggactccggtctattttctgcacccactgttccgttatccattaggaataatcactgggataactccccgtcgcctaacatgtacgggctgaataaagaagtggtccgtcagctctctcgcaggtacccacaactgcctcgggcagttgccactggaagagtctatgacatgaacactggtacactgcgcaattatgatccgcgcataaacctagtacctgtaaacagaagactgcctcatgctttagtcctccaccataatgaacacccacagagtgacttttcttcattcgtcagcaaattgaagggcagaactgtcctggtggtcggggaaaagttgtccgtcccaggcaaaatggttgactggttgtcagaccggcctgaggctaccttcagagctcggctggatttaggcatcccaggtgatgtgcccaaatatgacataatatttgttaatgtgaggaccccatataaataccatcactatcagcagtgtgaagaccatgccattaagcttagcatgttgaccaagaaagcttgtctgcatctgaatcccggcggaacctgtgtcagcataggttatggttacgctgacagggccagcgaaagcatcattggtgctatagcgcggcagttcaagttttcccgggtatgcaaaccgaaatcctcacttgaagagacggaagttctgtttgtattcattgggtacgatcgcaaggcccgtacgcacaatccttacaagctttcatcaaccttgaccaacatttatacaggttccagactccacgaagccggatgtgcaccctcatatcatgtggtgcgaggggatattgccacggccaccgaaggagtgattataaatgctgctaacagcaaaggacaacctggcggaggggtgtgcggagcgctgtataagaaattcccggaaagcttcgatttacagccgatcgaagtaggaaaagcgcgactggtcaaaggtgcagctaaacatatcattcatgccgtaggaccaaacttcaacaaagtttcggaggttgaaggtgacaaacagttggcagaggcttatgagtccatcgctaagattgtcaacgataacaattacaagtcagtagcgattccactgttgtccaccggcatcttttccgggaacaaagatcgactaacccaatcattgaaccatttgctgacagctttagacaccactgatgcagatgtagccatatactgcagggacaagaaatgggaaatgactctcaaggaagcagtggctaggagagaagcagtggaggagatatgcatatccgacgactcttcagtgacagaacctgatgcagagctggtgagggtgcatccgaagagttctttggctggaaggaagggctacagcacaagcgatggcaaaactttctcatatttggaagggaccaagtttcaccaggcggccaaggatatagcagaaattaatgccatgtggcccgttgcaacggaggccaatgagcaggtatgcatgtatatcctcggagaaagcatgagcagtattaggtcgaaatgccccgtcgaagagtcggaagcctccacaccacctagcacgctgccttgcttgtgcatccatgccatgactccagaaagagtacagcgcctaaaagcctcacgtccagaacaaattactgtgtgctcatcctttccattgccgaagtatagaatcactggtgtgcagaagatccaatgctcccagcctatattgttctcaccgaaagtgcctgcgtatattcatccaaggaagtatctcgtggaaacaccaccggtagacgagactccggagccatcggcagagaaccaatccacagaggggacacctgaacaaccaccacttataaccgaggatgagaccaggactagaacgcctgagccgatcatcatcgaagaggaagaagaggatagcataagtttgctgtcagatggcccgacccaccaggtgctgcaagtcgaggcagacattcacgggccgccctctgtatctagctcatcctggtccattcctcatgcatccgactttgatgtggacagtttatccatacttgacaccctggagggagctagcgtgaccagcggggcaacgtcagccgagactaactcttacttcgcaaagagtatggagtttctggcgcgaccggtgcctgcgcctcgaacagtattcaggaaccctccacatcccgctccgcgcacaagaacaccgtcacttgcacccagcagggcctgctcgagaaccagcctagtttccaccccgccaggcgtgaatagggtgatcactagagaggagctcgaggcgcttaccccgtcacgcactcctagcaggtcggtctcgagaaccagcctggtctccaacccgccaggcgtaaatagggtgattacaagagaggagtttgaggcgttcgtagcacaacaacaatgacggtttgatgcgggtgcatacatcttttcctccgacaccggtcaagggcatttacaacaaaaatcagtaaggcaaacggtgctatccgaagtggtgttggagaggaccgaattggagatttcgtatgccccgcgcctcgaccaagaaaaagaagaattactacgcaagaaattacagttaaatcccacacctgctaacagaagcagataccagtccaggaaggtggagaacatgaaagccataacagctagacgtattctgcaaggcctagggcattatttgaaggcagaaggaaaagtggagtgctaccgaaccctgcatcctgttcctttgtattcatctagtgtgaaccgtgccttttcaagccccaaggtcgcagtggaagcctgtaacgccatgttgaaagagaactttccgactgtggcttcttactgtattattccagagtacgatgcctatttggacatggttgacggagcttcatgctgcttagacactgccagtttttgccctgcaaagctgcgcagctttccaaagaaacactcctatttggaacccacaatacgatcggcagtgccttcagcgatccagaacacgctccagaacgtcctggcagctgccacaaaaagaaattgcaatgtcacgcaaatgagagaattgcccgtattggattcggcggcctttaatgtggaatgcttcaagaaatatgcgtgtaataatgaatattgggaaacgtttaaagaaaaccccatcaggcttactgaagaaaacgtggtaaattacattaccaaattaaaaggaccaaaagctgctgctctttttgcgaagacacataatttgaatatgttgcaggacataccaatggacaggtttgtaatggacttaaagagagacgtgaaagtgactccaggaacaaaacatactgaagaacggcccaaggtacaggtgatccaggctgccgatccgctagcaacagcgtatctgtgcggaatccaccgagagctggttaggagattaaatgcggtcctgcttccgaacattcatacactgtttgatatgtcggctgaagactttgacgctattatagccgagcacttccagcctggggattgtgttctggaaactgacatcgcgtcgtttgataaaagtgaggacgacgccatggctctgaccgcgttaatgattctggaagacttaggtgtggacgcagagctgttgacgctgattgaggcggctttcggcgaaatttcatcaatacatttgcccactaaaactaaatttaaattcggagccatgatgaaatctggaatgttcctcacactgtttgtgaacacagtcattaacattgtaatcgcaagcagagtgttgagagaacggctaaccggatcaccatgtgcagcattcattggagatgacaatatcgtgaaaggagtcaaatcggacaaattaatggcagacaggtgcgccacctggttgaatatggaagtcaagattatagatgctgtggtgggcgagaaagcgccttatttctgtggagggtttattttgtgtgactccgtgaccggcacagcgtgccgtgtggcagaccccctaaaaaggctgtttaagcttggcaaacctctggcagcagacgatgaacatgatgatgacaggagaagggcattgcatgaagagtcaacacgctggaaccgagtgggtattctttcagagctgtgcaaggcagtagaatcaaggtatgaaaccgtaggaacttccatcatagttatggccatgactactctagctagcagtgttaaatcattcagctacctgagaggggcccctataactctctacggctaacctgaatggactacgacatagtctagtccgccaagatgaggcctggcctgccctcctacctgatcatcctggccgtgtgcctgttcagccacctgctgtccagcagatacggcgccgaggccgtgagcgagcccctggacaaggctttccacctgctgctgaacacctacggcagacccatccggtttctgcgggagaacaccacccagtgcacctacaacagcagcctgcggaacagcaccgtcgtgagagagaacgccatcagcttcaactttttccagagctacaaccagtactacgtgttccacatgcccagatgcctgtttgccggccctctggccgagcagttcctgaaccaggtggacctgaccgagacactggaaagataccagcagcggctgaatacctacgccctggtgtccaaggacctggccagctaccggtcctttagccagcagctcaaggctcaggatagcctcggcgagcagcctaccaccgtgccccctcccatcgacctgagcatcccccacgtgtggatgcctccccagaccacccctcacggctggaccgagagccacaccacctccggcctgcacagaccccacttcaaccagacctgcatcctgttcgacggccacgacctgctgtttagcaccgtgaccccctgcctgcaccagggcttctacctgatcgacgagctgagatacgtgaagatcaccctgaccgaggatttcttcgtggtcaccgtgtccatcgacgacgacacccccatgctgctgatcttcggccacctgcccagagtgctgttcaaggccccctaccagcgggacaacttcatcctgcggcagaccgagaagcacgagctgctggtgctggtcaagaaggaccagctgaaccggcactcctacctgaaggaccccgacttcctggacgccgccctggacttcaactacctggacctgagcgccctgctgagaaacagcttccacagatacgccgtggacgtgctgaagtccggacggtgccagatgctcgatcggcggaccgtggagatggccttcgcctatgccctcgccctgttcgccgctgccagacaggaagaggctggcgcccaggtgtcagtgcccagagccctggatagacaggccgccctgctgcagatccaggaattcatgatcacctgcctgagccagaccccccctagaaccaccctgctgctgtaccccacagccgtggatctggccaagagggccctgtggacccccaaccagatcaccgacatcacaagcctcgtgcggctcgtgtacatcctgagcaagcagaaccagcagcacctgatcccccagtgggccctgagacagatcgccgacttcgccctgaagctgcacaagacccatctggccagctttctgagcgccttcgccaggcaggaactgtacctgatgggcagcctggtccacagcatgctggtgcataccaccgagcggcgggagatcttcatcgtggagacaggcctgtgtagcctggccgagctgtcccactttacccagctgctggcccaccctcaccacgagtacctgagcgacctgtacaccccctgcagcagcagcggcagacgggaccacagcctggaacggctgaccagactgttccccgatgccaccgtgcctgctacagtgcctgccgccctgtccatcctgtccaccatgcagcccagcaccctggaaaccttccccgacctgttctgcctgcccctgggcgagagctttagcgccctgaccgtgtccgagcacgtgtcctacatcgtgaccaatcagtacctgatcaagggcatcagctaccccgtgtccaccacagtcgtgggccagagcctgatcatcacccagaccgacagccagaccaagtgcgagctgacccggaacatgcacaccacacacagcatcaccgtggccctgaacatcagcctggaaaactgcgctttctgtcagtctgccctgctggaatacgacgatacccagggcgtgatcaacatcatgtacatgcacgacagcgacgacgtgctgttcgccctggacccctacaacgaggtggtggtgtccagcccccggacccactacctgatgctgctgaagaacggcaccgtgctggaagtgaccgacgtggtggtggacgccaccgactgataatctagattaaaacagctgtgggttgttcccacccacagggcccactgggcgctagcactctgattttacgaaatccttgtgcgcctgttttatatcccttccctaattcgaaacgtagaagcaatgcgcaccactgatcaatagtaggcgtaacgcgccagttacgtcatgatcaagcatatctgttcccccggactgagtatcaatagactgcttacgcggttgaaggagaaaacgttcgttatccggctaactacttcgagaagcccagtaacaccatggaagctgcagggtgtttcgctcagcacttcccccgtgtagatcaggtcgatgagccactgcaatccccacaggtgactgtggcagtggctgcgttggcggcctgcctatggggagacccataggacgctctaatgtggacatggtgcgaagagcctattgagctagttagtagtcctccggcccctgaatgcggctaatcctaactgcggagcacatgccttcaacccagagggtagtgtgtcgtaatgggcaactctgcagcggaaccgactactttgggtgtccgtgtttctttttattcttatattggctgcttatggtgacaattacagaattgttaccatatagctattggattggccatccggtgtgtaatagagctgttatatacctatttgttggctttgtaccactaactttaaaatctataactaccctcaactttatattaaccctcaatacagttgaacatgtgcagaaggcccgactgcggcttcagcttcagccctggacccgtgatcctgctgtggtgctgcctgctgctgcctatcgtgtcctctgccgccgtgtctgtggcccctacagccgccgagaaggtgccagccgagtgccccgagctgaccagaagatgcctgctgggcgaggtgttcgagggcgacaagtacgagagctggctgcggcccctggtcaacgtgaccggcagagatggccccctgagccagctgatccggtacagacccgtgacccccgaggccgccaatagcgtgctgctggacgaggccttcctggataccctggccctgctgtacaacaaccccgaccagctgagagccctgctgaccctgctgtccagcgacaccgcccccagatggatgaccgtgatgcggggctacagcgagtgtggagatggcagccctgccgtgtacacctgcgtggacgacctgtgcagaggctacgacctgaccagactgagctacggccggtccatcttcacagagcacgtgctgggcttcgagctggtgccccccagcctgttcaacgtggtggtggccatccggaacgaggccaccagaaccaacagagccgtgcggctgcctgtgtctacagccgctgcacctgagggcatcacactgttctacggcctgtacaacgccgtgaaagagttctgcctccggcaccagctggatccccccctgctgagacacctggacaagtactacgccggcctgcccccagagctgaagcagaccagagtgaacctgcccgcccacagcagatatggccctcaggccgtggacgccagatgataagcggccgcatacagcagcaattggcaagctgcttacatagaactcgcggcgattggcatgccgccttaaaatttttattttatttttcttttcttttccgaatcggattttgtttttaatatttcaaaaaaaaaaaaaaaaaaaaaaaaaaaaaaaaaaagggtcggcatggcatctccacctcctcgcggtccgacctgggcatccgaaggaggacgcacgtccactcggatggctaagggagagccacgtttaaacacgtgatatctggcctcatgggccttcctttcactgcccgctttccagtcgggaaacctgtcgtgccagctgcattaacatggtcatagctgtttccttgcgtattgggcgctctccgcttcctcgctcactgactcgctgcgctcggtcgttcgggtaaagcctggggtgcctaatgagcaaaaggccagcaaaaggccaggaaccgtaaaaaggccgcgttgctggcgtttttccataggctccgcccccctgacgagcatcacaaaaatcgacgctcaagtcagaggtggcgaaacccgacaggactataaagataccaggcgtttccccctggaagctccctcgtgcgctctcctgttccgaccctgccgcttaccggatacctgtccgcctttctcccttcgggaagcgtggcgctttctcatagctcacgctgtaggtatctcagttcggtgtaggtcgttcgctccaagctgggctgtgtgcacgaaccccccgttcagcccgaccgctgcgccttatccggtaactatcgtcttgagtccaacccggtaagacacgacttatcgccactggcagcagccactggtaacaggattagcagagcgaggtatgtaggcggtgctacagagttcttgaagtggtggcctaactacggctacactagaagaacagtatttggtatctgcgctctgctgaagccagttaccttcggaaaaagagttggtagctcttgatccggcaaacaaaccaccgctggtagcggtggtttttttgtttgcaagcagcagattacgcgcagaaaaaaaggatctcaagaagatcctttgatcttttctacggggtctgacgctcagtggaacgaaaactcacgttaagggattttggtcatgagattatcaaaaaggatcttcacctagatccttttaaattaaaaatgaagttttaaatcaatctaaagtatatatgagtaaacttggtctgacagttattagaaaaattcatccagcagacgataaaacgcaatacgctggctatccggtgccgcaatgccatacagcaccagaaaacgatccgcccattcgccgcccagttcttccgcaatatcacgggtggccagcgcaatatcctgataacgatccgccacgcccagacggccgcaatcaataaagccgctaaaacggccattttccaccataatgttcggcaggcacgcatcaccatgggtcaccaccagatcttcgccatccggcatgctcgctttcagacgcgcaaacagctctgccggtgccaggccctgatgttcttcatccagatcatcctgatccaccaggcccgcttccatacgggtacgcgcacgttcaatacgatgtttcgcctgatgatcaaacggacaggtcgccgggtccagggtatgcagacgacgcatggcatccgccataatgctcactttttctgccggcgccagatggctagacagcagatcctgacccggcacttcgcccagcagcagccaatcacggcccgcttcggtcaccacatccagcaccgccgcacacggaacaccggtggtggccagccagctcagacgcgccgcttcatcctgcagctcgttcagcgcaccgctcagatcggttttcacaaacagcaccggacgaccctgcgcgctcagacgaaacaccgccgcatcagagcagccaatggtctgctgcgcccaatcatagccaaacagacgttccacccacgctgccgggctacccgcatgcaggccatcctgttcaatcatactcttcctttttcaatattattgaagcatttatcagggttattgtctcatgagcggatacatatttgaatgtatttagaaaaataaacaaataggggttccgcgcacatttccccgaaaagtgccacctaaattgtaagcgttaatattttgttaaaattcgcgttaaatttttgttaaatcagctcattttttaaccaataggccgaaatcggcaaaatcccttataaatcaaaagaatagaccgagatagggttgagtggccgctacagggcgctcccattcgccattcaggctgcgcaactgttgggaagggcgtttcggtgcgggcctcttcgctattacgccagctggcgaaagggggatgtgctgcaaggcgattaagttgggtaacgccagggttttcccagtcacacgcgtaatacgactcactatag

SEQ ID NO: 61 - DNA, 13788 bp, Artificial Sequence
  source: /note="Description of Artificial Sequence: Synthetic polynucleotide"
ataggcggcgcatgagagaagcccagaccaattacctacccaaaatggagaaagttcacgttgacatcgaggaagacagcccattcctcagagctttgcagcggagcttcccgcagtttgaggtagaagccaagcaggtcactgataatgaccatgctaatgccagagcgttttcgcatctggcttcaaaactgatcgaaacggaggtggacccatccgacacgatccttgacattggaagtgcgcccgcccgcagaatgtattctaagcacaagtatcattgtatctgtccgatgagatgtgcggaagatccggacagattgtataagtatgcaactaagctgaagaaaaactgtaaggaaataactgataaggaattggacaagaaaatgaaggagctcgccgccgtcatgagcgaccctgacctggaaactgagactatgtgcctccacgacgacgagtcgtgtcgctacgaagggcaagtcgctgtttaccaggatgtatacgcggttgacggaccgacaagtctctatcaccaagccaataagggagttagagtcgcctactggataggctttgacaccaccccttttatgtttaagaacttggctggagcatatccatcatactctaccaactgggccgacgaaaccgtgttaacggctcgtaacataggcctatgcagctctgacgttatggagcggtcacgtagagggatgtccattcttagaaagaagtatttgaaaccatccaacaatgttctattctctgttggctcgaccatctaccacgagaagagggacttactgaggagctggcacctgccgtctgtatttcacttacgtggcaagcaaaattacacatgtcggtgtgagactatagttagttgcgacgggtacgtcgttaaaagaatagctatcagtccaggcctgtatgggaagccttcaggctatgctgctacgatgcaccgcgagggattcttgtgctgcaaagtgacagacacattgaacggggagagggtctcttttcccgtgtgcacgtatgtgccagctacattgtgtgaccaaatgactggcatactggcaacagatgtcagtgcggacgacgcgcaaaaactgctggttgggctcaaccagcgtatagtcgtcaacggtcgcacccagagaaacaccaataccatgaaaaattaccttttgcccgtagtggcccaggcatttgctaggtgggcaaaggaatataaggaagatcaagaagatgaaaggccactaggactacgagatagacagttagtcatggggtgttgttgggcttttagaaggcacaagataacatctatttataagcgcccggatacccaaaccatcatcaaagtgaacagcgatttccactcattcgtgctgcccaggataggcagtaacacattggagatcgggctgagaacaagaatcaggaaaatgttagaggagcacaaggagccgtcacctctcattaccgccgaggacgtacaagaagctaagtgcgcagccgatgaggctaaggaggtgcgtgaagccgaggagttgcgcgcagctctaccacctttggcagctgatgttgaggagcccactctggaagccgatgtcgacttgatgttacaagaggctggggccggctcagtggagacacctcgtggcttgataaaggttaccagctacgatggcgaggacaagatcggctcttacgctgtgctttctccgcaggctgtactcaagagtgaaaaattatcttgcatccaccctctcgctgaacaagtcatagtgataacacactctggccgaaaagggcgttatgccgtggaaccataccatggtaaagtagtggtgccagagggacatgcaatacccgtccaggactttcaagctctgagtgaaagtgccaccattgtgtacaacgaacgtgagttcgtaaacaggtacctgcaccatattgccacacatggaggagcgctgaacactgatgaagaatattacaaaactgtcaagcccagcgagcacgacggcgaatacctgtacgacatcgacaggaaacagtgcgtcaagaaagaactagtcactgggctagggctcacaggcgagctggtggatcctcccttccatgaattcgcctacgagagtctgagaacacgaccagccgctccttaccaagtaccaaccataggggtgtatggcgtgccaggatcaggcaagtctggcatcattaaaagcgcagtcaccaaaaaagatctagtggtgagcgccaagaaagaaaactgtgcagaaattataagggacgtcaagaaaatgaaagggctggacgtcaatgccagaactgtggactcagtgctcttgaatggatgcaaacaccccgtagagaccctgtatattgacgaagcttttgcttgtcatgcaggtactctcagagcgctcatagccattataagacctaaaaaggcagtgctctgcggggatcccaaacagtgcggtttttttaacatgatgtgcctgaaagtgcattttaaccacgagatttgcacacaagtcttccacaaaagcatctctcgccgttgcactaaatctgtgacttcggtcgtctcaaccttgttttacgacaaaaaaatgagaacgacgaatccgaaagagactaagattgtgattgacactaccggcagtaccaaacctaagcaggacgatctcattctcacttgtttcagagggtgggtgaagcagttgcaaatagattacaaaggcaacgaaataatgacggcagctgcctctcaagggctgacccgtaaaggtgtgtatgccgttcggtacaaggtgaatgaaaatcctctgtacgcacccacctcagaacatgtgaacgtcctactgacccgcacggaggaccgcatcgtgtggaaaacactagccggcgacccatggataaaaacactgactgccaagtaccctgggaatttcactgccacgatagaggagtggcaagcagagcatgatgccatcatgaggcacatcttggagagaccggaccctaccgacgtcttccagaataaggcaaacgtgtgttgggccaaggctttagtgccggtgctgaagaccgctggcatagacatgaccactgaacaatggaacactgtggattattttgaaacggacaaagctcactcagcagagatagtattgaaccaactatgcgtgaggttctttggactcgatctggactccggtctattttctgcacccactgttccgttatccattaggaataatcactgggataactccccgtcgcctaacatgtacgggctgaataaagaagtggtccgtcagctctctcgcaggtacccacaactgcctcgggcagttgccactggaagagtctatgacatgaacactggtacactgcgcaattatgatccgcgcataaacctagtacctgtaaacagaagactgcctcatgctttagtcctccaccataatgaacacccacagagtgacttttcttcattcgtcagcaaattgaagggcagaactgtcctggtggtcggggaaaagttgtccgtcccaggcaaaatggttgactggttgtcagaccggcctgaggctaccttcagagctcggctggatttaggcatcccaggtgatgtgcccaaatatgacataatatttgttaatgtgaggaccccatataaataccatcactatcagcagtgtgaagaccatgccattaagcttagcatgttgaccaagaaagcttgtctgcatctgaatcccggcggaacctgtgtcagcataggttatggttacgctgacagggccagcgaaagcatcattggtgctatagcgcggcagttcaagttttcccgggtatgcaaaccgaaatcctcacttgaagagacggaagttctgtttgtattcattgggtacgatcgcaaggcccgtacgcacaatccttacaagctttcatcaaccttgaccaacatttatacaggttccagactccacgaagccggatgtgcaccctcatatcatgtggtgcgaggggatattgccacggccaccgaaggagtgattataaatgctgctaacagcaaaggacaacctggcggaggggtgtgcggagcgctgtataagaaattcccggaaagcttcgatttacagccgatcgaagtaggaaaagcgcgactggtcaaaggtgcagctaaacatatcattcatgccgtaggaccaaacttcaacaaagtttcggaggttgaaggtgacaaacagttggcagaggcttatgagtccatcgctaagattgtcaacgataacaattacaagtcagtagcgattccactgttgtccaccggcatcttttccgggaacaaagatcgactaacccaatcattgaaccatttgctgacagctttagacaccactgatgcagatgtagccatatactgcagggacaagaaatgggaaatgactctcaaggaagcagtggctaggagagaagcagtggaggagatatgcatatccgacgactcttcagtgacagaacctgatgcagagctggtgagggtgcatccgaagagttctttggctggaaggaagggctacagcacaagcgatggcaaaactttctcatatttggaagggaccaagtttcaccaggcggccaaggatatagcagaaattaatgccatgtggcccgttgcaacggaggccaatgagcaggtatgcatgtatatcctcggagaaagcatgagcagtattaggtcgaaatgccccgtcgaagagtcggaagcctccacaccacctagcacgctgccttgcttgtgcatccatgccatgactccagaaagagtacagcgcctaaaagcctcacgtccagaacaaattactgtgtgctcatcctttccattgccgaagtatagaatcactggtgtgcagaagatccaatgctcccagcctatattgttctcaccgaaagtgcctgcgtatattcatccaaggaagtatctcgtggaaacaccaccggtagacgagactccggagccatcggcagagaaccaatccacagaggggacacctgaacaaccaccacttataaccgaggatgagaccaggactagaacgcctgagccgatcatcatcgaagaggaagaagaggatagcataagtttgctgtcagatggcccgacccaccaggtgctgcaagtcgaggcagacattcacgggccgccctctgtatctagctcatcctggtccattcctcatgcatccgactttgatgtggacagtttatccatacttgacaccctggagggagctagcgtgaccagcggggcaacgtcagccgagactaactcttacttcgcaaagagtatggagtttctggcgcgaccggtgcctgcgcctcgaacagtattcaggaaccctccacatcccgctccgcgcacaagaacaccgtcacttgcacccagcagggcctgctcgagaaccagcctagtttccaccccgccaggcgtgaatagggtgatcactagagaggagctcgaggcgcttaccccgtcacgcactcctagcaggtcggtctcgagaaccagcctggtctccaacccgccaggcgtaaatagggtgattacaagagaggagtttgaggcgttcgtagcacaacaacaatgacggtttgatgcgggtgcatacatcttttcctccgacaccggtcaagggcatttacaacaaaaatcagtaaggcaaacggtgctatccgaagtggtgttggagaggaccgaattggagatttcgtatgccccgcgcctcgaccaagaaaaagaagaattactacgcaagaaattacagttaaatcccacacctgctaacagaagcagataccagtccaggaaggtggagaacatgaaagccataacagctagacgtattctgcaaggcctagggcattatttgaaggcagaaggaaaagtggagtgctaccgaaccctgcatcctgttcctttgtattcatctagtgtgaaccgtgccttttcaagccccaaggtcgcagtggaagcctgtaacgccatgttgaaagagaactttccgactgtggcttcttactgtattattccagagtacgatgcctatttggacatggttgacggagcttcatgctgcttagacactgccagtttttgccctgcaaagctgcgcagctttccaaagaaacactcctatttggaacccacaatacgatcggcagtgccttcagcgatccagaacacgctccagaacgtcctggcagctgccacaaaaagaaattgcaatgtcacgcaaatgagagaattgcccgtattggattcggcggcctttaatgtggaatgcttcaagaaatatgcgtgtaataatgaatattgggaaacgtttaaagaaaaccccatcaggcttactgaagaaaacgtggtaaattacattaccaaattaaaaggaccaaaagctgctgctctttttgcgaagacacataatttgaatatgttgcaggacataccaatggacaggtttgtaatggacttaaagagagacgtgaaagtgactccaggaacaaaacatactgaagaacggcccaaggtacaggtgatccaggctgccgatccgctagcaacagcgtatctgtgcggaatccaccgagagctggttaggagattaaatgcggtcctgcttccgaacattcatacactgtttgatatgtcggctgaagactttgacgctattatagccgagcacttccagcctggggattgtgttctggaaactgacatcgcgtcgtttgataaaagtgaggacgacgccatggctctgaccgcgttaatgattctggaagacttaggtgtggacgcagagctgttgacgctgattgaggcggctttcggcgaaatttcatcaatacatttgcccactaaaactaaatttaaattcggagccatgatgaaatctggaatgttcctcacactgtttgtgaacacagtcattaacattgtaatcgcaagcagagtgttgagagaacggctaaccggatcaccatgtgcagcattcattggagatgacaatatcgtgaaaggagtcaaatcggacaaattaatggcagacaggtgcgccacctggttgaatatggaagtcaagattatagatgctgtggtgggcgagaaagcgccttatttctgtggagggtttattttgtgtgactccgtgaccggcacagcgtgccgtgtggcagaccccctaaaaaggctgtttaagcttggcaaacctctggcagcagacgatgaacatgatgatgacaggagaagggcattgcatgaagagtcaacacgctggaaccgagtgggtattctttcagagctgtgcaaggcagtagaatcaaggtatgaaaccgtaggaacttccatcatagttatggccatgactactctagctagcagtgttaaatcattcagctacctgagaggggcccctataactctctacggctaacctgaatggactacgacatagtctagtccgccaagatgtgcagaaggcccgactgcggcttcagcttcagccctggacccgtgatcctgctgtggtgctgcctgctgctgcctatcgtgtcctctgccgccgtgtctgtggcccctacagccgccgagaaggtgccagccgagtgccccgagctgaccagaagatgcctgctgggcgaggtgttcgagggcgacaagtacgagagctggctgcggcccctggtcaacgtgaccggcagagatggccccctgagccagctgatccggtacagacccgtgacccccgaggccgccaatagcgtgctgctggacgaggccttcctggataccctggccctgctgtacaacaaccccgaccagctgagagccctgctgaccctgctgtccagcgacaccgcccccagatggatgaccgtgatgcggggctacagcgagtgtggagatggcagccctgccgtgtacacctgcgtggacgacctgtgcagaggctacgacctgaccagactgagctacggccggtccatcttcacagagcacgtgctgggcttcgagctggtgccccccagcctgttcaacgtggtggtggccatccggaacgaggccaccagaaccaacagagccgtgcggctgcctgtgtctacagccgctgcacctgagggcatcacactgttctacggcctgtacaacgccgtgaaagagttctgcctccggcaccagctggatccccccctgctgagacacctggacaagtactacgccggcctgcccccagagctgaagcagaccagagtgaacctgcccgcccacagcagatatggccctcaggccgtggacgccagatgataatctagattaaaacagctgtgggttgttcccacccacagggcccactgggcgctagcactctgattttacgaaatccttgtgcgcctgttttatatcccttccctaattcgaaacgtagaagcaatgcgcaccactgatcaatagtaggcgtaacgcgccagttacgtcatgatcaagcatatctgttcccccggactgagtatcaatagactgcttacgcggttgaaggagaaaacgttcgttatccggctaactacttcgagaagcccagtaacaccatggaagctgcagggtgtttcgctcagcacttcccccgtgtagatcaggtcgatgagccactgcaatccccacaggtgactgtggcagtggctgcgttggcggcctgcctatggggagacccataggacgctctaatgtggacatggtgcgaagagcctattgagctagttagtagtcctccggcccctgaatgcggctaatcctaactgcggagcacatgccttcaacccagagggtagtgtgtcgtaatgggcaactctgcagcggaaccgactactttgggtgtccgtgtttctttttattcttatattggctgcttatggtgacaattacagaattgttaccatatagctattggattggccatccggtgtgtaatagagctgttatatacctatttgttggctttgtaccactaactttaaaatctataactaccctcaactttatattaaccctcaatacagttgaacatgaggcctggcctgccctcctacctgatcatcctggccgtgtgcctgttcagccacctgctgtccagcagatacggcgccgaggccgtgagcgagcccctggacaaggctttccacctgctgctgaacacctacggcagacccatccggtttctgcgggagaacaccacccagtgcacctacaacagcagcctgcggaacagcaccgtcgtgagagagaacgccatcagcttcaactttttccagagctacaaccagtactacgtgttccacatgcccagatgcctgtttgccggccctctggccgagcagttcctgaaccaggtggacctgaccgagacactggaaagataccagcagcggctgaatacctacgccctggtgtccaaggacctggccagctaccggtcctttagccagcagctcaaggctcaggatagcctcggcgagcagcctaccaccgtgccccctcccatcgacctgagcatcccccacgtgtggatgcctccccagaccacccctcacggctggaccgagagccacaccacctccggcctgcacagaccccacttcaaccagacctgcatcctgttcgacggccacgacctgctgtttagcaccgtgaccccctgcctgcaccagggcttctacctgatcgacgagctgagatacgtgaagatcaccctgaccgaggatttcttcgtggtcaccgtgtccatcgacgacgacacccccatgctgctgatcttcggccacctgcccagagtgctgttcaaggccccctaccagcgggacaacttcatcctgcggcagaccgagaagcacgagctgctggtgctggtcaagaaggaccagctgaaccggcactcctacctgaaggaccccgacttcctggacgccgccctggacttcaactacctggacctgagcgccctgctgagaaacagcttccacagatacgccgtggacgtgctgaagtccggacggtgccagatgctcgatcggcggaccgtggagatggccttcgcctatgccctcgccctgttcgccgctgccagacaggaagaggctggcgcccaggtgtcagtgcccagagccctggatagacaggccgccctgctgcagatccaggaattcatgatcacctgcctgagccagaccccccctagaaccaccctgctgctgtaccccacagccgtggatctggccaagagggccctgtggacccccaaccagatcaccgacatcacaagcctcgtgcggctcgtgtacatcctgagcaagcagaaccagcagcacctgatcccccagtgggccctgagacagatcgccgacttcgccctgaagctgcacaagacccatctggccagctttctgagcgccttcgccaggcaggaactgtacctgatgggcagcctggtccacagcatgctggtgcataccaccgagcggcgggagatcttcatcgtggagacaggcctgtgtagcctggccgagctgtcccactttacccagctgctggcccaccctcaccacgagtacctgagcgacctgtacaccccctgcagcagcagcggcagacgggaccacagcctggaacggctgaccagactgttccccgatgccaccgtgcctgctacagtgcctgccgccctgtccatcctgtccaccatgcagcccagcaccctggaaaccttccccgacctgttctgcctgcccctgggcgagagctttagcgccctgaccgtgtccgagcacgtgtcctacatcgtgaccaatcagtacctgatcaagggcatcagctaccccgtgtccaccacagtcgtgggccagagcctgatcatcacccagaccgacagccagaccaagtgcgagctgacccggaacatgcacaccacacacagcatcaccgtggccctgaacatcagcctggaaaactgcgctttctgtcagtctgccctgctggaatacgacgatacccagggcgtgatcaacatcatgtacatgcacgacagcgacgacgtgctgttcgccctggacccctacaacgaggtggtggtgtccagcccccggacccactacctgatgctgctgaagaacggcaccgtgctggaagtgaccgacgtggtggtggacgccaccgactgataagcggccgcatacagcagcaattggcaagctgcttacatagaactcgcggcgattggcatgccgccttaaaatttttattttatttttcttttcttttccgaatcggattttgtttttaatatttcaaaaaaaaaaaaaaaaaaaaaaaaaaaaaaaaaaagggtcggcatggcatctccacctcctcgcggtccgacctgggcatccgaaggaggacgcacgtccactcggatggctaagggagagccacgtttaaacacgtgatatctggcctcatgggccttcctttcactgcccgctttccagtcgggaaacctgtcgtgccagctgcattaacatggtcatagctgtttccttgcgtattgggcgctctccgcttcctcgctcactgactcgctgcgctcggtcgttcgggtaaagcctggggtgcctaatgagcaaaaggccagcaaaaggccaggaaccgtaaaaaggccgcgttgctggcgtttttccataggctccgcccccctgacgagcatcacaaaaatcgacgctcaagtcagaggtggcgaaacccgacaggactataaagataccaggcgtttccccctggaagctccctcgtgcgctctcctgttccgaccctgccgcttaccggatacctgtccgcctttctcccttcgggaagcgtggcgctttctcatagctcacgctgtaggtatctcagttcggtgtaggtcgttcgctccaagctgggctgtgtgcacgaaccccccgttcagcccgaccgctgcgccttatccggtaactatcgtcttgagtccaacccggtaagacacgacttatcgccactggcagcagccactggtaacaggattagcagagcgaggtatgtaggcggtgctacagagttcttgaagtggtggcctaactacggctacactagaagaacagtatttggtatctgcgctctgctgaagccagttaccttcggaaaaagagttggtagctcttgatccggcaaacaaaccaccgctggtagcggtggtttttttgtttgcaagcagcagattacgcgcagaaaaaaaggatctcaagaagatcctttgatcttttctacggggtctgacgctcagtggaacgaaaactcacgttaagggattttggtcatgagattatcaaaaaggatcttcacctagatccttttaaattaaaaatgaagttttaaatcaatctaaagtatatatgagtaaacttggtctgacagttattagaaaaattcatccagcagacgataaaacgcaatacgctggctatccggtgccgcaatgccatacagcaccagaaaacgatccgcccattcgccgcccagttcttccgcaatatcacgggtggccagcgcaatatcctgataacgatccgccacgcccagacggccgcaatcaataaagccgctaaaacggccattttccaccataatgttcggcaggcacgcatcaccatgggtcaccaccagatcttcgccatccggcatgctcgctttcagacgcgcaaacagctctgccggtgccaggccctgatgttcttcatccagatcatcctgatccaccaggcccgcttccatacgggtacgcgcacgttcaatacgatgtttcgcctgatgatcaaacggacaggtcgccgggtccagggtatgcagacgacgcatggcatccgccataatgctcactttttctgccggcgccagatggctagacagcagatcctgacccggcacttcgcccagcagcagccaatcacggcccgcttcggtcaccacatccagcaccgccgcacacggaacaccggtggtggccagccagctcagacgcgccgcttcatcctgcagctcgttcagcgcaccgctcagatcggttttcacaaacagcaccggacgaccctgcgcgctcagacgaaacaccgccgcatcagagcagccaatggtctgctgcgcccaatcatagccaaacagacgttccacccacgctgccgggctacccgcatgcaggccatcctgttcaatcatactcttcctttttcaatattattgaagcatttatcagggttattgtctcatgagcggatacatatttgaatgtatttagaaaaataaacaaataggggttccgcgcacatttccccgaaaagtgccacctaaattgtaagcgttaatattttgttaaaattcgcgttaaatttttgttaaatcagctcattttttaaccaataggccgaaatcggcaaaatcccttataaatcaaaagaatagaccgagatagggttgagtggccgctacagggcgctcccattcgccattcaggctgcgcaactgttgggaagggcgtttcggtgcgggcctcttcgctattacgccagctggcgaaagggggatgtgctgcaaggcgattaagttgggtaacgccagggttttcccagtcacacgcgtaatacgactcactatag

SEQ ID NO: 62 - DNA, 14202 bp, Artificial Sequence
  source: /note="Description of Artificial Sequence: Synthetic polynucleotide"
ataggcggcgcatgagagaagcccagaccaattacctacccaaaatggagaaagttcacgttgacatcgaggaagacagcccattcctcagagctttgcagcggagcttcccgcagtttgaggtagaagccaagcaggtcactgataatgaccatgctaatgccagagcgttttcgcatctggcttcaaaactgatcgaaacggaggtggacccatccgacacgatccttgacattggaagtgcgcccgcccgcagaatgtattctaagcacaagtatcattgtatctgtccgatgagatgtgcggaagatccggacagattgtataagtatgcaactaagctgaagaaaaactgtaaggaaataactgataaggaattggacaagaaaatgaaggagctcgccgccgtcatgagcgaccctgacctggaaactgagactatgtgcctccacgacgacgagtcgtgtcgctacgaagggcaagtcgctgtttaccaggatgtatacgcggttgacggaccgacaagtctctatcaccaagccaataagggagttagagtcgcctactggataggctttgacaccaccccttttatgtttaagaacttggctggagcatatccatcatactctaccaactgggccgacgaaaccgtgttaacggctcgtaacataggcctatgcagctctgacgttatggagcggtcacgtagagggatgtccattcttagaaagaagtatttgaaaccatccaacaatgttctattctctgttggctcgaccatctaccacgagaagagggacttactgaggagctggcacctgccgtctgtatttcacttacgtggcaagcaaaattacacatgtcggtgtgagactatagttagttgcgacgggtacgtcgttaaaagaatagctatcagtccaggcctgtatgggaagccttcaggctatgctgctacgatgcaccgcgagggattcttgtgctgcaaagtgacagacacattgaacggggagagggtctcttttcccgtgtgcacgtatgtgccagctacattgtgtgaccaaatgactggcatactggcaacagatgtcagtgcggacgacgcgcaaaaactgctggttgggctcaaccagcgtatagtcgtcaacggtcgcacccagagaaacaccaataccatgaaaaattaccttttgcccgtagtggcccaggcatttgctaggtgggcaaaggaatataaggaagatcaagaagatgaaaggccactaggactacgagatagacagttagtcatggggtgttgttgggcttttagaaggcacaagataacatctatttataagcgcccggatacccaaaccatcatcaaagtgaacagcgatttccactcattcgtgctgcccaggataggcagtaacacattggagatcgggctgagaacaagaatcaggaaaatgttagaggagcacaaggagccgtcacctctcattaccgccgaggacgtacaagaagctaagtgcgcagccgatgaggctaaggaggtgcgtgaagccgaggagttgcgcgcagctctaccacctttggcagctgatgttgaggagcccactctggaagccgatgtcgacttgatgttacaagaggctggggccggctcagtggagacacctcgtggcttgataaaggttaccagctacgatggcgaggacaagatcggctcttacgctgtgctttctccgcaggctgtactcaagagtgaaaaattatcttgcatccaccctctcgctgaacaagtcatagtgataacacactctggccgaaaagggcgttatgccgtggaaccataccatggtaaagtagtggtgccagagggacatgcaatacccgtccaggactttcaagctctgagtgaaagtgccaccattgtgtacaacgaacgtgagttcgtaaacaggtacctgcaccatattgccacacatggaggagcgctgaacactgatgaagaatattacaaaactgtcaagcccagcgagcacgacggcgaatacctgtacgacatcgacaggaaacagtgcgtcaagaaagaactagtcactgggctagggctcacaggcgagctggtggatcctcccttccatgaattcgcctacgagagtctgagaacacgaccagccgctccttaccaagtaccaaccataggggtgtatggcgtgccaggatcaggcaagtctggcatcattaaaagcgcagtcaccaaaaaagatctagtggtgagcgccaagaaagaaaactgtgcagaaattataagggacgtcaagaaaatgaaagggctggacgtcaatgccagaactgtggactcagtgctcttgaatggatgcaaacaccccgtagagaccctgtatattgacgaagcttttgcttgtcatgcaggtactctcagagcgctcatagccattataagacctaaaaaggcagtgctctgcggggatcccaaacagtgcggtttttttaacatgatgtgcctgaaagtgcattttaaccacgagatttgcacacaagtcttccacaaaagcatctctcgccgttgcactaaatctgtgacttcggtcgtctcaaccttgttttacgacaaaaaaatgagaacgacgaatccgaaagagactaagattgtgattgacactaccggcagtaccaaacctaagcaggacgatctcattctcacttgtttcagagggtgggtgaagcagttgcaaatagattacaaaggcaacgaaataatgacggcagctgcctctcaagggctgacccgtaaaggtgtgtatgccgttcggtacaaggtgaatgaaaatcctctgtacgcacccacctcagaacatgtgaacgtcctactgacccgcacggaggaccgcatcgtgtggaaaacactagccggcgacccatggataaaaacactgactgccaagtaccctgggaatttcactgccacgatagaggagtggcaagcagagcatgatgccatcatgaggcacatcttggagagaccggaccctaccgacgtcttccagaataaggcaaacgtgtgttgggccaaggctttagtgccggtgctgaagaccgctggcatagacatgaccactgaacaatggaacactgtggattattttgaaacggacaaagctcactcagcagagatagtattgaaccaactatgcgtgaggttctttggactcgatctggactccggtctattttctgcacccactgttccgttatccattaggaataatcactgggataactccccgtcgcctaacatgtacgggctgaataaagaagtggtccgtcagctctctcgcaggtacccacaactgcctcgggcagttgccactggaagagtctatgacatgaacactggtacactgcgcaattatgatccgcgcataaacctagtacctgtaaacagaagactgcctcatgctttagtcctccaccataatgaacacccacagagtgacttttcttcattcgtcagcaaattgaagggcagaactgtcctggtggtcggggaaaagttgtccgtcccaggcaaaatggttgactggttgtcagaccggcctgaggctaccttcagagctcggctggatttaggcatcccaggtgatgtgcccaaatatgacataatatttgttaatgtgaggaccccatataaataccatcactatcagcagtgtgaagaccatgccattaagcttagcatgttgaccaagaaagcttgtctgcatctgaatcccggcggaacctgtgtcagcataggttatggttacgctgacagggccagcgaaagcatcattggtgctatagcgcggcagttcaagttttcccgggtatgcaaaccgaaatcctcacttgaagagacggaagttctgtttgtattcattgggtacgatcgcaaggcccgtacgcacaatccttacaagctttcatcaaccttgaccaacatttatacaggttccagactccacgaagccggatgtgcaccctcatatcatgtggtgcgaggggatattgccacggccaccgaaggagtgattataaatgctgctaacagcaaaggacaacctggcggaggggtgtgcggagcgctgtataagaaattcccggaaagcttcgatttacagccgatcgaagtaggaaaagcgcgactggtcaaaggtgcagctaaacatatcattcatgccgtaggaccaaacttcaacaaagtttcggaggttgaaggtgacaaacagttggcagaggcttatgagtccatcgctaagattgtcaacgataacaattacaagtcagtagcgattccactgttgtccaccggcatcttttccgggaacaaagatcgactaacccaatcattgaaccatttgctgacagctttagacaccactgatgcagatgtagccatatactgcagggacaagaaatgggaaatgactctcaaggaagcagtggctaggagagaagcagtggaggagatatgcatatccgacgactcttcagtgacagaacctgatgcagagctggtgagggtgcatccgaagagttctttggctggaaggaagggctacagcacaagcgatggcaaaactttctcatatttggaagggaccaagtttcaccaggcggccaaggatatagcagaaattaatgccatgtggcccgttgcaacggaggccaatgagcaggtatgcatgtatatcctcggagaaagcatgagcagtattaggtcgaaatgccccgtcgaagagtcggaagcctccacaccacctagcacgctgccttgcttgtgcatccatgccatgactccagaaagagtacagcgcctaaaagcctcacgtccagaacaaattactgtgtgctcatcctttccattgccgaagtatagaatcactggtgtgcagaagatccaatgctcccagcctatattgttctcaccgaaagtgcctgcgtatattcatccaaggaagtatctcgtggaaacaccaccggtagacgagactccggagccatcggcagagaaccaatccacagaggggacacctgaacaaccaccacttataaccgaggatgagaccaggactagaacgcctgagccgatcatcatcgaagaggaagaagaggatagcataagtttgctgtcagatggcccgacccaccaggtgctgcaagtcgaggcagacattcacgggccgccctctgtatctagctcatcctggtccattcctcatgcatccgactttgatgtggacagtttatccatacttgacaccctggagggagctagcgtgaccagcggggcaacgtcagccgagactaactcttacttcgcaaagagtatggagtttctggcgcgaccggtgcctgcgcctcgaacagtattcaggaaccctccacatcccgctccgcgcacaagaacaccgtcacttgcacccagcagggcctgctcgagaaccagcctagtttccaccccgccaggcgtgaatagggtgatcactagagaggagctcgaggcgcttaccccgtcacgcactcctagcaggtcggtctcgagaaccagcctggtctccaacccgccaggcgtaaatagggtgattacaagagaggagtttgaggcgttcgtagcacaacaacaatgacggtttgatgcgggtgcatacatcttttcctccgacaccggtcaagggcatttacaacaaaaatcagtaaggcaaacggtgctatccgaagtggtgttggagaggaccgaattggagatttcgtatgccccgcgcctcgaccaagaaaaagaagaattactacgcaagaaattacagttaaatcccacacctgctaacagaagcagataccagtccaggaaggtggagaacatgaaagccataacagctagacgtattctgcaaggcctagggcattatttgaaggcagaaggaaaagtggagtgctaccgaaccctgcatcctgttcctttgtattcatctagtgtgaaccgtgccttttcaagccccaaggtcgcagtggaagcctgtaacgccatgttgaaagagaactttccgactgtggcttcttactgtattattccagagtacgatgcctatttggacatggttgacggagcttcatgctgcttagacactgccagtttttgccctgcaaagctgcgcagctttccaaagaaacactcctatttggaacccacaatacgatcggcagtgccttcagcgatccagaacacgctccagaacgtcctggcagctgccacaaaaagaaattgcaatgtcacgcaaatgagagaattgcccgtattggattcggcggcctttaatgtggaatgcttcaagaaatatgcgtgtaataatgaatattgggaaacgtttaaagaaaaccccatcaggcttactgaagaaaacgtggtaaattacattaccaaattaaaaggaccaaaagctgctgctctttttgcgaagacacataatttgaatatgttgcaggacataccaatggacaggtttgtaatggacttaaagagagacgtgaaagtgactccaggaacaaaacatactgaagaacggcccaaggtacaggtgatccaggctgccgatccgctagcaacagcgtatctgtgcggaatccaccgagagctggttaggagattaaatgcggtcctgcttccgaacattcatacactgtttgatatgtcggctgaagactttgacgctattatagccgagcacttccagcctggggattgtgttctggaaactgacatcgcgtcgtttgataaaagtgaggacgacgccatggctctgaccgcgttaatgattctggaagacttaggtgtggacgcagagctgttgacgctgattgaggcggctttcggcgaaatttcatcaatacatttgcccactaaaactaaatttaaattcggagccatgatgaaatctggaatgttcctcacactgtttgtgaacacagtcattaacattgtaatcgcaagcagagtgttgagagaacggctaaccggatcaccatgtgcagcattcattggagatgacaatatcgtgaaaggagtcaaatcggacaaattaatggcagacaggtgcgccacctggttgaatatggaagtcaagattatagatgctgtggtgggcgagaaagcgccttatttctgtggagggtttattttgtgtgactccgtgaccggcacagcgtgccgtgtggcagaccccctaaaaaggctgtttaagcttggcaaacctctggcagcagacgatgaacatgatgatgacaggagaagggcattgcatgaagagtcaacacgctggaaccgagtgggtattctttcagagctgtgcaaggcagtagaatcaaggtatgaaaccgtaggaacttccatcatagttatggccatgactactctagctagcagtgttaaatcattcagctacctgagaggggcccctataactctctacggctaacctgaatggactacgacatagtctagtccgccaagctattccagaagtagtgaggaggcttttttggaggcctaggcttttgcaaaaagcttgtatatccattttcggatctgatcaagagacaggatgaggatcgtttcgcatgattgaataagatggattgcacgtaggttctccggccgcttgggtggagaggctattcggctatgactgggcacaactgacaatcggctgctctgatgccgccgtgatccggttgtcagcgcaggggcgcccggttctttttgtcaagaccgacctgtccggtgccctgaatgaactgaaggacgaggcagcgcggctatcgtggctggccacgacgggcgttccttgcgcagtctagactggcgcgccaaacctgcaggttaaaacagctgtgggttgttcccacccacagggcccactgggcgctagcactctgattttacgaaatccttgtgcgcctgttttatatcccttccctaattcgaaacgtagaagcaatgcgcaccactgatcaatagtaggcgtaacgcgccagttacgtcatgatcaagcatatctgttcccccggactgagtatcaatagactgcttacgcggttgaaggagaaaacgttcgttatccggctaactacttcgagaagcccagtaacaccatggaagctgcagggtgtttcgctcagcacttcccccgtgtagatcaggtcgatgagccactgcaatccccacaggtgactgtggcagtggctgcgttggcggcctgcctatggggagacccataggacgctctaatgtggacatggtgcgaagagcctattgagctagttagtagtcctccggcccctgaatgcggctaatcctaactgcggagcacatgccttcaacccagagggtagtgtgtcgtaatgggcaactctgcagcggaaccgactactttgggtgtccgtgtttctttttattcttatattggctgcttatggtgacaattacagaattgttaccatatagctattggattggccatccggtgtgtaatagagctgttatatacctatttgttggctttgtaccactaactttaaaatctataactaccctcaactttatattaaccctcaatacagttgaacatgaggcctggcctgccctcctacctgatcatcctggccgtgtgcctgttcagccacctgctgtccagcagatacggcgccgaggccgtgagcgagcccctggacaaggctttccacctgctgctgaacacctacggcagacccatccggtttctgcgggagaacaccacccagtgcacctacaacagcagcctgcggaacagcaccgtcgtgagagagaacgccatcagcttcaactttttccagagctacaaccagtactacgtgttccacatgcccagatgcctgtttgccggccctctggccgagcagttcctgaaccaggtggacctgaccgagacactggaaagataccagcagcggctgaatacctacgccctggtgtccaaggacctggccagctaccggtcctttagccagcagctcaaggctcaggatagcctcggcgagcagcctaccaccgtgccccctcccatcgacctgagcatcccccacgtgtggatgcctccccagaccacccctcacggctggaccgagagccacaccacctccggcctgcacagaccccacttcaaccagacctgcatcctgttcgacggccacgacctgctgtttagcaccgtgaccccctgcctgcaccagggcttctacctgatcgacgagctgagatacgtgaagatcaccctgaccgaggatttcttcgtggtcaccgtgtccatcgacgacgacacccccatgctgctgatcttcggccacctgcccagagtgctgttcaaggccccctaccagcgggacaacttcatcctgcggcagaccgagaagcacgagctgctggtgctggtcaagaaggaccagctgaaccggcactcctacctgaaggaccccgacttcctggacgccgccctggacttcaactacctggacctgagcgccctgctgagaaacagcttccacagatacgccgtggacgtgctgaagtccggacggtgccagatgctcgatcggcggaccgtggagatggccttcgcctatgccctcgccctgttcgccgctgccagacaggaagaggctggcgcccaggtgtcagtgcccagagccctggatagacaggccgccctgctgcagatccaggaattcatgatcacctgcctgagccagaccccccctagaaccaccctgctgctgtaccccacagccgtggatctggccaagagggccctgtggacccccaaccagatcaccgacatcacaagcctcgtgcggctcgtgtacatcctgagcaagcagaaccagcagcacctgatcccccagtgggccctgagacagatcgccgacttcgccctgaagctgcacaagacccatctggccagctttctgagcgccttcgccaggcaggaactgtacctgatgggcagcctggtccacagcatgctggtgcataccaccgagcggcgggagatcttcatcgtggagacaggcctgtgtagcctggccgagctgtcccactttacccagctgctggcccaccctcaccacgagtacctgagcgacctgtacaccccctgcagcagcagcggcagacgggaccacagcctggaacggctgaccagactgttccccgatgccaccgtgcctgctacagtgcctgccgccctgtccatcctgtccaccatgcagcccagcaccctggaaaccttccccgacctgttctgcctgcccctgggcgagagctttagcgccctgaccgtgtccgagcacgtgtcctacatcgtgaccaatcagtacctgatcaagggcatcagctaccccgtgtccaccacagtcgtgggccagagcctgatcatcacccagaccgacagccagaccaagtgcgagctgacccggaacatgcacaccacacacagcatcaccgtggccctgaacatcagcctggaaaactgcgctttctgtcagtctgccctgctggaatacgacgatacccagggcgtgatcaacatcatgtacatgcacgacagcgacgacgtgctgttcgccctggacccctacaacgaggtggtggtgtccagcccccggacccactacctgatgctgctgaagaacggcaccgtgctggaagtgaccgacgtggtggtggacgccaccgacctgttgaattttgaccttcttaagcttgcgggagacgtcgagtccaaccccgggcccatgtgcagaaggcccgactgcggcttcagcttcagccctggacccgtgatcctgctgtggtgctgcctgctgctgcctatcgtgtcctctgccgccgtgtctgtggcccctacagccgccgagaaggtgccagccgagtgccccgagctgaccagaagatgcctgctgggcgaggtgttcgagggcgacaagtacgagagctggctgcggcccctggtcaacgtgaccggcagagatggccccctgagccagctgatccggtacagacccgtgacccccgaggccgccaatagcgtgctgctggacgaggccttcctggataccctggccctgctgtacaacaaccccgaccagctgagagccctgctgaccctgctgtccagcgacaccgcccccagatggatgaccgtgatgcggggctacagcgagtgtggagatggcagccctgccgtgtacacctgcgtggacgacctgtgcagaggctacgacctgaccagactgagctacggccggtccatcttcacagagcacgtgctgggcttcgagctggtgccccccagcctgttcaacgtggtggtggccatccggaacgaggccaccagaaccaacagagccgtgcggctgcctgtgtctacagccgctgcacctgagggcatcacactgttctacggcctgtacaacgccgtgaaagagttctgcctccggcaccagctggatccccccctgctgagacacctggacaagtactacgccggcctgcccccagagctgaagcagaccagagtgaacctgcccgcccacagcagatatggccctcaggccgtggacgccagatgataagcggccgcatacagcagcaattggcaagctgcttacatagaactcgcggcgattggcatgccgccttaaaatttttattttatttttcttttcttttccgaatcggattttgtttttaatatttcaaaaaaaaaaaaaaaaaaaaaaaaaaaaaaaaaaagggtcggcatggcatctccacctcctcgcggtccgacctgggcatccgaaggaggacgcacgtccactcggatggctaagggagagccacgtttaaacacgtgatatctggcctcatgggccttcctttcactgcccgctttccagtcgggaaacctgtcgtgccagctgcattaacatggtcatagctgtttccttgcgtattgggcgctctccgcttcctcgctcactgactcgctgcgctcggtcgttcgggtaaagcctggggtgcctaatgagcaaaaggccagcaaaaggccaggaaccgtaaaaaggccgcgttgctggcgtttttccataggctccgcccccctgacgagcatcacaaaaatcgacgctcaagtcagaggtggcgaaacccgacaggactataaagataccaggcgtttccccctggaagctccctcgtgcgctctcctgttccgaccctgccgcttaccggatacctgtccgcctttctcccttcgggaagcgtggcgctttctcatagctcacgctgtaggtatctcagttcggtgtaggtcgttcgctccaagctgggctgtgtgcacgaaccccccgttcagcccgaccgctgcgccttatccggtaactatcgtcttgagtccaacccggtaagacacgacttatcgccactggcagcagccactggtaacaggattagcagagcgaggtatgtaggcggtgctacagagttcttgaagtggtggcctaactacggctacactagaagaacagtatttggtatctgcgctctgctgaagccagttaccttcggaaaaagagttggtagctcttgatccggcaaacaaaccaccgctggtagcggtggtttttttgtttgcaagcagcagattacgcgcagaaaaaaaggatctcaagaagatcctttgatcttttctacggggtctgacgctcagtggaacgaaaactcacgttaagggattttggtcatgagattatcaaaaaggatcttcacctagatccttttaaattaaaaatgaagttttaaatcaatctaaagtatatatgagtaaacttggtctgacagttattagaaaaattcatccagcagacgataaaacgcaatacgctggctatccggtgccgcaatgccatacagcaccagaaaacgatccgcccattcgccgcccagttcttccgcaatatcacgggtggccagcgcaatatcctgataacgatccgccacgcccagacggccgcaatcaataaagccgctaaaacggccattttccaccataatgttcggcaggcacgcatcaccatgggtcaccaccagatcttcgccatccggcatgctcgctttcagacgcgcaaacagctctgccggtgccaggccctgatgttcttcatccagatcatcctgatccaccaggcccgcttccatacgggtacgcgcacgttcaatacgatgtttcgcctgatgatcaaacggacaggtcgccgggtccagggtatgcagacgacgcatggcatccgccataatgctcactttttctgccggcgccagatggctagacagcagatcctgacccggcacttcgcccagcagcagccaatcacggcccgcttcggtcaccacatccagcaccgccgcacacggaacaccggtggtggccagccagctcagacgcgccgcttcatcctgcagctcgttcagcgcaccgctcagatcggttttcacaaacagcaccggacgaccctgcgcgctcagacgaaacaccgccgcatcagagcagccaatggtctgctgcgcccaatcatagccaaacagacgttccacccacgctgccgggctacccgcatgcaggccatcctgttcaatcatactcttcctttttcaatattattgaagcatttatcagggttattgtctcatgagcggatacatatttgaatgtatttagaaaaataaacaaataggggttccgcgcacatttccccgaaaagtgccacctaaattgtaagcgttaatattttgttaaaattcgcgttaaatttttgttaaatcagctcattttttaaccaataggccgaaatcggcaaaatcccttataaatcaaaagaatagaccgagatagggttgagtggccgctacagggcgctcccattcgccattcaggctgcgcaactgttgggaagggcgtttcggtgcgggcctcttcgctattacgccagctggcgaaagggggatgtgctgcaaggcgattaagttgggtaacgccagggttttcccagtcacacgcgtaatacgactcactatag

SEQ ID NO: 63 - DNA, 14721 bp, Artificial Sequence
  source: /note="Description of Artificial Sequence: Synthetic polynucleotide"
ataggcggcgcatgagagaagcccagaccaattacctacccaaaatggagaaagttcacgttgacatcgaggaagacagcccattcctcagagctttgcagcggagcttcccgcagtttgaggtagaagccaagcaggtcactgataatgaccatgctaatgccagagcgttttcgcatctggcttcaaaactgatcgaaacggaggtggacccatccgacacgatccttgacattggaagtgcgcccgcccgcagaatgtattctaagcacaagtatcattgtatctgtccgatgagatgtgcggaagatccggacagattgtataagtatgcaactaagctgaagaaaaactgtaaggaaataactgataaggaattggacaagaaaatgaaggagctcgccgccgtcatgagcgaccctgacctggaaactgagactatgtgcctccacgacgacgagtcgtgtcgctacgaagggcaagtcgctgtttaccaggatgtatacgcggttgacggaccgacaagtctctatcaccaagccaataagggagttagagtcgcctactggataggctttgacaccaccccttttatgtttaagaacttggctggagcatatccatcatactctaccaactgggccgacgaaaccgtgttaacggctcgtaacataggcctatgcagctctgacgttatggagcggtcacgtagagggatgtccattcttagaaagaagtatttgaaaccatccaacaatgttctattctctgttggctcgaccatctaccacgagaagagggacttactgaggagctggcacctgccgtctgtatttcacttacgtggcaagcaaaattacacatgtcggtgtgagactatagttagttgcgacgggtacgtcgttaaaagaatagctatcagtccaggcctgtatgggaagccttcaggctatgctgctacgatgcaccgcgagggattcttgtgctgcaaagtgacagacacattgaacggggagagggtctcttttcccgtgtgcacgtatgtgccagctacattgtgtgaccaaatgactggcatactggcaacagatgtcagtgcggacgacgcgcaaaaactgctggttgggctcaaccagcgtatagtcgtcaacggtcgcacccagagaaacaccaataccatgaaaaattaccttttgcccgtagtggcccaggcatttgctaggtgggcaaaggaatataaggaagatcaagaagatgaaaggccactaggactacgagatagacagttagtcatggggtgttgttgggcttttagaaggcacaagataacatctatttataagcgcccggatacccaaaccatcatcaaagtgaacagcgatttccactcattcgtgctgcccaggataggcagtaacacattggagatcgggctgagaacaagaatcaggaaaatgttagaggagcacaaggagccgtcacctctcattaccgccgaggacgtacaagaagctaagtgcgcagccgatgaggctaaggaggtgcgtgaagccgaggagttgcgcgcagctctaccacctttggcagctgatgttgaggagcccactctggaagccgatgtcgacttgatgttacaagaggctggggccggctcagtggagacacctcgtggcttgataaaggttaccagctacgatggcgaggacaagatcggctcttacgctgtgctttctccgcaggctgtactcaagagtgaaaaattatcttgcatccaccctctcgctgaacaagtcatagtgataacacactctggccgaaaagggcgttatgccgtggaaccataccatggtaaagtagtggtgccagagggacatgcaatacccgtccaggactttcaagctctgagtgaaagtgccaccattgtgtacaacgaacgtgagttcgtaaacaggtacctgcaccatattgccacacatggaggagcgctgaacactgatgaagaatattacaaaactgtcaagcccagcgagcacgacggcgaatacctgtacgacatcgacaggaaacagtgcgtcaagaaagaactagtcactgggctagggctcacaggcgagctggtggatcctcccttccatgaattcgcctacgagagtctgagaacacgaccagccgctccttaccaagtaccaaccataggggtgtatggcgtgccaggatcaggcaagtctggcatcattaaaagcgcagtcaccaaaaaagatctagtggtgagcgccaagaaagaaaactgtgcagaaattataagggacgtcaagaaaatgaaagggctggacgtcaatgccagaactgtggactcagtgctcttgaatggatgcaaacaccccgtagagaccctgtatattgacgaagcttttgcttgtcatgcaggtactctcagagcgctcatagccattataagacctaaaaaggcagtgctctgcggggatcccaaacagtgcggtttttttaacatgatgtgcctgaaagtgcattttaaccacgagatttgcacacaagtcttccacaaaagcatctctcgccgttgcactaaatctgtgacttcggtcgtctcaaccttgttttacgacaaaaaaatgagaacgacgaatccgaaagagactaagattgtgattgacactaccggcagtaccaaacctaagcaggacgatctcattctcacttgtttcagagggtgggtgaagcagttgcaaatagattacaaaggcaacgaaataatgacggcagctgcctctcaagggctgacccgtaaaggtgtgtatgccgttcggtacaaggtgaatgaaaatcctctgtacgcacccacctcagaacatgtgaacgtcctactgacccgcacggaggaccgcatcgtgtggaaaacactagccggcgacccatggataaaaacactgactgccaagtaccctgggaatttcactgccacgatagaggagtggcaagcagagcatgatgccatcatgaggcacatcttggagagaccggaccctaccgacgtcttccagaataaggcaaacgtgtgttgggccaaggctttagtgccggtgctgaagaccgctggcatagacatgaccactgaacaatggaacactgtggattattttgaaacggacaaagctcactcagcagagatagtattgaaccaactatgcgtgaggttctttggactcgatctggactccggtctattttctgcacccactgttccgttatccattaggaataatcactgggataactccccgtcgcctaacatgtacgggctgaataaagaagtggtccgtcagctctctcgcaggtacccacaactgcctcgggcagttgccactggaagagtctatgacatgaacactggtacactgcgcaattatgatccgcgcataaacctagtacctgtaaacagaagactgcctcatgctttagtcctccaccataatgaacacccacagagtgacttttcttcattcgtcagcaaattgaagggcagaactgtcctggtggtcggggaaaagttgtccgtcccaggcaaaatggttgactggttgtcagaccggcctgaggctaccttcagagctcggctggatttaggcatcccaggtgatgtgcccaaatatgacataatatttgttaatgtgaggaccccatataaataccatcactatcagcagtgtgaagaccatgccattaagcttagcatgttgaccaagaaagcttgtctgcatctgaatcccggcggaacctgtgtcagcataggttatggttacgctgacagggccagcgaaagcatcattggtgctatagcgcggcagttcaagttttcccgggtatgcaaaccgaaatcctcacttgaagagacggaagttctgtttgtattcattgggtacgatcgcaaggcccgtacgcacaatccttacaagctttcatcaaccttgaccaacatttatacaggttccagactccacgaagccggatgtgcaccctcatatcatgtggtgcgaggggatattgccacggccaccgaaggagtgattataaatgctgctaacagcaaaggacaacctggcggaggggtgtgcggagcgctgtataagaaattcccggaaagcttcgatttacagccgatcgaagtaggaaaagcgcgactggtcaaaggtgcagctaaacatatcattcatgccgtaggaccaaacttcaacaaagtttcggaggttgaaggtgacaaacagttggcagaggcttatgagtccatcgctaagattgtcaacgataacaattacaagtcagtagcgattccactgttgtccaccggcatcttttccgggaacaaagatcgactaacccaatcattgaaccatttgctgacagctttagacaccactgatgcagatgtagccatatactgcagggacaagaaatgggaaatgactctcaaggaagcagtggctaggagagaagcagtggaggagatatgcatatccgacgactcttcagtgacagaacctgatgcagagctggtgagggtgcatccgaagagttctttggctggaaggaagggctacagcacaagcgatggcaaaactttctcatatttggaagggaccaagtttcaccaggcggccaaggatatagcagaaattaatgccatgtggcccgttgcaacggaggccaatgagcaggtatgcatgtatatcctcggagaaagcatgagcagtattaggtcgaaatgccccgtcgaagagtcggaagcctccacaccacctagcacgctgccttgcttgtgcatccatgccatgactccagaaagagtacagcgcctaaaagcctcacgtccagaacaaattactgtgtgctcatcctttccattgccgaagtatagaatcactggtgtgcagaagatccaatgctcccagcctatattgttctcaccgaaagtgcctgcgtatattcatccaaggaagtatctcgtggaaacaccaccggtagacgagactccggagccatcggcagagaaccaatccacagaggggacacctgaacaaccaccacttataaccgaggatgagaccaggactagaacgcctgagccgatcatcatcgaagaggaagaagaggatagcataagtttgctgtcagatggcccgacccaccaggtgctgcaagtcgaggcagacattcacgggccgccctctgtatctagctcatcctggtccattcctcatgcatccgactttgatgtggacagtttatccatacttgacaccctggagggagctagcgtgaccagcggggcaacgtcagccgagactaactcttacttcgcaaagagtatggagtttctggcgcgaccggtgcctgcgcctcgaacagtattcaggaaccctccacatcccgctccgcgcacaagaacaccgtcacttgcacccagcagggcctgctcgagaaccagcctagtttccaccccgccaggcgtgaatagggtgatcactagagaggagctcgaggcgcttaccccgtcacgcactcctagcaggtcggtctcgagaaccagcctggtctccaacccgccaggcgtaaatagggtgattacaagagaggagtttgaggcgttcgtagcacaacaacaatgacggtttgatgcgggtgcatacatcttttcctccgacaccggtcaagggcatttacaacaaaaatcagtaaggcaaacggtgctatccgaagtggtgttggagaggaccgaattggagatttcgtatgccccgcgcctcgaccaagaaaaagaagaattactacgcaagaaattacagttaaatcccacacctgctaacagaagcagataccagtccaggaaggtggagaacatgaaagccataacagctagacgtattctgcaaggcctagggcattatttgaaggcagaaggaaaagtggagtgctaccgaaccctgcatcctgttcctttgtattcatctagtgtgaaccgtgccttttcaagccccaaggtcgcagtggaagcctgtaacgccatgttgaaagagaactttccgactgtggcttcttactgtattattccagagtacgatgcctatttggacatggttgacggagcttcatgctgcttagacactgccagtttttgccctgcaaagctgcgcagctttccaaagaaacactcctatttggaacccacaatacgatcggcagtgccttcagcgatccagaacacgctccagaacgtcctggcagctgccacaaaaagaaattgcaatgtcacgcaaatgagagaattgcccgtattggattcggcggcctttaatgtggaatgcttcaagaaatatgcgtgtaataatgaatattgggaaacgtttaaagaaaaccccatcaggcttactgaagaaaacgtggtaaattacattaccaaattaaaaggaccaaaagctgctgctctttttgcgaagacacataatttgaatatgttgcaggacataccaatggacaggtttgtaatggacttaaagagagacgtgaaagtgactccaggaacaaaacatactgaagaacggcccaaggtacaggtgatccaggctgccgatccgctagcaacagcgtatctgtgcggaatccaccgagagctggttaggagattaaatgcggtcctgcttccgaacattcatacactgtttgatatgtcggctgaagactttgacgctattatagccgagcacttccagcctggggattgtgttctggaaactgacatcgcgtcgtttgataaaagtgaggacgacgccatggctctgaccgcgttaatgattctggaagacttaggtgtggacgcagagctgttgacgctgattgaggcggctttcggcgaaatttcatcaatacatttgcccactaaaactaaatttaaattcggagccatgatgaaatctggaatgttcctcacactgtttgtgaacacagtcattaacattgtaatcgcaagcagagtgttgagagaacggctaaccggatcaccatgtgcagcattcattggagatgacaatatcgtgaaaggagtcaaatcggacaaattaatggcagacaggtgcgccacctggttgaatatggaagtcaagattatagatgctgtggtgggcgagaaagcgccttatttctgtggagggtttattttgtgtgactccgtgaccggcacagcgtgccgtgtggcagaccccctaaaaaggctgtttaagcttggcaaacctctggcagcagacgatgaacatgatgatgacaggagaagggcattgcatgaagagtcaacacgctggaaccgagtgggtattctttcagagctgtgcaaggcagtagaatcaaggtatgaaaccgtaggaacttccatcatagttatggccatgactactctagctagcagtgttaaatcattcagctacctgagaggggcccctataactctctacggctaacctgaatggactacgacatagtctagtccgccaagctattccagaagtagtgaggaggcttttttggaggcctaggcttttgcaaaaagcttgtatatccattttcggatctgatcaagagacaggatgaggatcgtttcgcatgattgaataagatggattgcacgtaggttctccggccgcttgggtggagaggctattcggctatgactgggcacaactgacaatcggctgctctgatgccgccgtgatccggttgtcagcgcaggggcgcccggttctttttgtcaagaccgacctgtccggtgccctgaatgaactgaaggacgaggcagcgcggctatcgtggctggccacgacgggcgttccttgcgcagtctagactggcgcgccaaacctgcaggttaaaacagctgtgggttgttcccacccacagggcccactgggcgctagcactctgattttacgaaatccttgtgcgcctgttttatatcccttccctaattcgaaacgtagaagcaatgcgcaccactgatcaatagtaggcgtaacgcgccagttacgtcatgatcaagcatatctgttcccccggactgagtatcaatagactgcttacgcggttgaaggagaaaacgttcgttatccggctaactacttcgagaagcccagtaacaccatggaagctgcagggtgtttcgctcagcacttcccccgtgtagatcaggtcgatgagccactgcaatccccacaggtgactgtggcagtggctgcgttggcggcctgcctatggggagacccataggacgctctaatgtggacatggtgcgaagagcctattgagctagttagtagtcctccggcccctgaatgcggctaatcctaactgcggagcacatgccttcaacccagagggtagtgtgtcgtaatgggcaactctgcagcggaaccgactactttgggtgtccgtgtttctttttattcttatattggctgcttatggtgacaattacagaattgttaccatatagctattggattggccatccggtgtgtaatagagctgttatatacctatttgttggctttgtaccactaactttaaaatctataactaccctcaactttatattaaccctcaatacagttgaacatgaggcctggcctgccctcctacctgatcatcctggccgtgtgcctgttcagccacctgctgtccagcagatacggcgccgaggccgtgagcgagcccctggacaaggctttccacctgctgctgaacacctacggcagacccatccggtttctgcgggagaacaccacccagtgcacctacaacagcagcctgcggaacagcaccgtcgtgagagagaacgccatcagcttcaactttttccagagctacaaccagtactacgtgttccacatgcccagatgcctgtttgccggccctctggccgagcagttcctgaaccaggtggacctgaccgagacactggaaagataccagcagcggctgaatacctacgccctggtgtccaaggacctggccagctaccggtcctttagccagcagctcaaggctcaggatagcctcggcgagcagcctaccaccgtgccccctcccatcgacctgagcatcccccacgtgtggatgcctccccagaccacccctcacggctggaccgagagccacaccacctccggcctgcacagaccccacttcaaccagacctgcatcctgttcgacggccacgacctgctgtttagcaccgtgaccccctgcctgcaccagggcttctacctgatcgacgagctgagatacgtgaagatcaccctgaccgaggatttcttcgtggtcaccgtgtccatcgacgacgacacccccatgctgctgatcttcggccacctgcccagagtgctgttcaaggccccctaccagcgggacaacttcatcctgcggcagaccgagaagcacgagctgctggtgctggtcaagaaggaccagctgaaccggcactcctacctgaaggaccccgacttcctggacgccgccctggacttcaactacctggacctgagcgccctgctgagaaacagcttccacagatacgccgtggacgtgctgaagtccggacggtgccagatgctcgatcggcggaccgtggagatggccttcgcctatgccctcgccctgttcgccgctgccagacaggaagaggctggcgcccaggtgtcagtgcccagagccctggatagacaggccgccctgctgcagatccaggaattcatgatcacctgcctgagccagaccccccctagaaccaccctgctgctgtaccccacagccgtggatctggccaagagggccctgtggacccccaaccagatcaccgacatcacaagcctcgtgcggctcgtgtacatcctgagcaagcagaaccagcagcacctgatcccccagtgggccctgagacagatcgccgacttcgccctgaagctgcacaagacccatctggccagctttctgagcgccttcgccaggcaggaactgtacctgatgggcagcctggtccacagcatgctggtgcataccaccgagcggcgggagatcttcatcgtggagacaggcctgtgtagcctggccgagctgtcccactttacccagctgctggcccaccctcaccacgagtacctgagcgacctgtacaccccctgcagcagcagcggcagacgggaccacagcctggaacggctgaccagactgttccccgatgccaccgtgcctgctacagtgcctgccgccctgtccatcctgtccaccatgcagcccagcaccctggaaaccttccccgacctgttctgcctgcccctgggcgagagctttagcgccctgaccgtgtccgagcacgtgtcctacatcgtgaccaatcagtacctgatcaagggcatcagctaccccgtgtccaccacagtcgtgggccagagcctgatcatcacccagaccgacagccagaccaagtgcgagctgacccggaacatgcacaccacacacagcatcaccgtggccctgaacatcagcctggaaaactgcgctttctgtcagtctgccctgctggaatacgacgatacccagggcgtgatcaacatcatgtacatgcacgacagcgacgacgtgctgttcgccctggacccctacaacgaggtggtggtgtccagcccccggacccactacctgatgctgctgaagaacggcaccgtgctggaagtgaccgacgtggtggtggacgccaccgactgataacgccggcgcccccccctaacgttactggccgaagccgcttggaataaggccggtgtgcgtttgtctatatgttattttccaccatattgccgtcttttggcaatgtgagggcccggaaacctggccctgtcttcttgacgagcattcctaggggtctttcccctctcgccaaaggaatgcaaggtctgttgaatgtcgtgaaggaagcagttcctctggaagcttcttgaagacaaacaacgtctgtagcgaccctttgcaggcagcggaaccccccacctggcgacaggtgcctctgcggccaaaagccacgtgtataagatacacctgcaaaggcggcacaaccccagtgccacgttgtgagttggatagttgtggaaagagtcaaatggctctcctcaagcgtattcaacaaggggctgaaggatgcccagaaggtaccccattgtatgggatctgatctggggcctcggtgcacatgctttacatgtgtttagtcgaggttaaaaaaacgtctaggccccccgaaccacggggacgtggttttcctttgaaaaacacgataataatatgtgcagaaggcccgactgcggcttcagcttcagccctggacccgtgatcctgctgtggtgctgcctgctgctgcctatcgtgtcctctgccgccgtgtctgtggcccctacagccgccgagaaggtgccagccgagtgccccgagctgaccagaagatgcctgctgggcgaggtgttcgagggcgacaagtacgagagctggctgcggcccctggtcaacgtgaccggcagagatggccccctgagccagctgatccggtacagacccgtgacccccgaggccgccaatagcgtgctgctggacgaggccttcctggataccctggccctgctgtacaacaaccccgaccagctgagagccctgctgaccctgctgtccagcgacaccgcccccagatggatgaccgtgatgcggggctacagcgagtgtggagatggcagccctgccgtgtacacctgcgtggacgacctgtgcagaggctacgacctgaccagactgagctacggccggtccatcttcacagagcacgtgctgggcttcgagctggtgccccccagcctgttcaacgtggtggtggccatccggaacgaggccaccagaaccaacagagccgtgcggctgcctgtgtctacagccgctgcacctgagggcatcacactgttctacggcctgtacaacgccgtgaaagagttctgcctccggcaccagctggatccccccctgctgagacacctggacaagtactacgccggcctgcccccagagctgaagcagaccagagtgaacctgcccgcccacagcagatatggccctcaggccgtggacgccagatgataagcggccgcatacagcagcaattggcaagctgcttacatagaactcgcggcgattggcatgccgccttaaaatttttattttatttttcttttcttttccgaatcggattttgtttttaatatttcaaaaaaaaaaaaaaaaaaaaaaaaaaaaaaaaaaagggtcggcatggcatctccacctcctcgcggtccgacctgggcatccgaaggaggacgcacgtccactcggatggctaagggagagccacgtttaaacacgtgatatctggcctcatgggccttcctttcactgcccgctttccagtcgggaaacctgtcgtgccagctgcattaacatggtcatagctgtttccttgcgtattgggcgctctccgcttcctcgctcactgactcgctgcgctcggtcgttcgggtaaagcctggggtgcctaatgagcaaaaggccagcaaaaggccaggaaccgtaaaaaggccgcgttgctggcgtttttccataggctccgcccccctgacgagcatcacaaaaatcgacgctcaagtcagaggtggcgaaacccgacaggactataaagataccaggcgtttccccctggaagctccctcgtgcgctctcctgttccgaccctgccgcttaccggatacctgtccgcctttctcccttcgggaagcgtggcgctttctcatagctcacgctgtaggtatctcagttcggtgtaggtcgttcgctccaagctgggctgtgtgcacgaaccccccgttcagcccgaccgctgcgccttatccggtaactatcgtcttgagtccaacccggtaagacacgacttatcgccactggcagcagccactggtaacaggattagcagagcgaggtatgtaggcggtgctacagagttcttgaagtggtggcctaactacggctacactagaagaacagtatttggtatctgcgctctgctgaagccagttaccttcggaaaaagagttggtagctcttgatccggcaaacaaaccaccgctggtagcggtggtttttttgtttgcaagcagcagattacgcgcagaaaaaaaggatctcaagaagatcctttgatcttttctacggggtctgacgctcagtggaacgaaaactcacgttaagggattttggtcatgagattatcaaaaaggatcttcacctagatccttttaaattaaaaatgaagttttaaatcaatctaaagtatatatgagtaaacttggtctgacagttattagaaaaattcatccagcagacgataaaacgcaatacgctggctatccggtgccgcaatgccatacagcaccagaaaacgatccgcccattcgccgcccagttcttccgcaatatcacgggtggccagcgcaatatcctgataacgatccgccacgcccagacggccgcaatcaataaagccgctaaaacggccattttccaccataatgttcggcaggcacgcatcaccatgggtcaccaccagatcttcgccatccggcatgctcgctttcagacgcgcaaacagctctgccggtgccaggccctgatgttcttcatccagatcatcctgatccaccaggcccgcttccatacgggtacgcgcacgttcaatacgatgtttcgcctgatgatcaaacggacaggtcgccgggtccagggtatgcagacgacgcatggcatccgccataatgctcactttttctgccggcgccagatggctagacagcagatcctgacccggcacttcgcccagcagcagccaatcacggcccgcttcggtcaccacatccagcaccgccgcacacggaacaccggtggtggccagccagctcagacgcgccgcttcatcctgcagctcgttcagcgcaccgctcagatcggttttcacaaacagcaccggacgaccctgcgcgctcagacgaaacaccgccgcatcagagcagccaatggtctgctgcgcccaatcatagccaaacagacgttccacccacgctgccgggctacccgcatgcaggccatcctgttcaatcatactcttcctttttcaatattattgaagcatttatcagggttattgtctcatgagcggatacatatttgaatgtatttagaaaaataaacaaataggggttccgcgcacatttccccgaaaagtgccacctaaattgtaagcgttaatattttgttaaaattcgcgttaaatttttgttaaatcagctcattttttaaccaataggccgaaatcggcaaaatcccttataaatcaaaagaatagaccgagatagggttgagtggccgctacagggcgctcccattcgccattcaggctgcgcaactgttgggaagggcgtttcggtgcgggcctcttcgctattacgccagctggcgaaagggggatgtgctgcaaggcgattaagttgggtaacgccagggttttcccagtcacacgcgtaatacgactcactatag

SEQ ID NO: 64 - DNA, 14721 bp, Artificial Sequence
  source: /note="Description of Artificial Sequence: Synthetic polynucleotide"
ataggcggcgcatgagagaagcccagaccaattacctacccaaaatggagaaagttcacgttgacatcgaggaagacagcccattcctcagagctttgcagcggagcttcccgcagtttgaggtagaagccaagcaggtcactgataatgaccatgctaatgccagagcgttttcgcatctggcttcaaaactgatcgaaacggaggtggacccatccgacacgatccttgacattggaagtgcgcccgcccgcagaatgtattctaagcacaagtatcattgtatctgtccgatgagatgtgcggaagatccggacagattgtataagtatgcaactaagctgaagaaaaactgtaaggaaataactgataaggaattggacaagaaaatgaaggagctcgccgccgtcatgagcgaccctgacctggaaactgagactatgtgcctccacgacgacgagtcgtgtcgctacgaagggcaagtcgctgtttaccaggatgtatacgcggttgacggaccgacaagtctctatcaccaagccaataagggagttagagtcgcctactggataggctttgacaccaccccttttatgtttaagaacttggctggagcatatccatcatactctaccaactgggccgacgaaaccgtgttaacggctcgtaacataggcctatgcagctctgacgttatggagcggtcacgtagagggatgtccattcttagaaagaagtatttgaaaccatccaacaatgttctattctctgttggctcgaccatctaccacgagaagagggacttactgaggagctggcacctgccgtctgtatttcacttacgtggcaagcaaaattacacatgtcggtgtgagactatagttagttgcgacgggtacgtcgttaaaagaatagctatcagtccaggcctgtatgggaagccttcaggctatgctgctacgatgcaccgcgagggattcttgtgctgcaaagtgacagacacattgaacggggagagggtctcttttcccgtgtgcacgtatgtgccagctacattgtgtgaccaaatgactggcatactggcaacagatgtcagtgcggacgacgcgcaaaaactgctggttgggctcaaccagcgtatagtcgtcaacggtcgcacccagagaaacaccaataccatgaaaaattaccttttgcccgtagtggcccaggcatttgctaggtgggcaaaggaatataaggaagatcaagaagatgaaaggccactaggactacgagatagacagttagtcatggggtgttgttgggcttttagaaggcacaagataacatctatttataagcgcccggatacccaaaccatcatcaaagtgaacagcgatttccactcattcgtgctgcccaggataggcagtaacacattggagatcgggctgagaacaagaatcaggaaaatgttagaggagcacaaggagccgtcacctctcattaccgccgaggacgtacaagaagctaagtgcgcagccgatgaggctaaggaggtgcgtgaagccgaggagttgcgcgcagctctaccacctttggcagctgatgttgaggagcccactctggaagccgatgtcgacttgatgttacaagaggctggggccggctcagtggagacacctcgtggcttgataaaggttaccagctacgatggcgaggacaagatcggctcttacgctgtgctttctccgcaggctgtactcaagagtgaaaaattatcttgcatccaccctctcgctgaacaagtcatagtgataacacactctggccgaaaagggcgttatgccgtggaaccataccatggtaaagtagtggtgccagagggacatgcaatacccgtccaggactttcaagctctgagtgaaagtgccaccattgtgtacaacgaacgtgagttcgtaaacaggtacctgcaccatattgccacacatggaggagcgctgaacactgatgaagaatattacaaaactgtcaagcccagcgagcacgacggcgaatacctgtacgacatcgacaggaaacagtgcgtcaagaaagaactagtcactgggctagggctcacaggcgagctggtggatcctcccttccatgaattcgcctacgagagtctgagaacacgaccagccgctccttaccaagtaccaaccataggggtgtatggcgtgccaggatcaggcaagtctggcatcattaaaagcgcagtcaccaaaaaagatctagtggtgagcgccaagaaagaaaactgtgcagaaattataagggacgtcaagaaaatgaaagggctggacgtcaatgccagaactgtggactcagtgctcttgaatggatgcaaacaccccgtagagaccctgtatattgacgaagcttttgcttgtcatgcaggtactctcagagcgctcatagccattataagacctaaaaaggcagtgctctgcggggatcccaaacagtgcggtttttttaacatgatgtgcctgaaagtgcattttaaccacgagatttgcacacaagtcttccacaaaagcatctctcgccgttgcactaaatctgtgacttcggtcgtctcaaccttgttttacgacaaaaaaatgagaacgacgaatccgaaagagactaagattgtgattgacactaccggcagtaccaaacctaagcaggacgatctcattctcacttgtttcagagggtgggtgaagcagttgcaaatagattacaaaggcaacgaaataatgacggcagctgcctctcaagggctgacccgtaaaggtgtgtatgccgttcggtacaaggtgaatgaaaatcctctgtacgcacccacctcagaacatgtgaacgtcctactgacccgcacggaggaccgcatcgtgtggaaaacactagccggcgacccatggataaaaacactgactgccaagtaccctgggaatttcactgccacgatagaggagtggcaagcagagcatgatgccatcatgaggcacatcttggagagaccggaccctaccgacgtcttccagaataaggcaaacgtgtgttgggccaaggctttagtgccggtgctgaagaccgctggcatagacatgaccactgaacaatggaacactgtggattattttgaaacggacaaagctcactcagcagagatagtattgaaccaactatgcgtgaggttctttggactcgatctggactccggtctattttctgcacccactgttccgttatccattaggaataatcactgggataactccccgtcgcctaacatgtacgggctgaataaagaagtggtccgtcagctctctcgcaggtacccacaactgcctcgggcagttgccactggaagagtctatgacatgaacactggtacactgcgcaattatgatccgcgcataaacctagtacctgtaaacagaagactgcctcatgctttagtcctccaccataatgaacacccacagagtgacttttcttcattcgtcagcaaattgaagggcagaactgtcctggtggtcggggaaaagttgtccgtcccaggcaaaatggttgactggttgtcagaccggcctgaggctaccttcagagctcggctggatttaggcatcccaggtgatgtgcccaaatatgacataatatttgttaatgtgaggaccccatataaataccatcactatcagcagtgtgaagaccatgccattaagcttagcatgttgaccaagaaagcttgtctgcatctgaatcccggcggaacctgtgtcagcataggttatggttacgctgacagggccagcgaaagcatcattggtgctatagcgcggcagttcaagttttcccgggtatgcaaaccgaaatcctcacttgaagagacggaagttctgtttgtattcattgggtacgatcgcaaggcccgtacgcacaatccttacaagctttcatcaaccttgaccaacatttatacaggttccagactccacgaagccggatgtgcaccctcatatcatgtggtgcgaggggatattgccacggccaccgaaggagtgattataaatgctgctaacagcaaaggacaacctggcggaggggtgtgcggagcgctgtataagaaattcccggaaagcttcgatttacagccgatcgaagtaggaaaagcgcgactggtcaaaggtgcagctaaacatatcattcatgccgtaggaccaaacttcaacaaagtttcggaggttgaaggtgacaaacagttggcagaggcttatgagtccatcgctaagattgtcaacgataacaattacaagtcagtagcgattccactgttgtccaccggcatcttttccgggaacaaagatcgactaacccaatcattgaaccatttgctgacagctttagacaccactgatgcagatgtagccatatactgcagggacaagaaatgggaaatgactctcaaggaagcagtggctaggagagaagcagtggaggagatatgcatatccgacgactcttcagtgacagaacctgatgcagagctggtgagggtgcatccgaagagttctttggctggaaggaagggctacagcacaagcgatggcaaaactttctcatatttggaagggaccaagtttcaccaggcggccaaggatatagcagaaattaatgccatgtggcccgttgcaacggaggccaatgagcaggtatgcatgtatatcctcggagaaagcatgagcagtattaggtcgaaatgccccgtcgaagagtcggaagcctccacaccacctagcacgctgccttgcttgtgcatccatgccatgactccagaaagagtacagcgcctaaaagcctcacgtccagaacaaattactgtgtgctcatcctttccattgccgaagtatagaatcactggtgtgcagaagatccaatgctcccagcctatattgttctcaccgaaagtgcctgcgtatattcatccaaggaagtatctcgtggaaacaccaccggtagacgagactccggagccatcggcagagaaccaatccacagaggggacacctgaacaaccaccacttataaccgaggatgagaccaggactagaacgcctgagccgatcatcatcgaagaggaagaagaggatagcataagtttgctgtcagatggcccgacccaccaggtgctgcaagtcgaggcagacattcacgggccgccctctgtatctagctcatcctggtccattcctcatgcatccgactttgatgtggacagtttatccatacttgacaccctggagggagctagcgtgaccagcggggcaacgtcagccgagactaactcttacttcgcaaagagtatggagtttctggcgcgaccggtgcctgcgcctcgaacagtattcaggaaccctccacatcccgctccgcgcacaagaacaccgtcacttgcacccagcagggcctgctcgagaaccagcctagtttccaccccgccaggcgtgaatagggtgatcactagagaggagctcgaggcgcttaccccgtcacgcactcctagcaggtcggtctcgagaaccagcctggtctccaacccgccaggcgtaaatagggtgattacaagagaggagtttgaggcgttcgtagcacaacaacaatgacggtttgatgcgggtgcatacatcttttcctccgacaccggtcaagggcatttacaacaaaaatcagtaaggcaaacggtgctatccgaagtggtgttggagaggaccgaattggagatttcgtatgccccgcgcctcgaccaagaaaaagaagaattactacgcaagaaattacagttaaatcccacacctgctaacagaagcagataccagtccaggaaggtggagaacatgaaagccataacagctagacgtattctgcaaggcctagggcattatttgaaggcagaaggaaaagtggagtgctaccgaaccctgcatcctgttcctttgtattcatctagtgtgaaccgtgccttttcaagccccaaggtcgcagtggaagcctgtaacgccatgttgaaagagaactttccgactgtggcttcttactgtattattccagagtacgatgcctatttggacatggttgacggagcttcatgctgcttagacactgccagtttttgccctgcaaagctgcgcagctttccaaagaaacactcctatttggaacccacaatacgatcggcagtgccttcagcgatccagaacacgctccagaacgtcctggcagctgccacaaaaagaaattgcaatgtcacgcaaatgagagaattgcccgtattggattcggcggcctttaatgtggaatgcttcaagaaatatgcgtgtaataatgaatattgggaaacgtttaaagaaaaccccatcaggcttactgaagaaaacgtggtaaattacattaccaaattaaaaggaccaaaagctgctgctctttttgcgaagacacataatttgaatatgttgcaggacataccaatggacaggtttgtaatggacttaaagagagacgtgaaagtgactccaggaacaaaacatactgaagaacggcccaaggtacaggtgatccaggctgccgatccgctagcaacagcgtatctgtgcggaatccaccgagagctggttaggagattaaatgcggtcctgcttccgaacattcatacactgtttgatatgtcggctgaagactttgacgctattatagccgagcacttccagcctggggattgtgttctggaaactgacatcgcgtcgtttgataaaagtgaggacgacgccatggctctgaccgcgttaatgattctggaagacttaggtgtggacgcagagctgttgacgctgattgaggcggctttcggcgaaatttcatcaatacatttgcccactaaaactaaatttaaattcggagccatgatgaaatctggaatgttcctcacactgtttgtgaacacagtcattaacattgtaatcgcaagcagagtgttgagagaacggctaaccggatcaccatgtgcagcattcattggagatgacaatatcgtgaaaggagtcaaatcggacaaattaatggcagacaggtgcgccacctggttgaatatggaagtcaagattatagatgctgtggtgggcgagaaagcgccttatttctgtggagggtttattttgtgtgactccgtgaccggcacagcgtgccgtgtggcagaccccctaaaaaggctgtttaagcttggcaaacctctggcagcagacgatgaacatgatgatgacaggagaagggcattgcatgaagagtcaacacgctggaaccgagtgggtattctttcagagctgtgcaaggcagtagaatcaaggtatgaaaccgtaggaacttccatcatagttatggccatgactactctagctagcagtgttaaatcattcagctacctgagaggggcccctataactctctacggctaacctgaatggactacgacatagtctagtccgccaagctattccagaagtagtgaggaggcttttttggaggcctaggcttttgcaaaaagcttgtatatccattttcggatctgatcaagagacaggatgaggatcgtttcgcatgattgaataagatggattgcacgtaggttctccggccgcttgggtggagaggctattcggctatgactgggcacaactgacaatcggctgctctgatgccgccgtgatccggttgtcagcgcaggggcgcccggttctttttgtcaagaccgacctgtccggtgccctgaatgaactgaaggacgaggcagcgcggctatcgtggctggccacgacgggcgttccttgcgcagtctagactggcgcgccaaacctgcaggttaaaacagctgtgggttgttcccacccacagggcccactgggcgctagcactctgattttacgaaatccttgtgcgcctgttttatatcccttccctaattcgaaacgtagaagcaatgcgcaccactgatcaatagtaggcgtaacgcgccagttacgtcatgatcaagcatatctgttcccccggactgagtatcaatagactgcttacgcggttgaaggagaaaacgttcgttatccggctaactacttcgagaagcccagtaacaccatggaagctgcagggtgtttcgctcagcacttcccccgtgtagatcaggtcgatgagccactgcaatccccacaggtgactgtggcagtggctgcgttggcggcctgcctatggggagacccataggacgctctaatgtggacatggtgcgaagagcctattgagctagttagtagtcctccggcccctgaatgcggctaatcctaactgcggagcacatgccttcaacccagagggtagtgtgtcgtaatgggcaactctgcagcggaaccgactactttgggtgtccgtgtttctttttattcttatattggctgcttatggtgacaattacagaattgttaccatatagctattggattggccatccggtgtgtaatagagctgttatatacctatttgttggctttgtaccactaactttaaaatctataactaccctcaactttatattaaccctcaatacagttgaacatgtgcagaaggcccgactgcggcttcagcttcagccctggacccgtgatcctgctgtggtgctgcctgctgctgcctatcgtgtcctctgccgccgtgtctgtggcccctacagccgccgagaaggtgccagccgagtgccccgagctgaccagaagatgcctgctgggcgaggtgttcgagggcgacaagtacgagagctggctgcggcccctggtcaacgtgaccggcagagatggccccctgagccagctgatccggtacagacccgtgacccccgaggccgccaatagcgtgctgctggacgaggccttcctggataccctggccctgctgtacaacaaccccgaccagctgagagccctgctgaccctgctgtccagcgacaccgcccccagatggatgaccgtgatgcggggctacagcgagtgtggagatggcagccctgccgtgtacacctgcgtggacgacctgtgcagaggctacgacctgaccagactgagctacggccggtccatcttcacagagcacgtgctgggcttcgagctggtgccccccagcctgttcaacgtggtggtggccatccggaacgaggccaccagaaccaacagagccgtgcggctgcctgtgtctacagccgctgcacctgagggcatcacactgttctacggcctgtacaacgccgtgaaagagttctgcctccggcaccagctggatccccccctgctgagacacctggacaagtactacgccggcctgcccccagagctgaagcagaccagagtgaacctgcccgcccacagcagatatggccctcaggccgtggacgccagatgataacgccggcgcccccccctaacgttactggccgaagccgcttggaataaggccggtgtgcgtttgtctatatgttattttccaccatattgccgtcttttggcaatgtgagggcccggaaacctggccctgtcttcttgacgagcattcctaggggtctttcccctctcgccaaaggaatgcaaggtctgttgaatgtcgtgaaggaagcagttcctctggaagcttcttgaagacaaacaacgtctgtagcgaccctttgcaggcagcggaaccccccacctggcgacaggtgcctctgcggccaaaagccacgtgtataagatacacctgcaaaggcggcacaaccccagtgccacgttgtgagttggatagttgtggaaagagtcaaatggctctcctcaagcgtattcaacaaggggctgaaggatgcccagaaggtaccccattgtatgggatctgatctggggcctcggtgcacatgctttacatgtgtttagtcgaggttaaaaaaacgtctaggccccccgaaccacggggacgtggttttcctttgaaaaacacgataataatatgaggcctggcctgccctcctacctgatcatcctggccgtgtgcctgttcagccacctgctgtccagcagatacggcgccgaggccgtgagcgagcccctggacaaggctttccacctgctgctgaacacctacggcagacccatccggtttctgcgggagaacaccacccagtgcacctacaacagcagcctgcggaacagcaccgtcgtgagagagaacgccatcagcttcaactttttccagagctacaaccagtactacgtgttccacatgcccagatgcctgtttgccggccctctggccgagcagttcctgaaccaggtggacctgaccgagacactggaaagataccagcagcggctgaatacctacgccctggtgtccaaggacctggccagctaccggtcctttagccagcagctcaaggctcaggatagcctcggcgagcagcctaccaccgtgccccctcccatcgacctgagcatcccccacgtgtggatgcctccccagaccacccctcacggctggaccgagagccacaccacctccggcctgcacagaccccacttcaaccagacctgcatcctgttcgacggccacgacctgctgtttagcaccgtgaccccctgcctgcaccagggcttctacctgatcgacgagctgagatacgtgaagatcaccctgaccgaggatttcttcgtggtcaccgtgtccatcgacgacgacacccccatgctgctgatcttcggccacctgcccagagtgctgttcaaggccccctaccagcgggacaacttcatcctgcggcagaccgagaagcacgagctgctggtgctggtcaagaaggaccagctgaaccggcactcctacctgaaggaccccgacttcctggacgccgccctggacttcaactacctggacctgagcgccctgctgagaaacagcttccacagatacgccgtggacgtgctgaagtccggacggtgccagatgctcgatcggcggaccgtggagatggccttcgcctatgccctcgccctgttcgccgctgccagacaggaagaggctggcgcccaggtgtcagtgcccagagccctggatagacaggccgccctgctgcagatccaggaattcatgatcacctgcctgagccagaccccccctagaaccaccctgctgctgtaccccacagccgtggatctggccaagagggccctgtggacccccaaccagatcaccgacatcacaagcctcgtgcggctcgtgtacatcctgagcaagcagaaccagcagcacctgatcccccagtgggccctgagacagatcgccgacttcgccctgaagctgcacaagacccatctggccagctttctgagcgccttcgccaggcaggaactgtacctgatgggcagcctggtccacagcatgctggtgcataccaccgagcggcgggagatcttcatcgtggagacaggcctgtgtagcctggccgagctgtcccactttacccagctgctggcccaccctcaccacgagtacctgagcgacctgtacaccccctgcagcagcagcggcagacgggaccacagcctggaacggctgaccagactgttccccgatgccaccgtgcctgctacagtgcctgccgccctgtccatcctgtccaccatgcagcccagcaccctggaaaccttccccgacctgttctgcctgcccctgggcgagagctttagcgccctgaccgtgtccgagcacgtgtcctacatcgtgaccaatcagtacctgatcaagggcatcagctaccccgtgtccaccacagtcgtgggccagagcctgatcatcacccagaccgacagccagaccaagtgcgagctgacccggaacatgcacaccacacacagcatcaccgtggccctgaacatcagcctggaaaactgcgctttctgtcagtctgccctgctggaatacgacgatacccagggcgtgatcaacatcatgtacatgcacgacagcgacgacgtgctgttcgccctggacccctacaacgaggtggtggtgtccagcccccggacccactacctgatgctgctgaagaacggcaccgtgctggaagtgaccgacgtggtggtggacgccaccgactgataagcggccgcatacagcagcaattggcaagctgcttacatagaactcgcggcgattggcatgccgccttaaaatttttattttatttttcttttcttttccgaatcggattttgtttttaatatttcaaaaaaaaaaaaaaaaaaaaaaaaaaaaaaaaaaagggtcggcatggcatctccacctcctcgcggtccgacctgggcatccgaaggaggacgcacgtccactcggatggctaagggagagccacgtttaaacacgtgatatctggcctcatgggccttcctttcactgcccgctttccagtcgggaaacctgtcgtgccagctgcattaacatggtcatagctgtttccttgcgtattgggcgctctccgcttcctcgctcactgactcgctgcgctcggtcgttcgggtaaagcctggggtgcctaatgagcaaaaggccagcaaaaggccaggaaccgtaaaaaggccgcgttgctggcgtttttccataggctccgcccccctgacgagcatcacaaaaatcgacgctcaagtcagaggtggcgaaacccgacaggactataaagataccaggcgtttccccctggaagctccctcgtgcgctctcctgttccgaccctgccgcttaccggatacctgtccgcctttctcccttcgggaagcgtggcgctttctcatagctcacgctgtaggtatctcagttcggtgtaggtcgttcgctccaagctgggctgtgtgcacgaaccccccgttcagcccgaccgctgcgccttatccggtaactatcgtcttgagtccaacccggtaagacacgacttatcgccactggcagcagccactggtaacaggattagcagagcgaggtatgtaggcggtgctacagagttcttgaagtggtggcctaactacggctacactagaagaacagtatttggtatctgcgctctgctgaagccagttaccttcggaaaaagagttggtagctcttgatccggcaaacaaaccaccgctggtagcggtggtttttttgtttgcaagcagcagattacgcgcagaaaaaaaggatctcaagaagatcctttgatcttttctacggggtctgacgctcagtggaacgaaaactcacgttaagggattttggtcatgagattatcaaaaaggatcttcacctagatccttttaaattaaaaatgaagttttaaatcaatctaaagtatatatgagtaaacttggtctgacagttattagaaaaattcatccagcagacgataaaacgcaatacgctggctatccggtgccgcaatgccatacagcaccagaaaacgatccgcccattcgccgcccagttcttccgcaatatcacgggtggccagcgcaatatcctgataacgatccgccacgcccagacggccgcaatcaataaagccgctaaaacggccattttccaccataatgttcggcaggcacgcatcaccatgggtcaccaccagatcttcgccatccggcatgctcgctttcagacgcgcaaacagctctgccggtgccaggccctgatgttcttcatccagatcatcctgatccaccaggcccgcttccatacgggtacgcgcacgttcaatacgatgtttcgcctgatgatcaaacggacaggtcgccgggtccagggtatgcagacgacgcatggcatccgccataatgctcactttttctgccggcgccagatggctagacagcagatcctgacccggcacttcgcccagcagcagccaatcacggcccgcttcggtcaccacatccagcaccgccgcacacggaacaccggtggtggccagccagctcagacgcgccgcttcatcctgcagctcgttcagcgcaccgctcagatcggttttcacaaacagcaccggacgaccctgcgcgctcagacgaaacaccgccgcatcagagcagccaatggtctgctgcgcccaatcatagccaaacagacgttccacccacgctgccgggctacccgcatgcaggccatcctgttcaatcatactcttcctttttcaatattattgaagcatttatcagggttattgtctcatgagcggatacatatttgaatgtatttagaaaaataaacaaataggggttccgcgcacatttccccgaaaagtgccacctaaattgtaagcgttaatattttgttaaaattcgcgttaaatttttgttaaatcagctcattttttaaccaataggccgaaatcggcaaaatcccttataaatcaaaagaatagaccgagatagggttgagtggccgctacagggcgctcccattcgccattcaggctgcgcaactgttgggaagggcgtttcggtgcgggcctcttcgctattacgccagctggcgaaagggggatgtgctgcaaggcgattaagttgggtaacgccagggttttcccagtcacacgcgtaatacgactcactatag

SEQ ID NO: 65 - DNA, 15300 bp, Artificial Sequence
  source: /note="Description of Artificial Sequence: Synthetic polynucleotide"
ataggcggcgcatgagagaagcccagaccaattacctacccaaaatggagaaagttcacgttgacatcgaggaagacagcccattcctcagagctttgcagcggagcttcccgcagtttgaggtagaagccaagcaggtcactgataatgaccatgctaatgccagagcgttttcgcatctggcttcaaaactgatcgaaacggaggtggacccatccgacacgatccttgacattggaagtgcgcccgcccgcagaatgtattctaagcacaagtatcattgtatctgtccgatgagatgtgcggaagatccggacagattgtataagtatgcaactaagctgaagaaaaactgtaaggaaataactgataaggaattggacaagaaaatgaaggagctcgccgccgtcatgagcgaccctgacctggaaactgagactatgtgcctccacgacgacgagtcgtgtcgctacgaagggcaagtcgctgtttaccaggatgtatacgcggttgacggaccgacaagtctctatcaccaagccaataagggagttagagtcgcctactggataggctttgacaccaccccttttatgtttaagaacttggctggagcatatccatcatactctaccaactgggccgacgaaaccgtgttaacggctcgtaacataggcctatgcagctctgacgttatggagcggtcacgtagagggatgtccattcttagaaagaagtatttgaaaccatccaacaatgttctattctctgttggctcgaccatctaccacgagaagagggacttactgaggagctggcacctgccgtctgtatttcacttacgtggcaagcaaaattacacatgtcggtgtgagactatagttagttgcgacgggtacgtcgttaaaagaatagctatcagtccaggcctgtatgggaagccttcaggctatgctgctacgatgcaccgcgagggattcttgtgctgcaaagtgacagacacattgaacggggagagggtctcttttcccgtgtgcacgtatgtgccagctacattgtgtgaccaaatgactggcatactggcaacagatgtcagtgcggacgacgcgcaaaaactgctggttgggctcaaccagcgtatagtcgtcaacggtcgcacccagagaaacaccaataccatgaaaaattaccttttgcccgtagtggcccaggcatttgctaggtgggcaaaggaatataaggaagatcaagaagatgaaaggccactaggactacgagatagacagttagtcatggggtgttgttgggcttttagaaggcacaagataacatctatttataagcgcccggatacccaaaccatcatcaaagtgaacagcgatttccactcattcgtgctgcccaggataggcagtaacacattggagatcgggctgagaacaagaatcaggaaaatgttagaggagcacaaggagccgtcacctctcattaccgccgaggacgtacaagaagctaagtgcgcagccgatgaggctaaggaggtgcgtgaagccgaggagttgcgcgcagctctaccacctttggcagctgatgttgaggagcccactctggaagccgatgtagacttgatgttacaagaggctggggccggctcagtggagacacctcgtggcttgataaaggttaccagctacgatggcgaggacaagatcggctcttacgctgtgctttctccgcaggctgtactcaagagtgaaaaattatcttgcatccaccctctcgctgaacaagtcatagtgataacacactctggccgaaaagggcgttatgccgtggaaccataccatggtaaagtagtggtgccagagggacatgcaatacccgtccaggactttcaagctctgagtgaaagtgccaccattgtgtacaacgaacgtgagttcgtaaacaggtacctgcaccatattgccacacatggaggagcgctgaacactgatgaagaatattacaaaactgtcaagcccagcgagcacgacggcgaatacctgtacgacatcgacaggaaacagtgcgtcaagaaagaactagtcactgggctagggctcacaggcgagctggtggatcctcccttccatgaattcgcctacgagagtctgagaacacgaccagccgctccttaccaagtaccaaccataggggtgtatggcgtgccaggatcaggcaagtctggcatcattaaaagcgcagtcaccaaaaaagatctagtggtgagcgccaagaaagaaaactgtgcagaaattataagggacgtcaagaaaatgaaagggctggacgtcaatgccagaactgtggactcagtgctcttgaatggatgcaaacaccccgtagagaccctgtatattgacgaagcttttgcttgtcatgcaggtactctcagagcgctcatagccattataagacctaaaaaggcagtgctctgcggggatcccaaacagtgcggtttttttaacatgatgtgcctgaaagtgcattttaaccacgagatttgcacacaagtcttccacaaaagcatctctcgccgttgcactaaatctgtgacttcggtcgtctcaaccttgttttacgacaaaaaaatgagaacgacgaatccgaaagagactaagattgtgattgacactaccggcagtaccaaacctaagcaggacgatctcattctcacttgtttcagagggtgggtgaagcagttgcaaatagattacaaaggcaacgaaataatgacggcagctgcctctcaagggctgacccgtaaaggtgtgtatgccgttcggtacaaggtgaatgaaaatcctctgtacgcacccacctcagaacatgtgaacgtcctactgacccgcacggaggaccgcatcgtgtggaaaacactagccggcgacccatggataaaaacactgactgccaagtaccctgggaatttcactgccacgatagaggagtggcaagcagagcatgatgccatcatgaggcacatcttggagagaccggaccctaccgacgtcttccagaataaggcaaacgtgtgttgggccaaggctttagtgccggtgctgaagaccgctggcatagacatgaccactgaacaatggaacactgtggattattttgaaacggacaaagctcactcagcagagatagtattgaaccaactatgcgtgaggttctttggactcgatctggactccggtctattttctgcacccactgttccgttatccattaggaataatcactgggataactccccgtcgcctaacatgtacgggctgaataaagaagtggtccgtcagctctctcgcaggtacccacaactgcctcgggcagttgccactggaagagtctatgacatgaacactggtacactgcgcaattatgatccgcgcataaacctagtacctgtaaacagaagactgcctcatgctttagtcctccaccataatgaacacccacagagtgacttttcttcattcgtcagcaaattgaagggcagaactgtcctggtggtcggggaaaagttgtccgtcccaggcaaaatggttgactggttgtcagaccggcctgaggctaccttcagagctcggctggatttaggcatcccaggtgatgtgcccaaatatgacataatatttgttaatgtgaggaccccatataaataccatcactatcagcagtgtgaagaccatgccattaagcttagcatgttgaccaagaaagcttgtctgcatctgaatcccggcggaacctgtgtcagcataggttatggttacgctgacagggccagcgaaagcatcattggtgctatagcgcggcagttcaagttttcccgggtatgcaaaccgaaatcctcacttgaagagacggaagttctgtttgtattcattgggtacgatcgcaaggcccgtacgcacaatccttacaagctttcatcaaccttgaccaacatttatacaggttccagactccacgaagccggatgtgcaccctcatatcatgtggtgcgaggggatattgccacggccaccgaaggagtgattataaatgctgctaacagcaaaggacaacctggcggaggggtgtgcggagcgctgtataagaaattcccggaaagcttcgatttacagccgatcgaagtaggaaaagcgcgactggtcaaaggtgcagctaaacatatcattcatgccgtaggaccaaacttcaacaaagtttcggaggttgaaggtgacaaacagttggcagaggcttatgagtccatcgctaagattgtcaacgataacaattacaagtcagtagcgattccactgttgtccaccggcatcttttccgggaacaaagatcgactaacccaatcattgaaccatttgctgacagctttagacaccactgatgcagatgtagccatatactgcagggacaagaaatgggaaatgactctcaaggaagcagtggctaggagagaagcagtggaggagatatgcatatccgacgactcttcagtgacagaacctgatgcagagctggtgagggtgcatccgaagagttctttggctggaaggaagggctacagcacaagcgatggcaaaactttctcatatttggaagggaccaagtttcaccaggcggccaaggatatagcagaaattaatgccatgtggcccgttgcaacggaggccaatgagcaggtatgcatgtatatcctcggagaaagcatgagcagtattaggtcgaaatgccccgtcgaagagtcggaagcctccacaccacctagcacgctgccttgcttgtgcatccatgccatgactccagaaagagtacagcgcctaaaagcctcacgtccagaacaaattactgtgtgctcatcctttccattgccgaagtatagaatcactggtgtgcagaagatccaatgctcccagcctatattgttctcaccgaaagtgcctgcgtatattcatccaaggaagtatctcgtggaaacaccaccggtagacgagactccggagccatcggcagagaaccaatccacagaggggacacctgaacaaccaccacttataaccgaggatgagaccaggactagaacgcctgagccgatcatcatcgaagaggaagaagaggatagcataagtttgctgtcagatggcccgacccaccaggtgctgcaagtcgaggcagacattcacgggccgccctctgtatctagctcatcctggtccattcctcatgcatccgactttgatgtggacagtttatccatacttgacaccctggagggagctagcgtgaccagcggggcaacgtcagccgagactaactcttacttcgcaaagagtatggagtttctggcgcgaccggtgcctgcgcctcgaacagtattcaggaaccctccacatcccgctccgcgcacaagaacaccgtcacttgcacccagcagggcctgctcgagaaccagcctagtttccaccccgccaggcgtgaatagggtgatcactagagaggagctcgaggcgcttaccccgtcacgcactcctagcaggtcggtctcgagaaccagcctggtctccaacccgccaggcgtaaatagggtgattacaagagaggagtttgaggcgttcgtagcacaacaacaatgacggtttgatgcgggtgcatacatcttttcctccgacaccggtcaagggcatttacaacaaaaatcagtaaggcaaacggtgctatccgaagtggtgttggagaggaccgaattggagatttcgtatgccccgcgcctcgaccaagaaaaagaagaattactacgcaagaaattacagttaaatcccacacctgctaacagaagcagataccagtccaggaaggtggagaacatgaaagccataacagctagacgtattctgcaaggcctagggcattatttgaaggcagaaggaaaagtggagtgctaccgaaccctgcatcctgttcctttgtattcatctagtgtgaaccgtgccttttcaagccccaaggtcgcagtggaagcctgtaacgccatgttgaaagagaactttccgactgtggcttcttactgtattattccagagtacgatgcctatttggacatggttgacggagcttcatgctgcttagacactgccagtttttgccctgcaaagctgcgcagctttccaaagaaacactcctatttggaacccacaatacgatcggcagtgccttcagcgatccagaacacgctccagaacgtcctggcagctgccacaaaaagaaattgcaatgtcacgcaaatgagagaattgcccgtattggattcggcggcctttaatgtggaatgcttcaagaaatatgcgtgtaataatgaatattgggaaacgtttaaagaaaaccccatcaggcttactgaagaaaacgtggtaaattacattaccaaattaaaaggaccaaaagctgctgctctttttgcgaagacacataatttgaatatgttgcaggacataccaatggacaggtttgtaatggacttaaagagagacgtgaaagtgactccaggaacaaaacatactgaagaacggcccaaggtacaggtgatccaggctgccgatccgctagcaacagcgtatctgtgcggaatccaccgagagctggttaggagattaaatgcggtcctgcttccgaacattcatacactgtttgatatgtcggctgaagactttgacgctattatagccgagcacttccagcctggggattgtgttctggaaactgacatcgcgtcgtttgataaaagtgaggacgacgccatggctctgaccgcgttaatgattctggaagacttaggtgtggacgcagagctgttgacgctgattgaggcggctttcggcgaaatttcatcaatacatttgcccactaaaactaaatttaaattcggagccatgatgaaatctggaatgttcctcacactgtttgtgaacacagtcattaacattgtaatcgcaagcagagtgttgagagaacggctaaccggatcaccatgtgcagcattcattggagatgacaatatcgtgaaaggagtcaaatcggacaaattaatggcagacaggtgcgccacctggttgaatatggaagtcaagattatagatgctgtggtgggcgagaaagcgccttatttctgtggagggtttattttgtgtgactccgtgaccggcacagcgtgccgtgtggcagaccccctaaaaaggctgtttaagcttggcaaacctctggcagcagacgatgaacatgatgatgacaggagaagggcattgcatgaagagtcaacacgctggaaccgagtgggtattctttcagagctgtgcaaggcagtagaatcaaggtatgaaaccgtaggaacttccatcatagttatggccatgactactctagctagcagtgttaaatcattcagctacctgagaggggcccctataactctctacggctaacctgaatggactacgacatagtctagtccgccaagatgaggcctggcctgccctcctacctgatcatcctggccgtgtgcctgttcagccacctgctgtccagcagatacggcgccgaggccgtgagcgagcccctggacaaggctttccacctgctgctgaacacctacggcagacccatccggtttctgcgggagaacaccacccagtgcacctacaacagcagcctgcggaacagcaccgtcgtgagagagaacgccatcagcttcaactttttccagagctacaaccagtactacgtgttccacatgcccagatgcctgtttgccggccctctggccgagcagttcctgaaccaggtggacctgaccgagacactggaaagataccagcagcggctgaatacctacgccctggtgtccaaggacctggccagctaccggtcctttagccagcagctcaaggctcaggatagcctcggcgagcagcctaccaccgtgccccctcccatcgacctgagcatcccccacgtgtggatgcctccccagaccacccctcacggctggaccgagagccacaccacctccggcctgcacagaccccacttcaaccagacctgcatcctgttcgacggccacgacctgctgtttagcaccgtgaccccctgcctgcaccagggcttctacctgatcgacgagctgagatacgtgaagatcaccctgaccgaggatttcttcgtggtcaccgtgtccatcgacgacgacacccccatgctgctgatcttcggccacctgcccagagtgctgttcaaggccccctaccagcgggacaacttcatcctgcggcagaccgagaagcacgagctgctggtgctggtcaagaaggaccagctgaaccggcactcctacctgaaggaccccgacttcctggacgccgccctggacttcaactacctggacctgagcgccctgctgagaaacagcttccacagatacgccgtggacgtgctgaagtccggacggtgccagatgctcgatcggcggaccgtggagatggccttcgcctatgccctcgccctgttcgccgctgccagacaggaagaggctggcgcccaggtgtcagtgcccagagccctggatagacaggccgccctgctgcagatccaggaattcatgatcacctgcctgagccagaccccccctagaaccaccctgctgctgtaccccacagccgtggatctggccaagagggccctgtggacccccaaccagatcaccgacatcacaagcctcgtgcggctcgtgtacatcctgagcaagcagaaccagcagcacctgatcccccagtgggccctgagacagatcgccgacttcgccctgaagctgcacaagacccatctggccagctttctgagcgccttcgccaggcaggaactgtacctgatgggcagcctggtccacagcatgctggtgcataccaccgagcggcgggagatcttcatcgtggagacaggcctgtgtagcctggccgagctgtcccactttacccagctgctggcccaccctcaccacgagtacctgagcgacctgtacaccccctgcagcagcagcggcagacgggaccacagcctggaacggctgaccagactgttccccgatgccaccgtgcctgctacagtgcctgccgccctgtccatcctgtccaccatgcagcccagcaccctggaaaccttccccgacctgttctgcctgcccctgggcgagagctttagcgccctgaccgtgtccgagcacgtgtcctacatcgtgaccaatcagtacctgatcaagggcatcagctaccccgtgtccaccacagtcgtgggccagagcctgatcatcacccagaccgacagccagaccaagtgcgagctgacccggaacatgcacaccacacacagcatcaccgtggccctgaacatcagcctggaaaactgcgctttctgtcagtctgccctgctggaatacgacgatacccagggcgtgatcaacatcatgtacatgcacgacagcgacgacgtgctgttcgccctggacccctacaacgaggtggtggtgtccagcccccggacccactacctgatgctgctgaagaacggcaccgtgctggaagtgaccgacgtggtggtggacgccaccgacagcagactgctgatgatgagcgtgtacgccctgagcgccatcatcggcatctacctgctgtaccggatgctgaaaacctgctgataatctagaggcccctataactctctacggctaacctgaatggactacgacatagtctagtccgccaagatgtgcagaaggcccgactgcggcttcagcttcagccctggacccgtgatcctgctgtggtgctgcctgctgctgcctatcgtgtcctctgccgccgtgtctgtggcccctacagccgccgagaaggtgccagccgagtgccccgagctgaccagaagatgcctgctgggcgaggtgttcgagggcgacaagtacgagagctggctgcggcccctggtcaacgtgaccggcagagatggccccctgagccagctgatccggtacagacccgtgacccccgaggccgccaatagcgtgctgctggacgaggccttcctggataccctggccctgctgtacaacaaccccgaccagctgagagccctgctgaccctgctgtccagcgacaccgcccccagatggatgaccgtgatgcggggctacagcgagtgtggagatggcagccctgccgtgtacacctgcgtggacgacctgtgcagaggctacgacctgaccagactgagctacggccggtccatcttcacagagcacgtgctgggcttcgagctggtgccccccagcctgttcaacgtggtggtggccatccggaacgaggccaccagaaccaacagagccgtgcggctgcctgtgtctacagccgctgcacctgagggcatcacactgttctacggcctgtacaacgccgtgaaagagttctgcctccggcaccagctggatccccccctgctgagacacctggacaagtactacgccggcctgcccccagagctgaagcagaccagagtgaacctgcccgcccacagcagatatggccctcaggccgtggacgccagatgataacgccggcggcccctataactctctacggctaacctgaatggactacgacatagtctagtccgccaagatgagccccaaggacctgacccccttcctgacaaccctgtggctgctcctgggccatagcagagtgcctagagtgcgggccgaggaatgctgcgagttcatcaacgtgaaccacccccccgagcggtgctacgacttcaagatgtgcaaccggttcaccgtggccctgagatgccccgacggcgaagtgtgctacagccccgagaaaaccgccgagatccggggcatcgtgaccaccatgacccacagcctgacccggcaggtggtgcacaacaagctgaccagctgcaactacaaccccctgtacctggaagccgacggccggatcagatgcggcaaagtgaacgacaaggcccagtacctgctgggagccgccggaagcgtgccctaccggtggatcaacctggaatacgacaagatcacccggatcgtgggcctggaccagtacctggaaagcgtgaagaagcacaagcggctggacgtgtgcagagccaagatgggctacatgctgcagtgataaggcgcgccgcccctataactctctacggctaacctgaatggactacgacatagtctagtccgccaagatgctgcggctgctgctgagacaccacttccactgcctgctgctgtgtgccgtgtgggccaccccttgtctggccagcccttggagcaccctgaccgccaaccagaaccctagccccccttggtccaagctgacctacagcaagccccacgacgccgccaccttctactgcccctttctgtaccccagccctcccagaagccccctgcagttcagcggcttccagagagtgtccaccggccctgagtgccggaacgagacactgtacctgctgtacaaccgggagggccagacactggtggagcggagcagcacctgggtgaaaaaagtgatctggtatctgagcggccggaaccagaccatcctgcagcggatgcccagaaccgccagcaagcccagcgacggcaacgtgcagatcagcgtggaggacgccaaaatcttcggagcccacatggtgcccaagcagaccaagctgctgagattcgtggtcaacgacggcaccagatatcagatgtgcgtgatgaagctggaaagctgggcccacgtgttccgggactactccgtgagcttccaggtccggctgaccttcaccgaggccaacaaccagacctacaccttctgcacccaccccaacctgatcgtgtgataagcggccgcgcccctataactctctacggctaacctgaatggactacgacatagtctagtccgccaagatgcggctgtgcagagtgtggctgtccgtgtgcctgtgtgccgtggtgctgggccagtgccagagagagacagccgagaagaacgactactaccgggtgccccactactgggatgcctgcagcagagccctgcccgaccagacccggtacaaatacgtggagcagctcgtggacctgaccctgaactaccactacgacgccagccacggcctggacaacttcgacgtgctgaagcggatcaacgtgaccgaggtgtccctgctgatcagcgacttccggcggcagaacagaagaggcggcaccaacaagcggaccaccttcaacgccgctggctctctggcccctcacgccagatccctggaattcagcgtgcggctgttcgccaactgataacgttgcatcctgcaggatacagcagcaattggcaagctgcttacatagaactcgcggcgattggcatgccgccttaaaatttttattttatttttcttttcttttccgaatcggattttgtttttaatatttcaaaaaaaaaaaaaaaaaaaaaaaaaaaaaaaaaaagggtcggcatggcatctccacctcctcgcggtccgacctgggcatccgaaggaggacgcacgtccactcggatggctaagggagagccacgtttaaacgctagagcaagacgtttcccgttgaatatggctcataacaccccttgtattactgtttatgtaagcagacagttttattgttcatgatgatatatttttatcttgtgcaatgtaacatcagagattttgagacacaacgtggctttgttgaataaatcgaacttttgctgagttgaaggatcagatcacgcatcttcccgacaacgcagaccgttccgtggcaaagcaaaagttcaaaatcaccaactggtccacctacaacaaagctctcatcaaccgtggctccctcactttctggctggatgatggggcgattcaggcctggtatgagtcagcaacaccttcttcacgaggcagacctcagcgctagcggagtgtatactggcttactatgttggcactgatgagggtgtcagtgaagtgcttcatgtggcaggagaaaaaaggctgcaccggtgcgtcagcagaatatgtgatacaggatatattccgcttcctcgctcactgactcgctacgctcggtcgttcgactgcggcgagcggaaatggcttacgaacggggcggagatttcctggaagatgccaggaagatacttaacagggaagtgagagggccgcggcaaagccgtttttccataggctccgcccccctgacaagcatcacgaaatctgacgctcaaatcagtggtggcgaaacccgacaggactataaagataccaggcgtttcccctggcggctccctcgtgcgctctcctgttcctgcctttcggtttaccggtgtcattccgctgttatggccgcgtttgtctcattccacgcctgacactcagttccgggtaggcagttcgctccaagctggactgtatgcacgaaccccccgttcagtccgaccgctgcgccttatccggtaactatcgtcttgagtccaacccggaaagacatgcaaaagcaccactggcagcagccactggtaattgatttagaggagttagtcttgaagtcatgcgccggttaaggctaaactgaaaggacaagttttggtgactgcgctcctccaagccagttacctcggttcaaagagttggtagctcagagaaccttcgaaaaaccgccctgcaaggcggttttttcgttttcagagcaagagattacgcgcagaccaaaacgatctcaagaagatcatcttattaaggggtctgacgctcagtggaacgaaaactcacgttaagggattttggtcatgagattatcaaaaaggatcttcacctagatccttttaaattaaaaatgaagttttaaatcaatctaaagtatatatgagtaaacttggtctgacagttattagaaaaattcatccagcagacgataaaacgcaatacgctggctatccggtgccgcaatgccatacagcaccagaaaacgatccgcccattcgccgcccagttcttccgcaatatcacgggtggccagcgcaatatcctgataacgatccgccacgcccagacggccgcaatcaataaagccgctaaaacggccattttccaccataatgttcggcaggcacgcatcaccatgggtcaccaccagatcttcgccatccggcatgctcgctttcagacgcgcaaacagctctgccggtgccaggccctgatgttcttcatccagatcatcctgatccaccaggcccgcttccatacgggtacgcgcacgttcaatacgatgtttcgcctgatgatcaaacggacaggtcgccgggtccagggtatgcagacgacgcatggcatccgccataatgctcactttttctgccggcgccagatggctagacagcagatcctgacccggcacttcgcccagcagcagccaatcacggcccgcttcggtcaccacatccagcaccgccgcacacggaacaccggtggtggccagccagctcagacgcgccgcttcatcctgcagctcgttcagcgcaccgctcagatcggttttcacaaacagcaccggacgaccctgcgcgctcagacgaaacaccgccgcatcagagcagccaatggtctgctgcgcccaatcatagccaaacagacgttccacccacgctgccgggctacccgcatgcaggccatcctgttcaatcatactcttcctttttcaatattattgaagcatttatcagggttattgtctcatgagcggatacatatttgaatgtatttagaaaaataaacaaataggggttccgcgcacatttccccgaaaagtgccacctaaattgtaagcgttaatattttgttaaaattcgcgttaaatttttgttaaatcagctcattttttaaccaataggccgaaatcggcaaaatcccttataaatcaaaagaatagaccgagatagggttgagtggccgctacagggcgctcccattcgccattcaggctgcgcaactgttgggaagggcgtttcggtgcgggcctcttcgctattacgccagctggcgaaagggggatgtgctgcaaggcgattaagttgggtaacgccagggttttcccagtcacacgcgtaatacgactcactatag

SEQ ID NO: 66 - DNA, 16324 bp, Artificial Sequence
  source: /note="Description of Artificial Sequence: Synthetic polynucleotide"
ataggcggcgcatgagagaagcccagaccaattacctacccaaaatggagaaagttcacgttgacatcgaggaagacagcccattcctcagagctttgcagcggagcttcccgcagtttgaggtagaagccaagcaggtcactgataatgaccatgctaatgccagagcgttttcgcatctggcttcaaaactgatcgaaacggaggtggacccatccgacacgatccttgacattggaagtgcgcccgcccgcagaatgtattctaagcacaagtatcattgtatctgtccgatgagatgtgcggaagatccggacagattgtataagtatgcaactaagctgaagaaaaactgtaaggaaataactgataaggaattggacaagaaaatgaaggagctcgccgccgtcatgagcgaccctgacctggaaactgagactatgtgcctccacgacgacgagtcgtgtcgctacgaagggcaagtcgctgtttaccaggatgtatacgcggttgacggaccgacaagtctctatcaccaagccaataagggagttagagtcgcctactggataggctttgacaccaccccttttatgtttaagaacttggctggagcatatccatcatactctaccaactgggccgacgaaaccgtgttaacggctcgtaacataggcctatgcagctctgacgttatggagcggtcacgtagagggatgtccattcttagaaagaagtatttgaaaccatccaacaatgttctattctctgttggctcgaccatctaccacgagaagagggacttactgaggagctggcacctgccgtctgtatttcacttacgtggcaagcaaaattacacatgtcggtgtgagactatagttagttgcgacgggtacgtcgttaaaagaatagctatcagtccaggcctgtatgggaagccttcaggctatgctgctacgatgcaccgcgagggattcttgtgctgcaaagtgacagacacattgaacggggagagggtctcttttcccgtgtgcacgtatgtgccagctacattgtgtgaccaaatgactggcatactggcaacagatgtcagtgcggacgacgcgcaaaaactgctggttgggctcaaccagcgtatagtcgtcaacggtcgcacccagagaaacaccaataccatgaaaaattaccttttgcccgtagtggcccaggcatttgctaggtgggcaaaggaatataaggaagatcaagaagatgaaaggccactaggactacgagatagacagttagtcatggggtgttgttgggcttttagaaggcacaagataacatctatttataagcgcccggatacccaaaccatcatcaaagtgaacagcgatttccactcattcgtgctgcccaggataggcagtaacacattggagatcgggctgagaacaagaatcaggaaaatgttagaggagcacaaggagccgtcacctctcattaccgccgaggacgtacaagaagctaagtgcgcagccgatgaggctaaggaggtgcgtgaagccgaggagttgcgcgcagctctaccacctttggcagctgatgttgaggagcccactctggaagccgatgtagacttgatgttacaagaggctggggccggctcagtggagacacctcgtggcttgataaaggttaccagctacgatggcgaggacaagatcggctcttacgctgtgctttctccgcaggctgtactcaagagtgaaaaattatcttgcatccaccctctcgctgaacaagtcatagtgataacacactctggccgaaaagggcgttatgccgtggaaccataccatggtaaagtagtggtgccagagggacatgcaatacccgtccaggactttcaagctctgagtgaaagtgccaccattgtgtacaacgaacgtgagttcgtaaacaggtacctgcaccatattgccacacatggaggagcgctgaacactgatgaagaatattacaaaactgtcaagcccagcgagcacgacggcgaatacctgtacgacatcgacaggaaacagtgcgtcaagaaagaactagtcactgggctagggctcacaggcgagctggtggatcctcccttccatgaattcgcctacgagagtctgagaacacgaccagccgctccttaccaagtaccaaccataggggtgtatggcgtgccaggatcaggcaagtctggcatcattaaaagcgcagtcaccaaaaaagatctagtggtgagcgccaagaaagaaaactgtgcagaaattataagggacgtcaagaaaatgaaagggctggacgtcaatgccagaactgtggactcagtgctcttgaatggatgcaaacaccccgtagagaccctgtatattgacgaagcttttgcttgtcatgcaggtactctcagagcgctcatagccattataagacctaaaaaggcagtgctctgcggggatcccaaacagtgcggtttttttaacatgatgtgcctgaaagtgcattttaaccacgagatttgcacacaagtcttccacaaaagcatctctcgccgttgcactaaatctgtgacttcggtcgtctcaaccttgttttacgacaaaaaaatgagaacgacgaatccgaaagagactaagattgtgattgacactaccggcagtaccaaacctaagcaggacgatctcattctcacttgtttcagagggtgggtgaagcagttgcaaatagattacaaaggcaacgaaataatgacggcagctgcctctcaagggctgacccgtaaaggtgtgtatgccgttcggtacaaggtgaatgaaaatcctctgtacgcacccacctcagaacatgtgaacgtcctactgacccgcacggaggaccgcatcgtgtggaaaacactagccggcgacccatggataaaaacactgactgccaagtaccctgggaatttcactgccacgatagaggagtggcaagcagagcatgatgccatcatgaggcacatcttggagagaccggaccctaccgacgtcttccagaataaggcaaacgtgtgttgggccaaggctttagtgccggtgctgaagaccgctggcatagacatgaccactgaacaatggaacactgtggattattttgaaacggacaaagctcactcagcagagatagtattgaaccaactatgcgtgaggttctttggactcgatctggactccggtctattttctgcacccactgttccgttatccattaggaataatcactgggataactccccgtcgcctaacatgtacgggctgaataaagaagtggtccgtcagctctctcgcaggtacccacaactgcctcgggcagttgccactggaagagtctatgacatgaacactggtacactgcgcaattatgatccgcgcataaacctagtacctgtaaacagaagactgcctcatgctttagtcctccaccataatgaacacccacagagtgacttttcttcattcgtcagcaaattgaagggcagaactgtcctggtggtcggggaaaagttgtccgtcccaggcaaaatggttgactggttgtcagaccggcctgaggctaccttcagagctcggctggatttaggcatcccaggtgatgtgcccaaatatgacataatatttgttaatgtgaggaccccatataaataccatcactatcagcagtgtgaagaccatgccattaagcttagcatgttgaccaagaaagcttgtctgcatctgaatcccggcggaacctgtgtcagcataggttatggttacgctgacagggccagcgaaagcatcattggtgctatagcgcggcagttcaagttttcccgggtatgcaaaccgaaatcctcacttgaagagacggaagttctgtttgtattcattgggtacgatcgcaaggcccgtacgcacaatccttacaagctttcatcaaccttgaccaacatttatacaggttccagactccacgaagccggatgtgcaccctcatatcatgtggtgcgaggggatattgccacggccaccgaaggagtgattataaatgctgctaacagcaaaggacaacctggcggaggggtgtgcggagcgctgtataagaaattcccggaaagcttcgatttacagccgatcgaagtaggaaaagcgcgactggtcaaaggtgcagctaaacatatcattcatgccgtaggaccaaacttcaacaaagtttcggaggttgaaggtgacaaacagttggcagaggcttatgagtccatcgctaagattgtcaacgataacaattacaagtcagtagcgattccactgttgtccaccggcatcttttccgggaacaaagatcgactaacccaatcattgaaccatttgctgacagctttagacaccactgatgcagatgtagccatatactgcagggacaagaaatgggaaatgactctcaaggaagcagtggctaggagagaagcagtggaggagatatgcatatccgacgactcttcagtgacagaacctgatgcagagctggtgagggtgcatccgaagagttctttggctggaaggaagggctacagcacaagcgatggcaaaactttctcatatttggaagggaccaagtttcaccaggcggccaaggatatagcagaaattaatgccatgtggcccgttgcaacggaggccaatgagcaggtatgcatgtatatcctcggagaaagcatgagcagtattaggtcgaaatgccccgtcgaagagtcggaagcctccacaccacctagcacgctgccttgcttgtgcatccatgccatgactccagaaagagtacagcgcctaaaagcctcacgtccagaacaaattactgtgtgctcatcctttccattgccgaagtatagaatcactggtgtgcagaagatccaatgctcccagcctatattgttctcaccgaaagtgcctgcgtatattcatccaaggaagtatctcgtggaaacaccaccggtagacgagactccggagccatcggcagagaaccaatccacagaggggacacctgaacaaccaccacttataaccgaggatgagaccaggactagaacgcctgagccgatcatcatcgaagaggaagaagaggatagcataagtttgctgtcagatggcccgacccaccaggtgctgcaagtcgaggcagacattcacgggccgccctctgtatctagctcatcctggtccattcctcatgcatccgactttgatgtggacagtttatccatacttgacaccctggagggagctagcgtgaccagcggggcaacgtcagccgagactaactcttacttcgcaaagagtatggagtttctggcgcgaccggtgcctgcgcctcgaacagtattcaggaaccctccacatcccgctccgcgcacaagaacaccgtcacttgcacccagcagggcctgctcgagaaccagcctagtttccaccccgccaggcgtgaatagggtgatcactagagaggagctcgaggcgcttaccccgtcacgcactcctagcaggtcggtctcgagaaccagcctggtctccaacccgccaggcgtaaatagggtgattacaagagaggagtttgaggcgttcgtagcacaacaacaatgacggtttgatgcgggtgcatacatcttttcctccgacaccggtcaagggcatttacaacaaaaatcagtaaggcaaacggtgctatccgaagtggtgttggagaggaccgaattggagatttcgtatgccccgcgcctcgaccaagaaaaagaagaattactacgcaagaaattacagttaaatcccacacctgctaacagaagcagataccagtccaggaaggtggagaacatgaaagccataacagctagacgtattctgcaaggcctagggcattatttgaaggcagaaggaaaagtggagtgctaccgaaccctgcatcctgttcctttgtattcatctagtgtgaaccgtgccttttcaagccccaaggtcgcagtggaagcctgtaacgccatgttgaaagagaactttccgactgtggcttcttactgtattattccagagtacgatgcctatttggacatggttgacggagcttcatgctgcttagacactgccagtttttgccctgcaaagctgcgcagctttccaaagaaacactcctatttggaacccacaatacgatcggcagtgccttcagcgatccagaacacgctccagaacgtcctggcagctgccacaaaaagaaattgcaatgtcacgcaaatgagagaattgcccgtattggattcggcggcctttaatgtggaatgcttcaagaaatatgcgtgtaataatgaatattgggaaacgtttaaagaaaaccccatcaggcttactgaagaaaacgtggtaaattacattaccaaattaaaaggaccaaaagctgctgctctttttgcgaagacacataatttgaatatgttgcaggacataccaatggacaggtttgtaatggacttaaagagagacgtgaaagtgactccaggaacaaaacatactgaagaacggcccaaggtacaggtgatccaggctgccgatccgctagcaacagcgtatctgtgcggaatccaccgagagctggttaggagattaaatgcggtcctgcttccgaacattcatacactgtttgatatgtcggctgaagactttgacgctattatagccgagcacttccagcctggggattgtgttctggaaactgacatcgcgtcgtttgataaaagtgaggacgacgccatggctctgaccgcgttaatgattctggaagacttaggtgtggacgcagagctgttgacgctgattgaggcggctttcggcgaaatttcatcaatacatttgcccactaaaactaaatttaaattcggagccatgatgaaatctggaatgttcctcacactgtttgtgaacacagtcattaacattgtaatcgcaagcagagtgttgagagaacggctaaccggatcaccatgtgcagcattcattggagatgacaatatcgtgaaaggagtcaaatcggacaaattaatggcagacaggtgcgccacctggttgaatatggaagtcaagattatagatgctgtggtgggcgagaaagcgccttatttctgtggagggtttattttgtgtgactccgtgaccggcacagcgtgccgtgtggcagaccccctaaaaaggctgtttaagcttggcaaacctctggcagcagacgatgaacatgatgatgacaggagaagggcattgcatgaagagtcaacacgctggaaccgagtgggtattctttcagagctgtgcaaggcagtagaatcaaggtatgaaaccgtaggaacttccatcatagttatggccatgactactctagctagcagtgttaaatcattcagctacctgagaggggcccctataactctctacggctaacctgaatggactacgacatagtctagtccgccaagatgaggcctggcctgccctcctacctgatcatcctggccgtgtgcctgttcagccacctgctgtccagcagatacggcgccgaggccgtgagcgagcccctggacaaggctttccacctgctgctgaacacctacggcagacccatccggtttctgcgggagaacaccacccagtgcacctacaacagcagcctgcggaacagcaccgtcgtgagagagaacgccatcagcttcaactttttccagagctacaaccagtactacgtgttccacatgcccagatgcctgtttgccggccctctggccgagcagttcctgaaccaggtggacctgaccgagacactggaaagataccagcagcggctgaatacctacgccctggtgtccaaggacctggccagctaccggtcctttagccagcagctcaaggctcaggatagcctcggcgagcagcctaccaccgtgccccctcccatcgacctgagcatcccccacgtgtggatgcctccccagaccacccctcacggctggaccgagagccacaccacctccggcctgcacagaccccacttcaaccagacctgcatcctgttcgacggccacgacctgctgtttagcaccgtgaccccctgcctgcaccagggcttctacctgatcgacgagctgagatacgtgaagatcaccctgaccgaggatttcttcgtggtcaccgtgtccatcgacgacgacacccccatgctgctgatcttcggccacctgcccagagtgctgttcaaggccccctaccagcgggacaacttcatcctgcggcagaccgagaagcacgagctgctggtgctggtcaagaaggaccagctgaaccggcactcctacctgaaggaccccgacttcctggacgccgccctggacttcaactacctggacctgagcgccctgctgagaaacagcttccacagatacgccgtggacgtgctgaagtccggacggtgccagatgctcgatcggcggaccgtggagatggccttcgcctatgccctcgccctgttcgccgctgccagacaggaagaggctggcgcccaggtgtcagtgcccagagccctggatagacaggccgccctgctgcagatccaggaattcatgatcacctgcctgagccagaccccccctagaaccaccctgctgctgtaccccacagccgtggatctggccaagagggccctgtggacccccaaccagatcaccgacatcacaagcctcgtgcggctcgtgtacatcctgagcaagcagaaccagcagcacctgatcccccagtgggccctgagacagatcgccgacttcgccctgaagctgcacaagacccatctggccagctttctgagcgccttcgccaggcaggaactgtacctgatgggcagcctggtccacagcatgctggtgcataccaccgagcggcgggagatcttcatcgtggagacaggcctgtgtagcctggccgagctgtcccactttacccagctgctggcccaccctcaccacgagtacctgagcgacctgtacaccccctgcagcagcagcggcagacgggaccacagcctggaacggctgaccagactgttccccgatgccaccgtgcctgctacagtgcctgccgccctgtccatcctgtccaccatgcagcccagcaccctggaaaccttccccgacctgttctgcctgcccctgggcgagagctttagcgccctgaccgtgtccgagcacgtgtcctacatcgtgaccaatcagtacctgatcaagggcatcagctaccccgtgtccaccacagtcgtgggccagagcctgatcatcacccagaccgacagccagaccaagtgcgagctgacccggaacatgcacaccacacacagcatcaccgtggccctgaacatcagcctggaaaactgcgctttctgtcagtctgccctgctggaatacgacgatacccagggcgtgatcaacatcatgtacatgcacgacagcgacgacgtgctgttcgccctggacccctacaacgaggtggtggtgtccagcccccggacccactacctgatgctgctgaagaacggcaccgtgctggaagtgaccgacgtggtggtggacgccaccgactgataatctagaggcccctataactctctacggctaacctgaatggactacgacatagtctagtccgccaagatgtgcagaaggcccgactgcggcttcagcttcagccctggacccgtgatcctgctgtggtgctgcctgctgctgcctatcgtgtcctctgccgccgtgtctgtggcccctacagccgccgagaaggtgccagccgagtgccccgagctgaccagaagatgcctgctgggcgaggtgttcgagggcgacaagtacgagagctggctgcggcccctggtcaacgtgaccggcagagatggccccctgagccagctgatccggtacagacccgtgacccccgaggccgccaatagcgtgctgctggacgaggccttcctggataccctggccctgctgtacaacaaccccgaccagctgagagccctgctgaccctgctgtccagcgacaccgcccccagatggatgaccgtgatgcggggctacagcgagtgtggagatggcagccctgccgtgtacacctgcgtggacgacctgtgcagaggctacgacctgaccagactgagctacggccggtccatcttcacagagcacgtgctgggcttcgagctggtgccccccagcctgttcaacgtggtggtggccatccggaacgaggccaccagaaccaacagagccgtgcggctgcctgtgtctacagccgctgcacctgagggcatcacactgttctacggcctgtacaacgccgtgaaagagttctgcctccggcaccagctggatccccccctgctgagacacctggacaagtactacgccggcctgcccccagagctgaagcagaccagagtgaacctgcccgcccacagcagatatggccctcaggccgtggacgccagatgataacgccggcggcccctataactctctacggctaacctgaatggactacgacatagtctagtccgccaagatgagccccaaggacctgacccccttcctgacaaccctgtggctgctcctgggccatagcagagtgcctagagtgcgggccgaggaatgctgcgagttcatcaacgtgaaccacccccccgagcggtgctacgacttcaagatgtgcaaccggttcaccgtggccctgagatgccccgacggcgaagtgtgctacagccccgagaaaaccgccgagatccggggcatcgtgaccaccatgacccacagcctgacccggcaggtggtgcacaacaagctgaccagctgcaactacaaccccctgtacctggaagccgacggccggatcagatgcggcaaagtgaacgacaaggcccagtacctgctgggagccgccggaagcgtgccctaccggtggatcaacctggaatacgacaagatcacccggatcgtgggcctggaccagtacctggaaagcgtgaagaagcacaagcggctggacgtgtgcagagccaagatgggctacatgctgcagtgataaggcgcgccaacgttactggccgaagccgcttggaataaggccggtgtgcgtttgtctatatgttattttccaccatattgccgtcttttggcaatgtgagggcccggaaacctggccctgtcttcttgacgagcattcctaggggtctttcccctctcgccaaaggaatgcaaggtctgttgaatgtcgtgaaggaagcagttcctctggaagcttcttgaagacaaacaacgtctgtagcgaccctttgcaggcagcggaaccccccacctggcgacaggtgcctctgcggccaaaagccacgtgtataagatacacctgcaaaggcggcacaaccccagtgccacgttgtgagttggatagttgtggaaagagtcaaatggctctcctcaagcgtattcaacaaggggctgaaggatgcccagaaggtaccccattgtatgggatctgatctggggcctcggtgcacatgctttacatgtgtttagtcgaggttaaaaaaacgtctaggccccccgaaccacggggacgtggttttcctttgaaaaacacgataatatgctgcggctgctgctgagacaccacttccactgcctgctgctgtgtgccgtgtgggccaccccttgtctggccagcccttggagcaccctgaccgccaaccagaaccctagccccccttggtccaagctgacctacagcaagccccacgacgccgccaccttctactgcccctttctgtaccccagccctcccagaagccccctgcagttcagcggcttccagagagtgtccaccggccctgagtgccggaacgagacactgtacctgctgtacaaccgggagggccagacactggtggagcggagcagcacctgggtgaaaaaagtgatctggtatctgagcggccggaaccagaccatcctgcagcggatgcccagaaccgccagcaagcccagcgacggcaacgtgcagatcagcgtggaggacgccaaaatcttcggagcccacatggtgcccaagcagaccaagctgctgagattcgtggtcaacgacggcaccagatatcagatgtgcgtgatgaagctggaaagctgggcccacgtgttccgggactactccgtgagcttccaggtccggctgaccttcaccgaggccaacaaccagacctacaccttctgcacccaccccaacctgatcgtgtgataagtacctttgtacgcctgttttataccccctccctgatttgcaacttagaagcaacgcaaaccagatcaatagtaggtgtgacataccagtcgcatcttgatcaagcacttctgtatccccggaccgagtatcaatagactgtgcacacggttgaaggagaaaacgtccgttacccggctaactacttcgagaagcctagtaacgccattgaagttgcagagtgtttcgctcagcactccccccgtgtagatcaggtcgatgagtcaccgcattccccacgggcgaccgtggcggtggctgcgttggcggcctgcctatggggtaacccataggacgctctaatacggacatggcgtgaagagtctattgagctagttagtagtcctccggcccctgaatgcggctaatcctaactgcggagcacatacccttaatccaaagggcagtgtgtcgtaacgggcaactctgcagcggaaccgactactttgggtgtccgtgtttctttttattcttgtattggctgcttatggtgacaattaaagaattgttaccatatagctattggattggccatccagtgtcaaacagagctattgtatatctctttgttggattcacacctctcactcttgaaacgttacacaccctcaattacattatactgctgaacacgaagcgcatatgcggctgtgcagagtgtggctgtccgtgtgcctgtgtgccgtggtgctgggccagtgccagagagagacagccgagaagaacgactactaccgggtgccccactactgggatgcctgcagcagagccctgcccgaccagacccggtacaaatacgtggagcagctcgtggacctgaccctgaactaccactacgacgccagccacggcctggacaacttcgacgtgctgaagcggatcaacgtgaccgaggtgtccctgctgatcagcgacttccggcggcagaacagaagaggcggcaccaacaagcggaccaccttcaacgccgctggctctctggcccctcacgccagatccctggaattcagcgtgcggctgttcgccaactgataacgttgcatcctgcaggatacagcagcaattggcaagctgcttacatagaactcgcggcgattggcatgccgccttaaaatttttattttatttttcttttcttttccgaatcggattttgtttttaatatttcaaaaaaaaaaaaaaaaaaaaaaaaaaaaaaaaaaagggtcggcatggcatctccacctcctcgcggtccgacctgggcatccgaaggaggacgcacgtccactcggatggctaagggagagccacgtttaaacgctagagcaagacgtttcccgttgaatatggctcataacaccccttgtattactgtttatgtaagcagacagttttattgttcatgatgatatatttttatcttgtgcaatgtaacatcagagattttgagacacaacgtggctttgttgaataaatcgaacttttgctgagttgaaggatcagatcacgcatcttcccgacaacgcagaccgttccgtggcaaagcaaaagttcaaaatcaccaactggtccacctacaacaaagctctcatcaaccgtggctccctcactttctggctggatgatggggcgattcaggcctggtatgagtcagcaacaccttcttcacgaggcagacctcagcgctagcggagtgtatactggcttactatgttggcactgatgagggtgtcagtgaagtgcttcatgtggcaggagaaaaaaggctgcaccggtgcgtcagcagaatatgtgatacaggatatattccgcttcctcgctcactgactcgctacgctcggtcgttcgactgcggcgagcggaaatggcttacgaacggggcggagatttcctggaagatgccaggaagatacttaacagggaagtgagagggccgcggcaaagccgtttttccataggctccgcccccctgacaagcatcacgaaatctgacgctcaaatcagtggtggcgaaacccgacaggactataaagataccaggcgtttcccctggcggctccctcgtgcgctctcctgttcctgcctttcggtttaccggtgtcattccgctgttatggccgcgtttgtctcattccacgcctgacactcagttccgggtaggcagttcgctccaagctggactgtatgcacgaaccccccgttcagtccgaccgctgcgccttatccggtaactatcgtcttgagtccaacccggaaagacatgcaaaagcaccactggcagcagccactggtaattgatttagaggagttagtcttgaagtcatgcgccggttaaggctaaactgaaaggacaagttttggtgactgcgctcctccaagccagttacctcggttcaaagagttggtagctcagagaaccttcgaaaaaccgccctgcaaggcggttttttcgttttcagagcaagagattacgcgcagaccaaaacgatctcaagaagatcatcttattaaggggtctgacgctcagtggaacgaaaactcacgttaagggattttggtcatgagattatcaaaaaggatcttcacctagatccttttaaattaaaaatgaagttttaaatcaatctaaagtatatatgagtaaacttggtctgacagttattagaaaaattcatccagcagacgataaaacgcaatacgctggctatccggtgccgcaatgccatacagcaccagaaaacgatccgcccattcgccgcccagttcttccgcaatatcacgggtggccagcgcaatatcctgataacgatccgccacgcccagacggccgcaatcaataaagccgctaaaacggccattttccaccataatgttcggcaggcacgcatcaccatgggtcaccaccagatcttcgccatccggcatgctcgctttcagacgcgcaaacagctctgccggtgccaggccctgatgttcttcatccagatcatcctgatccaccaggcccgcttccatacgggtacgcgcacgttcaatacgatgtttcgcctgatgatcaaacggacaggtcgccgggtccagggtatgcagacgacgcatggcatccgccataatgctcactttttctgccggcgccagatggctagacagcagatcctgacccggcacttcgcccagcagcagccaatcacggcccgcttcggtcaccacatccagcaccgccgcacacggaacaccggtggtggccagccagctcagacgcgccgcttcatcctgcagctcgttcagcgcaccgctcagatcggttttcacaaacagcaccggacgaccctgcgcgctcagacgaaacaccgccgcatcagagcagccaatggtctgctgcgcccaatcatagccaaacagacgttccacccacgctgccgggctacccgcatgcaggccatcctgttcaatcatactcttcctttttcaatattattgaagcatttatcagggttattgtctcatgagcggatacatatttgaatgtatttagaaaaataaacaaataggggttccgcgcacatttccccgaaaagtgccacctaaattgtaagcgttaatattttgttaaaattcgcgttaaatttttgttaaatcagctcattttttaaccaataggccgaaatcggcaaaatcccttataaatcaaaagaatagaccgagatagggttgagtggccgctacagggcgctcccattcgccattcaggctgcgcaactgttgggaagggcgtttcggtgcgggcctcttcgctattacgccagctggcgaaagggggatgtgctgcaaggcgattaagttgggtaacgccagggttttcccagtcacacgcgtaatacgactcactatag

SEQ ID NO: 67 - DNA, 16360 bp, Artificial Sequence
  source: /note="Description of Artificial Sequence: Synthetic polynucleotide"
ataggcggcgcatgagagaagcccagaccaattacctacccaaaatggagaaagttcacgttgacatcgaggaagacagcccattcctcagagctttgcagcggagcttcccgcagtttgaggtagaagccaagcaggtcactgataatgaccatgctaatgccagagcgttttcgcatctggcttcaaaactgatcgaaacggaggtggacccatccgacacgatccttgacattggaagtgcgcccgcccgcagaatgtattctaagcacaagtatcattgtatctgtccgatgagatgtgcggaagatccggacagattgtataagtatgcaactaagctgaagaaaaactgtaaggaaataactgataaggaattggacaagaaaatgaaggagctcgccgccgtcatgagcgaccctgacctggaaactgagactatgtgcctccacgacgacgagtcgtgtcgctacgaagggcaagtcgctgtttaccaggatgtatacgcggttgacggaccgacaagtctctatcaccaagccaataagggagttagagtcgcctactggataggctttgacaccaccccttttatgtttaagaacttggctggagcatatccatcatactctaccaactgggccgacgaaaccgtgttaacggctcgtaacataggcctatgcagctctgacgttatggagcggtcacgtagagggatgtccattcttagaaagaagtatttgaaaccatccaacaatgttctattctctgttggctcgaccatctaccacgagaagagggacttactgaggagctggcacctgccgtctgtatttcacttacgtggcaagcaaaattacacatgtcggtgtgagactatagttagttgcgacgggtacgtcgttaaaagaatagctatcagtccaggcctgtatgggaagccttcaggctatgctgctacgatgcaccgcgagggattcttgtgctgcaaagtgacagacacattgaacggggagagggtctcttttcccgtgtgcacgtatgtgccagctacattgtgtgaccaaatgactggcatactggcaacagatgtcagtgcggacgacgcgcaaaaactgctggttgggctcaaccagcgtatagtcgtcaacggtcgcacccagagaaacaccaataccatgaaaaattaccttttgcccgtagtggcccaggcatttgctaggtgggcaaaggaatataaggaagatcaagaagatgaaaggccactaggactacgagatagacagttagtcatggggtgttgttgggcttttagaaggcacaagataacatctatttataagcgcccggatacccaaaccatcatcaaagtgaacagcgatttccactcattcgtgctgcccaggataggcagtaacacattggagatcgggctgagaacaagaatcaggaaaatgttagaggagcacaaggagccgtcacctctcattaccgccgaggacgtacaagaagctaagtgcgcagccgatgaggctaaggaggtgcgtgaagccgaggagttgcgcgcagctctaccacctttggcagctgatgttgaggagcccactctggaagccgatgtagacttgatgttacaagaggctggggccggctcagtggagacacctcgtggcttgataaaggttaccagctacgatggcgaggacaagatcggctcttacgctgtgctttctccgcaggctgtactcaagagtgaaaaattatcttgcatccaccctctcgctgaacaagtcatagtgataacacactctggccgaaaagggcgttatgccgtggaaccataccatggtaaagtagtggtgccagagggacatgcaatacccgtccaggactttcaagctctgagtgaaagtgccaccattgtgtacaacgaacgtgagttcgtaaacaggtacctgcaccatattgccacacatggaggagcgctgaacactgatgaagaatattacaaaactgtcaagcccagcgagcacgacggcgaatacctgtacgacatcgacaggaaacagtgcgtcaagaaagaactagtcactgggctagggctcacaggcgagctggtggatcctcccttccatgaattcgcctacgagagtctgagaacacgaccagccgctccttaccaagtaccaaccataggggtgtatggcgtgccaggatcaggcaagtctggcatcattaaaagcgcagtcaccaaaaaagatctagtggtgagcgccaagaaagaaaactgtgcagaaattataagggacgtcaagaaaatgaaagggctggacgtcaatgccagaactgtggactcagtgctcttgaatggatgcaaacaccccgtagagaccctgtatattgacgaagcttttgcttgtcatgcaggtactctcagagcgctcatagccattataagacctaaaaaggcagtgctctgcggggatcccaaacagtgcggtttttttaacatgatgtgcctgaaagtgcattttaaccacgagatttgcacacaagtcttccacaaaagcatctctcgccgttgcactaaatctgtgacttcggtcgtctcaaccttgttttacgacaaaaaaatgagaacgacgaatccgaaagagactaagattgtgattgacactaccggcagtaccaaacctaagcaggacgatctcattctcacttgtttcagagggtgggtgaagcagttgcaaatagattacaaaggcaacgaaataatgacggcagctgcctctcaagggctgacccgtaaaggtgtgtatgccgttcggtacaaggtgaatgaaaatcctctgtacgcacccacctcagaacatgtgaacgtcctactgacccgcacggaggaccgcatcgtgtggaaaacactagccggcgacccatggataaaaacactgactgccaagtaccctgggaatttcactgccacgatagaggagtggcaagcagagcatgatgccatcatgaggcacatcttggagagaccggaccctaccgacgtcttccagaataaggcaaacgtgtgttgggccaaggctttagtgccggtgctgaagaccgctggcatagacatgaccactgaacaatggaacactgtggattattttgaaacggacaaagctcactcagcagagatagtattgaaccaactatgcgtgaggttctttggactcgatctggactccggtctattttctgcacccactgttccgttatccattaggaataatcactgggataactccccgtcgcctaacatgtacgggctgaataaagaagtggtccgtcagctctctcgcaggtacccacaactgcctcgggcagttgccactggaagagtctatgacatgaacactggtacactgcgcaattatgatccgcgcataaacctagtacctgtaaacagaagactgcctcatgctttagtcctccaccataatgaacacccacagagtgacttttcttcattcgtcagcaaattgaagggcagaactgtcctggtggtcggggaaaagttgtccgtcccaggcaaaatggttgactggttgtcagaccggcctgaggctaccttcagagctcggctggatttaggcatcccaggtgatgtgcccaaatatgacataatatttgttaatgtgaggaccccatataaataccatcactatcagcagtgtgaagaccatgccattaagcttagcatgttgaccaagaaagcttgtctgcatctgaatcccggcggaacctgtgtcagcataggttatggttacgctgacagggccagcgaaagcatcattggtgctatagcgcggcagttcaagttttcccgggtatgcaaaccgaaatcctcacttgaagagacggaagttctgtttgtattcattgggtacgatcgcaaggcccgtacgcacaatccttacaagctttcatcaaccttgaccaacatttatacaggttccagactccacgaagccggatgtgcaccctcatatcatgtggtgcgaggggatattgccacggccaccgaaggagtgattataaatgctgctaacagcaaaggacaacctggcggaggggtgtgcggagcgctgtataagaaattcccggaaagcttcgatttacagccgatcgaagtaggaaaagcgcgactggtcaaaggtgcagctaaacatatcattcatgccgtaggaccaaacttcaacaaagtttcggaggttgaaggtgacaaacagttggcagaggcttatgagtccatcgctaagattgtcaacgataacaattacaagtcagtagcgattccactgttgtccaccggcatcttttccgggaacaaagatcgactaacccaatcattgaaccatttgctgacagctttagacaccactgatgcagatgtagccatatactgcagggacaagaaatgggaaatgactctcaaggaagcagtggctaggagagaagcagtggaggagatatgcatatccgacgactcttcagtgacagaacctgatgcagagctggtgagggtgcatccgaagagttctttggctggaaggaagggctacagcacaagcgatggcaaaactttctcatatttggaagggaccaagtttcaccaggcggccaaggatatagcagaaattaatgccatgtggcccgttgcaacggaggccaatgagcaggtatgcatgtatatcctcggagaaagcatgagcagtattaggtcgaaatgccccgtcgaagagtcggaagcctccacaccacctagcacgctgccttgcttgtgcatccatgccatgactccagaaagagtacagcgcctaaaagcctcacgtccagaacaaattactgtgtgctcatcctttccattgccgaagtatagaatcactggtgtgcagaagatccaatgctcccagcctatattgttctcaccgaaagtgcctgcgtatattcatccaaggaagtatctcgtggaaacaccaccggtagacgagactccggagccatcggcagagaaccaatccacagaggggacacctgaacaaccaccacttataaccgaggatgagaccaggactagaacgcctgagccgatcatcatcgaagaggaagaagaggatagcataagtttgctgtcagatggcccgacccaccaggtgctgcaagtcgaggcagacattcacgggccgccctctgtatctagctcatcctggtccattcctcatgcatccgactttgatgtggacagtttatccatacttgacaccctggagggagctagcgtgaccagcggggcaacgtcagccgagactaactcttacttcgcaaagagtatggagtttctggcgcgaccggtgcctgcgcctcgaacagtattcaggaaccctccacatcccgctccgcgcacaagaacaccgtcacttgcacccagcagggcctgctcgagaaccagcctagtttccaccccgccaggcgtgaatagggtgatcactagagaggagctcgaggcgcttaccccgtcacgcactcctagcaggtcggtctcgagaaccagcctggtctccaacccgccaggcgtaaatagggtgattacaagagaggagtttgaggcgttcgtagcacaacaacaatgacggtttgatgcgggtgcatacatcttttcctccgacaccggtcaagggcatttacaacaaaaatcagtaaggcaaacggtgctatccgaagtggtgttggagaggaccgaattggagatttcgtatgccccgcgcctcgaccaagaaaaagaagaattactacgcaagaaattacagttaaatcccacacctgctaacagaagcagataccagtccaggaaggtggagaacatgaaagccataacagctagacgtattctgcaaggcctagggcattatttgaaggcagaaggaaaagtggagtgctaccgaaccctgcatcctgttcctttgtattcatctagtgtgaaccgtgccttttcaagccccaaggtcgcagtggaagcctgtaacgccatgttgaaagagaactttccgactgtggcttcttactgtattattccagagtacgatgcctatttggacatggttgacggagcttcatgctgcttagacactgccagtttttgccctgcaaagctgcgcagctttccaaagaaacactcctatttggaacccacaatacgatcggcagtgccttcagcgatccagaacacgctccagaacgtcctggcagctgccacaaaaagaaattgcaatgtcacgcaaatgagagaattgcccgtattggattcggcggcctttaatgtggaatgcttcaagaaatatgcgtgtaataatgaatattgggaaacgtttaaagaaaaccccatcaggcttactgaagaaaacgtggtaaattacattaccaaattaaaaggaccaaaagctgctgctctttttgcgaagacacataatttgaatatgttgcaggacataccaatggacaggtttgtaatggacttaaagagagacgtgaaagtgactccaggaacaaaacatactgaagaacggcccaaggtacaggtgatccaggctgccgatccgctagcaacagcgtatctgtgcggaatccaccgagagctggttaggagattaaatgcggtcctgcttccgaacattcatacactgtttgatatgtcggctgaagactttgacgctattatagccgagcacttccagcctggggattgtgttctggaaactgacatcgcgtcgtttgataaaagtgaggacgacgccatggctctgaccgcgttaatgattctggaagacttaggtgtggacgcagagctgttgacgctgattgaggcggctttcggcgaaatttcatcaatacatttgcccactaaaactaaatttaaattcggagccatgatgaaatctggaatgttcctcacactgtttgtgaacacagtcattaacattgtaatcgcaagcagagtgttgagagaacggctaaccggatcaccatgtgcagcattcattggagatgacaatatcgtgaaaggagtcaaatcggacaaattaatggcagacaggtgcgccacctggttgaatatggaagtcaagattatagatgctgtggtgggcgagaaagcgccttatttctgtggagggtttattttgtgtgactccgtgaccggcacagcgtgccgtgtggcagaccccctaaaaaggctgtttaagcttggcaaacctctggcagcagacgatgaacatgatgatgacaggagaagggcattgcatgaagagtcaacacgctggaaccgagtgggtattctttcagagctgtgcaaggcagtagaatcaaggtatgaaaccgtaggaacttccatcatagttatggccatgactactctagctagcagtgttaaatcattcagctacctgagaggggcccctataactctctacggctaacctgaatggactacgacatagtctagtccgccaagatgaggcctggcctgccctcctacctgatcatcctggccgtgtgcctgttcagccacctgctgtccagcagatacggcgccgaggccgtgagcgagcccctggacaaggctttccacctgctgctgaacacctacggcagacccatccggtttctgcgggagaacaccacccagtgcacctacaacagcagcctgcggaacagcaccgtcgtgagagagaacgccatcagcttcaactttttccagagctacaaccagtactacgtgttccacatgcccagatgcctgtttgccggccctctggccgagcagttcctgaaccaggtggacctgaccgagacactggaaagataccagcagcggctgaatacctacgccctggtgtccaaggacctggccagctaccggtcctttagccagcagctcaaggctcaggatagcctcggcgagcagcctaccaccgtgccccctcccatcgacctgagcatcccccacgtgtggatgcctccccagaccacccctcacggctggaccgagagccacaccacctccggcctgcacagaccccacttcaaccagacctgcatcctgttcgacggccacgacctgctgtttagcaccgtgaccccctgcctgcaccagggcttctacctgatcgacgagctgagatacgtgaagatcaccctgaccgaggatttcttcgtggtcaccgtgtccatcgacgacgacacccccatgctgctgatcttcggccacctgcccagagtgctgttcaaggccccctaccagcgggacaacttcatcctgcggcagaccgagaagcacgagctgctggtgctggtcaagaaggaccagctgaaccggcactcctacctgaaggaccccgacttcctggacgccgccctggacttcaactacctggacctgagcgccctgctgagaaacagcttccacagatacgccgtggacgtgctgaagtccggacggtgccagatgctcgatcggcggaccgtggagatggccttcgcctatgccctcgccctgttcgccgctgccagacaggaagaggctggcgcccaggtgtcagtgcccagagccctggatagacaggccgccctgctgcagatccaggaattcatgatcacctgcctgagccagaccccccctagaaccaccctgctgctgtaccccacagccgtggatctggccaagagggccctgtggacccccaaccagatcaccgacatcacaagcctcgtgcggctcgtgtacatcctgagcaagcagaaccagcagcacctgatcccccagtgggccctgagacagatcgccgacttcgccctgaagctgcacaagacccatctggccagctttctgagcgccttcgccaggcaggaactgtacctgatgggcagcctggtccacagcatgctggtgcataccaccgagcggcgggagatcttcatcgtggagacaggcctgtgtagcctggccgagctgtcccactttacccagctgctggcccaccctcaccacgagtacctgagcgacctgtacaccccctgcagcagcagcggcagacgggaccacagcctggaacggctgaccagactgttccccgatgccaccgtgcctgctacagtgcctgccgccctgtccatcctgtccaccatgcagcccagcaccctggaaaccttccccgacctgttctgcctgcccctgggcgagagctttagcgccctgaccgtgtccgagcacgtgtcctacatcgtgaccaatcagtacctgatcaagggcatcagctaccccgtgtccaccacagtcgtgggccagagcctgatcatcacccagaccgacagccagaccaagtgcgagctgacccggaacatgcacaccacacacagcatcaccgtggccctgaacatcagcctggaaaactgcgctttctgtcagtctgccctgctggaatacgacgatacccagggcgtgatcaacatcatgtacatgcacgacagcgacgacgtgctgttcgccctggacccctacaacgaggtggtggtgtccagcccccggacccactacctgatgctgctgaagaacggcaccgtgctggaagtgaccgacgtggtggtggacgccaccgacggcagcggatctgggtcccaccatcaccatcaccattgataatctagaggcccctataactctctacggctaacctgaatggactacgacatagtctagtccgccaagatgtgcagaaggcccgactgcggcttcagcttcagccctggacccgtgatcctgctgtggtgctgcctgctgctgcctatcgtgtcctctgccgccgtgtctgtggcccctacagccgccgagaaggtgccagccgagtgccccgagctgaccagaagatgcctgctgggcgaggtgttcgagggcgacaagtacgagagctggctgcggcccctggtcaacgtgaccggcagagatggccccctgagccagctgatccggtacagacccgtgacccccgaggccgccaatagcgtgctgctggacgaggccttcctggataccctggccctgctgtacaacaaccccgaccagctgagagccctgctgaccctgctgtccagcgacaccgcccccagatggatgaccgtgatgcggggctacagcgagtgtggagatggcagccctgccgtgtacacctgcgtggacgacctgtgcagaggctacgacctgaccagactgagctacggccggtccatcttcacagagcacgtgctgggcttcgagctggtgccccccagcctgttcaacgtggtggtggccatccggaacgaggccaccagaaccaacagagccgtgcggctgcctgtgtctacagccgctgcacctgagggcatcacactgttctacggcctgtacaacgccgtgaaagagttctgcctccggcaccagctggatccccccctgctgagacacctggacaagtactacgccggcctgcccccagagctgaagcagaccagagtgaacctgcccgcccacagcagatatggccctcaggccgtggacgccagatgataacgccggcggcccctataactctctacggctaacctgaatggactacgacatagtctagtccgccaagatgagccccaaggacctgacccccttcctgacaaccctgtggctgctcctgggccatagcagagtgcctagagtgcgggccgaggaatgctgcgagttcatcaacgtgaaccacccccccgagcggtgctacgacttcaagatgtgcaaccggttcaccgtggccctgagatgccccgacggcgaagtgtgctacagccccgagaaaaccgccgagatccggggcatcgtgaccaccatgacccacagcctgacccggcaggtggtgcacaacaagctgaccagctgcaactacaaccccctgtacctggaagccgacggccggatcagatgcggcaaagtgaacgacaaggcccagtacctgctgggagccgccggaagcgtgccctaccggtggatcaacctggaatacgacaagatcacccggatcgtgggcctggaccagtacctggaaagcgtgaagaagcacaagcggctggacgtgtgcagagccaagatgggctacatgctgcagtgataaggcgcgccaacgttactggccgaagccgcttggaataaggccggtgtgcgtttgtctatatgttattttccaccatattgccgtcttttggcaatgtgagggcccggaaacctggccctgtcttcttgacgagcattcctaggggtctttcccctctcgccaaaggaatgcaaggtctgttgaatgtcgtgaaggaagcagttcctctggaagcttcttgaagacaaacaacgtctgtagcgaccctttgcaggcagcggaaccccccacctggcgacaggtgcctctgcggccaaaagccacgtgtataagatacacctgcaaaggcggcacaaccccagtgccacgttgtgagttggatagttgtggaaagagtcaaatggctctcctcaagcgtattcaacaaggggctgaaggatgcccagaaggtaccccattgtatgggatctgatctggggcctcggtgcacatgctttacatgtgtttagtcgaggttaaaaaaacgtctaggccccccgaaccacggggacgtggttttcctttgaaaaacacgataatatgctgcggctgctgctgagacaccacttccactgcctgctgctgtgtgccgtgtgggccaccccttgtctggccagcccttggagcaccctgaccgccaaccagaaccctagccccccttggtccaagctgacctacagcaagccccacgacgccgccaccttctactgcccctttctgtaccccagccctcccagaagccccctgcagttcagcggcttccagagagtgtccaccggccctgagtgccggaacgagacactgtacctgctgtacaaccgggagggccagacactggtggagcggagcagcacctgggtgaaaaaagtgatctggtatctgagcggccggaaccagaccatcctgcagcggatgcccagaaccgccagcaagcccagcgacggcaacgtgcagatcagcgtggaggacgccaaaatcttcggagcccacatggtgcccaagcagaccaagctgctgagattcgtggtcaacgacggcaccagatatcagatgtgcgtgatgaagctggaaagctgggcccacgtgttccgggactactccgtgagcttccaggtccggctgaccttcaccgaggccaacaaccagacctacaccttctgcacccaccccaacctgatcgtgtgataagtacctttgtacgcctgttttataccccctccctgatttgcaacttagaagcaacgcaaaccagatcaatagtaggtgtgacataccagtcgcatcttgatcaagcacttctgtatccccggaccgagtatcaatagactgtgcacacggttgaaggagaaaacgtccgttacccggctaactacttcgagaagcctagtaacgccattgaagttgcagagtgtttcgctcagcactccccccgtgtagatcaggtcgatgagtcaccgcattccccacgggcgaccgtggcggtggctgcgttggcggcctgcctatggggtaacccataggacgctctaatacggacatggcgtgaagagtctattgagctagttagtagtcctccggcccctgaatgcggctaatcctaactgcggagcacatacccttaatccaaagggcagtgtgtcgtaacgggcaactctgcagcggaaccgactactttgggtgtccgtgtttctttttattcttgtattggctgcttatggtgacaattaaagaattgttaccatatagctattggattggccatccagtgtcaaacagagctattgtatatctctttgttggattcacacctctcactcttgaaacgttacacaccctcaattacattatactgctgaacacgaagcgcatatgcggctgtgcagagtgtggctgtccgtgtgcctgtgtgccgtggtgctgggccagtgccagagagagacagccgagaagaacgactactaccgggtgccccactactgggatgcctgcagcagagccctgcccgaccagacccggtacaaatacgtggagcagctcgtggacctgaccctgaactaccactacgacgccagccacggcctggacaacttcgacgtgctgaagcggatcaacgtgaccgaggtgtccctgctgatcagcgacttccggcggcagaacagaagaggcggcaccaacaagcggaccaccttcaacgccgctggctctctggcccctcacgccagatccctggaattcagcgtgcggctgttcgccaactgataacgttgcatcctgcaggatacagcagcaattggcaagctgcttacatagaactcgcggcgattggcatgccgccttaaaatttttattttatttttcttttcttttccgaatcggattttgtttttaatatttcaaaaaaaaaaaaaaaaaaaaaaaaaaaaaaaaaaagggtcggcatggcatctccacctcctcgcggtccgacctgggcatccgaaggaggacgcacgtccactcggatggctaagggagagccacgtttaaacgctagagcaagacgtttcccgttgaatatggctcataacaccccttgtattactgtttatgtaagcagacagttttattgttcatgatgatatatttttatcttgtgcaatgtaacatcagagattttgagacacaacgtggctttgttgaataaatcgaacttttgctgagttgaaggatcagatcacgcatcttcccgacaacgcagaccgttccgtggcaaagcaaaagttcaaaatcaccaactggtccacctacaacaaagctctcatcaaccgtggctccctcactttctggctggatgatggggcgattcaggcctggtatgagtcagcaacaccttcttcacgaggcagacctcagcgctagcggagtgtatactggcttactatgttggcactgatgagggtgtcagtgaagtgcttcatgtggcaggagaaaaaaggctgcaccggtgcgtcagcagaatatgtgatacaggatatattccgcttcctcgctcactgactcgctacgctcggtcgttcgactgcggcgagcggaaatggcttacgaacggggcggagatttcctggaagatgccaggaagatacttaacagggaagtgagagggccgcggcaaagccgtttttccataggctccgcccccctgacaagcatcacgaaatctgacgctcaaatcagtggtggcgaaacccgacaggactataaagataccaggcgtttcccctggcggctccctcgtgcgctctcctgttcctgcctttcggtttaccggtgtcattccgctgttatggccgcgtttgtctcattccacgcctgacactcagttccgggtaggcagttcgctccaagctggactgtatgcacgaaccccccgttcagtccgaccgctgcgccttatccggtaactatcgtcttgagtccaacccggaaagacatgcaaaagcaccactggcagcagccactggtaattgatttagaggagttagtcttgaagtcatgcgccggttaaggctaaactgaaaggacaagttttggtgactgcgctcctccaagccagttacctcggttcaaagagttggtagctcagagaaccttcgaaaaaccgccctgcaaggcggttttttcgttttcagagcaagagattacgcgcagaccaaaacgatctcaagaagatcatcttattaaggggtctgacgctcagtggaacgaaaactcacgttaagggattttggtcatgagattatcaaaaaggatcttcacctagatccttttaaattaaaaatgaagttttaaatcaatctaaagtatatatgagtaaacttggtctgacagttattagaaaaattcatccagcagacgataaaacgcaatacgctggctatccggtgccgcaatgccatacagcaccagaaaacgatccgcccattcgccgcccagttcttccgcaatatcacgggtggccagcgcaatatcctgataacgatccgccacgcccagacggccgcaatcaataaagccgctaaaacggccattttccaccataatgttcggcaggcacgcatcaccatgggtcaccaccagatcttcgccatccggcatgctcgctttcagacgcgcaaacagctctgccggtgccaggccctgatgttcttcatccagatcatcctgatccaccaggcccgcttccatacgggtacgcgcacgttcaatacgatgtttcgcctgatgatcaaacggacaggtcgccgggtccagggtatgcagacgacgcatggcatccgccataatgctcactttttctgccggcgccagatggctagacagcagatcctgacccggcacttcgcccagcagcagccaatcacggcccgcttcggtcaccacatccagcaccgccgcacacggaacaccggtggtggccagccagctcagacgcgccgcttcatcctgcagctcgttcagcgcaccgctcagatcggttttcacaaacagcaccggacgaccctgcgcgctcagacgaaacaccgccgcatcagagcagccaatggtctgctgcgcccaatcatagccaaacagacgttccacccacgctgccgggctacccgcatgcaggccatcctgttcaatcatactcttcctttttcaatattattgaagcatttatcagggttattgtctcatgagcggatacatatttgaatgtatttagaaaaataaacaaataggggttccgcgcacatttccccgaaaagtgccacctaaattgtaagcgttaatattttgttaaaattcgcgttaaatttttgttaaatcagctcattttttaaccaataggccgaaatcggcaaaatcccttataaatcaaaagaatagaccgagatagggttgagtggccgctacagggcgctcccattcgccattcaggctgcgcaactgttgggaagggcgtttcggtgcgggcctcttcgctattacgccagctggcgaaagggggatgtgctgcaaggcgattaagttgggtaacgccagggttttcccagtcacacgcgtaatacgactcactatag

SEQ ID NO: 68 - protein, 868 aa, Varicella zoster virus
MFVTAVVSVSPSSFYESLQVEPTQSEDITRSAHLGDGDEIREAIHKSQDAETKPTFYVCPPPTGSTIVRLEPPRTCPDYHLGKNFTEGIAVVYKENIAAYKFKATVYYKDVIVSTAWAGSSYTQITNRYADRVPIPVSEITDTIDKFGKCSSKATYVRNNHKVEAFNEDKNPQDMPLIASKYNSVGSKAWHTTNDTYMVAGTPGTYRTGTSVNCIIEEVEARSIFPYDSFGLSTGDIIYMSPFFGLRDGAYREHSNYAMDRFHQFEGYRQRDLDTRALLEPAARNFLVTPHLTVGWNWKPKRTEVCSLVKWREVEDVVRDEYAHNFRFTMKTLSTTFISETNEFNLNQIHLSQCVKEEARAIINRIYTTRYNSSHVRTGDIQTYLARGGFVVVFQPLLSNSLARLYLQELVRENTNHSPQKHPTRNTRSRRSVPVELRANRTITTTSSVEFAMLQFTYDHIQEHVNEMLARISSSWCQLQNRERALWSGLFPINPSALASTILDQRVKARILGDVISVSNCPELGSDTRIILQNSMRVSGSTTRCYSRPLISIVSLNGSGTVEGQLGTDNELIMSRDLLEPCVANHKRYFLFGHHYVYYEDYRYVREIAVHDVGMISTYVDLNLTLLKDREFMPLQVYTRDELRDTGLLDYSEIQRRNQMHSLRFYDIDKVVQYDSGTAIMQGMAQFFQGLGTAGQAVGHVVLGATGALLSTVHGFTTFLSNPFGALAVGLLVLAGLVAAFFAYRYVLKLKTSPMKALYPLTTKGLKQLPEGMDPFAEKPNATDTPIEEIGDSQNTEPSVNSGFDPDKFREAQEMIKYMTLVSAAERQESKARKKNKTSALLTSRLTGLALRNRRGYSRVRTENVTGV

SEQ ID NO: 69 - protein, 841 aa, Varicella zoster virus
MFALVLAVVILPLWTTANKSYVTPTPATRSIGHMSALLREYSDRNMSLKLEAFYPTGFDEELIKSLHWGNDRKHVFLVIVKVNPTTHEGDVGLVIFPKYLLSPYHFKAEHRAPFPAGRFGFLSHPVTPDVSFFDSSFAPYLTTQHLVAFTTFPPNPLVWHLERAETAATAERPFGVSLLPARPTVPKNTILEHKAHFATWDALARHTFFSAEAIITNSTLRIHVPLFGSVWPIRYWATGSVLLTSDSGRVEVNIGVGFMSSLISLSSGLPIELIVVPHTVKLNAVTSDTTWFQLNPPGPDPGPSYRVYLLGRGLDMNFSKHATVDICAYPEESLDYRYHLSMAHTEALRMTTKADQHDINEESYYHIAARIATSIFALSEMGRTTEYFLLDEIVDVQYQLKFLNYILMRIGAGAHPNTISGTSDLIFADPSQLHDELSLLFGQVKPANVDYFISYDEARDQLKTAYALSRGQDHVNALSLARRVIMSIYKGLLVKQNLNATERQALFFASMILLNFREGLENSSRVLDGRTTLLLMTSMCTAAHATQAALNIQEGLAYLNPSKHMFTIPNVYSPCMGSLRTDLTEEIHVMNLLSAIPTRPGLNEVLHTQLDESEIFDAAFKTMMIFTTWTAKDLHILHTHVPEVFTCQDAAARNGEYVLILPAVQGHSYVITRNKPQRGLVYSLADVDVYNPISVVYLSKDTCVSEHGVIETVALPHPDNLKECLYCGSVFLRYLTTGAIMDIIIIDSKDTERQLAAMGNSTIPPFNPDMHGDDSKAVLLFPNGTVVTLLGFERRQAIRMSGQYLGASLGGAFLAVVGFGIIGWMLCGNSRLREYNKIPLT

SEQ ID NO: 70 - protein, 160 aa, Varicella zoster virus
MASHKWLLQMIVFLKTITIAYCLHLQDDTPLFFGAKPLSDVSLIITEPCVSSVYEAWDYAAPPVSNLSEALSGIVVKTKCPVPEVILWFKDKQMAYWTNPYVTLKGLTQSVGEEHKSGDIRDALLDALSGVWVDSTPSSTNIPENGCVWGADRLFQRVCQ

SEQ ID NO: 71 - protein, 354 aa, Varicella zoster virus
MFLIQCLISAVIFYIQVTNALIFKGDHVSLQVNSSLTSILIPMQNDNYTEIKGQLVFIGEQLPTGTNYSGTLELLYADTVAFCFRSVQVIRYDGCPRIRTSAFISCRYKHSWHYGNSTDRISTEPDAGVMLKITKPGINDAGVYVLLVRLDHSRSTDGFILGVNVYTAGSHHNIHGVIYTSPSLQNGYSTRALFQQARLCDLPATPKGSGTSLFQHMLDLRAGKSLEDNPWLHEDVVTTETKSVVKEGIENHVYPTDMSTLPEKSLNDPPENLLIIIPIVASVMILTAMVIVIVISVKRRRIKKHPIYRPNTKTRRGIQNATPESDVMLEAAIAQLATIREESPPHSVVNPFVK

SEQ ID NO: 72 - protein, 623 aa, Varicella zoster virus
MGTVNKPVVGVLMGFGIITGTLRITNPVRASVLRYDDFHIDEDKLDTNSVYEPYYHSDHAESSWVNRGESSRKAYDHNSPYIWPRNDYDGFLENAHEHHGVYNQGRGIDSGERLMQPTQMSAQEDLGDDTGIHVIPTLNGDDRHKIVNVDQRQYGDVFKGDLNPKPQGQRLIEVSVEENHPFTLRAPIQRIYGVRYTETWSFLPSLTCTGDAAPAIQHICLKHTTCFQDVVVDVDCAENTKEDQLAEISYRFQGKKEADQPWIVVNTSTLFDELELDPPEIEPGVLKVLRTEKQYLGVYIWNMRGSDGTSTYATFLVTWKGDEKTRNPTPAVTPQPRGAEFHMWNYHSHVFSVGDTFSLAMHLQYKIHEAPFDLLLEWLYVPIDPTCQPMRLYSTCLYHPNAPQCLSHMNSGCTFTSPHLAQRVASTVYQNCEHADNYTAYCLGISHMEPSFGLILHDGGTTLKFVDTPESLSGLYVFVVYFNGHVEAVAYTVVSTVDHFVNAIEERGFPPTAGQPPATTKPKEITPVNPGTSPLLRYAAWTGGLAAVVLLCLVIFLICTAKRMRVKAYRVDKSPYNQSMYYAGLPVDDFEDSESTDTEEEFGNAIGGSHGGSSYTVYIDKTR

SEQ ID NO: 73 - DNA, 13339 bp, Artificial Sequence
  source: /note="Description of Artificial Sequence: Synthetic polynucleotide"
ataggcggcgcatgagagaagcccagaccaattacctacccaaaatggagaaagttcacgttgacatcgaggaagacagcccattcctcagagctttgcagcggagcttcccgcagtttgaggtagaagccaagcaggtcactgataatgaccatgctaatgccagagcgttttcgcatctggcttcaaaactgatcgaaacggaggtggacccatccgacacgatccttgacattggaagtgcgcccgcccgcagaatgtattctaagcacaagtatcattgtatctgtccgatgagatgtgcggaagatccggacagattgtataagtatgcaactaagctgaagaaaaactgtaaggaaataactgataaggaattggacaagaaaatgaaggagctcgccgccgtcatgagcgaccctgacctggaaactgagactatgtgcctccacgacgacgagtcgtgtcgctacgaagggcaagtcgctgtttaccaggatgtatacgcggttgacggaccgacaagtctctatcaccaagccaataagggagttagagtcgcctactggataggctttgacaccaccccttttatgtttaagaacttggctggagcatatccatcatactctaccaactgggccgacgaaaccgtgttaacggctcgtaacataggcctatgcagctctgacgttatggagcggtcacgtagagggatgtccattcttagaaagaagtatttgaaaccatccaacaatgttctattctctgttggctcgaccatctaccacgagaagagggacttactgaggagctggcacctgccgtctgtatttcacttacgtggcaagcaaaattacacatgtcggtgtgagactatagttagttgcgacgggtacgtcgttaaaagaatagctatcagtccaggcctgtatgggaagccttcaggctatgctgctacgatgcaccgcgagggattcttgtgctgcaaagtgacagacacattgaacggggagagggtctcttttcccgtgtgcacgtatgtgccagctacattgtgtgaccaaatgactggcatactggcaacagatgtcagtgcggacgacgcgcaaaaactgctggttgggctcaaccagcgtatagtcgtcaacggtcgcacccagagaaacaccaataccatgaaaaattaccttttgcccgtagtggcccaggcatttgctaggtgggcaaaggaatataaggaagatcaagaagatgaaaggccactaggactacgagatagacagttagtcatggggtgttgttgggcttttagaaggcacaagataacatctatttataagcgcccggatacccaaaccatcatcaaagtgaacagcgatttccactcattcgtgctgcccaggataggcagtaacacattggagatcgggctgagaacaagaatcaggaaaatgttagaggagcacaaggagccgtcacctctcattaccgccgaggacgtacaagaagctaagtgcgcagccgatgaggctaaggaggtgcgtgaagccgaggagttgcgcgcagctctaccacctttggcagctgatgttgaggagcccactctggaagccgatgtagacttgatgttacaagaggctggggccggctcagtggagacacctcgtggcttgataaaggttaccagctacgatggcgaggacaagatcggctcttacgctgtgctttctccgcaggctgtactcaagagtgaaaaattatcttgcatccaccctctcgctgaacaagtcatagtgataacacactctggccgaaaagggcgttatgccgtggaaccataccatggtaaagtagtggtgccagagggacatgcaatacccgtccaggactttcaagctctgagtgaaagtgccaccattgtgtacaacgaacgtgagttcgtaaacaggtacctgcaccatattgccacacatggaggagcgctgaacactgatgaagaatattacaaaactgtcaagcccagcgagcacgacggcgaatacctgtacgacatcgacaggaaacagtgcgtcaagaaagaactagtcactgggctagggctcacaggcgagctggtggatcctcccttccatgaattcgcctacgagagtctgagaacacgaccagccgctccttaccaagtaccaaccataggggtgtatggcgtgccaggatcaggcaagtctggcatcattaaaagcgcagtcaccaaaaaagatctagtggtgagcgccaagaaagaaaactgtgcagaaattataagggacgtcaagaaaatgaaagggctggacgtcaatgccagaactgtggactcagtgctcttgaatggatgcaaacaccccgtagagaccctgtatattgacgaagcttttgcttgtcatgcaggtactctcagagcgctcatagccattataagacctaaaaaggcagtgctctgcggggatcccaaacagtgcggtttttttaacatgatgtgcctgaaagtgcattttaaccacgagatttgcacacaagtcttccacaaaagcatctctcgccgttgcactaaatctgtgacttcggtcgtctcaaccttgttttacgacaaaaaaatgagaacgacgaatccgaaagagactaagattgtgattgacactaccggcagtaccaaacctaagcaggacgatctcattctcacttgtttcagagggtgggtgaagcagttgcaaatagattacaaaggcaacgaaataatgacggcagctgcctctcaagggctgacccgtaaaggtgtgtatgccgttcggtacaaggtgaatgaaaatcctctgtacgcacccacctcagaacatgtgaacgtcctactgacccgcacggaggaccgcatcgtgtggaaaacactagccggcgacccatggataaaaacactgactgccaagtaccctgggaatttcactgccacgatagaggagtggcaagcagagcatgatgccatcatgaggcacatcttggagagaccggaccctaccgacgtcttccagaataaggcaaacgtgtgttgggccaaggctttagtgccggtgctgaagaccgctggcatagacatgaccactgaacaatggaacactgtggattattttgaaacggacaaagctcactcagcagagatagtattgaaccaactatgcgtgaggttctttggactcgatctggactccggtctattttctgcacccactgttccgttatccattaggaataatcactgggataactccccgtcgcctaacatgtacgggctgaataaagaagtggtccgtcagctctctcgcaggtacccacaactgcctcgggcagttgccactggaagagtctatgacatgaacactggtacactgcgcaattatgatccgcgcataaacctagtacctgtaaacagaagactgcctcatgctttagtcctccaccataatgaacacccacagagtgacttttcttcattcgtcagcaaattgaagggcagaactgtcctggtggtcggggaaaagttgtccgtcccaggcaaaatggttgactggttgtcagaccggcctgaggctaccttcagagctcggctggatttaggcatcccaggtgatgtgcccaaatatgacataatatttgttaatgtgaggaccccatataaataccatcactatcagcagtgtgaagaccatgccattaagcttagcatgttgaccaagaaagcttgtctgcatctgaatcccggcggaacctgtgtcagcataggttatggttacgctgacagggccagcgaaagcatcattggtgctatagcgcggcagttcaagttttcccgggtatgcaaaccgaaatcctcacttgaagagacggaagttctgtttgtattcattgggtacgatcgcaaggcccgtacgcacaatccttacaagctttcatcaaccttgaccaacatttatacaggttccagactccacgaagccggatgtgcaccctcatatcatgtggtgcgaggggatattgccacggccaccgaaggagtgattataaatgctgctaacagcaaaggacaacctggcggaggggtgtgcggagcgctgtataagaaattcccggaaagcttcgatttacagccgatcgaagtaggaaaagcgcgactggtcaaaggtgcagctaaacatatcattcatgccgtaggaccaaacttcaacaaagtttcggaggttgaaggtgacaaacagttggcagaggcttatgagtccatcgctaagattgtcaacgataacaattacaagtcagtagcgattccactgttgtccaccggcatcttttccgggaacaaagatcgactaacccaatcattgaaccatttgctgacagctttagacaccactgatgcagatgtagccatatactgcagggacaagaaatgggaaatgactctcaaggaagcagtggctaggagagaagcagtggaggagatatgcatatccgacgactcttcagtgacagaacctgatgcagagctggtgagggtgcatccgaagagttctttggctggaaggaagggctacagcacaagcgatggcaaaactttctcatatttggaagggaccaagtttcaccaggcggccaaggatatagcagaaattaatgccatgtggcccgttgcaacggaggccaatgagcaggtatgcatgtatatcctcggagaaagcatgagcagtattaggtcgaaatgccccgtcgaagagtcggaagcctccacaccacctagcacgctgccttgcttgtgcatccatgccatgactccagaaagagtacagcgcctaaaagcctcacgtccagaacaaattactgtgtgctcatcctttccattgccgaagtatagaatcactggtgtgcagaagatccaatgctcccagcctatattgttctcaccgaaagtgcctgcgtatattcatccaaggaagtatctcgtggaaacaccaccggtagacgagactccggagccatcggcagagaaccaatccacagaggggacacctgaacaaccaccacttataaccgaggatgagaccaggactagaacgcctgagccgatcatcatcgaagaggaagaagaggatagcataagtttgctgtcagatggcccgacccaccaggtgctgcaagtcgaggcagacattcacgggccgccctctgtatctagctcatcctggtccattcctcatgcatccgactttgatgtggacagtttatccatacttgacaccctggagggagctagcgtgaccagcggggcaacgtcagccgagactaactcttacttcgcaaagagtatggagtttctggcgcgaccggtgcctgcgcctcgaacagtattcaggaaccctccacatcccgctccgcgcacaagaacaccgtcacttgcacccagcagggcctgctcgagaaccagcctagtttccaccccgccaggcgtgaatagggtgatcactagagaggagctcgaggcgcttaccccgtcacgcactcctagcaggtcggtctcgagaaccagcctggtctccaacccgccaggcgtaaatagggtgattacaagagaggagtttgaggcgttcgtagcacaacaacaatgacggtttgatgcgggtgcatacatcttttcctccgacaccggtcaagggcatttacaacaaaaatcagtaaggcaaacggtgctatccgaagtggtgttggagaggaccgaattggagatttcgtatgccccgcgcctcgaccaagaaaaagaagaattactacgcaagaaattacagttaaatcccacacctgctaacagaagcagataccagtccaggaaggtggagaacatgaaagccataacagctagacgtattctgcaaggcctagggcattatttgaaggcagaaggaaaagtggagtgctaccgaaccctgcatcctgttcctttgtattcatctagtgtgaaccgtgccttttcaagccccaaggtcgcagtggaagcctgtaacgccatgttgaaagagaactttccgactgtggcttcttactgtattattccagagtacgatgcctatttggacatggttgacggagcttcatgctgcttagacactgccagtttttgccctgcaaagctgcgcagctttccaaagaaacactcctatttggaacccacaatacgatcggcagtgccttcagcgatccagaacacgctccagaacgtcctggcagctgccacaaaaagaaattgcaatgtcacgcaaatgagagaattgcccgtattggattcggcggcctttaatgtggaatgcttcaagaaatatgcgtgtaataatgaatattgggaaacgtttaaagaaaaccccatcaggcttactgaagaaaacgtggtaaattacattaccaaattaaaaggaccaaaagctgctgctctttttgcgaagacacataatttgaatatgttgcaggacataccaatggacaggtttgtaatggacttaaagagagacgtgaaagtgactccaggaacaaaacatactgaagaacggcccaaggtacaggtgatccaggctgccgatccgctagcaacagcgtatctgtgcggaatccaccgagagctggttaggagattaaatgcggtcctgcttccgaacattcatacactgtttgatatgtcggctgaagactttgacgctattatagccgagcacttccagcctggggattgtgttctggaaactgacatcgcgtcgtttgataaaagtgaggacgacgccatggctctgaccgcgttaatgattctggaagacttaggtgtggacgcagagctgttgacgctgattgaggcggctttcggcgaaatttcatcaatacatttgcccactaaaactaaatttaaattcggagccatgatgaaatctggaatgttcctcacactgtttgtgaacacagtcattaacattgtaatcgcaagcagagtgttgagagaacggctaaccggatcaccatgtgcagcattcattggagatgacaatatcgtgaaaggagtcaaatcggacaaattaatggcagacaggtgcgccacctggttgaatatggaagtcaagattatagatgctgtggtgggcgagaaagcgccttatttctgtggagggtttattttgtgtgactccgtgaccggcacagcgtgccgtgtggcagaccccctaaaaaggctgtttaagcttggcaaacctctggcagcagacgatgaacatgatgatgacaggagaagggcattgcatgaagagtcaacacgctggaaccgagtgggtattctttcagagctgtgcaaggcagtagaatcaaggtatgaaaccgtaggaacttccatcatagttatggccatgactactctagctagcagtgttaaatcattcagctacctgagaggggcccctataactctctacggctaacctgaatggactacgacatagtctagtcgagtctagtcgacgccaccatgttcgtgaccgccgtggtgtccgtgtcccccagcagcttttacgagagcctgcaggtcgagcccacccagagcgaggacatcacaagatctgcccacctgggcgacggcgacgagatcagagaggccatccacaagagccaggacgccgagacaaagcccaccttctacgtgtgccccccacctaccggctctacaattgtgcggctggaaccccccagaacctgccctgattaccacctgggcaagaacttcaccgagggaattgccgtggtgtacaaagagaatatcgccgcctacaagttcaaggccaccgtgtactacaaggacgtgatcgtgtccaccgcctgggccggcagcagctacacccagatcaccaacagatacgccgaccgggtgcccatccccgtgtctgagatcaccgacaccatcgacaagttcggcaagtgcagcagcaaggccacctacgtgcggaacaaccacaaggtggaagccttcaacgaggacaagaacccccaggacatgcccctgatcgccagcaagtacaacagcgtgggctccaaggcctggcacaccaccaacgacacctacatggtggccggcacccccggcacatacagaacaggcaccagcgtgaactgcatcatcgaggaagtggaagcccggtccatcttcccatacgacagcttcggcctgagcaccggcgacattatctacatgagccctttcttcggcctgcgggacggcgcctacagagagcacagcaactacgccatggaccggttccaccagttcgagggctacagacagcgggacctggacacaagagccctgctggaacctgccgccagaaacttcctggtcacccctcacctgaccgtgggctggaactggaagcccaagcggaccgaagtgtgcagcctggtcaagtggcgcgaggtggaagatgtcgtgcgggatgagtacgcccacaacttccggttcaccatgaagaccctgagcaccaccttcatcagcgagacaaacgagttcaacctgaaccagatccacctgagccagtgcgtgaaagaggaagccagagccatcatcaaccggatctacaccacccggtacaacagcagccacgtgcggaccggcgatatccagacctatctggctagaggcggcttcgtggtggtgtttcagcccctgctgagcaacagcctggctagactgtacctgcaggaactcgtcagagagaacaccaaccacagcccccagaagcaccccacccggaataccagatccagacgcagcgtgcccgtggaactgagagccaaccggaccatcaccaccaccagcagcgtggaattcgccatgctgcagttcacctacgaccacatccaggaacacgtgaacgagatgctggcccggatcagcagcagttggtgccagctgcagaatcgggaaagggccctgtggtccggcctgttccccatcaatccaagcgccctggccagcaccatcctggaccagagagtgaaggccagaatcctgggggacgtgatcagcgtgtccaactgtcctgagctgggcagcgacacccggatcatcctgcagaacagcatgcgggtgtccggcagcaccaccagatgctacagcagacccctgatcagcatcgtgtccctgaacggcagcggcacagtggaaggccagctgggcaccgataacgagctgatcatgagccgggacctgctcgaaccctgcgtggccaatcacaagcggtactttctgttcggccaccactacgtgtactatgaggactacagatacgtgcgcgagatcgccgtgcacgacgtgggcatgatcagcacctacgtggacctgaacctgaccctgctgaaggaccgcgagttcatgccactgcaggtctacacccgggacgagctgagagataccggcctgctggactacagcgagatccagcggcggaaccagatgcactccctgcggttctacgacatcgacaaggtggtgcagtacgacagcggcaccgccatcatgcagggcatggcccagttctttcagggcctgggaacagccggacaggccgtgggacatgtggtgctgggagctacaggcgccctgctgtctaccgtgcacggcttcaccacctttctgagcaaccccttcggagccctggctgtgggactgctggtcctggctggactggtggccgccttctttgcctaccgctacgtgctgaagctgaaaaccagccccatgaaggccctgtaccccctgaccaccaagggcctgaagcagctgcctgagggcatggaccccttcgccgagaagcccaatgccaccgacacccccatcgaggaaatcggcgacagccagaacaccgagccctccgtgaacagcggcttcgaccccgacaagtttcgcgaggcccaggaaatgatcaagtacatgaccctggtgtctgctgccgagcggcaggaaagcaaggcccggaagaagaacaagacctccgccctgctgaccagcagactgacaggactggccctgcggaacagacggggctatagcagagtgcggaccgagaatgtgaccggcgtgtaatctagacgcggccgcatacagcagcaattggcaagctgcttacatagaactcgcggcgattggcatgccgccttaaaatttttattttatttttcttttcttttccgaatcggattttgtttttaatatttcaaaaaaaaaaaaaaaaaaaaaaaaaaaaaaaaaaagggtcggcatggcatctccacctcctcgcggtccgacctgggcatccgaaggaggacgcacgtccactcggatggctaagggagagccacgtttaaaccagctccaattcgccctatagtgagtcgtattacgcgcgctcactggccgtcgttttacaacgtcgtgactgggaaaaccctggcgttacccaacttaatcgccttgcagcacatccccctttcgccagctggcgtaatagcgaagaggcccgcaccgatcgcccttcccaacagttgcgcagcctgaatggcgaatgggacgcgccctgtagcggcgcattaagcgcggcgggtgtggtggttacgcgcagcgtgaccgctacacttgccagcgccctagcgcccgctcctttcgctttcttcccttcctttctcgccacgttcgccggctttccccgtcaagctctaaatcgggggctccctttagggttccgatttagtgctttacggcacctcgaccccaaaaaacttgattagggtgatggttcacgtagtgggccatcgccctgatagacggtttttcgccctttgacgttggagtccacgttctttaatagtggactcttgttccaaactggaacaacactcaaccctatctcggtctattcttttgatttataagggattttgccgatttcggcctattggttaaaaaatgagctgatttaacaaaaatttaacgcgaattttaacaaaatattaacgcttacaatttaggtggcacttttcggggaaatgtgcgcggaacccctatttgtttatttttctaaatacattcaaatatgtatccgctcatgagacaataaccctgataaatgcttcaataatattgaaaaaggaagagtatgagtattcaacatttccgtgtcgcccttattcccttttttgcggcattttgccttcctgtttttgctcacccagaaacgctggtgaaagtaaaagatgctgaagatcagttgggtgcacgagtgggttacatcgaactggatctcaacagcggtaagatccttgagagttttcgccccgaagaacgttttccaatgatgagcacttttaaagttctgctatgtggcgcggtattatcccgtattgacgccgggcaagagcaactcggtcgccgcatacactattctcagaatgacttggttgagtactcaccagtcacagaaaagcatcttacggatggcatgacagtaagagaattatgcagtgctgccataaccatgagtgataacactgcggccaacttacttctgacaacgatcggaggaccgaaggagctaaccgcttttttgcacaacatgggggatcatgtaactcgccttgatcgttgggaaccggagctgaatgaagccataccaaacgacgagcgtgacaccacgatgcctgtagcaatggcaacaacgttgcgcaaactattaactggcgaactacttactctagcttcccggcaacaattaatagactggatggaggcggataaagttgcaggaccacttctgcgctcggcccttccggctggctggtttattgctgataaatctggagccggtgagcgtgggtctcgcggtatcattgcagcactggggccagatggtaagccctcccgtatcgtagttatctacacgacggggagtcaggcaactatggatgaacgaaatagacagatcgctgagataggtgcctcactgattaagcattggtaactgtcagaccaagtttactcatatatactttagattgatttaaaacttcatttttaatttaaaaggatctaggtgaagatcctttttgataatctcatgaccaaaatcccttaacgtgagttttcgttccactgagcgtcagaccccgtagaaaagatcaaaggatcttcttgagatcctttttttctgcgcgtaatctgctgcttgcaaacaaaaaaaccaccgctaccagcggtggtttgtttgccggatcaagagctaccaactctttttccgaaggtaactggcttcagcagagcgcagataccaaatactgttcttctagtgtagccgtagttaggccaccacttcaagaactctgtagcaccgcctacatacctcgctctgctaatcctgttaccagtggctgctgccagtggcgataagtcgtgtcttaccgggttggactcaagacgatagttaccggataaggcgcagcggtcgggctgaacggggggttcgtgcacacagcccagcttggagcgaacgacctacaccgaactgagatacctacagcgtgagctatgagaaagcgccacgcttcccgaagggagaaaggcggacaggtatccggtaagcggcagggtcggaacaggagagcgcacgagggagcttccagggggaaacgcctggtatctttatagtcctgtcgggtttcgccacctctgacttgagcgtcgatttttgtgatgctcgtcaggggggcggagcctatggaaaaacgccagcaacgcggcctttttacggttcctggccttttgctggccttttgctcacatgttctttcctgcgttatcccctgattctgtggataaccgtattaccgcctttgagtgagctgataccgctcgccgcagccgaacgaccgagcgcagcgagtcagtgagcgaggaagcggaagagcgcccaatacgcaaaccgcctctccccgcgcgttggccgattcattaatgcagctggcacgacaggtttcccgactggaaagcgggcagtgagcgcaacgcaattaatgtgagttagctcactcattaggcaccccaggctttacactttatgctcccggctcgtatgttgtgtggaattgtgagcggataacaatttcacacaggaaacagctatgaccatgattacgccaagcgcgcaattaaccctcactaaagggaacaaaagctgggtaccgggcccacgcgtaatacgactcactatag

SEQ ID NO: 74 - DNA, 13258 bp, Artificial Sequence
  source: /note="Description of Artificial Sequence: Synthetic polynucleotide"
ataggcggcgcatgagagaagcccagaccaattacctacccaaaatggagaaagttcacgttgacatcgaggaagacagcccattcctcagagctttgcagcggagcttcccgcagtttgaggtagaagccaagcaggtcactgataatgaccatgctaatgccagagcgttttcgcatctggcttcaaaactgatcgaaacggaggtggacccatccgacacgatccttgacattggaagtgcgcccgcccgcagaatgtattctaagcacaagtatcattgtatctgtccgatgagatgtgcggaagatccggacagattgtataagtatgcaactaagctgaagaaaaactgtaaggaaataactgataaggaattggacaagaaaatgaaggagctcgccgccgtcatgagcgaccctgacctggaaactgagactatgtgcctccacgacgacgagtcgtgtcgctacgaagggcaagtcgctgtttaccaggatgtatacgcggttgacggaccgacaagtctctatcaccaagccaataagggagttagagtcgcctactggataggctttgacaccaccccttttatgtttaagaacttggctggagcatatccatcatactctaccaactgggccgacgaaaccgtgttaacggctcgtaacataggcctatgcagctctgacgttatggagcggtcacgtagagggatgtccattcttagaaagaagtatttgaaaccatccaacaatgttctattctctgttggctcgaccatctaccacgagaagagggacttactgaggagctggcacctgccgtctgtatttcacttacgtggcaagcaaaattacacatgtcggtgtgagactatagttagttgcgacgggtacgtcgttaaaagaatagctatcagtccaggcctgtatgggaagccttcaggctatgctgctacgatgcaccgcgagggattcttgtgctgcaaagtgacagacacattgaacggggagagggtctcttttcccgtgtgcacgtatgtgccagctacattgtgtgaccaaatgactggcatactggcaacagatgtcagtgcggacgacgcgcaaaaactgctggttgggctcaaccagcgtatagtcgtcaacggtcgcacccagagaaacaccaataccatgaaaaattaccttttgcccgtagtggcccaggcatttgctaggtgggcaaaggaatataaggaagatcaagaagatgaaaggccactaggactacgagatagacagttagtcatggggtgttgttgggcttttagaaggcacaagataacatctatttataagcgcccggatacccaaaccatcatcaaagtgaacagcgatttccactcattcgtgctgcccaggataggcagtaacacattggagatcgggctgagaacaagaatcaggaaaatgttagaggagcacaaggagccgtcacctctcattaccgccgaggacgtacaagaagctaagtgcgcagccgatgaggctaaggaggtgcgtgaagccgaggagttgcgcgcagctctaccacctttggcagctgatgttgaggagcccactctggaagccgatgtagacttgatgttacaagaggctggggccggctcagtggagacacctcgtggcttgataaaggttaccagctacgatggcgaggacaagatcggctcttacgctgtgctttctccgcaggctgtactcaagagtgaaaaattatcttgcatccaccctctcgctgaacaagtcatagtgataacacactctggccgaaaagggcgttatgccgtggaaccataccatggtaaagtagtggtgccagagggacatgcaatacccgtccaggactttcaagctctgagtgaaagtgccaccattgtgtacaacgaacgtgagttcgtaaacaggtacctgcaccatattgccacacatggaggagcgctgaacactgatgaagaatattacaaaactgtcaagcccagcgagcacgacggcgaatacctgtacgacatcgacaggaaacagtgcgtcaagaaagaactagtcactgggctagggctcacaggcgagctggtggatcctcccttccatgaattcgcctacgagagtctgagaacacgaccagccgctccttaccaagtaccaaccataggggtgtatggcgtgccaggatcaggcaagtctggcatcattaaaagcgcagtcaccaaaaaagatctagtggtgagcgccaagaaagaaaactgtgcagaaattataagggacgtcaagaaaatgaaagggctggacgtcaatgccagaactgtggactcagtgctcttgaatggatgcaaacaccccgtagagaccctgtatattgacgaagcttttgcttgtcatgcaggtactctcagagcgctcatagccattataagacctaaaaaggcagtgctctgcggggatcccaaacagtgcggtttttttaacatgatgtgcctgaaagtgcattttaaccacgagatttgcacacaagtcttccacaaaagcatctctcgccgttgcactaaatctgtgacttcggtcgtctcaaccttgttttacgacaaaaaaatgagaacgacgaatccgaaagagactaagattgtgattgacactaccggcagtaccaaacctaagcaggacgatctcattctcacttgtttcagagggtgggtgaagcagttgcaaatagattacaaaggcaacgaaataatgacggcagctgcctctcaagggctgacccgtaaaggtgtgtatgccgttcggtacaaggtgaatgaaaatcctctgtacgcacccacctcagaacatgtgaacgtcctactgacccgcacggaggaccgcatcgtgtggaaaacactagccggcgacccatggataaaaacactgactgccaagtaccctgggaatttcactgccacgatagaggagtggcaagcagagcatgatgccatcatgaggcacatcttggagagaccggaccctaccgacgtcttccagaataaggcaaacgtgtgttgggccaaggctttagtgccggtgctgaagaccgctggcatagacatgaccactgaacaatggaacactgtggattattttgaaacggacaaagctcactcagcagagatagtattgaaccaactatgcgtgaggttctttggactcgatctggactccggtctattttctgcacccactgttccgttatccattaggaataatcactgggataactccccgtcgcctaacatgtacgggctgaataaagaagtggtccgtcagctctctcgcaggtacccacaactgcctcgggcagttgccactggaagagtctatgacatgaacactggtacactgcgcaattatgatccgcgcataaacctagtacctgtaaacagaagactgcctcatgctttagtcctccaccataatgaacacccacagagtgacttttcttcattcgtcagcaaattgaagggcagaactgtcctggtggtcggggaaaagttgtccgtcccaggcaaaatggttgactggttgtcagaccggcctgaggctaccttcagagctcggctggatttaggcatcccaggtgatgtgcccaaatatgacataatatttgttaatgtgaggaccccatataaataccatcactatcagcagtgtgaagaccatgccattaagcttagcatgttgaccaagaaagcttgtctgcatctgaatcccggcggaacctgtgtcagcataggttatggttacgctgacagggccagcgaaagcatcattggtgctatagcgcggcagttcaagttttcccgggtatgcaaaccgaaatcctcacttgaagagacggaagttctgtttgtattcattgggtacgatcgcaaggcccgtacgcacaatccttacaagctttcatcaaccttgaccaacatttatacaggttccagactccacgaagccggatgtgcaccctcatatcatgtggtgcgaggggatattgccacggccaccgaaggagtgattataaatgctgctaacagcaaaggacaacctggcggaggggtgtgcggagcgctgtataagaaattcccggaaagcttcgatttacagccgatcgaagtaggaaaagcgcgactggtcaaaggtgcagctaaacatatcattcatgccgtaggaccaaacttcaacaaagtttcggaggttgaaggtgacaaacagttggcagaggcttatgagtccatcgctaagattgtcaacgataacaattacaagtcagtagcgattccactgttgtccaccggcatcttttccgggaacaaagatcgactaacccaatcattgaaccatttgctgacagctttagacaccactgatgcagatgtagccatatactgcagggacaagaaatgggaaatgactctcaaggaagcagtggctaggagagaagcagtggaggagatatgcatatccgacgactcttcagtgacagaacctgatgcagagctggtgagggtgcatccgaagagttctttggctggaaggaagggctacagcacaagcgatggcaaaactttctcatatttggaagggaccaagtttcaccaggcggccaaggatatagcagaaattaatgccatgtggcccgttgcaacggaggccaatgagcaggtatgcatgtatatcctcggagaaagcatgagcagtattaggtcgaaatgccccgtcgaagagtcggaagcctccacaccacctagcacgctgccttgcttgtgcatccatgccatgactccagaaagagtacagcgcctaaaagcctcacgtccagaacaaattactgtgtgctcatcctttccattgccgaagtatagaatcactggtgtgcagaagatccaatgctcccagcctatattgttctcaccgaaagtgcctgcgtatattcatccaaggaagtatctcgtggaaacaccaccggtagacgagactccggagccatcggcagagaaccaatccacagaggggacacctgaacaaccaccacttataaccgaggatgagaccaggactagaacgcctgagccgatcatcatcgaagaggaagaagaggatagcataagtttgctgtcagatggcccgacccaccaggtgctgcaagtcgaggcagacattcacgggccgccctctgtatctagctcatcctggtccattcctcatgcatccgactttgatgtggacagtttatccatacttgacaccctggagggagctagcgtgaccagcggggcaacgtcagccgagactaactcttacttcgcaaagagtatggagtttctggcgcgaccggtgcctgcgcctcgaacagtattcaggaaccctccacatcccgctccgcgcacaagaacaccgtcacttgcacccagcagggcctgctcgagaaccagcctagtttccaccccgccaggcgtgaatagggtgatcactagagaggagctcgaggcgcttaccccgtcacgcactcctagcaggtcggtctcgagaaccagcctggtctccaacccgccaggcgtaaatagggtgattacaagagaggagtttgaggcgttcgtagcacaacaacaatgacggtttgatgcgggtgcatacatcttttcctccgacaccggtcaagggcatttacaacaaaaatcagtaaggcaaacggtgctatccgaagtggtgttggagaggaccgaattggagatttcgtatgccccgcgcctcgaccaagaaaaagaagaattactacgcaagaaattacagttaaatcccacacctgctaacagaagcagataccagtccaggaaggtggagaacatgaaagccataacagctagacgtattctgcaaggcctagggcattatttgaaggcagaaggaaaagtggagtgctaccgaaccctgcatcctgttcctttgtattcatctagtgtgaaccgtgccttttcaagccccaaggtcgcagtggaagcctgtaacgccatgttgaaagagaactttccgactgtggcttcttactgtattattccagagtacgatgcctatttggacatggttgacggagcttcatgctgcttagacactgccagtttttgccctgcaaagctgcgcagctttccaaagaaacactcctatttggaacccacaatacgatcggcagtgccttcagcgatccagaacacgctccagaacgtcctggcagctgccacaaaaagaaattgcaatgtcacgcaaatgagagaattgcccgtattggattcggcggcctttaatgtggaatgcttcaagaaatatgcgtgtaataatgaatattgggaaacgtttaaagaaaaccccatcaggcttactgaagaaaacgtggtaaattacattaccaaattaaaaggaccaaaagctgctgctctttttgcgaagacacataatttgaatatgttgcaggacataccaatggacaggtttgtaatggacttaaagagagacgtgaaagtgactccaggaacaaaacatactgaagaacggcccaaggtacaggtgatccaggctgccgatccgctagcaacagcgtatctgtgcggaatccaccgagagctggttaggagattaaatgcggtcctgcttccgaacattcatacactgtttgatatgtcggctgaagactttgacgctattatagccgagcacttccagcctggggattgtgttctggaaactgacatcgcgtcgtttgataaaagtgaggacgacgccatggctctgaccgcgttaatgattctggaagacttaggtgtggacgcagagctgttgacgctgattgaggcggctttcggcgaaatttcatcaatacatttgcccactaaaactaaatttaaattcggagccatgatgaaatctggaatgttcctcacactgtttgtgaacacagtcattaacattgtaatcgcaagcagagtgttgagagaacggctaaccggatcaccatgtgcagcattcattggagatgacaatatcgtgaaaggagtcaaatcggacaaattaatggcagacaggtgcgccacctggttgaatatggaagtcaagattatagatgctgtggtgggcgagaaagcgccttatttctgtggagggtttattttgtgtgactccgtgaccggcacagcgtgccgtgtggcagaccccctaaaaaggctgtttaagcttggcaaacctctggcagcagacgatgaacatgatgatgacaggagaagggcattgcatgaagagtcaacacgctggaaccgagtgggtattctttcagagctgtgcaaggcagtagaatcaaggtatgaaaccgtaggaacttccatcatagttatggccatgactactctagctagcagtgttaaatcattcagctacctgagaggggcccctataactctctacggctaacctgaatggactacgacatagtctagtcgagtctagtcgacgccaccatgttcgccctggtgctggccgtggtcatcctgcctctgtggaccaccgccaacaagagctacgtgacccccacacccgccaccagatccatcggacacatgagcgccctgctgagagagtacagcgaccggaacatgagcctgaagctggaagccttctaccccaccggcttcgacgaggaactgatcaagagcctgcactggggcaacgaccggaagcacgtgttcctcgtgatcgtgaaagtgaaccccaccacccacgagggcgacgtcggcctggtcatcttccccaagtacctgctgagcccctaccacttcaaggccgagcacagagcccccttccctgctggccgctttggctttctgagccaccctgtgacccccgacgtgtcattcttcgacagcagcttcgccccctacctgaccacacagcacctggtggccttcaccaccttcccccccaatcctctcgtgtggcacctggaaagagccgagacagccgccaccgccgaaagaccttttggcgtgtccctgctgcccgccagacctaccgtgcccaagaacaccatcctggaacacaaggcccacttcgccacctgggatgccctggccagacacaccttctttagcgccgaggccatcatcaccaacagcaccctgagaatccacgtgcccctgttcggcagcgtgtggcccatcagatactgggccacaggcagcgtgctgctgaccagcgatagcggcagagtggaagtgaacatcggcgtgggcttcatgagcagcctgatcagcctgagcagcggcctgcccatcgagctgattgtggtgccccacaccgtgaagctgaacgccgtgaccagcgacaccacctggttccagctgaacccccctggccctgatcctggccctagttacagagtgtacctgctgggcagaggcctggacatgaacttcagcaagcacgccaccgtggacatctgcgcctaccctgaggaaagcctggactacagataccacctgagcatggcccacaccgaggccctgagaatgaccaccaaggccgaccagcacgacatcaacgaggaaagctactaccacattgccgccagaatcgccaccagcatcttcgccctgagcgagatgggccggaccaccgagtactttctgctggacgagatcgtggacgtgcagtaccagctgaagttcctgaactacatcctgatgcggatcggcgctggcgcccaccctaataccatcagcggcaccagcgacctgatcttcgccgatcctagccagctgcacgacgagctgagcctgctgttcggccaggtcaaacccgccaacgtggactacttcatcagctacgacgaggcccgggaccagctgaaaacagcctacgccctgtccagaggccaggatcatgtgaacgccctgtccctggccaggcgcgtgatcatgagcatctacaagggcctgctggtcaagcagaacctgaacgccaccgagcggcaggccctgttcttcgccagcatgatcctgctgaacttcagagagggcctggaaaacagcagccgggtgctggatggcagaaccaccctgctgctgatgaccagcatgtgcacagccgcccatgccacacaggccgccctgaatatccaggaaggcctggcttacctgaaccccagcaagcacatgttcaccatccccaacgtgtacagcccctgcatgggcagcctgagaaccgacctgaccgaagagatccacgtgatgaacctgctgtccgccatccccaccagacccggactgaatgaggtgctgcacacccagctggacgagtccgagatcttcgacgccgccttcaagaccatgatgatctttaccacctggaccgccaaggacctgcacatcctgcacacacacgtgcccgaggtgttcacatgccaagatgccgccgctcggaacggcgagtatgtgctgattctgcctgccgtgcagggccacagctacgtgatcacccggaacaagccccagcggggcctggtgtatagcctggctgacgtggacgtgtacaaccccatcagcgtggtgtacctgagcaaggatacctgcgtgtccgagcacggcgtgatcgaaacagtggccctgccccaccccgacaacctgaaagagtgcctgtactgcggctccgtgttcctgcggtatctgaccaccggcgccatcatggacatcatcatcatcgacagcaaggacaccgagagacagctggccgccatgggcaacagcaccatcccccccttcaaccccgacatgcacggcgacgatagcaaggccgtgctgctgttccccaacggcaccgtggtcacactgctgggcttcgagcggagacaggccatcagaatgagcggccagtacctgggcgcctctctgggtggtgcctttctggccgtcgtgggctttggcatcatcggctggatgctgtgcggcaacagcagactgcgcgagtacaacaagatccccctgacctaatctagacgcggccgcatacagcagcaattggcaagctgcttacatagaactcgcggcgattggcatgccgccttaaaatttttattttatttttcttttcttttccgaatcggattttgtttttaatatttcaaaaaaaaaaaaaaaaaaaaaaaaaaaaaaaaaaagggtcggcatggcatctccacctcctcgcggtccgacctgggcatccgaaggaggacgcacgtccactcggatggctaagggagagccacgtttaaaccagctccaattcgccctatagtgagtcgtattacgcgcgctcactggccgtcgttttacaacgtcgtgactgggaaaaccctggcgttacccaacttaatcgccttgcagcacatccccctttcgccagctggcgtaatagcgaagaggcccgcaccgatcgcccttcccaacagttgcgcagcctgaatggcgaatgggacgcgccctgtagcggcgcattaagcgcggcgggtgtggtggttacgcgcagcgtgaccgctacacttgccagcgccctagcgcccgctcctttcgctttcttcccttcctttctcgccacgttcgccggctttccccgtcaagctctaaatcgggggctccctttagggttccgatttagtgctttacggcacctcgaccccaaaaaacttgattagggtgatggttcacgtagtgggccatcgccctgatagacggtttttcgccctttgacgttggagtccacgttctttaatagtggactcttgttccaaactggaacaacactcaaccctatctcggtctattcttttgatttataagggattttgccgatttcggcctattggttaaaaaatgagctgatttaacaaaaatttaacgcgaattttaacaaaatattaacgcttacaatttaggtggcacttttcggggaaatgtgcgcggaacccctatttgtttatttttctaaatacattcaaatatgtatccgctcatgagacaataaccctgataaatgcttcaataatattgaaaaaggaagagtatgagtattcaacatttccgtgtcgcccttattcccttttttgcggcattttgccttcctgtttttgctcacccagaaacgctggtgaaagtaaaagatgctgaagatcagttgggtgcacgagtgggttacatcgaactggatctcaacagcggtaagatccttgagagttttcgccccgaagaacgttttccaatgatgagcacttttaaagttctgctatgtggcgcggtattatcccgtattgacgccgggcaagagcaactcggtcgccgcatacactattctcagaatgacttggttgagtactcaccagtcacagaaaagcatcttacggatggcatgacagtaagagaattatgcagtgctgccataaccatgagtgataacactgcggccaacttacttctgacaacgatcggaggaccgaaggagctaaccgcttttttgcacaacatgggggatcatgtaactcgccttgatcgttgggaaccggagctgaatgaagccataccaaacgacgagcgtgacaccacgatgcctgtagcaatggcaacaacgttgcgcaaactattaactggcgaactacttactctagcttcccggcaacaattaatagactggatggaggcggataaagttgcaggaccacttctgcgctcggcccttccggctggctggtttattgctgataaatctggagccggtgagcgtgggtctcgcggtatcattgcagcactggggccagatggtaagccctcccgtatcgtagttatctacacgacggggagtcaggcaactatggatgaacgaaatagacagatcgctgagataggtgcctcactgattaagcattggtaactgtcagaccaagtttactcatatatactttagattgatttaaaacttcatttttaatttaaaaggatctaggtgaagatcctttttgataatctcatgaccaaaatcccttaacgtgagttttcgttccactgagcgtcagaccccgtagaaaagatcaaaggatcttcttgagatcctttttttctgcgcgtaatctgctgcttgcaaacaaaaaaaccaccgctaccagcggtggtttgtttgccggatcaagagctaccaactctttttccgaaggtaactggcttcagcagagcgcagataccaaatactgttcttctagtgtagccgtagttaggccaccacttcaagaactctgtagcaccgcctacatacctcgctctgctaatcctgttaccagtggctgctgccagtggcgataagtcgtgtcttaccgggttggactcaagacgatagttaccggataaggcgcagcggtcgggctgaacggggggttcgtgcacacagcccagcttggagcgaacgacctacaccgaactgagatacctacagcgtgagctatgagaaagcgccacgcttcccgaagggagaaaggcggacaggtatccggtaagcggcagggtcggaacaggagagcgcacgagggagcttccagggggaaacgcctggtatctttatagtcctgtcgggtttcgccacctctgacttgagcgtcgatttttgtgatgctcgtcaggggggcggagcctatggaaaaacgccagcaacgcggcctttttacggttcctggccttttgctggccttttgctcacatgttctttcctgcgttatcccctgattctgtggataaccgtattaccgcctttgagtgagctgataccgctcgccgcagccgaacgaccgagcgcagcgagtcagtgagcgaggaagcggaagagcgcccaatacgcaaaccgcctctccccgcgcgttggccgattcattaatgcagctggcacgacaggtttcccgactggaaagcgggcagtgagcgcaacgcaattaatgtgagttagctcactcattaggcaccccaggctttacactttatgctcccggctcgtatgttgtgtggaattgtgagcggataacaatttcacacaggaaacagctatgaccatgattacgccaagcgcgcaattaaccctcactaaagggaacaaaagctgggtaccgggcccacgcgtaatacgactcactatag

SEQ ID NO: 75 - DNA, 11215 bp, Artificial Sequence
  source: /note="Description of Artificial Sequence: Synthetic polynucleotide"
ataggcggcgcatgagagaagcccagaccaattacctacccaaaatggagaaagttcacgttgacatcgaggaagacagcccattcctcagagctttgcagcggagcttcccgcagtttgaggtagaagccaagcaggtcactgataatgaccatgctaatgccagagcgttttcgcatctggcttcaaaactgatcgaaacggaggtggacccatccgacacgatccttgacattggaagtgcgcccgcccgcagaatgtattctaagcacaagtatcattgtatctgtccgatgagatgtgcggaagatccggacagattgtataagtatgcaactaagctgaagaaaaactgtaaggaaataactgataaggaattggacaagaaaatgaaggagctcgccgccgtcatgagcgaccctgacctggaaactgagactatgtgcctccacgacgacgagtcgtgtcgctacgaagggcaagtcgctgtttaccaggatgtatacgcggttgacggaccgacaagtctctatcaccaagccaataagggagttagagtcgcctactggataggctttgacaccaccccttttatgtttaagaacttggctggagcatatccatcatactctaccaactgggccgacgaaaccgtgttaacggctcgtaacataggcctatgcagctctgacgttatggagcggtcacgtagagggatgtccattcttagaaagaagtatttgaaaccatccaacaatgttctattctctgttggctcgaccatctaccacgagaagagggacttactgaggagctggcacctgccgtctgtatttcacttacgtggcaagcaaaattacacatgtcggtgtgagactatagttagttgcgacgggtacgtcgttaaaagaatagctatcagtccaggcctgtatgggaagccttcaggctatgctgctacgatgcaccgcgagggattcttgtgctgcaaagtgacagacacattgaacggggagagggtctcttttcccgtgtgcacgtatgtgccagctacattgtgtgaccaaatgactggcatactggcaacagatgtcagtgcggacgacgcgcaaaaactgctggttgggctcaaccagcgtatagtcgtcaacggtcgcacccagagaaacaccaataccatgaaaaattaccttttgcccgtagtggcccaggcatttgctaggtgggcaaaggaatataaggaagatcaagaagatgaaaggccactaggactacgagatagacagttagtcatggggtgttgttgggcttttagaaggcacaagataacatctatttataagcgcccggatacccaaaccatcatcaaagtgaacagcgatttccactcattcgtgctgcccaggataggcagtaacacattggagatcgggctgagaacaagaatcaggaaaatgttagaggagcacaaggagccgtcacctctcattaccgccgaggacgtacaagaagctaagtgcgcagccgatgaggctaaggaggtgcgtgaagccgaggagttgcgcgcagctctaccacctttggcagctgatgttgaggagcccactctggaagccgatgtagacttgatgttacaagaggctggggccggctcagtggagacacctcgtggcttgataaaggttaccagctacgatggcgaggacaagatcggctcttacgctgtgctttctccgcaggctgtactcaagagtgaaaaattatcttgcatccaccctctcgctgaacaagtcatagtgataacacactctggccgaaaagggcgttatgccgtggaaccataccatggtaaagtagtggtgccagagggacatgcaatacccgtccaggactttcaagctctgagtgaaagtgccaccattgtgtacaacgaacgtgagttcgtaaacaggtacctgcaccatattgccacacatggaggagcgctgaacactgatgaagaatattacaaaactgtcaagcccagcgagcacgacggcgaatacctgtacgacatcgacaggaaacagtgcgtcaagaaagaactagtcactgggctagggctcacaggcgagctggtggatcctcccttccatgaattcgcctacgagagtctgagaacacgaccagccgctccttaccaagtaccaaccataggggtgtatggcgtgccaggatcaggcaagtctggcatcattaaaagcgcagtcaccaaaaaagatctagtggtgagcgccaagaaagaaaactgtgcagaaattataagggacgtcaagaaaatgaaagggctggacgtcaatgccagaactgtggactcagtgctcttgaatggatgcaaacaccccgtagagaccctgtatattgacgaagcttttgcttgtcatgcaggtactctcagagcgctcatagccattataagacctaaaaaggcagtgctctgcggggatcccaaacagtgcggtttttttaacatgatgtgcctgaaagtgcattttaaccacgagatttgcacacaagtcttccacaaaagcatctctcgccgttgcactaaatctgtgacttcggtcgtctcaaccttgttttacgacaaaaaaatgagaacgacgaatccgaaagagactaagattgtgattgacactaccggcagtaccaaacctaagcaggacgatctcattctcacttgtttcagagggtgggtgaagcagttgcaaatagattacaaaggcaacgaaataatgacggcagctgcctctcaagggctgacccgtaaaggtgtgtatgccgttcggtacaaggtgaatgaaaatcctctgtacgcacccacctcagaacatgtgaacgtcctactgacccgcacggaggaccgcatcgtgtggaaaacactagccggcgacccatggataaaaacactgactgccaagtaccctgggaatttcactgccacgatagaggagtggcaagcagagcatgatgccatcatgaggcacatcttggagagaccggaccctaccgacgtcttccagaataaggcaaacgtgtgttgggccaaggctttagtgccggtgctgaagaccgctggcatagacatgaccactgaacaatggaacactgtggattattttgaaacggacaaagctcactcagcagagatagtattgaaccaactatgcgtgaggttctttggactcgatctggactccggtctattttctgcacccactgttccgttatccattaggaataatcactgggataactccccgtcgcctaacatgtacgggctgaataaagaagtggtccgtcagctctctcgcaggtacccacaactgcctcgggcagttgccactggaagagtctatgacatgaacactggtacactgcgcaattatgatccgcgcataaacctagtacctgtaaacagaagactgcctcatgctttagtcctccaccataatgaacacccacagagtgacttttcttcattcgtcagcaaattgaagggcagaactgtcctggtggtcggggaaaagttgtccgtcccaggcaaaatggttgactggttgtcagaccggcctgaggctaccttcagagctcggctggatttaggcatcccaggtgatgtgcccaaatatgacataatatttgttaatgtgaggaccccatataaataccatcactatcagcagtgtgaagaccatgccattaagcttagcatgttgaccaagaaagcttgtctgcatctgaatcccggcggaacctgtgtcagcataggttatggttacgctgacagggccagcgaaagcatcattggtgctatagcgcggcagttcaagttttcccgggtatgcaaaccgaaatcctcacttgaagagacggaagttctgtttgtattcattgggtacgatcgcaaggcccgtacgcacaatccttacaagctttcatcaaccttgaccaacatttatacaggttccagactccacgaagccggatgtgcaccctcatatcatgtggtgcgaggggatattgccacggccaccgaaggagtgattataaatgctgctaacagcaaaggacaacctggcggaggggtgtgcggagcgctgtataagaaattcccggaaagcttcgatttacagccgatcgaagtaggaaaagcgcgactggtcaaaggtgcagctaaacatatcattcatgccgtaggaccaaacttcaacaaagtttcggaggttgaaggtgacaaacagttggcagaggcttatgagtccatcgctaagattgtcaacgataacaattacaagtcagtagcgattccactgttgtccaccggcatcttttccgggaacaaagatcgactaacccaatcattgaaccatttgctgacagctttagacaccactgatgcagatgtagccatatactgcagggacaagaaatgggaaatgactctcaaggaagcagtggctaggagagaagcagtggaggagatatgcatatccgacgactcttcagtgacagaacctgatgcagagctggtgagggtgcatccgaagagttctttggctggaaggaagggctacagcacaagcgatggcaaaactttctcatatttggaagggaccaagtttcaccaggcggccaaggatatagcagaaattaatgccatgtggcccgttgcaacggaggccaatgagcaggtatgcatgtatatcctcggagaaagcatgagcagtattaggtcgaaatgccccgtcgaagagtcggaagcctccacaccacctagcacgctgccttgcttgtgcatccatgccatgactccagaaagagtacagcgcctaaaagcctcacgtccagaacaaattactgtgtgctcatcctttccattgccgaagtatagaatcactggtgtgcagaagatccaatgctcccagcctatattgttctcaccgaaagtgcctgcgtatattcatccaaggaagtatctcgtggaaacaccaccggtagacgagactccggagccatcggcagagaaccaatccacagaggggacacctgaacaaccaccacttataaccgaggatgagaccaggactagaacgcctgagccgatcatcatcgaagaggaagaagaggatagcataagtttgctgtcagatggcccgacccaccaggtgctgcaagtcgaggcagacattcacgggccgccctctgtatctagctcatcctggtccattcctcatgcatccgactttgatgtggacagtttatccatacttgacaccctggagggagctagcgtgaccagcggggcaacgtcagccgagactaactcttacttcgcaaagagtatggagtttctggcgcgaccggtgcctgcgcctcgaacagtattcaggaaccctccacatcccgctccgcgcacaagaacaccgtcacttgcacccagcagggcctgctcgagaaccagcctagtttccaccccgccaggcgtgaatagggtgatcactagagaggagctcgaggcgcttaccccgtcacgcactcctagcaggtcggtctcgagaaccagcctggtctccaacccgccaggcgtaaatagggtgattacaagagaggagtttgaggcgttcgtagcacaacaacaatgacggtttgatgcgggtgcatacatcttttcctccgacaccggtcaagggcatttacaacaaaaatcagtaaggcaaacggtgctatccgaagtggtgttggagaggaccgaattggagatttcgtatgccccgcgcctcgaccaagaaaaagaagaattactacgcaagaaattacagttaaatcccacacctgctaacagaagcagataccagtccaggaaggtggagaacatgaaagccataacagctagacgtattctgcaaggcctagggcattatttgaaggcagaaggaaaagtggagtgctaccgaaccctgcatcctgttcctttgtattcatctagtgtgaaccgtgccttttcaagccccaaggtcgcagtggaagcctgtaacgccatgttgaaagagaactttccgactgtggcttcttactgtattattccagagtacgatgcctatttggacatggttgacggagcttcatgctgcttagacactgccagtttttgccctgcaaagctgcgcagctttccaaagaaacactcctatttggaacccacaatacgatcggcagtgccttcagcgatccagaacacgctccagaacgtcctggcagctgccacaaaaagaaattgcaatgtcacgcaaatgagagaattgcccgtattggattcggcggcctttaatgtggaatgcttcaagaaatatgcgtgtaataatgaatattgggaaacgtttaaagaaaaccccatcaggcttactgaagaaaacgtggtaaattacattaccaaattaaaaggaccaaaagctgctgctctttttgcgaagacacataatttgaatatgttgcaggacataccaatggacaggtttgtaatggacttaaagagagacgtgaaagtgactccaggaacaaaacatactgaagaacggcccaaggtacaggtgatccaggctgccgatccgctagcaacagcgtatctgtgcggaatccaccgagagctggttaggagattaaatgcggtcctgcttccgaacattcatacactgtttgatatgtcggctgaagactttgacgctattatagccgagcacttccagcctggggattgtgttctggaaactgacatcgcgtcgtttgataaaagtgaggacgacgccatggctctgaccgcgttaatgattctggaagacttaggtgtggacgcagagctgttgacgctgattgaggcggctttcggcgaaatttcatcaatacatttgcccactaaaactaaatttaaattcggagccatgatgaaatctggaatgttcctcacactgtttgtgaacacagtcattaacattgtaatcgcaagcagagtgttgagagaacggctaaccggatcaccatgtgcagcattcattggagatgacaatatcgtgaaaggagtcaaatcggacaaattaatggcagacaggtgcgccacctggttgaatatggaagtcaagattatagatgctgtggtgggcgagaaagcgccttatttctgtggagggtttattttgtgtgactccgtgaccggcacagcgtgccgtgtggcagaccccctaaaaaggctgtttaagcttggcaaacctctggcagcagacgatgaacatgatgatgacaggagaagggcattgcatgaagagtcaacacgctggaaccgagtgggtattctttcagagctgtgcaaggcagtagaatcaaggtatgaaaccgtaggaacttccatcatagttatggccatgactactctagctagcagtgttaaatcattcagctacctgagaggggcccctataactctctacggctaacctgaatggactacgacatagtctagtcgagtctagtcgacgccaccatggccagccacaagtggctgctgcagatgatcgtgttcctgaaaaccatcacaatcgcctactgcctgcatctgcaggacgacacccctctgttcttcggcgccaagcctctgagcgacgtgtccctgatcatcaccgagccttgcgtgtccagcgtgtacgaggcctgggattatgccgcccctcccgtgtccaatctgagcgaagccctgagcggcatcgtggtcaagaccaagtgccccgtgcccgaagtgatcctgtggttcaaggacaagcagatggcctactggaccaacccttacgtgaccctgaagggcctgacccagagcgtgggcgaggaacacaagagcggcgacatcagagatgccctgctggatgccctgtccggtgtctgggtggacagcacaccctccagcaccaacatccccgagaacggctgtgtgtggggagccgaccggctgttccagagagtgtgtcagtaatctagacgcggccgcatacagcagcaattggcaagctgcttacatagaactcgcggcgattggcatgccgccttaaaatttttattttatttttcttttcttttccgaatcggattttgtttttaatatttcaaaaaaaaaaaaaaaaaaaaaaaaaaaaaaaaaaagggtcggcatggcatctccacctcctcgcggtccgacctgggcatccgaaggaggacgcacgtccactcggatggctaagggagagccacgtttaaaccagctccaattcgccctatagtgagtcgtattacgcgcgctcactggccgtcgttttacaacgtcgtgactgggaaaaccctggcgttacccaacttaatcgccttgcagcacatccccctttcgccagctggcgtaatagcgaagaggcccgcaccgatcgcccttcccaacagttgcgcagcctgaatggcgaatgggacgcgccctgtagcggcgcattaagcgcggcgggtgtggtggttacgcgcagcgtgaccgctacacttgccagcgccctagcgcccgctcctttcgctttcttcccttcctttctcgccacgttcgccggctttccccgtcaagctctaaatcgggggctccctttagggttccgatttagtgctttacggcacctcgaccccaaaaaacttgattagggtgatggttcacgtagtgggccatcgccctgatagacggtttttcgccctttgacgttggagtccacgttctttaatagtggactcttgttccaaactggaacaacactcaaccctatctcggtctattcttttgatttataagggattttgccgatttcggcctattggttaaaaaatgagctgatttaacaaaaatttaacgcgaattttaacaaaatattaacgcttacaatttaggtggcacttttcggggaaatgtgcgcggaacccctatttgtttatttttctaaatacattcaaatatgtatccgctcatgagacaataaccctgataaatgcttcaataatattgaaaaaggaagagtatgagtattcaacatttccgtgtcgcccttattcccttttttgcggcattttgccttcctgtttttgctcacccagaaacgctggtgaaagtaaaagatgctgaagatcagttgggtgcacgagtgggttacatcgaactggatctcaacagcggtaagatccttgagagttttcgccccgaagaacgttttccaatgatgagcacttttaaagttctgctatgtggcgcggtattatcccgtattgacgccgggcaagagcaactcggtcgccgcatacactattctcagaatgacttggttgagtactcaccagtcacagaaaagcatcttacggatggcatgacagtaagagaattatgcagtgctgccataaccatgagtgataacactgcggccaacttacttctgacaacgatcggaggaccgaaggagctaaccgcttttttgcacaacatgggggatcatgtaactcgccttgatcgttgggaaccggagctgaatgaagccataccaaacgacgagcgtgacaccacgatgcctgtagcaatggcaacaacgttgcgcaaactattaactggcgaactacttactctagcttcccggcaacaattaatagactggatggaggcggataaagttgcaggaccacttctgcgctcggcccttccggctggctggtttattgctgataaatctggagccggtgagcgtgggtctcgcggtatcattgcagcactggggccagatggtaagccctcccgtatcgtagttatctacacgacggggagtcaggcaactatggatgaacgaaatagacagatcgctgagataggtgcctcactgattaagcattggtaactgtcagaccaagtttactcatatatactttagattgatttaaaacttcatttttaatttaaaaggatctaggtgaagatcctttttgataatctcatgaccaaaatcccttaacgtgagttttcgttccactgagcgtcagaccccgtagaaaagatcaaaggatcttcttgagatcctttttttctgcgcgtaatctgctgcttgcaaacaaaaaaaccaccgctaccagcggtggtttgtttgccggatcaagagctaccaactctttttccgaaggtaactggcttcagcagagcgcagataccaaatactgttcttctagtgtagccgtagttaggccaccacttcaagaactctgtagcaccgcctacatacctcgctctgctaatcctgttaccagtggctgctgccagtggcgataagtcgtgtcttaccgggttggactcaagacgatagttaccggataaggcgcagcggtcgggctgaacggggggttcgtgcacacagcccagcttggagcgaacgacctacaccgaactgagatacctacagcgtgagctatgagaaagcgccacgcttcccgaagggagaaaggcggacaggtatccggtaagcggcagggtcggaacaggagagcgcacgagggagcttccagggggaaacgcctggtatctttatagtcctgtcgggtttcgccacctctgacttgagcgtcgatttttgtgatgctcgtcaggggggcggagcctatggaaaaacgccagcaacgcggcctttttacggttcctggccttttgctggccttttgctcacatgttctttcctgcgttatcccctgattctgtggataaccgtattaccgcctttgagtgagctgataccgctcgccgcagccgaacgaccgagcgcagcgagtcagtgagcgaggaagcggaagagcgcccaatacgcaaaccgcctctccccgcgcgttggccgattcattaatgcagctggcacgacaggtttcccgactggaaagcgggcagtgagcgcaacgcaattaatgtgagttagctcactcattaggcaccccaggctttacactttatgctcccggctcgtatgttgtgtggaattgtgagcggataacaatttcacacaggaaacagctatgaccatgattacgccaagcgcgcaattaaccctcactaaagggaacaaaagctgggtaccgggcccacgcgtaatacgactcactatag

SEQ ID NO: 76 - DNA, 13827 bp, Artificial Sequence
  source: /note="Description of Artificial Sequence: Synthetic polynucleotide"
ataggcggcgcatgagagaagcccagaccaattacctacccaaaatggagaaagttcacgttgacatcgaggaagacagcccattcctcagagctttgcagcggagcttcccgcagtttgaggtagaagccaagcaggtcactgataatgaccatgctaatgccagagcgttttcgcatctggcttcaaaactgatcgaaacggaggtggacccatccgacacgatccttgacattggaagtgcgcccgcccgcagaatgtattctaagcacaagtatcattgtatctgtccgatgagatgtgcggaagatccggacagattgtataagtatgcaactaagctgaagaaaaactgtaaggaaataactgataaggaattggacaagaaaatgaaggagctcgccgccgtcatgagcgaccctgacctggaaactgagactatgtgcctccacgacgacgagtcgtgtcgctacgaagggcaagtcgctgtttaccaggatgtatacgcggttgacggaccgacaagtctctatcaccaagccaataagggagttagagtcgcctactggataggctttgacaccaccccttttatgtttaagaacttggctggagcatatccatcatactctaccaactgggccgacgaaaccgtgttaacggctcgtaacataggcctatgcagctctgacgttatggagcggtcacgtagagggatgtccattcttagaaagaagtatttgaaaccatccaacaatgttctattctctgttggctcgaccatctaccacgagaagagggacttactgaggagctggcacctgccgtctgtatttcacttacgtggcaagcaaaattacacatgtcggtgtgagactatagttagttgcgacgggtacgtcgttaaaagaatagctatcagtccaggcctgtatgggaagccttcaggctatgctgctacgatgcaccgcgagggattcttgtgctgcaaagtgacagacacattgaacggggagagggtctcttttcccgtgtgcacgtatgtgccagctacattgtgtgaccaaatgactggcatactggcaacagatgtcagtgcggacgacgcgcaaaaactgctggttgggctcaaccagcgtatagtcgtcaacggtcgcacccagagaaacaccaataccatgaaaaattaccttttgcccgtagtggcccaggcatttgctaggtgggcaaaggaatataaggaagatcaagaagatgaaaggccactaggactacgagatagacagttagtcatggggtgttgttgggcttttagaaggcacaagataacatctatttataagcgcccggatacccaaaccatcatcaaagtgaacagcgatttccactcattcgtgctgcccaggataggcagtaacacattggagatcgggctgagaacaagaatcaggaaaatgttagaggagcacaaggagccgtcacctctcattaccgccgaggacgtacaagaagctaagtgcgcagccgatgaggctaaggaggtgcgtgaagccgaggagttgcgcgcagctctaccacctttggcagctgatgttgaggagcccactctggaagccgatgtagacttgatgttacaagaggctggggccggctcagtggagacacctcgtggcttgataaaggttaccagctacgatggcgaggacaagatcggctcttacgctgtgctttctccgcaggctgtactcaagagtgaaaaattatcttgcatccaccctctcgctgaacaagtcatagtgataacacactctggccgaaaagggcgttatgccgtggaaccataccatggtaaagtagtggtgccagagggacatgcaatacccgtccaggactttcaagctctgagtgaaagtgccaccattgtgtacaacgaacgtgagttcgtaaacaggtacctgcaccatattgccacacatggaggagcgctgaacactgatgaagaatattacaaaactgtcaagcccagcgagcacgacggcgaatacctgtacgacatcgacaggaaacagtgcgtcaagaaagaactagtcactgggctagggctcacaggcgagctggtggatcctcccttccatgaattcgcctacgagagtctgagaacacgaccagccgctccttaccaagtaccaaccataggggtgtatggcgtgccaggatcaggcaagtctggcatcattaaaagcgcagtcaccaaaaaagatctagtggtgagcgccaagaaagaaaactgtgcagaaattataagggacgtcaagaaaatgaaagggctggacgtcaatgccagaactgtggactcagtgctcttgaatggatgcaaacaccccgtagagaccctgtatattgacgaagcttttgcttgtcatgcaggtactctcagagcgctcatagccattataagacctaaaaaggcagtgctctgcggggatcccaaacagtgcggtttttttaacatgatgtgcctgaaagtgcattttaaccacgagatttgcacacaagtcttccacaaaagcatctctcgccgttgcactaaatctgtgacttcggtcgtctcaaccttgttttacgacaaaaaaatgagaacgacgaatccgaaagagactaagattgtgattgacactaccggcagtaccaaacctaagcaggacgatctcattctcacttgtttcagagggtgggtgaagcagttgcaaatagattacaaaggcaacgaaataatgacggcagctgcctctcaagggctgacccgtaaaggtgtgtatgccgttcggtacaaggtgaatgaaaatcctctgtacgcacccacctcagaacatgtgaacgtcctactgacccgcacggaggaccgcatcgtgtggaaaacactagccggcgacccatggataaaaacactgactgccaagtaccctgggaatttcactgccacgatagaggagtggcaagcagagcatgatgccatcatgaggcacatcttggagagaccggaccctaccgacgtcttccagaataaggcaaacgtgtgttgggccaaggctttagtgccggtgctgaagaccgctggcatagacatgaccactgaacaatggaacactgtggattattttgaaacggacaaagctcactcagcagagatagtattgaaccaactatgcgtgaggttctttggactcgatctggactccggtctattttctgcacccactgttccgttatccattaggaataatcactgggataactccccgtcgcctaacatgtacgggctgaataaagaagtggtccgtcagctctctcgcaggtacccacaactgcctcgggcagttgccactggaagagtctatgacatgaacactggtacactgcgcaattatgatccgcgcataaacctagtacctgtaaacagaagactgcctcatgctttagtcctccaccataatgaacacccacagagtgacttttcttcattcgtcagcaaattgaagggcagaactgtcctggtggtcggggaaaagttgtccgtcccaggcaaaatggttgactggttgtcagaccggcctgaggctaccttcagagctcggctggatttaggcatcccaggtgatgtgcccaaatatgacataatatttgttaatgtgaggaccccatataaataccatcactatcagcagtgtgaagaccatgccattaagcttagcatgttgaccaagaaagcttgtctgcatctgaatcccggcggaacctgtgtcagcataggttatggttacgctgacagggccagcgaaagcatcattggtgctatagcgcggcagttcaagttttcccgggtatgcaaaccgaaatcctcacttgaagagacggaagttctgtttgtattcattgggtacgatcgcaaggcccgtacgcacaatccttacaagctttcatcaaccttgaccaacatttatacaggttccagactccacgaagccggatgtgcaccctcatatcatgtggtgcgaggggatattgccacggccaccgaaggagtgattataaatgctgctaacagcaaaggacaacctggcggaggggtgtgcggagcgctgtataagaaattcccggaaagcttcgatttacagccgatcgaagtaggaaaagcgcgactggtcaaaggtgcagctaaacatatcattcatgccgtaggaccaaacttcaacaaagtttcggaggttgaaggtgacaaacagttggcagaggcttatgagtccatcgctaagattgtcaacgataacaattacaagtcagtagcgattccactgttgtccaccggcatcttttccgggaacaaagatcgactaacccaatcattgaaccatttgctgacagctttagacaccactgatgcagatgtagccatatactgcagggacaagaaatgggaaatgactctcaaggaagcagtggctaggagagaagcagtggaggagatatgcatatccgacgactcttcagtgacagaacctgatgcagagctggtgagggtgcatccgaagagttctttggctggaaggaagggctacagcacaagcgatggcaaaactttctcatatttggaagggaccaagtttcaccaggcggccaaggatatagcagaaattaatgccatgtggcccgttgcaacggaggccaatgagcaggtatgcatgtatatcctcggagaaagcatgagcagtattaggtcgaaatgccccgtcgaagagtcggaagcctccacaccacctagcacgctgccttgcttgtgcatccatgccatgactccagaaagagtacagcgcctaaaagcctcacgtccagaacaaattactgtgtgctcatcctttccattgccgaagtatagaatcactggtgtgcagaagatccaatgctcccagcctatattgttctcaccgaaagtgcctgcgtatattcatccaaggaagtatctcgtggaaacaccaccggtagacgagactccggagccatcggcagagaaccaatccacagaggggacacctgaacaaccaccacttataaccgaggatgagaccaggactagaacgcctgagccgatcatcatcgaagaggaagaagaggatagcataagtttgctgtcagatggcccgacccaccaggtgctgcaagtcgaggcagacattcacgggccgccctctgtatctagctcatcctggtccattcctcatgcatccgactttgatgtggacagtttatccatacttgacaccctggagggagctagcgtgaccagcggggcaacgtcagccgagactaactcttacttcgcaaagagtatggagtttctggcgcgaccggtgcctgcgcctcgaacagtattcaggaaccctccacatcccgctccgcgcacaagaacaccgtcacttgcacccagcagggcctgctcgagaaccagcctagtttccaccccgccaggcgtgaatagggtgatcactagagaggagctcgaggcgcttaccccgtcacgcactcctagcaggtcggtctcgagaaccagcctggtctccaacccgccaggcgtaaatagggtgattacaagagaggagtttgaggcgttcgtagcacaacaacaatgacggtttgatgcgggtgcatacatcttttcctccgacaccggtcaagggcatttacaacaaaaatcagtaaggcaaacggtgctatccgaagtggtgttggagaggaccgaattggagatttcgtatgccccgcgcctcgaccaagaaaaagaagaattactacgcaagaaattacagttaaatcccacacctgctaacagaagcagataccagtccaggaaggtggagaacatgaaagccataacagctagacgtattctgcaaggcctagggcattatttgaaggcagaaggaaaagtggagtgctaccgaaccctgcatcctgttcctttgtattcatctagtgtgaaccgtgccttttcaagccccaaggtcgcagtggaagcctgtaacgccatgttgaaagagaactttccgactgtggcttcttactgtattattccagagtacgatgcctatttggacatggttgacggagcttcatgctgcttagacactgccagtttttgccctgcaaagctgcgcagctttccaaagaaacactcctatttggaacccacaatacgatcggcagtgccttcagcgatccagaacacgctccagaacgtcctggcagctgccacaaaaagaaattgcaatgtcacgcaaatgagagaattgcccgtattggattcggcggcctttaatgtggaatgcttcaagaaatatgcgtgtaataatgaatattgggaaacgtttaaagaaaaccccatcaggcttactgaagaaaacgtggtaaattacattaccaaattaaaaggaccaaaagctgctgctctttttgcgaagacacataatttgaatatgttgcaggacataccaatggacaggtttgtaatggacttaaagagagacgtgaaagtgactccaggaacaaaacatactgaagaacggcccaaggtacaggtgatccaggctgccgatccgctagcaacagcgtatctgtgcggaatccaccgagagctggttaggagattaaatgcggtcctgcttccgaacattcatacactgtttgatatgtcggctgaagactttgacgctattatagccgagcacttccagcctggggattgtgttctggaaactgacatcgcgtcgtttgataaaagtgaggacgacgccatggctctgaccgcgttaatgattctggaagacttaggtgtggacgcagagctgttgacgctgattgaggcggctttcggcgaaatttcatcaatacatttgcccactaaaactaaatttaaattcggagccatgatgaaatctggaatgttcctcacactgtttgtgaacacagtcattaacattgtaatcgcaagcagagtgttgagagaacggctaaccggatcaccatgtgcagcattcattggagatgacaatatcgtgaaaggagtcaaatcggacaaattaatggcagacaggtgcgccacctggttgaatatggaagtcaagattatagatgctgtggtgggcgagaaagcgccttatttctgtggagggtttattttgtgtgactccgtgaccggcacagcgtgccgtgtggcagaccccctaaaaaggctgtttaagcttggcaaacctctggcagcagacgatgaacatgatgatgacaggagaagggcattgcatgaagagtcaacacgctggaaccgagtgggtattctttcagagctgtgcaaggcagtagaatcaaggtatgaaaccgtaggaacttccatcatagttatggccatgactactctagctagcagtgttaaatcattcagctacctgagaggggcccctataactctctacggctaacctgaatggactacgacatagtctagtcgagtctagtcgacgccaccatgttcgccctggtgctggccgtggtcatcctgcctctgtggaccaccgccaacaagagctacgtgacccccacacccgccaccagatccatcggacacatgagcgccctgctgagagagtacagcgaccggaacatgagcctgaagctggaagccttctaccccaccggcttcgacgaggaactgatcaagagcctgcactggggcaacgaccggaagcacgtgttcctcgtgatcgtgaaagtgaaccccaccacccacgagggcgacgtcggcctggtcatcttccccaagtacctgctgagcccctaccacttcaaggccgagcacagagcccccttccctgctggccgctttggctttctgagccaccctgtgacccccgacgtgtcattcttcgacagcagcttcgccccctacctgaccacacagcacctggtggccttcaccaccttcccccccaatcctctcgtgtggcacctggaaagagccgagacagccgccaccgccgaaagaccttttggcgtgtccctgctgcccgccagacctaccgtgcccaagaacaccatcctggaacacaaggcccacttcgccacctgggatgccctggccagacacaccttctttagcgccgaggccatcatcaccaacagcaccctgagaatccacgtgcccctgttcggcagcgtgtggcccatcagatactgggccacaggcagcgtgctgctgaccagcgatagcggcagagtggaagtgaacatcggcgtgggcttcatgagcagcctgatcagcctgagcagcggcctgcccatcgagctgattgtggtgccccacaccgtgaagctgaacgccgtgaccagcgacaccacctggttccagctgaacccccctggccctgatcctggccctagttacagagtgtacctgctgggcagaggcctggacatgaacttcagcaagcacgccaccgtggacatctgcgcctaccctgaggaaagcctggactacagataccacctgagcatggcccacaccgaggccctgagaatgaccaccaaggccgaccagcacgacatcaacgaggaaagctactaccacattgccgccagaatcgccaccagcatcttcgccctgagcgagatgggccggaccaccgagtactttctgctggacgagatcgtggacgtgcagtaccagctgaagttcctgaactacatcctgatgcggatcggcgctggcgcccaccctaataccatcagcggcaccagcgacctgatcttcgccgatcctagccagctgcacgacgagctgagcctgctgttcggccaggtcaaacccgccaacgtggactacttcatcagctacgacgaggcccgggaccagctgaaaacagcctacgccctgtccagaggccaggatcatgtgaacgccctgtccctggccaggcgcgtgatcatgagcatctacaagggcctgctggtcaagcagaacctgaacgccaccgagcggcaggccctgttcttcgccagcatgatcctgctgaacttcagagagggcctggaaaacagcagccgggtgctggatggcagaaccaccctgctgctgatgaccagcatgtgcacagccgcccatgccacacaggccgccctgaatatccaggaaggcctggcttacctgaaccccagcaagcacatgttcaccatccccaacgtgtacagcccctgcatgggcagcctgagaaccgacctgaccgaagagatccacgtgatgaacctgctgtccgccatccccaccagacccggactgaatgaggtgctgcacacccagctggacgagtccgagatcttcgacgccgccttcaagaccatgatgatctttaccacctggaccgccaaggacctgcacatcctgcacacacacgtgcccgaggtgttcacatgccaagatgccgccgctcggaacggcgagtatgtgctgattctgcctgccgtgcagggccacagctacgtgatcacccggaacaagccccagcggggcctggtgtatagcctggctgacgtggacgtgtacaaccccatcagcgtggtgtacctgagcaaggatacctgcgtgtccgagcacggcgtgatcgaaacagtggccctgccccaccccgacaacctgaaagagtgcctgtactgcggctccgtgttcctgcggtatctgaccaccggcgccatcatggacatcatcatcatcgacagcaaggacaccgagagacagctggccgccatgggcaacagcaccatcccccccttcaaccccgacatgcacggcgacgatagcaaggccgtgctgctgttccccaacggcaccgtggtcacactgctgggcttcgagcggagacaggccatcagaatgagcggccagtacctgggcgcctctctgggtggtgcctttctggccgtcgtgggctttggcatcatcggctggatgctgtgcggcaacagcagactgcgcgagtacaacaagatccccctgacctaatctagacgtcgcgaccacccaggatccgcctataactctctacggctaacctgaatggactacgacatagtctagtcgacgccaccatggccagccacaagtggctgctgcagatgatcgtgttcctgaaaaccatcacaatcgcctactgcctgcatctgcaggacgacacccctctgttcttcggcgccaagcctctgagcgacgtgtccctgatcatcaccgagccttgcgtgtccagcgtgtacgaggcctgggattatgccgcccctcccgtgtccaatctgagcgaagccctgagcggcatcgtggtcaagaccaagtgccccgtgcccgaagtgatcctgtggttcaaggacaagcagatggcctactggaccaacccttacgtgaccctgaagggcctgacccagagcgtgggcgaggaacacaagagcggcgacatcagagatgccctgctggatgccctgtccggtgtctgggtggacagcacaccctccagcaccaacatccccgagaacggctgtgtgtggggagccgaccggctgttccagagagtgtgtcagtaatctagacgcggccgcatacagcagcaattggcaagctgcttacatagaactcgcggcgattggcatgccgccttaaaatttttattttatttttcttttcttttccgaatcggattttgtttttaatatttcaaaaaaaaaaaaaaaaaaaaaaaaaaaaaaaaaaagggtcggcatggcatctccacctcctcgcggtccgacctgggcatccgaaggaggacgcacgtccactcggatggctaagggagagccacgtttaaaccagctccaattcgccctatagtgagtcgtattacgcgcgctcactggccgtcgttttacaacgtcgtgactgggaaaaccctggcgttacccaacttaatcgccttgcagcacatccccctttcgccagctggcgtaatagcgaagaggcccgcaccgatcgcccttcccaacagttgcgcagcctgaatggcgaatgggacgcgccctgtagcggcgcattaagcgcggcgggtgtggtggttacgcgcagcgtgaccgctacacttgccagcgccctagcgcccgctcctttcgctttcttcccttcctttctcgccacgttcgccggctttccccgtcaagctctaaatcgggggctccctttagggttccgatttagtgctttacggcacctcgaccccaaaaaacttgattagggtgatggttcacgtagtgggccatcgccctgatagacggtttttcgccctttgacgttggagtccacgttctttaatagtggactcttgttccaaactggaacaacactcaaccctatctcggtctattcttttgatttataagggattttgccgatttcggcctattggttaaaaaatgagctgatttaacaaaaatttaacgcgaattttaacaaaatattaacgcttacaatttaggtggcacttttcggggaaatgtgcgcggaacccctatttgtttatttttctaaatacattcaaatatgtatccgctcatgagacaataaccctgataaatgcttcaataatattgaaaaaggaagagtatgagtattcaacatttccgtgtcgcccttattcccttttttgcggcattttgccttcctgtttttgctcacccagaaacgctggtgaaagtaaaagatgctgaagatcagttgggtgcacgagtgggttacatcgaactggatctcaacagcggtaagatccttgagagttttcgccccgaagaacgttttccaatgatgagcacttttaaagttctgctatgtggcgcggtattatcccgtattgacgccgggcaagagcaactcggtcgccgcatacactattctcagaatgacttggttgagtactcaccagtcacagaaaagcatcttacggatggcatgacagtaagagaattatgcagtgctgccataaccatgagtgataacactgcggccaacttacttctgacaacgatcggaggaccgaaggagctaaccgcttttttgcacaacatgggggatcatgtaactcgccttgatcgttgggaaccggagctgaatgaagccataccaaacgacgagcgtgacaccacgatgcctgtagcaatggcaacaacgttgcgcaaactattaactggcgaactacttactctagcttcccggcaacaattaatagactggatggaggcggataaagttgcaggaccacttctgcgctcggcccttccggctggctggtttattgctgataaatctggagccggtgagcgtgggtctcgcggtatcattgcagcactggggccagatggtaagccctcccgtatcgtagttatctacacgacggggagtcaggcaactatggatgaacgaaatagacagatcgctgagataggtgcctcactgattaagcattggtaactgtcagaccaagtttactcatatatactttagattgatttaaaacttcatttttaatttaaaaggatctaggtgaagatcctttttgataatctcatgaccaaaatcccttaacgtgagttttcgttccactgagcgtcagaccccgtagaaaagatcaaaggatcttcttgagatcctttttttctgcgcgtaatctgctgcttgcaaacaaaaaaaccaccgctaccagcggtggtttgtttgccggatcaagagctaccaactctttttccgaaggtaactggcttcagcagagcgcagataccaaatactgttcttctagtgtagccgtagttaggccaccacttcaagaactctgtagcaccgcctacatacctcgctctgctaatcctgttaccagtggctgctgccagtggcgataagtcgtgtcttaccgggttggactcaagacgatagttaccggataaggcgcagcggtcgggctgaacggggggttcgtgcacacagcccagcttggagcgaacgacctacaccgaactgagatacctacagcgtgagctatgagaaagcgccacgcttcccgaagggagaaaggcggacaggtatccggtaagcggcagggtcggaacaggagagcgcacgagggagcttccagggggaaacgcctggtatctttatagtcctgtcgggtttcgccacctctgacttgagcgtcgatttttgtgatgctcgtcaggggggcggagcctatggaaaaacgccagcaacgcggcctttttacggttcctggccttttgctggccttttgctcacatgttctttcctgcgttatcccctgattctgtggataaccgtattaccgcctttgagtgagctgataccgctcgccgcagccgaacgaccgagcgcagcgagtcagtgagcgaggaagcggaagagcgcccaatacgcaaaccgcctctccccgcgcgttggccgattcattaatgcagctggcacgacaggtttcccgactggaaagcgggcagtgagcgcaacgcaattaatgtgagttagctcactcattaggcaccccaggctttacactttatgctcccggctcgtatgttgtgtggaattgtgagcggataacaatttcacacaggaaacagctatgaccatgattacgccaagcgcgcaattaaccctcactaaagggaacaaaagctgggtaccgggcccacgcgtaatacgactcactatag

SEQ ID NO: 77 - DNA, 12604 bp, Artificial Sequence
  source: /note="Description of Artificial Sequence: Synthetic polynucleotide"
ataggcggcgcatgagagaagcccagaccaattacctacccaaaatggagaaagttcacgttgacatcgaggaagacagcccattcctcagagctttgcagcggagcttcccgcagtttgaggtagaagccaagcaggtcactgataatgaccatgctaatgccagagcgttttcgcatctggcttcaaaactgatcgaaacggaggtggacccatccgacacgatccttgacattggaagtgcgcccgcccgcagaatgtattctaagcacaagtatcattgtatctgtccgatgagatgtgcggaagatccggacagattgtataagtatgcaactaagctgaagaaaaactgtaaggaaataactgataaggaattggacaagaaaatgaaggagctcgccgccgtcatgagcgaccctgacctggaaactgagactatgtgcctccacgacgacgagtcgtgtcgctacgaagggcaagtcgctgtttaccaggatgtatacgcggttgacggaccgacaagtctctatcaccaagccaataagggagttagagtcgcctactggataggctttgacaccaccccttttatgtttaagaacttggctggagcatatccatcatactctaccaactgggccgacgaaaccgtgttaacggctcgtaacataggcctatgcagctctgacgttatggagcggtcacgtagagggatgtccattcttagaaagaagtatttgaaaccatccaacaatgttctattctctgttggctcgaccatctaccacgagaagagggacttactgaggagctggcacctgccgtctgtatttcacttacgtggcaagcaaaattacacatgtcggtgtgagactatagttagttgcgacgggtacgtcgttaaaagaatagctatcagtccaggcctgtatgggaagccttcaggctatgctgctacgatgcaccgcgagggattcttgtgctgcaaagtgacagacacattgaacggggagagggtctcttttcccgtgtgcacgtatgtgccagctacattgtgtgaccaaatgactggcatactggcaacagatgtcagtgcggacgacgcgcaaaaactgctggttgggctcaaccagcgtatagtcgtcaacggtcgcacccagagaaacaccaataccatgaaaaattaccttttgcccgtagtggcccaggcatttgctaggtgggcaaaggaatataaggaagatcaagaagatgaaaggccactaggactacgagatagacagttagtcatggggtgttgttgggcttttagaaggcacaagataacatctatttataagcgcccggatacccaaaccatcatcaaagtgaacagcgatttccactcattcgtgctgcccaggataggcagtaacacattggagatcgggctgagaacaagaatcaggaaaatgttagaggagcacaaggagccgtcacctctcattaccgccgaggacgtacaagaagctaagtgcgcagccgatgaggctaaggaggtgcgtgaagccgaggagttgcgcgcagctctaccacctttggcagctgatgttgaggagcccactctggaagccgatgtagacttgatgttacaagaggctggggccggctcagtggagacacctcgtggcttgataaaggttaccagctacgatggcgaggacaagatcggctcttacgctgtgctttctccgcaggctgtactcaagagtgaaaaattatcttgcatccaccctctcgctgaacaagtcatagtgataacacactctggccgaaaagggcgttatgccgtggaaccataccatggtaaagtagtggtgccagagggacatgcaatacccgtccaggactttcaagctctgagtgaaagtgccaccattgtgtacaacgaacgtgagttcgtaaacaggtacctgcaccatattgccacacatggaggagcgctgaacactgatgaagaatattacaaaactgtcaagcccagcgagcacgacggcgaatacctgtacgacatcgacaggaaacagtgcgtcaagaaagaactagtcactgggctagggctcacaggcgagctggtggatcctcccttccatgaattcgcctacgagagtctgagaacacgaccagccgctccttaccaagtaccaaccataggggtgtatggcgtgccaggatcaggcaagtctggcatcattaaaagcgcagtcaccaaaaaagatctagtggtgagcgccaagaaagaaaactgtgcagaaattataagggacgtcaagaaaatgaaagggctggacgtcaatgccagaactgtggactcagtgctcttgaatggatgcaaacaccccgtagagaccctgtatattgacgaagcttttgcttgtcatgcaggtactctcagagcgctcatagccattataagacctaaaaaggcagtgctctgcggggatcccaaacagtgcggtttttttaacatgatgtgcctgaaagtgcattttaaccacgagatttgcacacaagtcttccacaaaagcatctctcgccgttgcactaaatctgtgacttcggtcgtctcaaccttgttttacgacaaaaaaatgagaacgacgaatccgaaagagactaagattgtgattgacactaccggcagtaccaaacctaagcaggacgatctcattctcacttgtttcagagggtgggtgaagcagttgcaaatagattacaaaggcaacgaaataatgacggcagctgcctctcaagggctgacccgtaaaggtgtgtatgccgttcggtacaaggtgaatgaaaatcctctgtacgcacccacctcagaacatgtgaacgtcctactgacccgcacggaggaccgcatcgtgtggaaaacactagccggcgacccatggataaaaacactgactgccaagtaccctgggaatttcactgccacgatagaggagtggcaagcagagcatgatgccatcatgaggcacatcttggagagaccggaccctaccgacgtcttccagaataaggcaaacgtgtgttgggccaaggctttagtgccggtgctgaagaccgctggcatagacatgaccactgaacaatggaacactgtggattattttgaaacggacaaagctcactcagcagagatagtattgaaccaactatgcgtgaggttctttggactcgatctggactccggtctattttctgcacccactgttccgttatccattaggaataatcactgggataactccccgtcgcctaacatgtacgggctgaataaagaagtggtccgtcagctctctcgcaggtacccacaactgcctcgggcagttgccactggaagagtctatgacatgaacactggtacactgcgcaattatgatccgcgcataaacctagtacctgtaaacagaagactgcctcatgctttagtcctccaccataatgaacacccacagagtgacttttcttcattcgtcagcaaattgaagggcagaactgtcctggtggtcggggaaaagttgtccgtcccaggcaaaatggttgactggttgtcagaccggcctgaggctaccttcagagctcggctggatttaggcatcccaggtgatgtgcccaaatatgacataatatttgttaatgtgaggaccccatataaataccatcactatcagcagtgtgaagaccatgccattaagcttagcatgttgaccaagaaagcttgtctgcatctgaatcccggcggaacctgtgtcagcataggttatggttacgctgacagggccagcgaaagcatcattggtgctatagcgcggcagttcaagttttcccgggtatgcaaaccgaaatcctcacttgaagagacggaagttctgtttgtattcattgggtacgatcgcaaggcccgtacgcacaatccttacaagctttcatcaaccttgaccaacatttatacaggttccagactccacgaagccggatgtgcaccctcatatcatgtggtgcgaggggatattgccacggccaccgaaggagtgattataaatgctgctaacagcaaaggacaacctggcggaggggtgtgcggagcgctgtataagaaattcccggaaagcttcgatttacagccgatcgaagtaggaaaagcgcgactggtcaaaggtgcagctaaacatatcattcatgccgtaggaccaaacttcaacaaagtttcggaggttgaaggtgacaaacagttggcagaggcttatgagtccatcgctaagattgtcaacgataacaattacaagtcagtagcgattccactgttgtccaccggcatcttttccgggaacaaagatcgactaacccaatcattgaaccatttgctgacagctttagacaccactgatgcagatgtagccatatactgcagggacaagaaatgggaaatgactctcaaggaagcagtggctaggagagaagcagtggaggagatatgcatatccgacgactcttcagtgacagaacctgatgcagagctggtgagggtgcatccgaagagttctttggctggaaggaagggctacagcacaagcgatggcaaaactttctcatatttggaagggaccaagtttcaccaggcggccaaggatatagcagaaattaatgccatgtggcccgttgcaacggaggccaatgagcaggtatgcatgtatatcctcggagaaagcatgagcagtattaggtcgaaatgccccgtcgaagagtcggaagcctccacaccacctagcacgctgccttgcttgtgcatccatgccatgactccagaaagagtacagcgcctaaaagcctcacgtccagaacaaattactgtgtgctcatcctttccattgccgaagtatagaatcactggtgtgcagaagatccaatgctcccagcctatattgttctcaccgaaagtgcctgcgtatattcatccaaggaagtatctcgtggaaacaccaccggtagacgagactccggagccatcggcagagaaccaatccacagaggggacacctgaacaaccaccacttataaccgaggatgagaccaggactagaacgcctgagccgatcatcatcgaagaggaagaagaggatagcataagtttgctgtcagatggcccgacccaccaggtgctgcaagtcgaggcagacattcacgggccgccctctgtatctagctcatcctggtccattcctcatgcatccgactttgatgtggacagtttatccatacttgacaccctggagggagctagcgtgaccagcggggcaacgtcagccgagactaactcttacttcgcaaagagtatggagtttctggcgcgaccggtgcctgcgcctcgaacagtattcaggaaccctccacatcccgctccgcgcacaagaacaccgtcacttgcacccagcagggcctgctcgagaaccagcctagtttccaccccgccaggcgtgaatagggtgatcactagagaggagctcgaggcgcttaccccgtcacgcactcctagcaggtcggtctcgagaaccagcctggtctccaacccgccaggcgtaaatagggtgattacaagagaggagtttgaggcgttcgtagcacaacaacaatgacggtttgatgcgggtgcatacatcttttcctccgacaccggtcaagggcatttacaacaaaaatcagtaaggcaaacggtgctatccgaagtggtgttggagaggaccgaattggagatttcgtatgccccgcgcctcgaccaagaaaaagaagaattactacgcaagaaattacagttaaatcccacacctgctaacagaagcagataccagtccaggaaggtggagaacatgaaagccataacagctagacgtattctgcaaggcctagggcattatttgaaggcagaaggaaaagtggagtgctaccgaaccctgcatcctgttcctttgtattcatctagtgtgaaccgtgccttttcaagccccaaggtcgcagtggaagcctgtaacgccatgttgaaagagaactttccgactgtggcttcttactgtattattccagagtacgatgcctatttggacatggttgacggagcttcatgctgcttagacactgccagtttttgccctgcaaagctgcgcagctttccaaagaaacactcctatttggaacccacaatacgatcggcagtgccttcagcgatccagaacacgctccagaacgtcctggcagctgccacaaaaagaaattgcaatgtcacgcaaatgagagaattgcccgtattggattcggcggcctttaatgtggaatgcttcaagaaatatgcgtgtaataatgaatattgggaaacgtttaaagaaaaccccatcaggcttactgaagaaaacgtggtaaattacattaccaaattaaaaggaccaaaagctgctgctctttttgcgaagacacataatttgaatatgttgcaggacataccaatggacaggtttgtaatggacttaaagagagacgtgaaagtgactccaggaacaaaacatactgaagaacggcccaaggtacaggtgatccaggctgccgatccgctagcaacagcgtatctgtgcggaatccaccgagagctggttaggagattaaatgcggtcctgcttccgaacattcatacactgtttgatatgtcggctgaagactttgacgctattatagccgagcacttccagcctggggattgtgttctggaaactgacatcgcgtcgtttgataaaagtgaggacgacgccatggctctgaccgcgttaatgattctggaagacttaggtgtggacgcagagctgttgacgctgattgaggcggctttcggcgaaatttcatcaatacatttgcccactaaaactaaatttaaattcggagccatgatgaaatctggaatgttcctcacactgtttgtgaacacagtcattaacattgtaatcgcaagcagagtgttgagagaacggctaaccggatcaccatgtgcagcattcattggagatgacaatatcgtgaaaggagtcaaatcggacaaattaatggcagacaggtgcgccacctggttgaatatggaagtcaagattatagatgctgtggtgggcgagaaagcgccttatttctgtggagggtttattttgtgtgactccgtgaccggcacagcgtgccgtgtggcagaccccctaaaaaggctgtttaagcttggcaaacctctggcagcagacgatgaacatgatgatgacaggagaagggcattgcatgaagagtcaacacgctggaaccgagtgggtattctttcagagctgtgcaaggcagtagaatcaaggtatgaaaccgtaggaacttccatcatagttatggccatgactactctagctagcagtgttaaatcattcagctacctgagaggggcccctataactctctacggctaacctgaatggactacgacatagtctagtcgagtctagtcgacgccaccatgggcaccgtgaacaagcctgtcgtgggcgtgctgatgggcttcggcatcatcaccggcaccctgagaatcaccaaccctgtgcgggccagcgtgctgagatacgacgacttccacatcgacgaggacaagctggacaccaacagcgtgtacgagccctactaccacagcgaccacgccgagagcagctgggtcaacagaggcgagagcagccggaaggcctacgaccacaacagcccctacatctggccccggaacgactacgacggcttcctggaaaacgcccacgagcaccacggcgtgtacaatcagggcagaggcatcgacagcggcgagagactgatgcagcccacacagatgagcgcccaggaagatctgggcgacgacacaggcatccacgtgatccccaccctgaacggcgacgaccggcacaagatcgtgaacgtggaccagcggcagtacggcgacgtgttcaagggcgacctgaaccctaagccccagggccagagactgatcgaggtgtccgtggaagagaaccaccccttcaccctgagagcccccatccagagaatctacggcgtgcggtataccgagacttggagcttcctgcccagcctgacctgtacaggcgacgccgctcctgccatccagcacatctgcctgaagcacaccacctgtttccaggacgtggtggtggacgtggactgcgccgagaacaccaaagaggaccagctggccgagatcagctaccggttccagggcaagaaagaggccgaccagccctggatcgtggtcaataccagcaccctgttcgacgagctggaactggacccccccgagattgaacccggcgtgctgaaggtgctgcggaccgagaagcagtacctgggcgtgtacatctggaacatgcggggctccgacggcacctctacctacgccaccttcctggtcacatggaagggcgacgagaaaacccggaaccctacccctgccgtgacccctcagcctagaggcgccgagttccatatgtggaattaccactcccacgtgttcagcgtgggcgacaccttcagcctggccatgcatctgcagtacaagatccacgaggcccccttcgacctgctgctggaatggctgtacgtgcccatcgaccctacctgccagcccatgcggctgtacagcacctgtctgtaccaccccaacgcccctcagtgcctgagccacatgaacagcggctgcaccttcaccagccctcacctggctcagagggtggccagcaccgtgtaccagaattgcgagcacgccgacaactacaccgcctactgcctgggcatcagccacatggaacccagcttcggcctgatcctgcacgatggcggcaccaccctgaagttcgtggacacacccgagagcctgagcggcctgtacgtgttcgtggtgtacttcaacggccacgtggaagccgtggcctacaccgtggtgtccaccgtggaccacttcgtgaacgccatcgaggaaagaggcttcccacccacagccggacagcctccagccaccaccaagcccaaagaaatcacccccgtgaaccccggcaccagccccctgctgagatatgctgcttggacaggcggactggccgctgtggtgctgctgtgcctggtcatcttcctgatctgcaccgccaagcggatgagagtgaaggcctaccgggtggacaagtccccctacaaccagagcatgtactacgccggcctgcccgtggacgatttcgaggatagcgagagcaccgacaccgaggaagagttcggcaacgccatcggcggatctcacggcggcagcagctacaccgtgtacatcgacaagaccagataatctagacgcggccgcatacagcagcaattggcaagctgcttacatagaactcgcggcgattggcatgccgccttaaaatttttattttatttttcttttcttttccgaatcggattttgtttttaatatttcaaaaaaaaaaaaaaaaaaaaaaaaaaaaaaaaaaagggtcggcatggcatctccacctcctcgcggtccgacctgggcatccgaaggaggacgcacgtccactcggatggctaagggagagccacgtttaaaccagctccaattcgccctatagtgagtcgtattacgcgcgctcactggccgtcgttttacaacgtcgtgactgggaaaaccctggcgttacccaacttaatcgccttgcagcacatccccctttcgccagctggcgtaatagcgaagaggcccgcaccgatcgcccttcccaacagttgcgcagcctgaatggcgaatgggacgcgccctgtagcggcgcattaagcgcggcgggtgtggtggttacgcgcagcgtgaccgctacacttgccagcgccctagcgcccgctcctttcgctttcttcccttcctttctcgccacgttcgccggctttccccgtcaagctctaaatcgggggctccctttagggttccgatttagtgctttacggcacctcgaccccaaaaaacttgattagggtgatggttcacgtagtgggccatcgccctgatagacggtttttcgccctttgacgttggagtccacgttctttaatagtggactcttgttccaaactggaacaacactcaaccctatctcggtctattcttttgatttataagggattttgccgatttcggcctattggttaaaaaatgagctgatttaacaaaaatttaacgcgaattttaacaaaatattaacgcttacaatttaggtggcacttttcggggaaatgtgcgcggaacccctatttgtttatttttctaaatacattcaaatatgtatccgctcatgagacaataaccctgataaatgcttcaataatattgaaaaaggaagagtatgagtattcaacatttccgtgtcgcccttattcccttttttgcggcattttgccttcctgtttttgctcacccagaaacgctggtgaaagtaaaagatgctgaagatcagttgggtgcacgagtgggttacatcgaactggatctcaacagcggtaagatccttgagagttttcgccccgaagaacgttttccaatgatgagcacttttaaagttctgctatgtggcgcggtattatcccgtattgacgccgggcaagagcaactcggtcgccgcatacactattctcagaatgacttggttgagtactcaccagtcacagaaaagcatcttacggatggcatgacagtaagagaattatgcagtgctgccataaccatgagtgataacactgcggccaacttacttctgacaacgatcggaggaccgaaggagctaaccgcttttttgcacaacatgggggatcatgtaactcgccttgatcgttgggaaccggagctgaatgaagccataccaaacgacgagcgtgacaccacgatgcctgtagcaatggcaacaacgttgcgcaaactattaactggcgaactacttactctagcttcccggcaacaattaatagactggatggaggcggataaagttgcaggaccacttctgcgctcggcccttccggctggctggtttattgctgataaatctggagccggtgagcgtgggtctcgcggtatcattgcagcactggggccagatggtaagccctcccgtatcgtagttatctacacgacggggagtcaggcaactatggatgaacgaaatagacagatcgctgagataggtgcctcactgattaagcattggtaactgtcagaccaagtttactcatatatactttagattgatttaaaacttcatttttaatttaaaaggatctaggtgaagatcctttttgataatctcatgaccaaaatcccttaacgtgagttttcgttccactgagcgtcagaccccgtagaaaagatcaaaggatcttcttgagatcctttttttctgcgcgtaatctgctgcttgcaaacaaaaaaaccaccgctaccagcggtggtttgtttgccggatcaagagctaccaactctttttccgaaggtaactggcttcagcagagcgcagataccaaatactgttcttctagtgtagccgtagttaggccaccacttcaagaactctgtagcaccgcctacatacctcgctctgctaatcctgttaccagtggctgctgccagtggcgataagtcgtgtcttaccgggttggactcaagacgatagttaccggataaggcgcagcggtcgggctgaacggggggttcgtgcacacagcccagcttggagcgaacgacctacaccgaactgagatacctacagcgtgagctatgagaaagcgccacgcttcccgaagggagaaaggcggacaggtatccggtaagcggcagggtcggaacaggagagcgcacgagggagcttccagggggaaacgcctggtatctttatagtcctgtcgggtttcgccacctctgacttgagcgtcgatttttgtgatgctcgtcaggggggcggagcctatggaaaaacgccagcaacgcggcctttttacggttcctggccttttgctggccttttgctcacatgttctttcctgcgttatcccctgattctgtggataaccgtattaccgcctttgagtgagctgataccgctcgccgcagccgaacgaccgagcgcagcgagtcagtgagcgaggaagcggaagagcgcccaatacgcaaaccgcctctccccgcgcgttggccgattcattaatgcagctggcacgacaggtttcccgactggaaagcgggcagtgagcgcaacgcaattaatgtgagttagctcactcattaggcaccccaggctttacactttatgctcccggctcgtatgttgtgtggaattgtgagcggataacaatttcacacaggaaacagctatgaccatgattacgccaagcgcgcaattaaccctcactaaagggaacaaaagctgggtaccgggcccacgcgtaatacgactcactatag

SEQ ID NO: 78 - DNA, 11797 bp, Artificial Sequence
  source: /note="Description of Artificial Sequence: Synthetic polynucleotide"
ataggcggcgcatgagagaagcccagaccaattacctacccaaaatggagaaagttcacgttgacatcgaggaagacagcccattcctcagagctttgcagcggagcttcccgcagtttgaggtagaagccaagcaggtcactgataatgaccatgctaatgccagagcgttttcgcatctggcttcaaaactgatcgaaacggaggtggacccatccgacacgatccttgacattggaagtgcgcccgcccgcagaatgtattctaagcacaagtatcattgtatctgtccgatgagatgtgcggaagatccggacagattgtataagtatgcaactaagctgaagaaaaactgtaaggaaataactgataaggaattggacaagaaaatgaaggagctcgccgccgtcatgagcgaccctgacctggaaactgagactatgtgcctccacgacgacgagtcgtgtcgctacgaagggcaagtcgctgtttaccaggatgtatacgcggttgacggaccgacaagtctctatcaccaagccaataagggagttagagtcgcctactggataggctttgacaccaccccttttatgtttaagaacttggctggagcatatccatcatactctaccaactgggccgacgaaaccgtgttaacggctcgtaacataggcctatgcagctctgacgttatggagcggtcacgtagagggatgtccattcttagaaagaagtatttgaaaccatccaacaatgttctattctctgttggctcgaccatctaccacgagaagagggacttactgaggagctggcacctgccgtctgtatttcacttacgtggcaagcaaaattacacatgtcggtgtgagactatagttagttgcgacgggtacgtcgttaaaagaatagctatcagtccaggcctgtatgggaagccttcaggctatgctgctacgatgcaccgcgagggattcttgtgctgcaaagtgacagacacattgaacggggagagggtctcttttcccgtgtgcacgtatgtgccagctacattgtgtgaccaaatgactggcatactggcaacagatgtcagtgcggacgacgcgcaaaaactgctggttgggctcaaccagcgtatagtcgtcaacggtcgcacccagagaaacaccaataccatgaaaaattaccttttgcccgtagtggcccaggcatttgctaggtgggcaaaggaatataaggaagatcaagaagatgaaaggccactaggactacgagatagacagttagtcatggggtgttgttgggcttttagaaggcacaagataacatctatttataagcgcccggatacccaaaccatcatcaaagtgaacagcgatttccactcattcgtgctgcccaggataggcagtaacacattggagatcgggctgagaacaagaatcaggaaaatgttagaggagcacaaggagccgtcacctctcattaccgccgaggacgtacaagaagctaagtgcgcagccgatgaggctaaggaggtgcgtgaagccgaggagttgcgcgcagctctaccacctttggcagctgatgttgaggagcccactctggaagccgatgtagacttgatgttacaagaggctggggccggctcagtggagacacctcgtggcttgataaaggttaccagctacgatggcgaggacaagatcggctcttacgctgtgctttctccgcaggctgtactcaagagtgaaaaattatcttgcatccaccctctcgctgaacaagtcatagtgataacacactctggccgaaaagggcgttatgccgtggaaccataccatggtaaagtagtggtgccagagggacatgcaatacccgtccaggactttcaagctctgagtgaaagtgccaccattgtgtacaacgaacgtgagttcgtaaacaggtacctgcaccatattgccacacatggaggagcgctgaacactgatgaagaatattacaaaactgtcaagcccagcgagcacgacggcgaatacctgtacgacatcgacaggaaacagtgcgtcaagaaagaactagtcactgggctagggctcacaggcgagctggtggatcctcccttccatgaattcgcctacgagagtctgagaacacgaccagccgctccttaccaagtaccaaccataggggtgtatggcgtgccaggatcaggcaagtctggcatcattaaaagcgcagtcaccaaaaaagatctagtggtgagcgccaagaaagaaaactgtgcagaaattataagggacgtcaagaaaatgaaagggctggacgtcaatgccagaactgtggactcagtgctcttgaatggatgcaaacaccccgtagagaccctgtatattgacgaagcttttgcttgtcatgcaggtactctcagagcgctcatagccattataagacctaaaaaggcagtgctctgcggggatcccaaacagtgcggtttttttaacatgatgtgcctgaaagtgcattttaaccacgagatttgcacacaagtcttccacaaaagcatctctcgccgttgcactaaatctgtgacttcggtcgtctcaaccttgttttacgacaaaaaaatgagaacgacgaatccgaaagagactaagattgtgattgacactaccggcagtaccaaacctaagcaggacgatctcattctcacttgtttcagagggtgggtgaagcagttgcaaatagattacaaaggcaacgaaataatgacggcagctgcctctcaagggctgacccgtaaaggtgtgtatgccgttcggtacaaggtgaatgaaaatcctctgtacgcacccacctcagaacatgtgaacgtcctactgacccgcacggaggaccgcatcgtgtggaaaacactagccggcgacccatggataaaaacactgactgccaagtaccctgggaatttcactgccacgatagaggagtggcaagcagagcatgatgccatcatgaggcacatcttggagagaccggaccctaccgacgtcttccagaataaggcaaacgtgtgttgggccaaggctttagtgccggtgctgaagaccgctggcatagacatgaccactgaacaatggaacactgtggattattttgaaacggacaaagctcactcagcagagatagtattgaaccaactatgcgtgaggttctttggactcgatctggactccggtctattttctgcacccactgttccgttatccattaggaataatcactgggataactccccgtcgcctaacatgtacgggctgaataaagaagtggtccgtcagctctctcgcaggtacccacaactgcctcgggcagttgccactggaagagtctatgacatgaacactggtacactgcgcaattatgatccgcgcataaacctagtacctgtaaacagaagactgcctcatgctttagtcctccaccataatgaacacccacagagtgacttttcttcattcgtcagcaaattgaagggcagaactgtcctggtggtcggggaaaagttgtccgtcccaggcaaaatggttgactggttgtcagaccggcctgaggctaccttcagagctcggctggatttaggcatcccaggtgatgtgcccaaatatgacataatatttgttaatgtgaggaccccatataaataccatcactatcagcagtgtgaagaccatgccattaagcttagcatgttgaccaagaaagcttgtctgcatctgaatcccggcggaacctgtgtcagcataggttatggttacgctgacagggccagcgaaagcatcattggtgctatagcgcggcagttcaagttttcccgggtatgcaaaccgaaatcctcacttgaagagacggaagttctgtttgtattcattgggtacgatcgcaaggcccgtacgcacaatccttacaagctttcatcaaccttgaccaacatttatacaggttccagactccacgaagccggatgtgcaccctcatatcatgtggtgcgaggggatattgccacggccaccgaaggagtgattataaatgctgctaacagcaaaggacaacctggcggaggggtgtgcggagcgctgtataagaaattcccggaaagcttcgatttacagccgatcgaagtaggaaaagcgcgactggtcaaaggtgcagctaaacatatcattcatgccgtaggaccaaacttcaacaaagtttcggaggttgaaggtgacaaacagttggcagaggcttatgagtccatcgctaagattgtcaacgataacaattacaagtcagtagcgattccactgttgtccaccggcatcttttccgggaacaaagatcgactaacccaatcattgaaccatttgctgacagctttagacaccactgatgcagatgtagccatatactgcagggacaagaaatgggaaatgactctcaaggaagcagtggctaggagagaagcagtggaggagatatgcatatccgacgactcttcagtgacagaacctgatgcagagctggtgagggtgcatccgaagagttctttggctggaaggaagggctacagcacaagcgatggcaaaactttctcatatttggaagggaccaagtttcaccaggcggccaaggatatagcagaaattaatgccatgtggcccgttgcaacggaggccaatgagcaggtatgcatgtatatcctcggagaaagcatgagcagtattaggtcgaaatgccccgtcgaagagtcggaagcctccacaccacctagcacgctgccttgcttgtgcatccatgccatgactccagaaagagtacagcgcctaaaagcctcacgtccagaacaaattactgtgtgctcatcctttccattgccgaagtatagaatcactggtgtgcagaagatccaatgctcccagcctatattgttctcaccgaaagtgcctgcgtatattcatccaaggaagtatctcgtggaaacaccaccggtagacgagactccggagccatcggcagagaaccaatccacagaggggacacctgaacaaccaccacttataaccgaggatgagaccaggactagaacgcctgagccgatcatcatcgaagaggaagaagaggatagcataagtttgctgtcagatggcccgacccaccaggtgctgcaagtcgaggcagacattcacgggccgccctctgtatctagctcatcctggtccattcctcatgcatccgactttgatgtggacagtttatccatacttgacaccctggagggagctagcgtgaccagcggggcaacgtcagccgagactaactcttacttcgcaaagagtatggagtttctggcgcgaccggtgcctgcgcctcgaacagtattcaggaaccctccacatcccgctccgcgcacaagaacaccgtcacttgcacccagcagggcctgctcgagaaccagcctagtttccaccccgccaggcgtgaatagggtgatcactagagaggagctcgaggcgcttaccccgtcacgcactcctagcaggtcggtctcgagaaccagcctggtctccaacccgccaggcgtaaatagggtgattacaagagaggagtttgaggcgttcgtagcacaacaacaatgacggtttgatgcgggtgcatacatcttttcctccgacaccggtcaagggcatttacaacaaaaatcagtaaggcaaacggtgctatccgaagtggtgttggagaggaccgaattggagatttcgtatgccccgcgcctcgaccaagaaaaagaagaattactacgcaagaaattacagttaaatcccacacctgctaacagaagcagataccagtccaggaaggtggagaacatgaaagccataacagctagacgtattctgcaaggcctagggcattatttgaaggcagaaggaaaagtggagtgctaccgaaccctgcatcctgttcctttgtattcatctagtgtgaaccgtgccttttcaagccccaaggtcgcagtggaagcctgtaacgccatgttgaaagagaactttccgactgtggcttcttactgtattattccagagtacgatgcctatttggacatggttgacggagcttcatgctgcttagacactgccagtttttgccctgcaaagctgcgcagctttccaaagaaacactcctatttggaacccacaatacgatcggcagtgccttcagcgatccagaacacgctccagaacgtcctggcagctgccacaaaaagaaattgcaatgtcacgcaaatgagagaattgcccgtattggattcggcggcctttaatgtggaatgcttcaagaaatatgcgtgtaataatgaatattgggaaacgtttaaagaaaaccccatcaggcttactgaagaaaacgtggtaaattacattaccaaattaaaaggaccaaaagctgctgctctttttgcgaagacacataatttgaatatgttgcaggacataccaatggacaggtttgtaatggacttaaagagagacgtgaaagtgactccaggaacaaaacatactgaagaacggcccaaggtacaggtgatccaggctgccgatccgctagcaacagcgtatctgtgcggaatccaccgagagctggttaggagattaaatgcggtcctgcttccgaacattcatacactgtttgatatgtcggctgaagactttgacgctattatagccgagcacttccagcctggggattgtgttctggaaactgacatcgcgtcgtttgataaaagtgaggacgacgccatggctctgaccgcgttaatgattctggaagacttaggtgtggacgcagagctgttgacgctgattgaggcggctttcggcgaaatttcatcaatacatttgcccactaaaactaaatttaaattcggagccatgatgaaatctggaatgttcctcacactgtttgtgaacacagtcattaacattgtaatcgcaagcagagtgttgagagaacggctaaccggatcaccatgtgcagcattcattggagatgacaatatcgtgaaaggagtcaaatcggacaaattaatggcagacaggtgcgccacctggttgaatatggaagtcaagattatagatgctgtggtgggcgagaaagcgccttatttctgtggagggtttattttgtgtgactccgtgaccggcacagcgtgccgtgtggcagaccccctaaaaaggctgtttaagcttggcaaacctctggcagcagacgatgaacatgatgatgacaggagaagggcattgcatgaagagtcaacacgctggaaccgagtgggtattctttcagagctgtgcaaggcagtagaatcaaggtatgaaaccgtaggaacttccatcatagttatggccatgactactctagctagcagtgttaaatcattcagctacctgagaggggcccctataactctctacggctaacctgaatggactacgacatagtctagtcgagtctagtcgacgccaccatgtttctgatccagtgcctgatcagcgccgtgatcttctatattcaagtcacaaacgccctgatctttaagggcgaccacgtgtcactgcaggtcaacagcagcctgaccagcatcctgatccccatgcagaacgacaattacaccgagatcaagggccagctggtgttcatcggcgagcagctgcccaccggcaccaattacagcggcaccctggaactgctgtacgccgataccgtggccttctgcttcagaagcgtgcaggtcatcagatacgacggctgcccccggatcagaaccagcgccttcatcagctgccggtacaagcacagctggcactacggcaacagcaccgaccggatcagcaccgaacctgatgccggcgtgatgctgaagatcaccaagcccggcatcaacgacgccggcgtgtacgtgctgctcgtgcggctggatcacagcagaagcaccgacggcttcatcctgggcgtgaacgtgtacaccgccggcagccaccacaacatccacggcgtgatctacaccagccccagcctgcagaacggctacagcaccagagccctgttccagcaggccagactgtgcgatctgcccgccacacctaagggcagcggcacaagcctgtttcagcacatgctggacctgagagccggcaagagcctggaagataacccctggctgcacgaggacgtggtcaccaccgagacaaagagcgtggtcaaagagggcatcgagaaccacgtgtaccccaccgacatgagcaccctgcccgagaagtccctgaacgacccccctgagaacctgctgatcatcatccccatcgtggccagcgtgatgatcctgaccgccatggtcatcgtgatcgtgatcagcgtgaagcggcggagaatcaagaagcaccccatctaccggcccaacaccaagaccagacggggcatccagaacgccacccctgagtccgacgtgatgctggaagccgccattgcccagctggccaccatcagagaggaaagcccccctcacagcgtcgtgaaccccttcgtgaagtaatctagacgcggccgcatacagcagcaattggcaagctgcttacatagaactcgcggcgattggcatgccgccttaaaatttttattttatttttcttttcttttccgaatcggattttgtttttaatatttcaaaaaaaaaaaaaaaaaaaaaaaaaaaaaaaaaaagggtcggcatggcatctccacctcctcgcggtccgacctgggcatccgaaggaggacgcacgtccactcggatggctaagggagagccacgtttaaaccagctccaattcgccctatagtgagtcgtattacgcgcgctcactggccgtcgttttacaacgtcgtgactgggaaaaccctggcgttacccaacttaatcgccttgcagcacatccccctttcgccagctggcgtaatagcgaagaggcccgcaccgatcgcccttcccaacagttgcgcagcctgaatggcgaatgggacgcgccctgtagcggcgcattaagcgcggcgggtgtggtggttacgcgcagcgtgaccgctacacttgccagcgccctagcgcccgctcctttcgctttcttcccttcctttctcgccacgttcgccggctttccccgtcaagctctaaatcgggggctccctttagggttccgatttagtgctttacggcacctcgaccccaaaaaacttgattagggtgatggttcacgtagtgggccatcgccctgatagacggtttttcgccctttgacgttggagtccacgttctttaatagtggactcttgttccaaactggaacaacactcaaccctatctcggtctattcttttgatttataagggattttgccgatttcggcctattggttaaaaaatgagctgatttaacaaaaatttaacgcgaattttaacaaaatattaacgcttacaatttaggtggcacttttcggggaaatgtgcgcggaacccctatttgtttatttttctaaatacattcaaatatgtatccgctcatgagacaataaccctgataaatgcttcaataatattgaaaaaggaagagtatgagtattcaacatttccgtgtcgcccttattcccttttttgcggcattttgccttcctgtttttgctcacccagaaacgctggtgaaagtaaaagatgctgaagatcagttgggtgcacgagtgggttacatcgaactggatctcaacagcggtaagatccttgagagttttcgccccgaagaacgttttccaatgatgagcacttttaaagttctgctatgtggcgcggtattatcccgtattgacgccgggcaagagcaactcggtcgccgcatacactattctcagaatgacttggttgagtactcaccagtcacagaaaagcatcttacggatggcatgacagtaagagaattatgcagtgctgccataaccatgagtgataacactgcggccaacttacttctgacaacgatcggaggaccgaaggagctaaccgcttttttgcacaacatgggggatcatgtaactcgccttgatcgttgggaaccggagctgaatgaagccataccaaacgacgagcgtgacaccacgatgcctgtagcaatggcaacaacgttgcgcaaactattaactggcgaactacttactctagcttcccggcaacaattaatagactggatggaggcggataaagttgcaggaccacttctgcgctcggcccttccggctggctggtttattgctgataaatctggagccggtgagcgtgggtctcgcggtatcattgcagcactggggccagatggtaagccctcccgtatcgtagttatctacacgacggggagtcaggcaactatggatgaacgaaatagacagatcgctgagataggtgcctcactgattaagcattggtaactgtcagaccaagtttactcatatatactttagattgatttaaaacttcatttttaatttaaaaggatctaggtgaagatcctttttgataatctcatgaccaaaatcccttaacgtgagttttcgttccactgagcgtcagaccccgtagaaaagatcaaaggatcttcttgagatcctttttttctgcgcgtaatctgctgcttgcaaacaaaaaaaccaccgctaccagcggtggtttgtttgccggatcaagagctaccaactctttttccgaaggtaactggcttcagcagagcgcagataccaaatactgttcttctagtgtagccgtagttaggccaccacttcaagaactctgtagcaccgcctacatacctcgctctgctaatcctgttaccagtggctgctgccagtggcgataagtcgtgtcttaccgggttggactcaagacgatagttaccggataaggcgcagcggtcgggctgaacggggggttcgtgcacacagcccagcttggagcgaacgacctacaccgaactgagatacctacagcgtgagctatgagaaagcgccacgcttcccgaagggagaaaggcggacaggtatccggtaagcggcagggtcggaacaggagagcgcacgagggagcttccagggggaaacgcctggtatctttatagtcctgtcgggtttcgccacctctgacttgagcgtcgatttttgtgatgctcgtcaggggggcggagcctatggaaaaacgccagcaacgcggcctttttacggttcctggccttttgctggccttttgctcacatgttctttcctgcgttatcccctgattctgtggataaccgtattaccgcctttgagtgagctgataccgctcgccgcagccgaacgaccgagcgcagcgagtcagtgagcgaggaagcggaagagcgcccaatacgcaaaccgcctctccccgcgcgttggccgattcattaatgcagctggcacgacaggtttcccgactggaaagcgggcagtgagcgcaacgcaattaatgtgagttagctcactcattaggcaccccaggctttacactttatgctcccggctcgtatgttgtgtggaattgtgagcggataacaatttcacacaggaaacagctatgaccatgattacgccaagcgcgcaattaaccctcactaaagggaacaaaagctgggtaccgggcccacgcgtaatacgactcactatag

SEQ ID NO: 79 - DNA, 13755 bp, Artificial Sequence
  source: /note="Description of Artificial Sequence: Synthetic polynucleotide"
ataggcggcgcatgagagaagcccagaccaattacctacccaaaatggagaaagttcacgttgacatcgaggaagacagcccattcctcagagctttgcagcggagcttcccgcagtttgaggtagaagccaagcaggtcactgataatgaccatgctaatgccagagcgttttcgcatctggcttcaaaactgatcgaaacggaggtggacccatccgacacgatccttgacattggaagtgcgcccgcccgcagaatgtattctaagcacaagtatcattgtatctgtccgatgagatgtgcggaagatccggacagattgtataagtatgcaactaagctgaagaaaaactgtaaggaaataactgataaggaattggacaagaaaatgaaggagctcgccgccgtcatgagcgaccctgacctggaaactgagactatgtgcctccacgacgacgagtcgtgtcgctacgaagggcaagtcgctgtttaccaggatgtatacgcggttgacggaccgacaagtctctatcaccaagccaataagggagttagagtcgcctactggataggctttgacaccaccccttttatgtttaagaacttggctggagcatatccatcatactctaccaactgggccgacgaaaccgtgttaacggctcgtaacataggcctatgcagctctgacgttatggagcggtcacgtagagggatgtccattcttagaaagaagtatttgaaaccatccaacaatgttctattctctgttggctcgaccatctaccacgagaagagggacttactgaggagctggcacctgccgtctgtatttcacttacgtggcaagcaaaattacacatgtcggtgtgagactatagttagttgcgacgggtacgtcgttaaaagaatagctatcagtccaggcctgtatgggaagccttcaggctatgctgctacgatgcaccgcgagggattcttgtgctgcaaagtgacagacacattgaacggggagagggtctcttttcccgtgtgcacgtatgtgccagctacattgtgtgaccaaatgactggcatactggcaacagatgtcagtgcggacgacgcgcaaaaactgctggttgggctcaaccagcgtatagtcgtcaacggtcgcacccagagaaacaccaataccatgaaaaattaccttttgcccgtagtggcccaggcatttgctaggtgggcaaaggaatataaggaagatcaagaagatgaaaggccactaggactacgagatagacagttagtcatggggtgttgttgggcttttagaaggcacaagataacatctatttataagcgcccggatacccaaaccatcatcaaagtgaacagcgatttccactcattcgtgctgcccaggataggcagtaacacattggagatcgggctgagaacaagaatcaggaaaatgttagaggagcacaaggagccgtcacctctcattaccgccgaggacgtacaagaagctaagtgcgcagccgatgaggctaaggaggtgcgtgaagccgaggagttgcgcgcagctctaccacctttggcagctgatgttgaggagcccactctggaagccgatgtagacttgatgttacaagaggctggggccggctcagtggagacacctcgtggcttgataaaggttaccagctacgatggcgaggacaagatcggctcttacgctgtgctttctccgcaggctgtactcaagagtgaaaaattatcttgcatccaccctctcgctgaacaagtcatagtgataacacactctggccgaaaagggcgttatgccgtggaaccataccatggtaaagtagtggtgccagagggacatgcaatacccgtccaggactttcaagctctgagtgaaagtgccaccattgtgtacaacgaacgtgagttcgtaaacaggtacctgcaccatattgccacacatggaggagcgctgaacactgatgaagaatattacaaaactgtcaagcccagcgagcacgacggcgaatacctgtacgacatcgacaggaaacagtgcgtcaagaaagaactagtcactgggctagggctcacaggcgagctggtggatcctcccttccatgaattcgcctacgagagtctgagaacacgaccagccgctccttaccaagtaccaaccataggggtgtatggcgtgccaggatcaggcaagtctggcatcattaaaagcgcagtcaccaaaaaagatctagtggtgagcgccaagaaagaaaactgtgcagaaattataagggacgtcaagaaaatgaaagggctggacgtcaatgccagaactgtggactcagtgctcttgaatggatgcaaacaccccgtagagaccctgtatattgacgaagcttttgcttgtcatgcaggtactctcagagcgctcatagccattataagacctaaaaaggcagtgctctgcggggatcccaaacagtgcggtttttttaacatgatgtgcctgaaagtgcattttaaccacgagatttgcacacaagtcttccacaaaagcatctctcgccgttgcactaaatctgtgacttcggtcgtctcaaccttgttttacgacaaaaaaatgagaacgacgaatccgaaagagactaagattgtgattgacactaccggcagtaccaaacctaagcaggacgatctcattctcacttgtttcagagggtgggtgaagcagttgcaaatagattacaaaggcaacgaaataatgacggcagctgcctctcaagggctgacccgtaaaggtgtgtatgccgttcggtacaaggtgaatgaaaatcctctgtacgcacccacctcagaacatgtgaacgtcctactgacccgcacggaggaccgcatcgtgtggaaaacactagccggcgacccatggataaaaacactgactgccaagtaccctgggaatttcactgccacgatagaggagtggcaagcagagcatgatgccatcatgaggcacatcttggagagaccggaccctaccgacgtcttccagaataaggcaaacgtgtgttgggccaaggctttagtgccggtgctgaagaccgctggcatagacatgaccactgaacaatggaacactgtggattattttgaaacggacaaagctcactcagcagagatagtattgaaccaactatgcgtgaggttctttggactcgatctggactccggtctattttctgcacccactgttccgttatccattaggaataatcactgggataactccccgtcgcctaacatgtacgggctgaataaagaagtggtccgtcagctctctcgcaggtacccacaactgcctcgggcagttgccactggaagagtctatgacatgaacactggtacactgcgcaattatgatccgcgcataaacctagtacctgtaaacagaagactgcctcatgctttagtcctccaccataatgaacacccacagagtgacttttcttcattcgtcagcaaattgaagggcagaactgtcctggtggtcggggaaaagttgtccgtcccaggcaaaatggttgactggttgtcagaccggcctgaggctaccttcagagctcggctggatttaggcatcccaggtgatgtgcccaaatatgacataatatttgttaatgtgaggaccccatataaataccatcactatcagcagtgtgaagaccatgccattaagcttagcatgttgaccaagaaagcttgtctgcatctgaatcccggcggaacctgtgtcagcataggttatggttacgctgacagggccagcgaaagcatcattggtgctatagcgcggcagttcaagttttcccgggtatgcaaaccgaaatcctcacttgaagagacggaagttctgtttgtattcattgggtacgatcgcaaggcccgtacgcacaatccttacaagctttcatcaaccttgaccaacatttatacaggttccagactccacgaagccggatgtgcaccctcatatcatgtggtgcgaggggatattgccacggccaccgaaggagtgattataaatgctgctaacagcaaaggacaacctggcggaggggtgtgcggagcgctgtataagaaattcccggaaagcttcgatttacagccgatcgaagtaggaaaagcgcgactggtcaaaggtgcagctaaacatatcattcatgccgtaggaccaaacttcaacaaagtttcggaggttgaaggtgacaaacagttggcagaggcttatgagtccatcgctaagattgtcaacgataacaattacaagtcagtagcgattccactgttgtccaccggcatcttttccgggaacaaagatcgactaacccaatcattgaaccatttgctgacagctttagacaccactgatgcagatgtagccatatactgcagggacaagaaatgggaaatgactctcaaggaagcagtggctaggagagaagcagtggaggagatatgcatatccgacgactcttcagtgacagaacctgatgcagagctggtgagggtgcatccgaagagttctttggctggaaggaagggctacagcacaagcgatggcaaaactttctcatatttggaagggaccaagtttcaccaggcggccaaggatatagcagaaattaatgccatgtggcccgttgcaacggaggccaatgagcaggtatgcatgtatatcctcggagaaagcatgagcagtattaggtcgaaatgccccgtcgaagagtcggaagcctccacaccacctagcacgctgccttgcttgtgcatccatgccatgactccagaaagagtacagcgcctaaaagcctcacgtccagaacaaattactgtgtgctcatcctttccattgccgaagtatagaatcactggtgtgcagaagatccaatgctcccagcctatattgttctcaccgaaagtgcctgcgtatattcatccaaggaagtatctcgtggaaacaccaccggtagacgagactccggagccatcggcagagaaccaatccacagaggggacacctgaacaaccaccacttataaccgaggatgagaccaggactagaacgcctgagccgatcatcatcgaagaggaagaagaggatagcataagtttgctgtcagatggcccgacccaccaggtgctgcaagtcgaggcagacattcacgggccgccctctgtatctagctcatcctggtccattcctcatgcatccgactttgatgtggacagtttatccatacttgacaccctggagggagctagcgtgaccagcggggcaacgtcagccgagactaactcttacttcgcaaagagtatggagtttctggcgcgaccggtgcctgcgcctcgaacagtattcaggaaccctccacatcccgctccgcgcacaagaacaccgtcacttgcacccagcagggcctgctcgagaaccagcctagtttccaccccgccaggcgtgaatagggtgatcactagagaggagctcgaggcgcttaccccgtcacgcactcctagcaggtcggtctcgagaaccagcctggtctccaacccgccaggcgtaaatagggtgattacaagagaggagtttgaggcgttcgtagcacaacaacaatgacggtttgatgcgggtgcatacatcttttcctccgacaccggtcaagggcatttacaacaaaaatcagtaaggcaaacggtgctatccgaagtggtgttggagaggaccgaattggagatttcgtatgccccgcgcctcgaccaagaaaaagaagaattactacgcaagaaattacagttaaatcccacacctgctaacagaagcagataccagtccaggaaggtggagaacatgaaagccataacagctagacgtattctgcaaggcctagggcattatttgaaggcagaaggaaaagtggagtgctaccgaaccctgcatcctgttcctttgtattcatctagtgtgaaccgtgccttttcaagccccaaggtcgcagtggaagcctgtaacgccatgttgaaagagaactttccgactgtggcttcttactgtattattccagagtacgatgcctatttggacatggttgacggagcttcatgctgcttagacactgccagtttttgccctgcaaagctgcgcagctttccaaagaaacactcctatttggaacccacaatacgatcggcagtgccttcagcgatccagaacacgctccagaacgtcctggcagctgccacaaaaagaaattgcaatgtcacgcaaatgagagaattgcccgtattggattcggcggcctttaatgtggaatgcttcaagaaatatgcgtgtaataatgaatattgggaaacgtttaaagaaaaccccatcaggcttactgaagaaaacgtggtaaattacattaccaaattaaaaggaccaaaagctgctgctctttttgcgaagacacataatttgaatatgttgcaggacataccaatggacaggtttgtaatggacttaaagagagacgtgaaagtgactccaggaacaaaacatactgaagaacggcccaaggtacaggtgatccaggctgccgatccgctagcaacagcgtatctgtgcggaatccaccgagagctggttaggagattaaatgcggtcctgcttccgaacattcatacactgtttgatatgtcggctgaagactttgacgctattatagccgagcacttccagcctggggattgtgttctggaaactgacatcgcgtcgtttgataaaagtgaggacgacgccatggctctgaccgcgttaatgattctggaagacttaggtgtggacgcagagctgttgacgctgattgaggcggctttcggcgaaatttcatcaatacatttgcccactaaaactaaatttaaattcggagccatgatgaaatctggaatgttcctcacactgtttgtgaacacagtcattaacattgtaatcgcaagcagagtgttgagagaacggctaaccggatcaccatgtgcagcattcattggagatgacaatatcgtgaaaggagtcaaatcggacaaattaatggcagacaggtgcgccacctggttgaatatggaagtcaagattatagatgctgtggtgggcgagaaagcgccttatttctgtggagggtttattttgtgtgactccgtgaccggcacagcgtgccgtgtggcagaccccctaaaaaggctgtttaagcttggcaaacctctggcagcagacgatgaacatgatgatgacaggagaagggcattgcatgaagagtcaacacgctggaaccgagtgggtattctttcagagctgtgcaaggcagtagaatcaaggtatgaaaccgtaggaacttccatcatagttatggccatgactactctagctagcagtgttaaatcattcagctacctgagaggggcccctataactctctacggctaacctgaatggactacgacatagtctagtcgagtctagtcgacgccaccatgggcaccgtgaacaagcctgtcgtgggcgtgctgatgggcttcggcatcatcaccggcaccctgagaatcaccaaccctgtgcgggccagcgtgctgagatacgacgacttccacatcgacgaggacaagctggacaccaacagcgtgtacgagccctactaccacagcgaccacgccgagagcagctgggtcaacagaggcgagagcagccggaaggcctacgaccacaacagcccctacatctggccccggaacgactacgacggcttcctggaaaacgcccacgagcaccacggcgtgtacaatcagggcagaggcatcgacagcggcgagagactgatgcagcccacacagatgagcgcccaggaagatctgggcgacgacacaggcatccacgtgatccccaccctgaacggcgacgaccggcacaagatcgtgaacgtggaccagcggcagtacggcgacgtgttcaagggcgacctgaaccctaagccccagggccagagactgatcgaggtgtccgtggaagagaaccaccccttcaccctgagagcccccatccagagaatctacggcgtgcggtataccgagacttggagcttcctgcccagcctgacctgtacaggcgacgccgctcctgccatccagcacatctgcctgaagcacaccacctgtttccaggacgtggtggtggacgtggactgcgccgagaacaccaaagaggaccagctggccgagatcagctaccggttccagggcaagaaagaggccgaccagccctggatcgtggtcaataccagcaccctgttcgacgagctggaactggacccccccgagattgaacccggcgtgctgaaggtgctgcggaccgagaagcagtacctgggcgtgtacatctggaacatgcggggctccgacggcacctctacctacgccaccttcctggtcacatggaagggcgacgagaaaacccggaaccctacccctgccgtgacccctcagcctagaggcgccgagttccatatgtggaattaccactcccacgtgttcagcgtgggcgacaccttcagcctggccatgcatctgcagtacaagatccacgaggcccccttcgacctgctgctggaatggctgtacgtgcccatcgaccctacctgccagcccatgcggctgtacagcacctgtctgtaccaccccaacgcccctcagtgcctgagccacatgaacagcggctgcaccttcaccagccctcacctggctcagagggtggccagcaccgtgtaccagaattgcgagcacgccgacaactacaccgcctactgcctgggcatcagccacatggaacccagcttcggcctgatcctgcacgatggcggcaccaccctgaagttcgtggacacacccgagagcctgagcggcctgtacgtgttcgtggtgtacttcaacggccacgtggaagccgtggcctacaccgtggtgtccaccgtggaccacttcgtgaacgccatcgaggaaagaggcttcccacccacagccggacagcctccagccaccaccaagcccaaagaaatcacccccgtgaaccccggcaccagccccctgctgagatatgctgcttggacaggcggactggccgctgtggtgctgctgtgcctggtcatcttcctgatctgcaccgccaagcggatgagagtgaaggcctaccgggtggacaagtccccctacaaccagagcatgtactacgccggcctgcccgtggacgatttcgaggatagcgagagcaccgacaccgaggaagagttcggcaacgccatcggcggatctcacggcggcagcagctacaccgtgtacatcgacaagaccagataatctagacgtcgcgaccacccaggatccgcctataactctctacggctaacctgaatggactacgacatagtctagtcgacgccaccatgtttctgatccagtgcctgatcagcgccgtgatcttctatattcaagtcacaaacgccctgatctttaagggcgaccacgtgtcactgcaggtcaacagcagcctgaccagcatcctgatccccatgcagaacgacaattacaccgagatcaagggccagctggtgttcatcggcgagcagctgcccaccggcaccaattacagcggcaccctggaactgctgtacgccgataccgtggccttctgcttcagaagcgtgcaggtcatcagatacgacggctgcccccggatcagaaccagcgccttcatcagctgccggtacaagcacagctggcactacggcaacagcaccgaccggatcagcaccgaacctgatgccggcgtgatgctgaagatcaccaagcccggcatcaacgacgccggcgtgtacgtgctgctcgtgcggctggatcacagcagaagcaccgacggcttcatcctgggcgtgaacgtgtacaccgccggcagccaccacaacatccacggcgtgatctacaccagccccagcctgcagaacggctacagcaccagagccctgttccagcaggccagactgtgcgatctgcccgccacacctaagggcagcggcacaagcctgtttcagcacatgctggacctgagagccggcaagagcctggaagataacccctggctgcacgaggacgtggtcaccaccgagacaaagagcgtggtcaaagagggcatcgagaaccacgtgtaccccaccgacatgagcaccctgcccgagaagtccctgaacgacccccctgagaacctgctgatcatcatccccatcgtggccagcgtgatgatcctgaccgccatggtcatcgtgatcgtgatcagcgtgaagcggcggagaatcaagaagcaccccatctaccggcccaacaccaagaccagacggggcatccagaacgccacccctgagtccgacgtgatgctggaagccgccattgcccagctggccaccatcagagaggaaagcccccctcacagcgtcgtgaaccccttcgtgaagtaatctagacgcggccgcatacagcagcaattggcaagctgcttacatagaactcgcggcgattggcatgccgccttaaaatttttattttatttttcttttcttttccgaatcggattttgtttttaatatttcaaaaaaaaaaaaaaaaaaaaaaaaaaaaaaaaaaagggtcggcatggcatctccacctcctcgcggtccgacctgggcatccgaaggaggacgcacgtccactcggatggctaagggagagccacgtttaaaccagctccaattcgccctatagtgagtcgtattacgcgcgctcactggccgtcgttttacaacgtcgtgactgggaaaaccctggcgttacccaacttaatcgccttgcagcacatccccctttcgccagctggcgtaatagcgaagaggcccgcaccgatcgcccttcccaacagttgcgcagcctgaatggcgaatgggacgcgccctgtagcggcgcattaagcgcggcgggtgtggtggttacgcgcagcgtgaccgctacacttgccagcgccctagcgcccgctcctttcgctttcttcccttcctttctcgccacgttcgccggctttccccgtcaagctctaaatcgggggctccctttagggttccgatttagtgctttacggcacctcgaccccaaaaaacttgattagggtgatggttcacgtagtgggccatcgccctgatagacggtttttcgccctttgacgttggagtccacgttctttaatagtggactcttgttccaaactggaacaacactcaaccctatctcggtctattcttttgatttataagggattttgccgatttcggcctattggttaaaaaatgagctgatttaacaaaaatttaacgcgaattttaacaaaatattaacgcttacaatttaggtggcacttttcggggaaatgtgcgcggaacccctatttgtttatttttctaaatacattcaaatatgtatccgctcatgagacaataaccctgataaatgcttcaataatattgaaaaaggaagagtatgagtattcaacatttccgtgtcgcccttattcccttttttgcggcattttgccttcctgtttttgctcacccagaaacgctggtgaaagtaaaagatgctgaagatcagttgggtgcacgagtgggttacatcgaactggatctcaacagcggtaagatccttgagagttttcgccccgaagaacgttttccaatgatgagcacttttaaagttctgctatgtggcgcggtattatcccgtattgacgccgggcaagagcaactcggtcgccgcatacactattctcagaatgacttggttgagtactcaccagtcacagaaaagcatcttacggatggcatgacagtaagagaattatgcagtgctgccataaccatgagtgataacactgcggccaacttacttctgacaacgatcggaggaccgaaggagctaaccgcttttttgcacaacatgggggatcatgtaactcgccttgatcgttgggaaccggagctgaatgaagccataccaaacgacgagcgtgacaccacgatgcctgtagcaatggcaacaacgttgcgcaaactattaactggcgaactacttactctagcttcccggcaacaattaatagactggatggaggcggataaagttgcaggaccacttctgcgctcggcccttccggctggctggtttattgctgataaatctggagccggtgagcgtgggtctcgcggtatcattgcagcactggggccagatggtaagccctcccgtatcgtagttatctacacgacggggagtcaggcaactatggatgaacgaaatagacagatcgctgagataggtgcctcactgattaagcattggtaactgtcagaccaagtttactcatatatactttagattgatttaaaacttcatttttaatttaaaaggatctaggtgaagatcctttttgataatctcatgaccaaaatcccttaacgtgagttttcgttccactgagcgtcagaccccgtagaaaagatcaaaggatcttcttgagatcctttttttctgcgcgtaatctgctgcttgcaaacaaaaaaaccaccgctaccagcggtggtttgtttgccggatcaagagctaccaactctttttccgaaggtaactggcttcagcagagcgcagataccaaatactgttcttctagtgtagccgtagttaggccaccacttcaagaactctgtagcaccgcctacatacctcgctctgctaatcctgttaccagtggctgctgccagtggcgataagtcgtgtcttaccgggttggactcaagacgatagttaccggataaggcgcagcggtcgggctgaacggggggttcgtgcacacagcccagcttggagcgaacgacctacaccgaactgagatacctacagcgtgagctatgagaaagcgccacgcttcccgaagggagaaaggcggacaggtatccggtaagcggcagggtcggaacaggagagcgcacgagggagcttccagggggaaacgcctggtatctttatagtcctgtcgggtttcgccacctctgacttgagcgtcgatttttgtgatgctcgtcaggggggcggagcctatggaaaaacgccagcaacgcggcctttttacggttcctggccttttgctggccttttgctcacatgttctttcctgcgttatcccctgattctgtggataaccgtattaccgcctttgagtgagctgataccgctcgccgcagccgaacgaccgagcgcagcgagtcagtgagcgaggaagcggaagagcgcccaatacgcaaaccgcctctccccgcgcgttggccgattcattaatgcagctggcacgacaggtttcccgactggaaagcgggcagtgagcgcaacgcaattaatgtgagttagctcactcattaggcaccccaggctttacactttatgctcccggctcgtatgttgtgtggaattgtgagcggataacaatttcacacaggaaacagctatgaccatgattacgccaagcgcgcaattaaccctcactaaagggaacaaaagctgggtaccgggcccacgcgtaatacgactcactatag

SEQ ID NO: 80 - DNA, 11459 bp, Artificial Sequence
  source: /note="Description of Artificial Sequence: Synthetic polynucleotide"
ataggcggcgcatgagagaagcccagaccaattacctacccaaaatggagaaagttcacgttgacatcgaggaagacagcccattcctcagagctttgcagcggagcttcccgcagtttgaggtagaagccaagcaggtcactgataatgaccatgctaatgccagagcgttttcgcatctggcttcaaaactgatcgaaacggaggtggacccatccgacacgatccttgacattggaagtgcgcccgcccgcagaatgtattctaagcacaagtatcattgtatctgtccgatgagatgtgcggaagatccggacagattgtataagtatgcaactaagctgaagaaaaactgtaaggaaataactgataaggaattggacaagaaaatgaaggagctcgccgccgtcatgagcgaccctgacctggaaactgagactatgtgcctccacgacgacgagtcgtgtcgctacgaagggcaagtcgctgtttaccaggatgtatacgcggttgacggaccgacaagtctctatcaccaagccaataagggagttagagtcgcctactggataggctttgacaccaccccttttatgtttaagaacttggctggagcatatccatcatactctaccaactgggccgacgaaaccgtgttaacggctcgtaacataggcctatgcagctctgacgttatggagcggtcacgtagagggatgtccattcttagaaagaagtatttgaaaccatccaacaatgttctattctctgttggctcgaccatctaccacgagaagagggacttactgaggagctggcacctgccgtctgtatttcacttacgtggcaagcaaaattacacatgtcggtgtgagactatagttagttgcgacgggtacgtcgttaaaagaatagctatcagtccaggcctgtatgggaagccttcaggctatgctgctacgatgcaccgcgagggattcttgtgctgcaaagtgacagacacattgaacggggagagggtctcttttcccgtgtgcacgtatgtgccagctacattgtgtgaccaaatgactggcatactggcaacagatgtcagtgcggacgacgcgcaaaaactgctggttgggctcaaccagcgtatagtcgtcaacggtcgcacccagagaaacaccaataccatgaaaaattaccttttgcccgtagtggcccaggcatttgctaggtgggcaaaggaatataaggaagatcaagaagatgaaaggccactaggactacgagatagacagttagtcatggggtgttgttgggcttttagaaggcacaagataacatctatttataagcgcccggatacccaaaccatcatcaaagtgaacagcgatttccactcattcgtgctgcccaggataggcagtaacacattggagatcgggctgagaacaagaatcaggaaaatgttagaggagcacaaggagccgtcacctctcattaccgccgaggacgtacaagaagctaagtgcgcagccgatgaggctaaggaggtgcgtgaagccgaggagttgcgcgcagctctaccacctttggcagctgatgttgaggagcccactctggaagccgatgtagacttgatgttacaagaggctggggccggctcagtggagacacctcgtggcttgataaaggttaccagctacgatggcgaggacaagatcggctcttacgctgtgctttctccgcaggctgtactcaagagtgaaaaattatcttgcatccaccctctcgctgaacaagtcatagtgataacacactctggccgaaaagggcgttatgccgtggaaccataccatggtaaagtagtggtgccagagggacatgcaatacccgtccaggactttcaagctctgagtgaaagtgccaccattgtgtacaacgaacgtgagttcgtaaacaggtacctgcaccatattgccacacatggaggagcgctgaacactgatgaagaatattacaaaactgtcaagcccagcgagcacgacggcgaatacctgtacgacatcgacaggaaacagtgcgtcaagaaagaactagtcactgggctagggctcacaggcgagctggtggatcctcccttccatgaattcgcctacgagagtctgagaacacgaccagccgctccttaccaagtaccaaccataggggtgtatggcgtgccaggatcaggcaagtctggcatcattaaaagcgcagtcaccaaaaaagatctagtggtgagcgccaagaaagaaaactgtgcagaaattataagggacgtcaagaaaatgaaagggctggacgtcaatgccagaactgtggactcagtgctcttgaatggatgcaaacaccccgtagagaccctgtatattgacgaagcttttgcttgtcatgcaggtactctcagagcgctcatagccattataagacctaaaaaggcagtgctctgcggggatcccaaacagtgcggtttttttaacatgatgtgcctgaaagtgcattttaaccacgagatttgcacacaagtcttccacaaaagcatctctcgccgttgcactaaatctgtgacttcggtcgtctcaaccttgttttacgacaaaaaaatgagaacgacgaatccgaaagagactaagattgtgattgacactaccggcagtaccaaacctaagcaggacgatctcattctcacttgtttcagagggtgggtgaagcagttgcaaatagattacaaaggcaacgaaataatgacggcagctgcctctcaagggctgacccgtaaaggtgtgtatgccgttcggtacaaggtgaatgaaaatcctctgtacgcacccacctcagaacatgtgaacgtcctactgacccgcacggaggaccgcatcgtgtggaaaacactagccggcgacccatggataaaaacactgactgccaagtaccctgggaatttcactgccacgatagaggagtggcaagcagagcatgatgccatcatgaggcacatcttggagagaccggaccctaccgacgtcttccagaataaggcaaacgtgtgttgggccaaggctttagtgccggtgctgaagaccgctggcatagacatgaccactgaacaatggaacactgtggattattttgaaacggacaaagctcactcagcagagatagtattgaaccaactatgcgtgaggttctttggactcgatctggactccggtctattttctgcacccactgttccgttatccattaggaataatcactgggataactccccgtcgcctaacatgtacgggctgaataaagaagtggtccgtcagctctctcgcaggtacccacaactgcctcgggcagttgccactggaagagtctatgacatgaacactggtacactgcgcaattatgatccgcgcataaacctagtacctgtaaacagaagactgcctcatgctttagtcctccaccataatgaacacccacagagtgacttttcttcattcgtcagcaaattgaagggcagaactgtcctggtggtcggggaaaagttgtccgtcccaggcaaaatggttgactggttgtcagaccggcctgaggctaccttcagagctcggctggatttaggcatcccaggtgatgtgcccaaatatgacataatatttgttaatgtgaggaccccatataaataccatcactatcagcagtgtgaagaccatgccattaagcttagcatgttgaccaagaaagcttgtctgcatctgaatcccggcggaacctgtgtcagcataggttatggttacgctgacagggccagcgaaagcatcattggtgctatagcgcggcagttcaagttttcccgggtatgcaaaccgaaatcctcacttgaagagacggaagttctgtttgtattcattgggtacgatcgcaaggcccgtacgcacaatccttacaagctttcatcaaccttgaccaacatttatacaggttccagactccacgaagccggatgtgcaccctcatatcatgtggtgcgaggggatattgccacggccaccgaaggagtgattataaatgctgctaacagcaaaggacaacctggcggaggggtgtgcggagcgctgtataagaaattcccggaaagcttcgatttacagccgatcgaagtaggaaaagcgcgactggtcaaaggtgcagctaaacatatcattcatgccgtaggaccaaacttcaacaaagtttcggaggttgaaggtgacaaacagttggcagaggcttatgagtccatcgctaagattgtcaacgataacaattacaagtcagtagcgattccactgttgtccaccggcatcttttccgggaacaaagatcgactaacccaatcattgaaccatttgctgacagctttagacaccactgatgcagatgtagccatatactgcagggacaagaaatgggaaatgactctcaaggaagcagtggctaggagagaagcagtggaggagatatgcatatccgacgactcttcagtgacagaacctgatgcagagctggtgagggtgcatccgaagagttctttggctggaaggaagggctacagcacaagcgatggcaaaactttctcatatttggaagggaccaagtttcaccaggcggccaaggatatagcagaaattaatgccatgtggcccgttgcaacggaggccaatgagcaggtatgcatgtatatcctcggagaaagcatgagcagtattaggtcgaaatgccccgtcgaagagtcggaagcctccacaccacctagcacgctgccttgcttgtgcatccatgccatgactccagaaagagtacagcgcctaaaagcctcacgtccagaacaaattactgtgtgctcatcctttccattgccgaagtatagaatcactggtgtgcagaagatccaatgctcccagcctatattgttctcaccgaaagtgcctgcgtatattcatccaaggaagtatctcgtggaaacaccaccggtagacgagactccggagccatcggcagagaaccaatccacagaggggacacctgaacaaccaccacttataaccgaggatgagaccaggactagaacgcctgagccgatcatcatcgaagaggaagaagaggatagcataagtttgctgtcagatggcccgacccaccaggtgctgcaagtcgaggcagacattcacgggccgccctctgtatctagctcatcctggtccattcctcatgcatccgactttgatgtggacagtttatccatacttgacaccctggagggagctagcgtgaccagcggggcaacgtcagccgagactaactcttacttcgcaaagagtatggagtttctggcgcgaccggtgcctgcgcctcgaacagtattcaggaaccctccacatcccgctccgcgcacaagaacaccgtcacttgcacccagcagggcctgctcgagaaccagcctagtttccaccccgccaggcgtgaatagggtgatcactagagaggagctcgaggcgcttaccccgtcacgcactcctagcaggtcggtctcgagaaccagcctggtctccaacccgccaggcgtaaatagggtgattacaagagaggagtttgaggcgttcgtagcacaacaacaatgacggtttgatgcgggtgcatacatcttttcctccgacaccggtcaagggcatttacaacaaaaatcagtaaggcaaacggtgctatccgaagtggtgttggagaggaccgaattggagatttcgtatgccccgcgcctcgaccaagaaaaagaagaattactacgcaagaaattacagttaaatcccacacctgctaacagaagcagataccagtccaggaaggtggagaacatgaaagccataacagctagacgtattctgcaaggcctagggcattatttgaaggcagaaggaaaagtggagtgctaccgaaccctgcatcctgttcctttgtattcatctagtgtgaaccgtgccttttcaagccccaaggtcgcagtggaagcctgtaacgccatgttgaaagagaactttccgactgtggcttcttactgtattattccagagtacgatgcctatttggacatggttgacggagcttcatgctgcttagacactgccagtttttgccctgcaaagctgcgcagctttccaaagaaacactcctatttggaacccacaatacgatcggcagtgccttcagcgatccagaacacgctccagaacgtcctggcagctgccacaaaaagaaattgcaatgtcacgcaaatgagagaattgcccgtattggattcggcggcctttaatgtggaatgcttcaagaaatatgcgtgtaataatgaatattgggaaacgtttaaagaaaaccccatcaggcttactgaagaaaacgtggtaaattacattaccaaattaaaaggaccaaaagctgctgctctttttgcgaagacacataatttgaatatgttgcaggacataccaatggacaggtttgtaatggacttaaagagagacgtgaaagtgactccaggaacaaaacatactgaagaacggcccaaggtacaggtgatccaggctgccgatccgctagcaacagcgtatctgtgcggaatccaccgagagctggttaggagattaaatgcggtcctgcttccgaacattcatacactgtttgatatgtcggctgaagactttgacgctattatagccgagcacttccagcctggggattgtgttctggaaactgacatcgcgtcgtttgataaaagtgaggacgacgccatggctctgaccgcgttaatgattctggaagacttaggtgtggacgcagagctgttgacgctgattgaggcggctttcggcgaaatttcatcaatacatttgcccactaaaactaaatttaaattcggagccatgatgaaatctggaatgttcctcacactgtttgtgaacacagtcattaacattgtaatcgcaagcagagtgttgagagaacggctaaccggatcaccatgtgcagcattcattggagatgacaatatcgtgaaaggagtcaaatcggacaaattaatggcagacaggtgcgccacctggttgaatatggaagtcaagattatagatgctgtggtgggcgagaaagcgccttatttctgtggagggtttattttgtgtgactccgtgaccggcacagcgtgccgtgtggcagaccccctaaaaaggctgtttaagcttggcaaacctctggcagcagacgatgaacatgatgatgacaggagaagggcattgcatgaagagtcaacacgctggaaccgagtgggtattctttcagagctgtgcaaggcagtagaatcaaggtatgaaaccgtaggaacttccatcatagttatggccatgactactctagctagcagtgttaaatcattcagctacctgagaggggcccctataactctctacggctaacctgaatggactacgacatagtctagtcgacgccaccatggtgagcaagggcgaggagctgttcaccggggtggtgcccatcctggtcgagctggacggcgacgtaaacggccacaagttcagcgtgtccggcgagggcgagggcgatgccacctacggcaagctgaccctgaagttcatctgcaccaccggcaagctgcccgtgccctggcccaccctcgtgaccaccctgacctacggcgtgcagtgcttcagccgctaccccgaccacatgaagcagcacgacttcttcaagtccgccatgcccgaaggctacgtccaggagcgcaccatcttcttcaaggacgacggcaactacaagacccgcgccgaggtgaagttcgagggcgacaccctggtgaaccgcatcgagctgaagggcatcgacttcaaggaggacggcaacatcctggggcacaagctggagtacaactacaacagccacaacgtctatatcatggccgacaagcagaagaacggcatcaaggtgaacttcaagatccgccacaacatcgaggacggcagcgtgcagctcgccgaccactaccagcagaacacccccatcggcgacggccccgtgctgctgcccgacaaccactacctgagcacccagtccgccctgagcaaagaccccaacgagaagcgcgatcacatggtcctgctggagttcgtgaccgccgccgggatcactctcggcatggacgagctgtacaagtgataatctagacggcgcgcccacccagcggccgcatacagcagcaattggcaagctgcttacatagaactcgcggcgattggcatgccgccttaaaatttttattttatttttcttttcttttccgaatcggattttgtttttaatatttcaaaaaaaaaaaaaaaaaaaaaaaaaaaaaaaaaaagggtcggcatggcatctccacctcctcgcggtccgacctgggcatccgaaggaggacgcacgtccactcggatggctaagggagagccacgtttaaaccagctccaattcgccctatagtgagtcgtattacgcgcgctcactggccgtcgttttacaacgtcgtgactgggaaaaccctggcgttacccaacttaatcgccttgcagcacatccccctttcgccagctggcgtaatagcgaagaggcccgcaccgatcgcccttcccaacagttgcgcagcctgaatggcgaatgggacgcgccctgtagcggcgcattaagcgcggcgggtgtggtggttacgcgcagcgtgaccgctacacttgccagcgccctagcgcccgctcctttcgctttcttcccttcctttctcgccacgttcgccggctttccccgtcaagctctaaatcgggggctccctttagggttccgatttagtgctttacggcacctcgaccccaaaaaacttgattagggtgatggttcacgtagtgggccatcgccctgatagacggtttttcgccctttgacgttggagtccacgttctttaatagtggactcttgttccaaactggaacaacactcaaccctatctcggtctattcttttgatttataagggattttgccgatttcggcctattggttaaaaaatgagctgatttaacaaaaatttaacgcgaattttaacaaaatattaacgcttacaatttaggtggcacttttcggggaaatgtgcgcggaacccctatttgtttatttttctaaatacattcaaatatgtatccgctcatgagacaataaccctgataaatgcttcaataatattgaaaaaggaagagtatgagtattcaacatttccgtgtcgcccttattcccttttttgcggcattttgccttcctgtttttgctcacccagaaacgctggtgaaagtaaaagatgctgaagatcagttgggtgcacgagtgggttacatcgaactggatctcaacagcggtaagatccttgagagttttcgccccgaagaacgttttccaatgatgagcacttttaaagttctgctatgtggcgcggtattatcccgtattgacgccgggcaagagcaactcggtcgccgcatacactattctcagaatgacttggttgagtactcaccagtcacagaaaagcatcttacggatggcatgacagtaagagaattatgcagtgctgccataaccatgagtgataacactgcggccaacttacttctgacaacgatcggaggaccgaaggagctaaccgcttttttgcacaacatgggggatcatgtaactcgccttgatcgttgggaaccggagctgaatgaagccataccaaacgacgagcgtgacaccacgatgcctgtagcaatggcaacaacgttgcgcaaactattaactggcgaactacttactctagcttcccggcaacaattaatagactggatggaggcggataaagttgcaggaccacttctgcgctcggcccttccggctggctggtttattgctgataaatctggagccggtgagcgtgggtctcgcggtatcattgcagcactggggccagatggtaagccctcccgtatcgtagttatctacacgacggggagtcaggcaactatggatgaacgaaatagacagatcgctgagataggtgcctcactgattaagcattggtaactgtcagaccaagtttactcatatatactttagattgatttaaaacttcatttttaatttaaaaggatctaggtgaagatcctttttgataatctcatgaccaaaatcccttaacgtgagttttcgttccactgagcgtcagaccccgtagaaaagatcaaaggatcttcttgagatcctttttttctgcgcgtaatctgctgcttgcaaacaaaaaaaccaccgctaccagcggtggtttgtttgccggatcaagagctaccaactctttttccgaaggtaactggcttcagcagagcgcagataccaaatactgttcttctagtgtagccgtagttaggccaccacttcaagaactctgtagcaccgcctacatacctcgctctgctaatcctgttaccagtggctgctgccagtggcgataagtcgtgtcttaccgggttggactcaagacgatagttaccggataaggcgcagcggtcgggctgaacggggggttcgtgcacacagcccagcttggagcgaacgacctacaccgaactgagatacctacagcgtgagctatgagaaagcgccacgcttcccgaagggagaaaggcggacaggtatccggtaagcggcagggtcggaacaggagagcgcacgagggagcttccagggggaaacgcctggtatctttatagtcctgtcgggtttcgccacctctgacttgagcgtcgatttttgtgatgctcgtcaggggggcggagcctatggaaaaacgccagcaacgcggcctttttacggttcctggccttttgctggccttttgctcacatgttctttcctgcgttatcccctgattctgtggataaccgtattaccgcctttgagtgagctgataccgctcgccgcagccgaacgaccgagcgcagcgagtcagtgagcgaggaagcggaagagcgcccaatacgcaaaccgcctctccccgcgcgttggccgattcattaatgcagctggcacgacaggtttcccgactggaaagcgggcagtgagcgcaacgcaattaatgtgagttagctcactcattaggcaccccaggctttacactttatgctcccggctcgtatgttgtgtggaattgtgagcggataacaatttcacacaggaaacagctatgaccatgattacgccaagcgcgcaattaaccctcactaaagggaacaaaagctgggtaccgggcccacgcgtaatacgactcactatag

SEQ ID NO: 81 - DNA, 3567 bp, Artificial Sequence
  source: /note="Description of Artificial Sequence: Synthetic polynucleotide"
ataggcggcgcatgagagaagcccagaccaattacctacccaaataggagaaagttcacgttgacatcgaggaagacagcccattcctcagagctttgcagcggagcttcccgcagtttgaggtagaagccaagcaggtcactgataatgaccatgctaatgccagagcgttttcgcatctggcttcaaaactgatcgaaacggaggtggacccatccgacacgatccttgacattggacggaccgaccatgttcccgttccagccaatgtatccgatgcagccaatgccctatcgcaacccgttcgcggccccgcgcaggccctggttccccagaaccgacccttttctggcgatgcaggtgcaggaattaacccgctcgatggctaacctgacgttcaagcaacgccgggacgcgccacctgaggggccatccgctaagaaaccgaagaaggaggcctcgcaaaaacagaaagggggaggccaagggaagaagaagaagaaccaagggaagaagaaggctaagacagggccgcctaatccgaaggcacagaatggaaacaagaagaagaccaacaagaaaccaggcaagagacagcgcatggtcatgaaattggaatctgacaagacgttcccaatcatgttggaagggaagataaacggctacgcttgtgtggtcggagggaagttattcaggccgatgggtgtggaaggcaagatcgacaacgacgttctggccgcgcttaagacgaagaaagcatccaaatacgatcttgagtatgcagatgtgccacagaacatgcgggccgatacattcaaatacacccatgagaaaccccaaggctattacagctggcatcatggagcagtccaatatgaaaatgggcgtttcacggtgccgaaaggagttggggccaagggagacagcggacgacccattctggataaccagggacgggtggtcgctattgtgctgggaggtgtgaatgaaggatctaggacagccctttcagtcgtcatgtggaacgagaagggagttaccgtgaagtatactccggagaactgcgagcaatggtaatagtaagcggccgcatacagcagcaattggcaagctgcttacatagaactcgcggcgattggcatgccgccttaaaatttttattttatttttcttttcttttccgaatcggattttgtttttaatatttcaaaaaaaaaaaaaaaaaaaaaaaaaaaaaaaaaaagggtcggcatggcatctccacctcctcgcggtccgacctgggcatccgaaggaggacgcacgtccactcggatggctaagggagagccacgtttaaacacgtgatatctggcctcatgggccttcctttcactgcccgctttccagtcgggaaacctgtcgtgccagctgcattaacatggtcatagctgtttccttgcgtattgggcgctctccgcttcctcgctcactgactcgctgcgctcggtcgttcgggtaaagcctggggtgcctaatgagcaaaaggccagcaaaaggccaggaaccgtaaaaaggccgcgttgctggcgtttttccataggctccgcccccctgacgagcatcacaaaaatcgacgctcaagtcagaggtggcgaaacccgacaggactataaagataccaggcgtttccccctggaagctccctcgtgcgctctcctgttccgaccctgccgcttaccggatacctgtccgcctttctcccttcgggaagcgtggcgctttctcatagctcacgctgtaggtatctcagttcggtgtaggtcgttcgctccaagctgggctgtgtgcacgaaccccccgttcagcccgaccgctgcgccttatccggtaactatcgtcttgagtccaacccggtaagacacgacttatcgccactggcagcagccactggtaacaggattagcagagcgaggtatgtaggcggtgctacagagttcttgaagtggtggcctaactacggctacactagaagaacagtatttggtatctgcgctctgctgaagccagttaccttcggaaaaagagttggtagctcttgatccggcaaacaaaccaccgctggtagcggtggtttttttgtttgcaagcagcagattacgcgcagaaaaaaaggatctcaagaagatcctttgatcttttctacggggtctgacgctcagtggaacgaaaactcacgttaagggattttggtcatgagattatcaaaaaggatcttcacctagatccttttaaattaaaaatgaagttttaaatcaatctaaagtatatatgagtaaacttggtctgacagttattagaaaaattcatccagcagacgataaaacgcaatacgctggctatccggtgccgcaatgccatacagcaccagaaaacgatccgcccattcgccgcccagttcttccgcaatatcacgggtggccagcgcaatatcctgataacgatccgccacgcccagacggccgcaatcaataaagccgctaaaacggccattttccaccataatgttcggcaggcacgcatcaccatgggtcaccaccagatcttcgccatccggcatgctcgctttcagacgcgcaaacagctctgccggtgccaggccctgatgttcttcatccagatcatcctgatccaccaggcccgcttccatacgggtacgcgcacgttcaatacgatgtttcgcctgatgatcaaacggacaggtcgccgggtccagggtatgcagacgacgcatggcatccgccataatgctcactttttctgccggcgccagatggctagacagcagatcctgacccggcacttcgcccagcagcagccaatcacggcccgcttcggtcaccacatccagcaccgccgcacacggaacaccggtggtggccagccagctcagacgcgccgcttcatcctgcagctcgttcagcgcaccgctcagatcggttttcacaaacagcaccggacgaccctgcgcgctcagacgaaacaccgccgcatcagagcagccaatggtctgctgcgcccaatcatagccaaacagacgttccacccacgctgccgggctacccgcatgcaggccatcctgttcaatcatactcttcctttttcaatattattgaagcatttatcagggttattgtctcatgagcggatacatatttgaatgtatttagaaaaataaacaaataggggttccgcgcacatttccccgaaaagtgccacctaaattgtaagcgttaatattttgttaaaattcgcgttaaatttttgttaaatcagctcattttttaaccaataggccgaaatcggcaaaatcccttataaatcaaaagaatagaccgagatagggttgagtggccgctacagggcgctcccattcgccattcaggctgcgcaactgttgggaagggcgtttcggtgcgggcctcttcgctattacgccagctggcgaaagggggatgtgctgcaaggcgattaagttgggtaacgccagggttttcccagtcacacgcgtaatacgactcactatag

SEQ ID NO: 82 - DNA, 5685 bp, Artificial Sequence
  source: /note="Description of Artificial Sequence: Synthetic polynucleotide"
ataggcggcgcatgagagaagcccagaccaattacctacccaaataggagaaagttcacgttgacatcgaggaagacagcccattcctcagagctttgcagcggagcttcccgcagtttgaggtagaagccaagcaggtcactgataatgaccatgctaatgccagagcgttttcgcatctggcttcaaaactgatcgaaacggaggtggacccatccgacacgatccttgacattggacggaccgaccatgtcactagtgaccaccatgtgtctgctcgccaatgtgacgttcccatgtgctcaaccaccaatttgctacgacagaaaaccagcagagactttggccatgctcagcgttaacgttgacaacccgggctacgatgagctgctggaagcagctgttaagtgccccggaaggaaaaggagatccaccgaggagctgtttaatgagtataagctaacgcgcccttacatggccagatgcatcagatgtgcagttgggagctgccatagtccaatagcaatcgaggcagtaaagagcgacgggcacgacggttatgttagacttcagacttcctcgcagtatggcctggattcctccggcaacttaaagggcaggaccatgcggtatgacatgcacgggaccattaaagagataccactacatcaagtgtcactctatacatctcgcccgtgtcacattgtggatgggcacggttatttcctgcttgccaggtgcccggcaggggactccatcaccatggaatttaagaaagattccgtcagacactcctgctcggtgccgtatgaagtgaaatttaatcctgtaggcagagaactctatactcatcccccagaacacggagtagagcaagcgtgccaagtctacgcacatgatgcacagaacagaggagcttatgtcgagatgcacctcccgggctcagaagtggacagcagtttggtttccttgagcggcagttcagtcaccgtgacacctcctgatgggactagcgccctggtggaatgcgagtgtggcggcacaaagatctccgagaccatcaacaagacaaaacagttcagccagtgcacaaagaaggagcagtgcagagcatatcggctgcagaacgataagtgggtgtataattctgacaaactgcccaaagcagcgggagccaccttaaaaggaaaactgcatgtcccattcttgctggcagacggcaaatgcaccgtgcctctagcaccagaacctatgataaccttcggtttcagatcagtgtcactgaaactgcaccctaagaatcccacatatctaatcacccgccaacttgctgatgagcctcactacacgcacgagctcatatctgaaccagctgttaggaattttaccgtcaccgaaaaagggtgggagtttgtatggggaaaccacccgccgaaaaggttttgggcacaggaaacagcacccggaaatccacatgggctaccgcacgaggtgataactcattattaccacagataccctatgtccaccatcctgggtttgtcaatttgtgccgccattgcaaccgtttccgttgcagcgtctacctggctgttttgcagatctagagttgcgtgcctaactccttaccggctaacacctaacgctaggataccattttgtctggctgtgctttgctgcgcccgcactgcccgggccgagaccacctgggagtccttggatcacctatggaacaataaccaacagatgttctggattcaattgctgatccctctggccgccttgatcgtagtgactcgcctgctcaggtgcgtgtgctgtgtcgtgccttttttagtcatggccggcgccgcaggcgccggcgcctacgagcacgcgaccacgatgccgagccaagcgggaatctcgtataacactatagtcaacagagcaggctacgcaccactccctatcagcataacaccaacaaagatcaagctgatacctacagtgaacttggagtacgtcacctgccactacaaaacaggaatggattcaccagccatcaaatgctgcggatctcaggaatgcactccaacttacaggcctgatgaacagtgcaaagtcttcacaggggtttacccgttcatgtggggtggtgcatattgcttttgcgacactgagaacacccaagtcagcaaggcctacgtaatgaaatctgacgactgccttgcggatcatgctgaagcatataaagcgcacacagcctcagtgcaggcgttcctcaacatcacagtgggagaacactctattgtgactaccgtgtatgtgaatggagaaactcctgtgaatttcaatggggtcaaaataactgcaggtccgctttccacagcttggacaccctttgatcgcaaaatcgtgcagtatgccggggagatctataattatgattttcctgagtatggggcaggacaaccaggagcatttggagatatacaatccagaacagtctcaagctctgatctgtatgccaataccaacctagtgctgcagagacccaaagcaggagcgatccacgtgccatacactcaggcaccttcgggttttgagcaatggaagaaagataaagctccatcattgaaatttaccgcccctttcggatgcgaaatatatacaaaccccattcgcgccgaaaactgtgctgtagggtcaattccattagcctttgacattcccgacgccttgttcaccagggtgtcagaaacaccgacactttcagcggccgaatgcactcttaacgagtgcgtgtattcttccgactttggtgggatcgccacggtcaagtactcggccagcaagtcaggcaagtgcgcagtccatgtgccatcagggactgctaccctaaaagaagcagcagtcgagctaaccgagcaagggtcggcgactatccatttctcgaccgcaaatatccacccggagttcaggctccaaatatgcacatcatatgttacgtgcaaaggtgattgtcaccccccgaaagaccatattgtgacacaccctcagtatcacgcccaaacatttacagccgcggtgtcaaaaaccgcgtggacgtggttaacatccctgctgggaggatcagccgtaattattataattggcttggtgctggctactattgtggccatgtacgtgctgaccaaccagaaacataattaatagtaagcggccgcatacagcagcaattggcaagctgcttacatagaactcgcggcgattggcatgccgccttaaaatttttattttatttttcttttcttttccgaatcggattttgtttttaatatttcaaaaaaaaaaaaaaaaaaaaaaaaaaaaaaaaaaagggtcggcatggcatctccacctcctcgcggtccgacctgggcatccgaaggaggacgcacgtccactcggatggctaagggagagccacgtttaaacacgtgatatctggcctcatgggccttcctttcactgcccgctttccagtcgggaaacctgtcgtgccagctgcattaacatggtcatagctgtttccttgcgtattgggcgctctccgcttcctcgctcactgactcgctgcgctcggtcgttcgggtaaagcctggggtgcctaatgagcaaaaggccagcaaaaggccaggaaccgtaaaaaggccgcgttgctggcgtttttccataggctccgcccccctgacgagcatcacaaaaatcgacgctcaagtcagaggtggcgaaacccgacaggactataaagataccaggcgtttccccctggaagctccctcgtgcgctctcctgttccgaccctgccgcttaccggatacctgtccgcctttctcccttcgggaagcgtggcgctttctcatagctcacgctgtaggtatctcagttcggtgtaggtcgttcgctccaagctgggctgtgtgcacgaaccccccgttcagcccgaccgctgcgccttatccggtaactatcgtcttgagtccaacccggtaagacacgacttatcgccactggcagcagccactggtaacaggattagcagagcgaggtatgtaggcggtgctacagagttcttgaagtggtggcctaactacggctacactagaagaacagtatttggtatctgcgctctgctgaagccagttaccttcggaaaaagagttggtagctcttgatccggcaaacaaaccaccgctggtagcggtggtttttttgtttgcaagcagcagattacgcgcagaaaaaaaggatctcaagaagatcctttgatcttttctacggggtctgacgctcagtggaacgaaaactcacgttaagggattttggtcatgagattatcaaaaaggatcttcacctagatccttttaaattaaaaatgaagttttaaatcaatctaaagtatatatgagtaaacttggtctgacagttattagaaaaattcatccagcagacgataaaacgcaatacgctggctatccggtgccgcaatgccatacagcaccagaaaacgatccgcccattcgccgcccagttcttccgcaatatcacgggtggccagcgcaatatcctgataacgatccgccacgcccagacggccgcaatcaataaagccgctaaaacggccattttccaccataatgttcggcaggcacgcatcaccatgggtcaccaccagatcttcgccatccggcatgctcgctttcagacgcgcaaacagctctgccggtgccaggccctgatgttcttcatccagatcatcctgatccaccaggcccgcttccatacgggtacgcgcacgttcaatacgatgtttcgcctgatgatcaaacggacaggtcgccgggtccagggtatgcagacgacgcatggcatccgccataatgctcactttttctgccggcgccagatggctagacagcagatcctgacccggcacttcgcccagcagcagccaatcacggcccgcttcggtcaccacatccagcaccgccgcacacggaacaccggtggtggccagccagctcagacgcgccgcttcatcctgcagctcgttcagcgcaccgctcagatcggttttcacaaacagcaccggacgaccctgcgcgctcagacgaaacaccgccgcatcagagcagccaatggtctgctgcgcccaatcatagccaaacagacgttccacccacgctgccgggctacccgcatgcaggccatcctgttcaatcatactcttcctttttcaatattattgaagcatttatcagggttattgtctcatgagcggatacatatttgaatgtatttagaaaaataaacaaataggggttccgcgcacatttccccgaaaagtgccacctaaattgtaagcgttaatattttgttaaaattcgcgttaaatttttgttaaatcagctcattttttaaccaataggccgaaatcggcaaaatcccttataaatcaaaagaatagaccgagatagggttgagtggccgctacagggcgctcccattcgccattcaggctgcgcaactgttgggaagggcgtttcggtgcgggcctcttcgctattacgccagctggcgaaagggggatgtgctgcaaggcgattaagttgggtaacgccagggttttcccagtcacacgcgtaatacgactcactatag

SEQ ID NO: 83 - DNA, 13364 bp, Artificial Sequence
  source: /note="Description of Artificial Sequence: Synthetic polynucleotide"
ataggcggcgcatgagagaagcccagaccaattacctacccaaaatggagaaagttcacgttgacatcgaggaagacagcccattcctcagagctttgcagcggagcttcccgcagtttgaggtagaagccaagcaggtcactgataatgaccatgctaatgccagagcgttttcgcatctggcttcaaaactgatcgaaacggaggtggacccatccgacacgatccttgacattggaagtgcgcccgcccgcagaatgtattctaagcacaagtatcattgtatctgtccgatgagatgtgcggaagatccggacagattgtataagtatgcaactaagctgaagaaaaactgtaaggaaataactgataaggaattggacaagaaaatgaaggagctcgccgccgtcatgagcgaccctgacctggaaactgagactatgtgcctccacgacgacgagtcgtgtcgctacgaagggcaagtcgctgtttaccaggatgtatacgcggttgacggaccgacaagtctctatcaccaagccaataagggagttagagtcgcctactggataggctttgacaccaccccttttatgtttaagaacttggctggagcatatccatcatactctaccaactgggccgacgaaaccgtgttaacggctcgtaacataggcctatgcagctctgacgttatggagcggtcacgtagagggatgtccattcttagaaagaagtatttgaaaccatccaacaatgttctattctctgttggctcgaccatctaccacgagaagagggacttactgaggagctggcacctgccgtctgtatttcacttacgtggcaagcaaaattacacatgtcggtgtgagactatagttagttgcgacgggtacgtcgttaaaagaatagctatcagtccaggcctgtatgggaagccttcaggctatgctgctacgatgcaccgcgagggattcttgtgctgcaaagtgacagacacattgaacggggagagggtctcttttcccgtgtgcacgtatgtgccagctacattgtgtgaccaaatgactggcatactggcaacagatgtcagtgcggacgacgcgcaaaaactgctggttgggctcaaccagcgtatagtcgtcaacggtcgcacccagagaaacaccaataccatgaaaaattaccttttgcccgtagtggcccaggcatttgctaggtgggcaaaggaatataaggaagatcaagaagatgaaaggccactaggactacgagatagacagttagtcatggggtgttgttgggcttttagaaggcacaagataacatctatttataagcgcccggatacccaaaccatcatcaaagtgaacagcgatttccactcattcgtgctgcccaggataggcagtaacacattggagatcgggctgagaacaagaatcaggaaaatgttagaggagcacaaggagccgtcacctctcattaccgccgaggacgtacaagaagctaagtgcgcagccgatgaggctaaggaggtgcgtgaagccgaggagttgcgcgcagctctaccacctttggcagctgatgttgaggagcccactctggaagccgatgtagacttgatgttacaagaggctggggccggctcagtggagacacctcgtggcttgataaaggttaccagctacgatggcgaggacaagatcggctcttacgctgtgctttctccgcaggctgtactcaagagtgaaaaattatcttgcatccaccctctcgctgaacaagtcatagtgataacacactctggccgaaaagggcgttatgccgtggaaccataccatggtaaagtagtggtgccagagggacatgcaatacccgtccaggactttcaagctctgagtgaaagtgccaccattgtgtacaacgaacgtgagttcgtaaacaggtacctgcaccatattgccacacatggaggagcgctgaacactgatgaagaatattacaaaactgtcaagcccagcgagcacgacggcgaatacctgtacgacatcgacaggaaacagtgcgtcaagaaagaactagtcactgggctagggctcacaggcgagctggtggatcctcccttccatgaattcgcctacgagagtctgagaacacgaccagccgctccttaccaagtaccaaccataggggtgtatggcgtgccaggatcaggcaagtctggcatcattaaaagcgcagtcaccaaaaaagatctagtggtgagcgccaagaaagaaaactgtgcagaaattataagggacgtcaagaaaatgaaagggctggacgtcaatgccagaactgtggactcagtgctcttgaatggatgcaaacaccccgtagagaccctgtatattgacgaagcttttgcttgtcatgcaggtactctcagagcgctcatagccattataagacctaaaaaggcagtgctctgcggggatcccaaacagtgcggtttttttaacatgatgtgcctgaaagtgcattttaaccacgagatttgcacacaagtcttccacaaaagcatctctcgccgttgcactaaatctgtgacttcggtcgtctcaaccttgttttacgacaaaaaaatgagaacgacgaatccgaaagagactaagattgtgattgacactaccggcagtaccaaacctaagcaggacgatctcattctcacttgtttcagagggtgggtgaagcagttgcaaatagattacaaaggcaacgaaataatgacggcagctgcctctcaagggctgacccgtaaaggtgtgtatgccgttcggtacaaggtgaatgaaaatcctctgtacgcacccacctcagaacatgtgaacgtcctactgacccgcacggaggaccgcatcgtgtggaaaacactagccggcgacccatggataaaaacactgactgccaagtaccctgggaatttcactgccacgatagaggagtggcaagcagagcatgatgccatcatgaggcacatcttggagagaccggaccctaccgacgtcttccagaataaggcaaacgtgtgttgggccaaggctttagtgccggtgctgaagaccgctggcatagacatgaccactgaacaatggaacactgtggattattttgaaacggacaaagctcactcagcagagatagtattgaaccaactatgcgtgaggttctttggactcgatctggactccggtctattttctgcacccactgttccgttatccattaggaataatcactgggataactccccgtcgcctaacatgtacgggctgaataaagaagtggtccgtcagctctctcgcaggtacccacaactgcctcgggcagttgccactggaagagtctatgacatgaacactggtacactgcgcaattatgatccgcgcataaacctagtacctgtaaacagaagactgcctcatgctttagtcctccaccataatgaacacccacagagtgacttttcttcattcgtcagcaaattgaagggcagaactgtcctggtggtcggggaaaagttgtccgtcccaggcaaaatggttgactggttgtcagaccggcctgaggctaccttcagagctcggctggatttaggcatcccaggtgatgtgcccaaatatgacataatatttgttaatgtgaggaccccatataaataccatcactatcagcagtgtgaagaccatgccattaagcttagcatgttgaccaagaaagcttgtctgcatctgaatcccggcggaacctgtgtcagcataggttatggttacgctgacagggccagcgaaagcatcattggtgctatagcgcggcagttcaagttttcccgggtatgcaaaccgaaatcctcacttgaagagacggaagttctgtttgtattcattgggtacgatcgcaaggcccgtacgcacaatccttacaagctttcatcaaccttgaccaacatttatacaggttccagactccacgaagccggatgtgcaccctcatatcatgtggtgcgaggggatattgccacggccaccgaaggagtgattataaatgctgctaacagcaaaggacaacctggcggaggggtgtgcggagcgctgtataagaaattcccggaaagcttcgatttacagccgatcgaagtaggaaaagcgcgactggtcaaaggtgcagctaaacatatcattcatgccgtaggaccaaacttcaacaaagtttcggaggttgaaggtgacaaacagttggcagaggcttatgagtccatcgctaagattgtcaacgataacaattacaagtcagtagcgattccactgttgtccaccggcatcttttccgggaacaaagatcgactaacccaatcattgaaccatttgctgacagctttagacaccactgatgcagatgtagccatatactgcagggacaagaaatgggaaatgactctcaaggaagcagtggctaggagagaagcagtggaggagatatgcatatccgacgactcttcagtgacagaacctgatgcagagctggtgagggtgcatccgaagagttctttggctggaaggaagggctacagcacaagcgatggcaaaactttctcatatttggaagggaccaagtttcaccaggcggccaaggatatagcagaaattaatgccatgtggcccgttgcaacggaggccaatgagcaggtatgcatgtatatcctcggagaaagcatgagcagtattaggtcgaaatgccccgtcgaagagtcggaagcctccacaccacctagcacgctgccttgcttgtgcatccatgccatgactccagaaagagtacagcgcctaaaagcctcacgtccagaacaaattactgtgtgctcatcctttccattgccgaagtatagaatcactggtgtgcagaagatccaatgctcccagcctatattgttctcaccgaaagtgcctgcgtatattcatccaaggaagtatctcgtggaaacaccaccggtagacgagactccggagccatcggcagagaaccaatccacagaggggacacctgaacaaccaccacttataaccgaggatgagaccaggactagaacgcctgagccgatcatcatcgaagaggaagaagaggatagcataagtttgctgtcagatggcccgacccaccaggtgctgcaagtcgaggcagacattcacgggccgccctctgtatctagctcatcctggtccattcctcatgcatccgactttgatgtggacagtttatccatacttgacaccctggagggagctagcgtgaccagcggggcaacgtcagccgagactaactcttacttcgcaaagagtatggagtttctggcgcgaccggtgcctgcgcctcgaacagtattcaggaaccctccacatcccgctccgcgcacaagaacaccgtcacttgcacccagcagggcctgctcgagaaccagcctagtttccaccccgccaggcgtgaatagggtgatcactagagaggagctcgaggcgcttaccccgtcacgcactcctagcaggtcggtctcgagaaccagcctggtctccaacccgccaggcgtaaatagggtgattacaagagaggagtttgaggcgttcgtagcacaacaacaatgacggtttgatgcgggtgcatacatcttttcctccgacaccggtcaagggcatttacaacaaaaatcagtaaggcaaacggtgctatccgaagtggtgttggagaggaccgaattggagatttcgtatgccccgcgcctcgaccaagaaaaagaagaattactacgcaagaaattacagttaaatcccacacctgctaacagaagcagataccagtccaggaaggtggagaacatgaaagccataacagctagacgtattctgcaaggcctagggcattatttgaaggcagaaggaaaagtggagtgctaccgaaccctgcatcctgttcctttgtattcatctagtgtgaaccgtgccttttcaagccccaaggtcgcagtggaagcctgtaacgccatgttgaaagagaactttccgactgtggcttcttactgtattattccagagtacgatgcctatttggacatggttgacggagcttcatgctgcttagacactgccagtttttgccctgcaaagctgcgcagctttccaaagaaacactcctatttggaacccacaatacgatcggcagtgccttcagcgatccagaacacgctccagaacgtcctggcagctgccacaaaaagaaattgcaatgtcacgcaaatgagagaattgcccgtattggattcggcggcctttaatgtggaatgcttcaagaaatatgcgtgtaataatgaatattgggaaacgtttaaagaaaaccccatcaggcttactgaagaaaacgtggtaaattacattaccaaattaaaaggaccaaaagctgctgctctttttgcgaagacacataatttgaatatgttgcaggacataccaatggacaggtttgtaatggacttaaagagagacgtgaaagtgactccaggaacaaaacatactgaagaacggcccaaggtacaggtgatccaggctgccgatccgctagcaacagcgtatctgtgcggaatccaccgagagctggttaggagattaaatgcggtcctgcttccgaacattcatacactgtttgatatgtcggctgaagactttgacgctattatagccgagcacttccagcctggggattgtgttctggaaactgacatcgcgtcgtttgataaaagtgaggacgacgccatggctctgaccgcgttaatgattctggaagacttaggtgtggacgcagagctgttgacgctgattgaggcggctttcggcgaaatttcatcaatacatttgcccactaaaactaaatttaaattcggagccatgatgaaatctggaatgttcctcacactgtttgtgaacacagtcattaacattgtaatcgcaagcagagtgttgagagaacggctaaccggatcaccatgtgcagcattcattggagatgacaatatcgtgaaaggagtcaaatcggacaaattaatggcagacaggtgcgccacctggttgaatatggaagtcaagattatagatgctgtggtgggcgagaaagcgccttatttctgtggagggtttattttgtgtgactccgtgaccggcacagcgtgccgtgtggcagaccccctaaaaaggctgtttaagcttggcaaacctctggcagcagacgatgaacatgatgatgacaggagaagggcattgcatgaagagtcaacacgctggaaccgagtgggtattctttcagagctgtgcaaggcagtagaatcaaggtatgaaaccgtaggaacttccatcatagttatggccatgactactctagctagcagtgttaaatcattcagctacctgagaggggcccctataactctctacggctaacctgaatggactacgacatagtctagtcgacgccaccatgaggcctggcctgccctcctacctgatcatcctggccgtgtgcctgttcagccacctgctgtccagcagatacggcgccgaggccgtgagcgagcccctggacaaggctttccacctgctgctgaacacctacggcagacccatccggtttctgcgggagaacaccacccagtgcacctacaacagcagcctgcggaacagcaccgtcgtgagagagaacgccatcagcttcaactttttccagagctacaaccagtactacgtgttccacatgcccagatgcctgtttgccggccctctggccgagcagttcctgaaccaggtggacctgaccgagacactggaaagataccagcagcggctgaatacctacgccctggtgtccaaggacctggccagctaccggtcctttagccagcagctcaaggctcaggatagcctcggcgagcagcctaccaccgtgccccctcccatcgacctgagcatcccccacgtgtggatgcctccccagaccacccctcacggctggaccgagagccacaccacctccggcctgcacagaccccacttcaaccagacctgcatcctgttcgacggccacgacctgctgtttagcaccgtgaccccctgcctgcaccagggcttctacctgatcgacgagctgagatacgtgaagatcaccctgaccgaggatttcttcgtggtcaccgtgtccatcgacgacgacacccccatgctgctgatcttcggccacctgcccagagtgctgttcaaggccccctaccagcgggacaacttcatcctgcggcagaccgagaagcacgagctgctggtgctggtcaagaaggaccagctgaaccggcactcctacctgaaggaccccgacttcctggacgccgccctggacttcaactacctggacctgagcgccctgctgagaaacagcttccacagatacgccgtggacgtgctgaagtccggacggtgccagatgctcgatcggcggaccgtggagatggccttcgcctatgccctcgccctgttcgccgctgccagacaggaagaggctggcgcccaggtgtcagtgcccagagccctggatagacaggccgccctgctgcagatccaggaattcatgatcacctgcctgagccagaccccccctagaaccaccctgctgctgtaccccacagccgtggatctggccaagagggccctgtggacccccaaccagatcaccgacatcacaagcctcgtgcggctcgtgtacatcctgagcaagcagaaccagcagcacctgatcccccagtgggccctgagacagatcgccgacttcgccctgaagctgcacaagacccatctggccagctttctgagcgccttcgccaggcaggaactgtacctgatgggcagcctggtccacagcatgctggtgcataccaccgagcggcgggagatcttcatcgtggagacaggcctgtgtagcctggccgagctgtcccactttacccagctgctggcccaccctcaccacgagtacctgagcgacctgtacaccccctgcagcagcagcggcagacgggaccacagcctggaacggctgaccagactgttccccgatgccaccgtgcctgctacagtgcctgccgccctgtccatcctgtccaccatgcagcccagcaccctggaaaccttccccgacctgttctgcctgcccctgggcgagagctttagcgccctgaccgtgtccgagcacgtgtcctacatcgtgaccaatcagtacctgatcaagggcatcagctaccccgtgtccaccacagtcgtgggccagagcctgatcatcacccagaccgacagccagaccaagtgcgagctgacccggaacatgcacaccacacacagcatcaccgtggccctgaacatcagcctggaaaactgcgctttctgtcagtctgccctgctggaatacgacgatacccagggcgtgatcaacatcatgtacatgcacgacagcgacgacgtgctgttcgccctggacccctacaacgaggtggtggtgtccagcccccggacccactacctgatgctgctgaagaacggcaccgtgctggaagtgaccgacgtggtggtggacgccaccgacagcagactgctgatgatgagcgtgtacgccctgagcgccatcatcggcatctacctgctgtaccggatgctgaaaacctgctgataatctagacggcgcgcccacccagcggccgcctataactctctacggctaacctgaatggactacgacatagtctagtcgacgccaccatgtgcagaaggcccgactgcggcttcagcttcagccctggacccgtgatcctgctgtggtgctgcctgctgctgcctatcgtgtcctctgccgccgtgtctgtggcccctacagccgccgagaaggtgccagccgagtgccccgagctgaccagaagatgcctgctgggcgaggtgttcgagggcgacaagtacgagagctggctgcggcccctggtcaacgtgaccggcagagatggccccctgagccagctgatccggtacagacccgtgacccccgaggccgccaatagcgtgctgctggacgaggccttcctggataccctggccctgctgtacaacaaccccgaccagctgagagccctgctgaccctgctgtccagcgacaccgcccccagatggatgaccgtgatgcggggctacagcgagtgtggagatggcagccctgccgtgtacacctgcgtggacgacctgtgcagaggctacgacctgaccagactgagctacggccggtccatcttcacagagcacgtgctgggcttcgagctggtgccccccagcctgttcaacgtggtggtggccatccggaacgaggccaccagaaccaacagagccgtgcggctgcctgtgtctacagccgctgcacctgagggcatcacactgttctacggcctgtacaacgccgtgaaagagttctgcctccggcaccagctggatccccccctgctgagacacctggacaagtactacgccggcctgcccccagagctgaagcagaccagagtgaacctgcccgcccacagcagatatggccctcaggccgtggacgccagatgataatctagacggcgcgcccacccacctgcaggatacagcagcaattggcaagctgcttacatagaactcgcggcgattggcatgccgccttaaaatttttattttatttttcttttcttttccgaatcggattttgtttttaatatttcaaaaaaaaaaaaaaaaaaaaaaaaaaaaaaaaaaagggtcggcatggcatctccacctcctcgcggtccgacctgggcatccgaaggaggacgcacgtccactcggatggctaagggagagccacgtttaaacgctagagcaagacgtttcccgttgaatatggctcataacaccccttgtattactgtttatgtaagcagacagttttattgttcatgatgatatatttttatcttgtgcaatgtaacatcagagattttgagacacaacgtggctttgttgaataaatcgaacttttgctgagttgaaggatcagatcacgcatcttcccgacaacgcagaccgttccgtggcaaagcaaaagttcaaaatcaccaactggtccacctacaacaaagctctcatcaaccgtggctccctcactttctggctggatgatggggcgattcaggcctggtatgagtcagcaacaccttcttcacgaggcagacctcagcgctagcggagtgtatactggcttactatgttggcactgatgagggtgtcagtgaagtgcttcatgtggcaggagaaaaaaggctgcaccggtgcgtcagcagaatatgtgatacaggatatattccgcttcctcgctcactgactcgctacgctcggtcgttcgactgcggcgagcggaaatggcttacgaacggggcggagatttcctggaagatgccaggaagatacttaacagggaagtgagagggccgcggcaaagccgtttttccataggctccgcccccctgacaagcatcacgaaatctgacgctcaaatcagtggtggcgaaacccgacaggactataaagataccaggcgtttcccctggcggctccctcgtgcgctctcctgttcctgcctttcggtttaccggtgtcattccgctgttatggccgcgtttgtctcattccacgcctgacactcagttccgggtaggcagttcgctccaagctggactgtatgcacgaaccccccgttcagtccgaccgctgcgccttatccggtaactatcgtcttgagtccaacccggaaagacatgcaaaagcaccactggcagcagccactggtaattgatttagaggagttagtcttgaagtcatgcgccggttaaggctaaactgaaaggacaagttttggtgactgcgctcctccaagccagttacctcggttcaaagagttggtagctcagagaaccttcgaaaaaccgccctgcaaggcggttttttcgttttcagagcaagagattacgcgcagaccaaaacgatctcaagaagatcatcttattaaggggtctgacgctcagtggaacgaaaactcacgttaagggattttggtcatgagattatcaaaaaggatcttcacctagatccttttaaattaaaaatgaagttttaaatcaatctaaagtatatatgagtaaacttggtctgacagttaccaatgcttaatcagtgaggcacctatctcagcgatctgtctatttcgttcatccatagttgcctgactccccgtcgtgtagataactacgatacgggagggcttaccatctggccccagtgctgcaatgataccgcgagacccacgctcaccggctccagatttatcagcaataaaccagccagccggaagggccgagcgcagaagtggtcctgcaactttatccgcctccatccagtctattaattgttgccgggaagctagagtaagtagttcgccagttaatagtttgcgcaacgttgttgccattgctgcaggcatcgtggtgtcacgctcgtcgtttggtatggcttcattcagctccggttcccaacgatcaaggcgagttacatgatcccccatgttgtgcaaaaaagcggttagctccttcggtcctccgatcgttgtcagaagtaagttggccgcagtgttatcactcatggttatggcagcactgcataattctcttactgtcatgccatccgtaagatgcttttctgtgactggtgagtactcaaccaagtcattctgagaatagtgtatgcggcgaccgagttgctcttgcccggcgtcaacacgggataataccgcgccacatagcagaactttaaaagtgctcatcattggaaaacgttcttcggggcgaaaactctcaaggatcttaccgctgttgagatccagttcgatgtaacccactcgtgcacccaactgatcttcagcatcttttactttcaccagcgtttctgggtgagcaaaaacaggaaggcaaaatgccgcaaaaaagggaataagggcgacacggaaatgttgaatactcatactcttcctttttcaatattattgaagcatttatcagggttattgtctcatgagcggatacatatttgaatgtatttagaaaaataaacaaataggggttccgcgcacatttccccgaaaagtgccacctgacgtgtcgagacgcgtaatacgactcactatag

SEQ ID NO: 84 - DNA, 13283 bp, Artificial Sequence
  source: /note="Description of Artificial Sequence: Synthetic polynucleotide"
ataggcggcgcatgagagaagcccagaccaattacctacccaaaatggagaaagttcacgttgacatcgaggaagacagcccattcctcagagctttgcagcggagcttcccgcagtttgaggtagaagccaagcaggtcactgataatgaccatgctaatgccagagcgttttcgcatctggcttcaaaactgatcgaaacggaggtggacccatccgacacgatccttgacattggaagtgcgcccgcccgcagaatgtattctaagcacaagtatcattgtatctgtccgatgagatgtgcggaagatccggacagattgtataagtatgcaactaagctgaagaaaaactgtaaggaaataactgataaggaattggacaagaaaatgaaggagctcgccgccgtcatgagcgaccctgacctggaaactgagactatgtgcctccacgacgacgagtcgtgtcgctacgaagggcaagtcgctgtttaccaggatgtatacgcggttgacggaccgacaagtctctatcaccaagccaataagggagttagagtcgcctactggataggctttgacaccaccccttttatgtttaagaacttggctggagcatatccatcatactctaccaactgggccgacgaaaccgtgttaacggctcgtaacataggcctatgcagctctgacgttatggagcggtcacgtagagggatgtccattcttagaaagaagtatttgaaaccatccaacaatgttctattctctgttggctcgaccatctaccacgagaagagggacttactgaggagctggcacctgccgtctgtatttcacttacgtggcaagcaaaattacacatgtcggtgtgagactatagttagttgcgacgggtacgtcgttaaaagaatagctatcagtccaggcctgtatgggaagccttcaggctatgctgctacgatgcaccgcgagggattcttgtgctgcaaagtgacagacacattgaacggggagagggtctcttttcccgtgtgcacgtatgtgccagctacattgtgtgaccaaatgactggcatactggcaacagatgtcagtgcggacgacgcgcaaaaactgctggttgggctcaaccagcgtatagtcgtcaacggtcgcacccagagaaacaccaataccatgaaaaattaccttttgcccgtagtggcccaggcatttgctaggtgggcaaaggaatataaggaagatcaagaagatgaaaggccactaggactacgagatagacagttagtcatggggtgttgttgggcttttagaaggcacaagataacatctatttataagcgcccggatacccaaaccatcatcaaagtgaacagcgatttccactcattcgtgctgcccaggataggcagtaacacattggagatcgggctgagaacaagaatcaggaaaatgttagaggagcacaaggagccgtcacctctcattaccgccgaggacgtacaagaagctaagtgcgcagccgatgaggctaaggaggtgcgtgaagccgaggagttgcgcgcagctctaccacctttggcagctgatgttgaggagcccactctggaagccgatgtagacttgatgttacaagaggctggggccggctcagtggagacacctcgtggcttgataaaggttaccagctacgatggcgaggacaagatcggctcttacgctgtgctttctccgcaggctgtactcaagagtgaaaaattatcttgcatccaccctctcgctgaacaagtcatagtgataacacactctggccgaaaagggcgttatgccgtggaaccataccatggtaaagtagtggtgccagagggacatgcaatacccgtccaggactttcaagctctgagtgaaagtgccaccattgtgtacaacgaacgtgagttcgtaaacaggtacctgcaccatattgccacacatggaggagcgctgaacactgatgaagaatattacaaaactgtcaagcccagcgagcacgacggcgaatacctgtacgacatcgacaggaaacagtgcgtcaagaaagaactagtcactgggctagggctcacaggcgagctggtggatcctcccttccatgaattcgcctacgagagtctgagaacacgaccagccgctccttaccaagtaccaaccataggggtgtatggcgtgccaggatcaggcaagtctggcatcattaaaagcgcagtcaccaaaaaagatctagtggtgagcgccaagaaagaaaactgtgcagaaattataagggacgtcaagaaaatgaaagggctggacgtcaatgccagaactgtggactcagtgctcttgaatggatgcaaacaccccgtagagaccctgtatattgacgaagcttttgcttgtcatgcaggtactctcagagcgctcatagccattataagacctaaaaaggcagtgctctgcggggatcccaaacagtgcggtttttttaacatgatgtgcctgaaagtgcattttaaccacgagatttgcacacaagtcttccacaaaagcatctctcgccgttgcactaaatctgtgacttcggtcgtctcaaccttgttttacgacaaaaaaatgagaacgacgaatccgaaagagactaagattgtgattgacactaccggcagtaccaaacctaagcaggacgatctcattctcacttgtttcagagggtgggtgaagcagttgcaaatagattacaaaggcaacgaaataatgacggcagctgcctctcaagggctgacccgtaaaggtgtgtatgccgttcggtacaaggtgaatgaaaatcctctgtacgcacccacctcagaacatgtgaacgtcctactgacccgcacggaggaccgcatcgtgtggaaaacactagccggcgacccatggataaaaacactgactgccaagtaccctgggaatttcactgccacgatagaggagtggcaagcagagcatgatgccatcatgaggcacatcttggagagaccggaccctaccgacgtcttccagaataaggcaaacgtgtgttgggccaaggctttagtgccggtgctgaagaccgctggcatagacatgaccactgaacaatggaacactgtggattattttgaaacggacaaagctcactcagcagagatagtattgaaccaactatgcgtgaggttctttggactcgatctggactccggtctattttctgcacccactgttccgttatccattaggaataatcactgggataactccccgtcgcctaacatgtacgggctgaataaagaagtggtccgtcagctctctcgcaggtacccacaactgcctcgggcagttgccactggaagagtctatgacatgaacactggtacactgcgcaattatgatccgcgcataaacctagtacctgtaaacagaagactgcctcatgctttagtcctccaccataatgaacacccacagagtgacttttcttcattcgtcagcaaattgaagggcagaactgtcctggtggtcggggaaaagttgtccgtcccaggcaaaatggttgactggttgtcagaccggcctgaggctaccttcagagctcggctggatttaggcatcccaggtgatgtgcccaaatatgacataatatttgttaatgtgaggaccccatataaataccatcactatcagcagtgtgaagaccatgccattaagcttagcatgttgaccaagaaagcttgtctgcatctgaatcccggcggaacctgtgtcagcataggttatggttacgctgacagggccagcgaaagcatcattggtgctatagcgcggcagttcaagttttcccgggtatgcaaaccgaaatcctcacttgaagagacggaagttctgtttgtattcattgggtacgatcgcaaggcccgtacgcacaatccttacaagctttcatcaaccttgaccaacatttatacaggttccagactccacgaagccggatgtgcaccctcatatcatgtggtgcgaggggatattgccacggccaccgaaggagtgattataaatgctgctaacagcaaaggacaacctggcggaggggtgtgcggagcgctgtataagaaattcccggaaagcttcgatttacagccgatcgaagtaggaaaagcgcgactggtcaaaggtgcagctaaacatatcattcatgccgtaggaccaaacttcaacaaagtttcggaggttgaaggtgacaaacagttggcagaggcttatgagtccatcgctaagattgtcaacgataacaattacaagtcagtagcgattccactgttgtccaccggcatcttttccgggaacaaagatcgactaacccaatcattgaaccatttgctgacagctttagacaccactgatgcagatgtagccatatactgcagggacaagaaatgggaaatgactctcaaggaagcagtggctaggagagaagcagtggaggagatatgcatatccgacgactcttcagtgacagaacctgatgcagagctggtgagggtgcatccgaagagttctttggctggaaggaagggctacagcacaagcgatggcaaaactttctcatatttggaagggaccaagtttcaccaggcggccaaggatatagcagaaattaatgccatgtggcccgttgcaacggaggccaatgagcaggtatgcatgtatatcctcggagaaagcatgagcagtattaggtcgaaatgccccgtcgaagagtcggaagcctccacaccacctagcacgctgccttgcttgtgcatccatgccatgactccagaaagagtacagcgcctaaaagcctcacgtccagaacaaattactgtgtgctcatcctttccattgccgaagtatagaatcactggtgtgcagaagatccaatgctcccagcctatattgttctcaccgaaagtgcctgcgtatattcatccaaggaagtatctcgtggaaacaccaccggtagacgagactccggagccatcggcagagaaccaatccacagaggggacacctgaacaaccaccacttataaccgaggatgagaccaggactagaacgcctgagccgatcatcatcgaagaggaagaagaggatagcataagtttgctgtcagatggcccgacccaccaggtgctgcaagtcgaggcagacattcacgggccgccctctgtatctagctcatcctggtccattcctcatgcatccgactttgatgtggacagtttatccatacttgacaccctggagggagctagcgtgaccagcggggcaacgtcagccgagactaactcttacttcgcaaagagtatggagtttctggcgcgaccggtgcctgcgcctcgaacagtattcaggaaccctccacatcccgctccgcgcacaagaacaccgtcacttgcacccagcagggcctgctcgagaaccagcctagtttccaccccgccaggcgtgaatagggtgatcactagagaggagctcgaggcgcttaccccgtcacgcactcctagcaggtcggtctcgagaaccagcctggtctccaacccgccaggcgtaaatagggtgattacaagagaggagtttgaggcgttcgtagcacaacaacaatgacggtttgatgcgggtgcatacatcttttcctccgacaccggtcaagggcatttacaacaaaaatcagtaaggcaaacggtgctatccgaagtggtgttggagaggaccgaattggagatttcgtatgccccgcgcctcgaccaagaaaaagaagaattactacgcaagaaattacagttaaatcccacacctgctaacagaagcagataccagtccaggaaggtggagaacatgaaagccataacagctagacgtattctgcaaggcctagggcattatttgaaggcagaaggaaaagtggagtgctaccgaaccctgcatcctgttcctttgtattcatctagtgtgaaccgtgccttttcaagccccaaggtcgcagtggaagcctgtaacgccatgttgaaagagaactttccgactgtggcttcttactgtattattccagagtacgatgcctatttggacatggttgacggagcttcatgctgcttagacactgccagtttttgccctgcaaagctgcgcagctttccaaagaaacactcctatttggaacccacaatacgatcggcagtgccttcagcgatccagaacacgctccagaacgtcctggcagctgccacaaaaagaaattgcaatgtcacgcaaatgagagaattgcccgtattggattcggcggcctttaatgtggaatgcttcaagaaatatgcgtgtaataatgaatattgggaaacgtttaaagaaaaccccatcaggcttactgaagaaaacgtggtaaattacattaccaaattaaaaggaccaaaagctgctgctctttttgcgaagacacataatttgaatatgttgcaggacataccaatggacaggtttgtaatggacttaaagagagacgtgaaagtgactccaggaacaaaacatactgaagaacggcccaaggtacaggtgatccaggctgccgatccgctagcaacagcgtatctgtgcggaatccaccgagagctggttaggagattaaatgcggtcctgcttccgaacattcatacactgtttgatatgtcggctgaagactttgacgctattatagccgagcacttccagcctggggattgtgttctggaaactgacatcgcgtcgtttgataaaagtgaggacgacgccatggctctgaccgcgttaatgattctggaagacttaggtgtggacgcagagctgttgacgctgattgaggcggctttcggcgaaatttcatcaatacatttgcccactaaaactaaatttaaattcggagccatgatgaaatctggaatgttcctcacactgtttgtgaacacagtcattaacattgtaatcgcaagcagagtgttgagagaacggctaaccggatcaccatgtgcagcattcattggagatgacaatatcgtgaaaggagtcaaatcggacaaattaatggcagacaggtgcgccacctggttgaatatggaagtcaagattatagatgctgtggtgggcgagaaagcgccttatttctgtggagggtttattttgtgtgactccgtgaccggcacagcgtgccgtgtggcagaccccctaaaaaggctgtttaagcttggcaaacctctggcagcagacgatgaacatgatgatgacaggagaagggcattgcatgaagagtcaacacgctggaaccgagtgggtattctttcagagctgtgcaaggcagtagaatcaaggtatgaaaccgtaggaacttccatcatagttatggccatgactactctagctagcagtgttaaatcattcagctacctgagaggggcccctataactctctacggctaacctgaatggactacgacatagtctagtcgacgccaccatgaggcctggcctgccctcctacctgatcatcctggccgtgtgcctgttcagccacctgctgtccagcagatacggcgccgaggccgtgagcgagcccctggacaaggctttccacctgctgctgaacacctacggcagacccatccggtttctgcgggagaacaccacccagtgcacctacaacagcagcctgcggaacagcaccgtcgtgagagagaacgccatcagcttcaactttttccagagctacaaccagtactacgtgttccacatgcccagatgcctgtttgccggccctctggccgagcagttcctgaaccaggtggacctgaccgagacactggaaagataccagcagcggctgaatacctacgccctggtgtccaaggacctggccagctaccggtcctttagccagcagctcaaggctcaggatagcctcggcgagcagcctaccaccgtgccccctcccatcgacctgagcatcccccacgtgtggatgcctccccagaccacccctcacggctggaccgagagccacaccacctccggcctgcacagaccccacttcaaccagacctgcatcctgttcgacggccacgacctgctgtttagcaccgtgaccccctgcctgcaccagggcttctacctgatcgacgagctgagatacgtgaagatcaccctgaccgaggatttcttcgtggtcaccgtgtccatcgacgacgacacccccatgctgctgatcttcggccacctgcccagagtgctgttcaaggccccctaccagcgggacaacttcatcctgcggcagaccgagaagcacgagctgctggtgctggtcaagaaggaccagctgaaccggcactcctacctgaaggaccccgacttcctggacgccgccctggacttcaactacctggacctgagcgccctgctgagaaacagcttccacagatacgccgtggacgtgctgaagtccggacggtgccagatgctcgatcggcggaccgtggagatggccttcgcctatgccctcgccctgttcgccgctgccagacaggaagaggctggcgcccaggtgtcagtgcccagagccctggatagacaggccgccctgctgcagatccaggaattcatgatcacctgcctgagccagaccccccctagaaccaccctgctgctgtaccccacagccgtggatctggccaagagggccctgtggacccccaaccagatcaccgacatcacaagcctcgtgcggctcgtgtacatcctgagcaagcagaaccagcagcacctgatcccccagtgggccctgagacagatcgccgacttcgccctgaagctgcacaagacccatctggccagctttctgagcgccttcgccaggcaggaactgtacctgatgggcagcctggtccacagcatgctggtgcataccaccgagcggcgggagatcttcatcgtggagacaggcctgtgtagcctggccgagctgtcccactttacccagctgctggcccaccctcaccacgagtacctgagcgacctgtacaccccctgcagcagcagcggcagacgggaccacagcctggaacggctgaccagactgttccccgatgccaccgtgcctgctacagtgcctgccgccctgtccatcctgtccaccatgcagcccagcaccctggaaaccttccccgacctgttctgcctgcccctgggcgagagctttagcgccctgaccgtgtccgagcacgtgtcctacatcgtgaccaatcagtacctgatcaagggcatcagctaccccgtgtccaccacagtcgtgggccagagcctgatcatcacccagaccgacagccagaccaagtgcgagctgacccggaacatgcacaccacacacagcatcaccgtggccctgaacatcagcctggaaaactgcgctttctgtcagtctgccctgctggaatacgacgatacccagggcgtgatcaacatcatgtacatgcacgacagcgacgacgtgctgttcgccctggacccctacaacgaggtggtggtgtccagcccccggacccactacctgatgctgctgaagaacggcaccgtgctggaagtgaccgacgtggtggtggacgccaccgactgataatctagacggcgcgcccacccagcggccgcctataactctctacggctaacctgaatggactacgacatagtctagtcgacgccaccatgtgcagaaggcccgactgcggcttcagcttcagccctggacccgtgatcctgctgtggtgctgcctgctgctgcctatcgtgtcctctgccgccgtgtctgtggcccctacagccgccgagaaggtgccagccgagtgccccgagctgaccagaagatgcctgctgggcgaggtgttcgagggcgacaagtacgagagctggctgcggcccctggtcaacgtgaccggcagagatggccccctgagccagctgatccggtacagacccgtgacccccgaggccgccaatagcgtgctgctggacgaggccttcctggataccctggccctgctgtacaacaaccccgaccagctgagagccctgctgaccctgctgtccagcgacaccgcccccagatggatgaccgtgatgcggggctacagcgagtgtggagatggcagccctgccgtgtacacctgcgtggacgacctgtgcagaggctacgacctgaccagactgagctacggccggtccatcttcacagagcacgtgctgggcttcgagctggtgccccccagcctgttcaacgtggtggtggccatccggaacgaggccaccagaaccaacagagccgtgcggctgcctgtgtctacagccgctgcacctgagggcatcacactgttctacggcctgtacaacgccgtgaaagagttctgcctccggcaccagctggatccccccctgctgagacacctggacaagtactacgccggcctgcccccagagctgaagcagaccagagtgaacctgcccgcccacagcagatatggccctcaggccgtggacgccagatgataatctagacggcgcgcccacccacctgcaggatacagcagcaattggcaagctgcttacatagaactcgcggcgattggcatgccgccttaaaatttttattttatttttcttttcttttccgaatcggattttgtttttaatatttcaaaaaaaaaaaaaaaaaaaaaaaaaaaaaaaaaaagggtcggcatggcatctccacctcctcgcggtccgacctgggcatccgaaggaggacgcacgtccactcggatggctaagggagagccacgtttaaacgctagagcaagacgtttcccgttgaatatggctcataacaccccttgtattactgtttatgtaagcagacagttttattgttcatgatgatatatttttatcttgtgcaatgtaacatcagagattttgagacacaacgtggctttgttgaataaatcgaacttttgctgagttgaaggatcagatcacgcatcttcccgacaacgcagaccgttccgtggcaaagcaaaagttcaaaatcaccaactggtccacctacaacaaagctctcatcaaccgtggctccctcactttctggctggatgatggggcgattcaggcctggtatgagtcagcaacaccttcttcacgaggcagacctcagcgctagcggagtgtatactggcttactatgttggcactgatgagggtgtcagtgaagtgcttcatgtggcaggagaaaaaaggctgcaccggtgcgtcagcagaatatgtgatacaggatatattccgcttcctcgctcactgactcgctacgctcggtcgttcgactgcggcgagcggaaatggcttacgaacggggcggagatttcctggaagatgccaggaagatacttaacagggaagtgagagggccgcggcaaagccgtttttccataggctccgcccccctgacaagcatcacgaaatctgacgctcaaatcagtggtggcgaaacccgacaggactataaagataccaggcgtttcccctggcggctccctcgtgcgctctcctgttcctgcctttcggtttaccggtgtcattccgctgttatggccgcgtttgtctcattccacgcctgacactcagttccgggtaggcagttcgctccaagctggactgtatgcacgaaccccccgttcagtccgaccgctgcgccttatccggtaactatcgtcttgagtccaacccggaaagacatgcaaaagcaccactggcagcagccactggtaattgatttagaggagttagtcttgaagtcatgcgccggttaaggctaaactgaaaggacaagttttggtgactgcgctcctccaagccagttacctcggttcaaagagttggtagctcagagaaccttcgaaaaaccgccctgcaaggcggttttttcgttttcagagcaagagattacgcgcagaccaaaacgatctcaagaagatcatcttattaaggggtctgacgctcagtggaacgaaaactcacgttaagggattttggtcatgagattatcaaaaaggatcttcacctagatccttttaaattaaaaatgaagttttaaatcaatctaaagtatatatgagtaaacttggtctgacagttaccaatgcttaatcagtgaggcacctatctcagcgatctgtctatttcgttcatccatagttgcctgactccccgtcgtgtagataactacgatacgggagggcttaccatctggccccagtgctgcaatgataccgcgagacccacgctcaccggctccagatttatcagcaataaaccagccagccggaagggccgagcgcagaagtggtcctgcaactttatccgcctccatccagtctattaattgttgccgggaagctagagtaagtagttcgccagttaatagtttgcgcaacgttgttgccattgctgcaggcatcgtggtgtcacgctcgtcgtttggtatggcttcattcagctccggttcccaacgatcaaggcgagttacatgatcccccatgttgtgcaaaaaagcggttagctccttcggtcctccgatcgttgtcagaagtaagttggccgcagtgttatcactcatggttatggcagcactgcataattctcttactgtcatgccatccgtaagatgcttttctgtgactggtgagtactcaaccaagtcattctgagaatagtgtatgcggcgaccgagttgctcttgcccggcgtcaacacgggataataccgcgccacatagcagaactttaaaagtgctcatcattggaaaacgttcttcggggcgaaaactctcaaggatcttaccgctgttgagatccagttcgatgtaacccactcgtgcacccaactgatcttcagcatcttttactttcaccagcgtttctgggtgagcaaaaacaggaaggcaaaatgccgcaaaaaagggaataagggcgacacggaaatgttgaatactcatactcttcctttttcaatattattgaagcatttatcagggttattgtctcatgagcggatacatatttgaatgtatttagaaaaataaacaaataggggttccgcgcacatttccccgaaaagtgccacctgacgtgtcgagacgcgtaatacgactcactatag

SEQ ID NO: 85 - DNA, 13463 bp, Artificial Sequence
  source: /note="Description of Artificial Sequence: Synthetic polynucleotide"
ataggcggcgcatgagagaagcccagaccaattacctacccaaaatggagaaagttcacgttgacatcgaggaagacagcccattcctcagagctttgcagcggagcttcccgcagtttgaggtagaagccaagcaggtcactgataatgaccatgctaatgccagagcgttttcgcatctggcttcaaaactgatcgaaacggaggtggacccatccgacacgatccttgacattggaagtgcgcccgcccgcagaatgtattctaagcacaagtatcattgtatctgtccgatgagatgtgcggaagatccggacagattgtataagtatgcaactaagctgaagaaaaactgtaaggaaataactgataaggaattggacaagaaaatgaaggagctcgccgccgtcatgagcgaccctgacctggaaactgagactatgtgcctccacgacgacgagtcgtgtcgctacgaagggcaagtcgctgtttaccaggatgtatacgcggttgacggaccgacaagtctctatcaccaagccaataagggagttagagtcgcctactggataggctttgacaccaccccttttatgtttaagaacttggctggagcatatccatcatactctaccaactgggccgacgaaaccgtgttaacggctcgtaacataggcctatgcagctctgacgttatggagcggtcacgtagagggatgtccattcttagaaagaagtatttgaaaccatccaacaatgttctattctctgttggctcgaccatctaccacgagaagagggacttactgaggagctggcacctgccgtctgtatttcacttacgtggcaagcaaaattacacatgtcggtgtgagactatagttagttgcgacgggtacgtcgttaaaagaatagctatcagtccaggcctgtatgggaagccttcaggctatgctgctacgatgcaccgcgagggattcttgtgctgcaaagtgacagacacattgaacggggagagggtctcttttcccgtgtgcacgtatgtgccagctacattgtgtgaccaaatgactggcatactggcaacagatgtcagtgcggacgacgcgcaaaaactgctggttgggctcaaccagcgtatagtcgtcaacggtcgcacccagagaaacaccaataccatgaaaaattaccttttgcccgtagtggcccaggcatttgctaggtgggcaaaggaatataaggaagatcaagaagatgaaaggccactaggactacgagatagacagttagtcatggggtgttgttgggcttttagaaggcacaagataacatctatttataagcgcccggatacccaaaccatcatcaaagtgaacagcgatttccactcattcgtgctgcccaggataggcagtaacacattggagatcgggctgagaacaagaatcaggaaaatgttagaggagcacaaggagccgtcacctctcattaccgccgaggacgtacaagaagctaagtgcgcagccgatgaggctaaggaggtgcgtgaagccgaggagttgcgcgcagctctaccacctttggcagctgatgttgaggagcccactctggaagccgatgtagacttgatgttacaagaggctggggccggctcagtggagacacctcgtggcttgataaaggttaccagctacgatggcgaggacaagatcggctcttacgctgtgctttctccgcaggctgtactcaagagtgaaaaattatcttgcatccaccctctcgctgaacaagtcatagtgataacacactctggccgaaaagggcgttatgccgtggaaccataccatggtaaagtagtggtgccagagggacatgcaatacccgtccaggactttcaagctctgagtgaaagtgccaccattgtgtacaacgaacgtgagttcgtaaacaggtacctgcaccatattgccacacatggaggagcgctgaacactgatgaagaatattacaaaactgtcaagcccagcgagcacgacggcgaatacctgtacgacatcgacaggaaacagtgcgtcaagaaagaactagtcactgggctagggctcacaggcgagctggtggatcctcccttccatgaattcgcctacgagagtctgagaacacgaccagccgctccttaccaagtaccaaccataggggtgtatggcgtgccaggatcaggcaagtctggcatcattaaaagcgcagtcaccaaaaaagatctagtggtgagcgccaagaaagaaaactgtgcagaaattataagggacgtcaagaaaatgaaagggctggacgtcaatgccagaactgtggactcagtgctcttgaatggatgcaaacaccccgtagagaccctgtatattgacgaagcttttgcttgtcatgcaggtactctcagagcgctcatagccattataagacctaaaaaggcagtgctctgcggggatcccaaacagtgcggtttttttaacatgatgtgcctgaaagtgcattttaaccacgagatttgcacacaagtcttccacaaaagcatctctcgccgttgcactaaatctgtgacttcggtcgtctcaaccttgttttacgacaaaaaaatgagaacgacgaatccgaaagagactaagattgtgattgacactaccggcagtaccaaacctaagcaggacgatctcattctcacttgtttcagagggtgggtgaagcagttgcaaatagattacaaaggcaacgaaataatgacggcagctgcctctcaagggctgacccgtaaaggtgtgtatgccgttcggtacaaggtgaatgaaaatcctctgtacgcacccacctcagaacatgtgaacgtcctactgacccgcacggaggaccgcatcgtgtggaaaacactagccggcgacccatggataaaaacactgactgccaagtaccctgggaatttcactgccacgatagaggagtggcaagcagagcatgatgccatcatgaggcacatcttggagagaccggaccctaccgacgtcttccagaataaggcaaacgtgtgttgggccaaggctttagtgccggtgctgaagaccgctggcatagacatgaccactgaacaatggaacactgtggattattttgaaacggacaaagctcactcagcagagatagtattgaaccaactatgcgtgaggttctttggactcgatctggactccggtctattttctgcacccactgttccgttatccattaggaataatcactgggataactccccgtcgcctaacatgtacgggctgaataaagaagtggtccgtcagctctctcgcaggtacccacaactgcctcgggcagttgccactggaagagtctatgacatgaacactggtacactgcgcaattatgatccgcgcataaacctagtacctgtaaacagaagactgcctcatgctttagtcctccaccataatgaacacccacagagtgacttttcttcattcgtcagcaaattgaagggcagaactgtcctggtggtcggggaaaagttgtccgtcccaggcaaaatggttgactggttgtcagaccggcctgaggctaccttcagagctcggctggatttaggcatcccaggtgatgtgcccaaatatgacataatatttgttaatgtgaggaccccatataaataccatcactatcagcagtgtgaagaccatgccattaagcttagcatgttgaccaagaaagcttgtctgcatctgaatcccggcggaacctgtgtcagcataggttatggttacgctgacagggccagcgaaagcatcattggtgctatagcgcggcagttcaagttttcccgggtatgcaaaccgaaatcctcacttgaagagacggaagttctgtttgtattcattgggtacgatcgcaaggcccgtacgcacaatccttacaagctttcatcaaccttgaccaacatttatacaggttccagactccacgaagccggatgtgcaccctcatatcatgtggtgcgaggggatattgccacggccaccgaaggagtgattataaatgctgctaacagcaaaggacaacctggcggaggggtgtgcggagcgctgtataagaaattcccggaaagcttcgatttacagccgatcgaagtaggaaaagcgcgactggtcaaaggtgcagctaaacatatcattcatgccgtaggaccaaacttcaacaaagtttcggaggttgaaggtgacaaacagttggcagaggcttatgagtccatcgctaagattgtcaacgataacaattacaagtcagtagcgattccactgttgtccaccggcatcttttccgggaacaaagatcgactaacccaatcattgaaccatttgctgacagctttagacaccactgatgcagatgtagccatatactgcagggacaagaaatgggaaatgactctcaaggaagcagtggctaggagagaagcagtggaggagatatgcatatccgacgactcttcagtgacagaacctgatgcagagctggtgagggtgcatccgaagagttctttggctggaaggaagggctacagcacaagcgatggcaaaactttctcatatttggaagggaccaagtttcaccaggcggccaaggatatagcagaaattaatgccatgtggcccgttgcaacggaggccaatgagcaggtatgcatgtatatcctcggagaaagcatgagcagtattaggtcgaaatgccccgtcgaagagtcggaagcctccacaccacctagcacgctgccttgcttgtgcatccatgccatgactccagaaagagtacagcgcctaaaagcctcacgtccagaacaaattactgtgtgctcatcctttccattgccgaagtatagaatcactggtgtgcagaagatccaatgctcccagcctatattgttctcaccgaaagtgcctgcgtatattcatccaaggaagtatctcgtggaaacaccaccggtagacgagactccggagccatcggcagagaaccaatccacagaggggacacctgaacaaccaccacttataaccgaggatgagaccaggactagaacgcctgagccgatcatcatcgaagaggaagaagaggatagcataagtttgctgtcagatggcccgacccaccaggtgctgcaagtcgaggcagacattcacgggccgccctctgtatctagctcatcctggtccattcctcatgcatccgactttgatgtggacagtttatccatacttgacaccctggagggagctagcgtgaccagcggggcaacgtcagccgagactaactcttacttcgcaaagagtatggagtttctggcgcgaccggtgcctgcgcctcgaacagtattcaggaaccctccacatcccgctccgcgcacaagaacaccgtcacttgcacccagcagggcctgctcgagaaccagcctagtttccaccccgccaggcgtgaatagggtgatcactagagaggagctcgaggcgcttaccccgtcacgcactcctagcaggtcggtctcgagaaccagcctggtctccaacccgccaggcgtaaatagggtgattacaagagaggagtttgaggcgttcgtagcacaacaacaatgacggtttgatgcgggtgcatacatcttttcctccgacaccggtcaagggcatttacaacaaaaatcagtaaggcaaacggtgctatccgaagtggtgttggagaggaccgaattggagatttcgtatgccccgcgcctcgaccaagaaaaagaagaattactacgcaagaaattacagttaaatcccacacctgctaacagaagcagataccagtccaggaaggtggagaacatgaaagccataacagctagacgtattctgcaaggcctagggcattatttgaaggcagaaggaaaagtggagtgctaccgaaccctgcatcctgttcctttgtattcatctagtgtgaaccgtgccttttcaagccccaaggtcgcagtggaagcctgtaacgccatgttgaaagagaactttccgactgtggcttcttactgtattattccagagtacgatgcctatttggacatggttgacggagcttcatgctgcttagacactgccagtttttgccctgcaaagctgcgcagctttccaaagaaacactcctatttggaacccacaatacgatcggcagtgccttcagcgatccagaacacgctccagaacgtcctggcagctgccacaaaaagaaattgcaatgtcacgcaaatgagagaattgcccgtattggattcggcggcctttaatgtggaatgcttcaagaaatatgcgtgtaataatgaatattgggaaacgtttaaagaaaaccccatcaggcttactgaagaaaacgtggtaaattacattaccaaattaaaaggaccaaaagctgctgctctttttgcgaagacacataatttgaatatgttgcaggacataccaatggacaggtttgtaatggacttaaagagagacgtgaaagtgactccaggaacaaaacatactgaagaacggcccaaggtacaggtgatccaggctgccgatccgctagcaacagcgtatctgtgcggaatccaccgagagctggttaggagattaaatgcggtcctgcttccgaacattcatacactgtttgatatgtcggctgaagactttgacgctattatagccgagcacttccagcctggggattgtgttctggaaactgacatcgcgtcgtttgataaaagtgaggacgacgccatggctctgaccgcgttaatgattctggaagacttaggtgtggacgcagagctgttgacgctgattgaggcggctttcggcgaaatttcatcaatacatttgcccactaaaactaaatttaaattcggagccatgatgaaatctggaatgttcctcacactgtttgtgaacacagtcattaacattgtaatcgcaagcagagtgttgagagaacggctaaccggatcaccatgtgcagcattcattggagatgacaatatcgtgaaaggagtcaaatcggacaaattaatggcagacaggtgcgccacctggttgaatatggaagtcaagattatagatgctgtggtgggcgagaaagcgccttatttctgtggagggtttattttgtgtgactccgtgaccggcacagcgtgccgtgtggcagaccccctaaaaaggctgtttaagcttggcaaacctctggcagcagacgatgaacatgatgatgacaggagaagggcattgcatgaagagtcaacacgctggaaccgagtgggtattctttcagagctgtgcaaggcagtagaatcaaggtatgaaaccgtaggaacttccatcatagttatggccatgactactctagctagcagtgttaaatcattcagctacctgagaggggcccctataactctctacggctaacctgaatggactacgacatagtctagtcgacgccaccatggaaagccggatctggtgcctggtcgtgtgcgtgaacctgtgcatcgtgtgcctgggagccgccgtgagcagcagcagcaccagaggcaccagcgccacacacagccaccacagcagccacaccacctctgccgcccacagcagatccggcagcgtgtcccagagagtgaccagcagccagaccgtgtcccacggcgtgaacgagacaatctacaacaccaccctgaagtacggcgacgtcgtgggcgtgaataccaccaagtacccctacagagtgtgcagcatggcccagggcaccgacctgatcagattcgagcggaacatcgtgtgcaccagcatgaagcccatcaacgaggacctggacgagggcatcatggtggtgtacaagagaaacatcgtggcccacaccttcaaagtgcgggtgtaccagaaggtgctgaccttccggcggagctacgcctacatccacaccacatacctgctgggcagcaacaccgagtacgtggcccctcccatgtgggagatccaccacatcaacagccacagccagtgctacagcagctacagccgcgtgatcgccggcacagtgttcgtggcctaccaccgggacagctacgagaacaagaccatgcagctgatgcccgacgactacagcaacacccacagcaccagatacgtgaccgtgaaggaccagtggcacagcagaggcagcacctggctgtaccgggagacatgcaacctgaactgcatggtcaccatcaccaccgccagaagcaagtacccttaccacttcttcgccacctccaccggcgacgtggtggacatcagccccttctacaacggcaccaaccggaacgccagctacttcggcgagaacgccgacaagttcttcatcttccccaactacaccatcgtgtccgacttcggcagacccaacagcgctctggaaacccacagactggtggcctttctggaacgggccgacagcgtgatcagctgggacatccaggacgagaagaacgtgacctgccagctgaccttctgggaggcctctgagagaaccatcagaagcgaggccgaggacagctaccacttcagcagcgccaagatgaccgccaccttcctgagcaagaaacaggaagtgaacatgagcgactccgccctggactgcgtgagggacgaggccatcaacaagctgcagcagatcttcaacaccagctacaaccagacctacgagaagtatggcaatgtgtccgtgttcgagacaacaggcggcctggtggtgttctggcagggcatcaagcagaaaagcctggtggagctggaacggctcgccaaccggtccagcctgaacctgacccacaaccggaccaagcggagcaccgacggcaacaacgcaacccacctgtccaacatggaaagcgtgcacaacctggtgtacgcacagctgcagttcacctacgacaccctgcggggctacatcaacagagccctggcccagatcgccgaggcttggtgcgtggaccagcggcggaccctggaagtgttcaaagagctgtccaagatcaaccccagcgccatcctgagcgccatctacaacaagcctatcgccgccagattcatgggcgacgtgctgggcctggccagctgcgtgaccatcaaccagaccagcgtgaaggtgctgcgggacatgaacgtgaaagagagcccaggccgctgctactccagacccgtggtcatcttcaacttcgccaacagctcctacgtgcagtacggccagctgggcgaggacaacgagatcctgctggggaaccaccggaccgaggaatgccagctgcccagcctgaagatctttatcgccggcaacagcgcctacgagtatgtggactacctgttcaagcggatgatcgacctgagcagcatctccaccgtggacagcatgatcgccctggacatcgaccccctggaaaacaccgacttccgggtgctggaactgtacagccagaaagagctgcggagcagcaacgtgttcgacctggaagagatcatgcgggagttcaacagctacaagcagcgcgtgaaatacgtggaggacaaggtggtggaccccctgcctccttacctgaagggcctggacgacctgatgagcggactgggcgctgccggaaaagccgtgggagtggccattggagctgtgggcggagctgtggcctctgtcgtggaaggcgtcgccacctttctgaagaaccccttcggcgccttcaccatcatcctggtggccattgccgtcgtgatcatcacctacctgatctacacccggcagcggagactgtgtacccagcccctgcagaacctgttcccctacctggtgtccgccgatggcaccacagtgaccagcggctccaccaaggataccagcctgcaggccccacccagctacgaagagagcgtgtacaacagcggcagaaagggccctggccctcccagctctgatgccagcacagccgcccctccctacaccaacgagcaggcctaccagatgctgctggccctggctagactggatgccgagcagagggcccagcagaacggcaccgacagcctggatggcagaaccggcacccaggacaagggccagaagcccaacctgctggaccggctgcggcaccggaagaacggctaccggcacctgaaggacagcgacgaggaagagaacgtctgataatctagacggcgcgcccacccagcggccgcatacagcagcaattggcaagctgcttacatagaactcgcggcgattggcatgccgccttaaaatttttattttatttttcttttcttttccgaatcggattttgtttttaatatttcaaaaaaaaaaaaaaaaaaaaaaaaaaaaaaaaaaagggtcggcatggcatctccacctcctcgcggtccgacctgggcatccgaaggaggacgcacgtccactcggatggctaagggagagccacgtttaaaccagctccaattcgccctatagtgagtcgtattacgcgcgctcactggccgtcgttttacaacgtcgtgactgggaaaaccctggcgttacccaacttaatcgccttgcagcacatccccctttcgccagctggcgtaatagcgaagaggcccgcaccgatcgcccttcccaacagttgcgcagcctgaatggcgaatgggacgcgccctgtagcggcgcattaagcgcggcgggtgtggtggttacgcgcagcgtgaccgctacacttgccagcgccctagcgcccgctcctttcgctttcttcccttcctttctcgccacgttcgccggctttccccgtcaagctctaaatcgggggctccctttagggttccgatttagtgctttacggcacctcgaccccaaaaaacttgattagggtgatggttcacgtagtgggccatcgccctgatagacggtttttcgccctttgacgttggagtccacgttctttaatagtggactcttgttccaaactggaacaacactcaaccctatctcggtctattcttttgatttataagggattttgccgatttcggcctattggttaaaaaatgagctgatttaacaaaaatttaacgcgaattttaacaaaatattaacgcttacaatttaggtggcacttttcggggaaatgtgcgcggaacccctatttgtttatttttctaaatacattcaaatatgtatccgctcatgagacaataaccctgataaatgcttcaataatattgaaaaaggaagagtatgagtattcaacatttccgtgtcgcccttattcccttttttgcggcattttgccttcctgtttttgctcacccagaaacgctggtgaaagtaaaagatgctgaagatcagttgggtgcacgagtgggttacatcgaactggatctcaacagcggtaagatccttgagagttttcgccccgaagaacgttttccaatgatgagcacttttaaagttctgctatgtggcgcggtattatcccgtattgacgccgggcaagagcaactcggtcgccgcatacactattctcagaatgacttggttgagtactcaccagtcacagaaaagcatcttacggatggcatgacagtaagagaattatgcagtgctgccataaccatgagtgataacactgcggccaacttacttctgacaacgatcggaggaccgaaggagctaaccgcttttttgcacaacatgggggatcatgtaactcgccttgatcgttgggaaccggagctgaatgaagccataccaaacgacgagcgtgacaccacgatgcctgtagcaatggcaacaacgttgcgcaaactattaactggcgaactacttactctagcttcccggcaacaattaatagactggatggaggcggataaagttgcaggaccacttctgcgctcggcccttccggctggctggtttattgctgataaatctggagccggtgagcgtgggtctcgcggtatcattgcagcactggggccagatggtaagccctcccgtatcgtagttatctacacgacggggagtcaggcaactatggatgaacgaaatagacagatcgctgagataggtgcctcactgattaagcattggtaactgtcagaccaagtttactcatatatactttagattgatttaaaacttcatttttaatttaaaaggatctaggtgaagatcctttttgataatctcatgaccaaaatcccttaacgtgagttttcgttccactgagcgtcagaccccgtagaaaagatcaaaggatcttcttgagatcctttttttctgcgcgtaatctgctgcttgcaaacaaaaaaaccaccgctaccagcggtggtttgtttgccggatcaagagctaccaactctttttccgaaggtaactggcttcagcagagcgcagataccaaatactgttcttctagtgtagccgtagttaggccaccacttcaagaactctgtagcaccgcctacatacctcgctctgctaatcctgttaccagtggctgctgccagtggcgataagtcgtgtcttaccgggttggactcaagacgatagttaccggataaggcgcagcggtcgggctgaacggggggttcgtgcacacagcccagcttggagcgaacgacctacaccgaactgagatacctacagcgtgagctatgagaaagcgccacgcttcccgaagggagaaaggcggacaggtatccggtaagcggcagggtcggaacaggagagcgcacgagggagcttccagggggaaacgcctggtatctttatagtcctgtcgggtttcgccacctctgacttgagcgtcgatttttgtgatgctcgtcaggggggcggagcctatggaaaaacgccagcaacgcggcctttttacggttcctggccttttgctggccttttgctcacatgttctttcctgcgttatcccctgattctgtggataaccgtattaccgcctttgagtgagctgataccgctcgccgcagccgaacgaccgagcgcagcgagtcagtgagcgaggaagcggaagagcgcccaatacgcaaaccgcctctccccgcgcgttggccgattcattaatgcagctggcacgacaggtttcccgactggaaagcgggcagtgagcgcaacgcaattaatgtgagttagctcactcattaggcaccccaggctttacactttatgctcccggctcgtatgttgtgtggaattgtgagcggataacaatttcacacaggaaacagctatgaccatgattacgccaagcgcgcaattaaccctcactaaagggaacaaaagctgggtaccgggcccacgcgtaatacgactcactatag